European Patent Application EP 4 321 015 A2, published February 14, 2024. Title: DOUBLE-FLOWERING DWARF CALIBRACHOA. Applicant: KLEMM & SOHN GMBH & CO. KG. Application EP, filed October 16, 2020. The sequence listing filed with the application follows.

SEQUENCE LISTING (7 sequences)

SEQ ID NO: 1 - DNA, 544 bp, Calibrachoa sp.
  source 1..544: mol_type = genomic DNA
ccctcatctttctctttcagaagagcctactttcgcccatggttcgcgtcgctatcgtgcttggtccgttcgctactctcttttcagccattattgtatgcgtgtagcctaagtctacccttcgattggactttctccagatcctttgacacccgctcatcttacttcccattctggtaggttggtgcgtgatgattcgtggagtacaaggctctctctggttgggtacgtaggctggtcctgcagmttgtggaggtgaccagcgctgcatgcccgaatggaatattgactatcccgtagaactgacctagtcgctcgtsaaggagctggtcattatggaatatactatatgtaggcgcaggtcttcctagagcgaacctccatgtgttttatattaaacatataaaaatcaacagtggaagaggcactggttgtgcgagatcattatgactggaggaagcccattcgacaaccataataggctctataaccggatcacgcacgctaagaacacagcggattagaggggacaagaggttccact

SEQ ID NO: 2 - DNA, 114 bp, Calibrachoa sp.
  source 1..114: mol_type = genomic DNA
atrccaccactgaaccaccrgctgcaatggcggagaaggtgtstgatgaaccatttttggtggtgggacacggtggattcttgggctgaaaaaacaagaatggaaaacgcagtg

SEQ ID NO: 3 - DNA, 544 bp, Calibrachoa sp.
  source 1..544: mol_type = genomic DNA
ccctcatctttctctttcagaagagcctactttcgcccatggttcgcgtcgctatcgtgcttggtccgttcgctactctcttttcagccattattgtatgcgtgtagcctaagtctacccttcgattggactttctccagatcctttgacacccgctcatcttacttcccattctggtaggttggtgcgtgatgattcgtggagtacaaggctctctctggttgggtacgtaggctggtcctgcagcttgtggaggtgaccagcgctgcatgcccgaatggaatattgactatcccgtagaactgacctagtcgctcgtcaaggagctggtcattatggaatatactatatgtaggcgcaggtcttcctagagcgaacctccatgtgttttatattaaacatataaaaatcaacagtggaagaggcactggttgtgcgagatcattatgactggaggaagcccattcgacaaccataataggctctataaccggatcacgcacgctaagaacacagcggattagaggggacaagaggttccact

SEQ ID NO: 4 - DNA, 544 bp, Calibrachoa sp.
  source 1..544: mol_type = genomic DNA
ccctcatctttctctttcagaagagcctactttcgcccatggttcgcgtcgctatcgtgcttggtccgttcgctactctcttttcagccattattgtatgcgtgtagcctaagtctacccttcgattggactttctccagatcctttgacacccgctcatcttacttcccattctggtaggttggtgcgtgatgattcgtggagtacaaggctctctctggttgggtacgtaggctggtcctgcagattgtggaggtgaccagcgctgcatgcccgaatggaatattgactatcccgtagaactgacctagtcgctcgtgaaggagctggtcattatggaatatactatatgtaggcgcaggtcttcctagagcgaacctccatgtgttttatattaaacatataaaaatcaacagtggaagaggcactggttgtgcgagatcattatgactggaggaagcccattcgacaaccataataggctctataaccggatcacgcacgctaagaacacagcggattagaggggacaagaggttccact

SEQ ID NO: 5 - DNA, 114 bp, Calibrachoa sp.
  source 1..114: mol_type = genomic DNA
atrccaccactgaaccaccrgctgcaatggcggagaaggtgtctgatgaaccatttttggtggtgggacacggtggattcttgggctgaaaaaacaagaatggaaaacgcagtg

SEQ ID NO: 6 - DNA, 114 bp, Calibrachoa sp.
  source 1..114: mol_type = genomic DNA
atrccaccactgaaccaccrgctgcaatggcggagaaggtgtgtgatgaaccatttttggtggtgggacacggtggattcttgggctgaaaaaacaagaatggaaaacgcagtg

SEQ ID NO: 7 - DNA, 465789 bp, Calibrachoa sp.
  misc_feature 24511: note = n is a, c, g, or t
  misc_feature 24513..24515: note = n is a, c, g, or t
  misc_feature 24518..24519: note = n is a, c, g, or t
  misc_feature 24521: note = n is a, c, g, or t
  misc_feature 42971..42977: note = n is a, c, g, or t
  misc_feature 148862..148863: note = n is a, c, g, or t
  misc_feature 157905: note = n is a, c, g, or t
  misc_feature 293054: note = n is a, c, g, or t
  misc_feature 293985: note = n is a, c, g, or t
  misc_feature 294064: note = n is a, c, g, or t
  misc_feature 294372: note = n is a, c, g, or t
  misc_feature 294386: note = n is a, c, g, or t
  misc_feature 294412: note = n is a, c, g, or t
  misc_feature 298184..298186: note = n is a, c, g, or t
  misc_feature 417943..417944: note = n is a, c, g, or t
  misc_feature 465621: note = n is a, c, g, or t
  misc_feature 465754: note = n is a, c, g, or t
  misc_feature 465764: note = n is a, c, g, or t
  misc_feature 465770: note = n is a, c, g, or t
  misc_feature 465776: note = n is a, c, g, or t
  source 1..465789: mol_type = genomic DNA
wymytrtystykhhgtvggtaghswhavatstdhawtgtatatagkwdahcymaawratccgahvcctcvratkcawyaycatatcatggccgtbyctawsadttgctytttgtgatgcagcggaaccatggcaattaggatctmaagmcgcagmammrycwmtmaykywwgrmakwwmwrmswtacmwsamgatgtttywghattcgttattctgattttgggtttcgtatcatggatcttgggtcgcgctttatggcatttccactataaaaaaaatccaatcccgcaaaggattgttcatggaactactatcgagattcttcggaccatatttcctagtatcatccctatgttcattgctataccatcatttgctctgttatactcaatggacgaggtagtagtagatccagccattactataaaagctattggacatcaatggtatcggagtgcgcctcttcacgagggtgattaaagtgcaacgaaatgccttaaagttgaatatggttcgcgaagcatctggcttaccggtaatctcccattcccgccgtcgagagactttaataactatagcatgccagaaacggggagttgaggtggttagacctataccccgaaatgctcccagcataggagcctatggttccattcttgttgttgctggaggtacacatccctcttctcggtgtggaacgatatacgagaaatagatgctcagcctgcaatgtccgataacggcgctgaagtagtgaatctatcggcaccatagcagtggtatacaactttggacctaacggccggcctagtaacctttcggaatgggggatccccgttggcaacaaccacggtagtagttgcggaactactgggccgggagaggacaacctcttgttcctgctcctctttcttcgcttcggggacggaggtcctacggtaggtaacagcaggcacaagcaagttgaccgaaggggaccagcgcttctactcctccaccgaggagccgttcttgcgagaagcaagggatgtcgtgaacggtgggaggtcacagagaattgacctattcatagagtgatcctatgatcgatacaggatatagactatctcattctttattctattctatttctgaaaaaaaaaagaagggtgactcaacttctcagctagagttggtggtgggacctcttggcataatgcacgctggaacgtgggaattcgaggtctcatgaactactactaaaaaccgactttgtttttgttttgtttgtggacaaacgatatccggtcaggcctatggctggatccttttagatctacgggccggccggccccggccgtttacatgagcatagggaatctatactcgagcgttccactgggcccctgacaggataggtgaggaatcactctggatcttctttttttgggctacaacttcgccgagccgactagcatccctttccactgtgcatttttcgaacaaagaagacgactataggatcgaattcgctcttcaagaaactgctcgtcccataccttctgcctgtctcatatgtgtggaacctggtctttttcggttccagcctctccctcgaatacatagggtaggtagggctgggtgataaagggttccctcttgccaataaactttccccggccttcgattaaccttactcataaagggtcttacggtcgggagaactacctaactaaagaaaaatagtgttctttctaagagtaggcgtggagagctttttgcggggaaacttgcaagtacagtttggggggaggcgggcgtcgaccctaccttatgagtattcggactataacagttccgatgaacagtcactcacttttgacagttatacgattccagaagatgatccagaattgggtcaatcacgtttattagaagtcgacaatagagtggttgtaccagcaaaaagttatatacgttttattgtaacatctgctgatgtacctcatagttgggctgtaccttccttaggtgtcaaatgtgatgctgtacctggtcgtttaaatcagacctctatttcggtacaacgagaaggagtttactatggtcagtgcagtgagatttgtggaactaatcatgcctttatgcctatcgtcgtagaagctgttcctaggaaagattatgggtctcgggtatccaatcaattaatcccacaaaccgcagaagcttctccagtcttcgtcggttccccaaaagaagacactattctttttgggagacccgtcgtcgacgaagatgagctctacgaagcggcttaccaccccttctacgcggccaacgtagtccacatccctggggaaattgaagacccctttactctggctaaattaagtaaattaaatgggactctcctagccatagcggatctctttttcaacggccagataaggggatcgtacactaaagagctgcaacttgaattgaatgcgaccgaagaaggcgagctggcggctaagctggaagagctgcggattagggaaaagcggcgctataatttacgctagggtgagcaagcgctagctctttctcttgcggtgaaataaccgccgtatagaggcgaacagcccttatagcaatagcaaacggcctacttatagcctttcaacaggtcagtcaatatcagtaagtaggggtcctcttgcctaacggagtcagcccaacatggacaatgataggcagaccaaagatttacgcagtcgttgcgtgcttgctttgcgcaccggcatagcagaattagaatccgctggctcagatgagtggctcttggcttcgtaaacatatctatgttgttgctttttcactaccaatgagtaggcagctttggatgcttatggagatatggcttggcccaggactattggctttccgtcaagtgtcagttcagccatagacattcaattcaatctcggagatagtcaaaatgccattgtccgttctaaatgaaaggaatgagataggccgcttacacacgcttcaagtcttcttttgctgattcaataacagtctggaaattcgactgaataagtcttagtgtggttaagccggggccagggtcagaagttcttccatctcctgagataagatcagacagagcctatacgccttcttgctttgctgcagctaccgggtattcattcaaaaagaatgcatttaccttttctcccccttccttcggcatccctgactcgggcatccctttcaggtgcagttgacgtacaatttaggtaatttataaggactaaacgtactgatgaaagggaaaacttaggaaagaatagctaaggagaatccttcgtttgaggaaagagatgataaaataagtcatgaaaaaaacccagtttgttttaaggctctcatgaagccttagggcgaattcctctcacattggaaacttcgctcacttcctatattattcgcgcacctacctaccacaatccggttccaagtcctttattttaaaatcgaggagtagttcaacttttctctcttcgggactaagagaacttacttactaattgaaaaaaaaagacaactagaacgaggtttttttttacgtgatcggaaatcacccgtcggtgatgaaccagtacgcacttaggatagcacttcgggagagtgagatccaggtggcatatcaaaaagacttatcaaaatcgccaccatacgagacttgcagggcatgcccgccagaaagtgaagagaggtttataagcaccccgacttaggaatcatgacccaccgaagaaaagaagactcgaggaaaactattgatccctttgatgactctcctcttcatcttcgcgggttgcagagaagaatccgaactgaggaaatgaaaaaaaaaaagaaaagtatctctttctctttctacgatcacctgtagcgtccttaaaaagtcttagaaggagaatctaactattctcgaagagattcttgccaacaccattaggaagatgagggaaaggggaaaagaagtcaaattcgctatttccgacagctacggtagtagagaaggagagggactacttatgagaaagaggagttctctcttctactcccgggtattgaaccgggatgctttggtactagactgggcgggcgagccataatcacagggggagaaaggcgcagatcttttcatcctccgccaacaagcagagccgacaccgagctacttcgtacctttttcattcaaacgggaatgactccactctcagtcccagtgtggcttagactagtagaaggcgtaaggatgctagaccgctgctcaatactggataatccacgttcatcggtctgcagcaagcactgacttttagggggcggcaactaaagaggtagcgagactaagcgcaatttcaggaagagttggacccttgcctctaagcttccttctacccttgtgctaaaggacaggaaaaacaacttctttctttctttttttttaatatattgaataatggaataactcgaaccctactaaagagtggctttcagctcctcccccttctttcattcagcgactgggtacgcacttcgccatgaaagatcttggtgatcttcatttctttcttaggaatcgaagtcaaaggtacatcgacttctctagtcttgactcagactaaatacaccttggaattactcgaactcatttgcaagactccaagccatgtcccacaccccttgcgtctggcttaaagctctctgcatacgatggtcctcctctctctgatgcaacggaatatcgtagcattgttggcgcccttcaatacctcactctcaccaccgtatatctccaggctgtaaaaggcatcttacggtatatgaagggttttcttgggcttggcctaaccatcactcagggactttaaaccaccttctttgcattctccgatgccgactgggctggctgtcccgatagcagacggtccactacttgcttctgcgtatttctcggaaacaacctactgacttgggtttcaaaaaaaaaaaagaaaccgattctttccaggtctagtgccgaagcagagtacaaggcactcgctcttactacctctgaactcttatgactttcttacttactacgcgatctagcggtgccgtttcgctatcaatttttcgtgcactgtgataatgctagcgctacacacttggtggccaatcctgtgttccatgtccgctctaagtacatagaagttgactaccacttcgttcgtgacctcgtcgtcgcaggcaaattgctcattcgacttgttcgtagcaacaatcaagtggcggaccttttcactaaaggattacctgaaccccccttccatcattttctgctgtctcccgcctgcccttctcgaaagaatgggctcctggccgtcctatctcattgaaaaggacaaaaaccatttacttttccaatcaaagaaagtgaagccaccaaaaaaaaagaaaaagggtatagtaatatatatataaagtcaaagttcaatggtaacgacttcttccattgacttcaggattgcttggtttcagggaaagtctctcgctcctctccttatagcgctggcctctgtctttgatcttggctcgagctctgtcctctcctctccctatgtgagagtggctgcttgaagcttttcgtatgaatagtcaaagctcggacttaggagctgctggcctttgttgatccgcttgaagagagttctcacgaccctgctacatcgcgatcgtttattcccaaggaatagagaatacaaagcacacaaggcgcatgatgaacaagagtaacttcccgtcccttactccatttcttgtcttaaatagacaaaatagtgggcttcctgcccccttctcaaagagaggaggacgggttattcattcatatttcatttgatggtcagaggcgaattgaaagctaagcagtgggaattctaaagattccccgggggaaaaatagagatgtctcctacgttacccataatatgtggaagtatcgacgtaatttcatagagtcattcggtctgaatgctacatgaagaacataagccagatgacggaacgggaagacccaggatgtagaagatcataacatgagtgattcggcagatttggattcatatatatatccacccatgtggtacttcattctacgatatatataagatccatctgtatagatatcatcatctacatccagaaagccgtatgctttggaagaagcttgtacagtttgggaaggggttttgattgatcaaaagaagaatctacttcaaccgatatgcccttaggcacggccatacataacatagaaatcacacttggaaagggtggacaattagctagagcagcgggtgctgtagcgaaactgattgcaaaagaggggaaatcggccacattaaaattaccttctggagaggtccgtttgatatccaaaaactgctcagcaacagtcggacaagtggggaatgttggggtgaaccagaaaagtttgggtagagccggatctaagcgttggctaggtaagcgtcctgtagtaagaggagtagttatgaaccctgtagaccatcccymkmcmtgtgggtcgagcctccttttcagtcgccctctacaactaagtcagttgagctctctcggctcctagaccagctgtgatctttcctcctgttggtttgcttagttaaatatatgcatccttagagtcagtccctttttttggagaaaaattccgagccggtaagcaagacaaagcaagtcaacgtgggaaaaagctctcgatggccatagacctgaatggttggagtgtggaggatcactcctgaaactttcttcctttatataaggaatcctcttggttggtcgaagctagaagacggctggacgaactgctattttgcatagggggagtaagataggctaggtgcttttactcaactcgtgaaggttcatttctagttagcaaggataaggaagcaaaggtagagtcctttaataatatgtctgtcattacgtgcgactatctccactatagaaagaaaaaaaggaaagaacaacattttcagcacatttatacgaaaaagtctttattattatattagcataagtaggaaacattttccactagggtttttcccatacatgcaaacataaaaaagaaaagcaaacaaagataattagcatagataggagtctatctccagtaagcatcggagtagatctccactaaaaaagacaaagaacaccctaaattaaaacacattactttgcgtctacagacacttatttaaaccttctaaaactaaaaagagtcgacggactcttctattctagtctccctggcgaccacgggtgacagcacccacaattaggtcttcctgtttttggaggagggcccgtttcctgtcttccaggacgctaatgcggtcccggatccgctgcatggctgcagccacaagtgcaggatcgatgggaggcaggtgctcccaaaaggcagccagggtttgctccgattggagcttctcctcttccacttgagagatttcttgcgaaatttcttgaagtcttataaaagaatccatggctacactcaaagcttttttttgccgacttctaagttcctctccgtctccctttgccaaatagagactgaaagaagcttctatttataggcgttggaggcccttaaccctttcttattattagtaagataggttgtcttggttccgtaacatggatcatttcaaacctggcttttcatgaatatggaaccccctccactagattttagtgtgctgaataattatcttcgtactccaatccgtacgaagggcccctttcttttggcgggtatcgccacgtggcttaatcccggatcactccttaaggaataggacacaataatatagcgcacatcagagaagagagtaccccctttattataagacaggccccacgcgtcctttcttaagagatggagcaatcgtcactcgacagctcaaagctgaccggtacaacccgcgtgcttgcctactcgtctttcaccggcctatttgtacccagctacaatctcttcccttagaaaagaaaaagggcccctcggccaatcgtcactcgacagctcgaaagcggatcagtacaaaaccatgtgatctgtacttgtttacgtactgccccttaggcctagggcttcgtcgtaccctgcttactcctctttcactttcactggcttctacttgtcttttttttttttattggcttatttagaaaatggtatcagcatttgagacgactctccccggccaatcctcagtcgtccgtccttgcttaggagaaaaccgaaccactatctcttgatagatctgtttttttctacctttacagctcgctctgtaagttcactagcaatacagcactagcactagctatagcagtaactagtacaatgagttaggggtcgggtcgggtgaattcaataatagacgcctgttggcattccagccttcctatccgaaagagaatccattatttcttggtcgtgaatatctgaactggttgttcactgttcaagaattcttgtttagacaattcagaccatccatacatagtcttttaatctaagattgaaattcttccatattttattgctaaaatattgttccatggagctaaggtccaaaatatggaagaaagaagtgtttccacgactctccagtcaattctgttccacttaatccctctttcatggcaacatctctttccggctaaggaatgggaaatctttctcctgttacatgaatcaagttttcattttatccggaaaagcccctttccagctgacgctgtcagtccactaacagcggtatacagtaagtcagtataagtcagtacaggaagggcacgcgaaatagacaactacttactaggctagggtagtagttttttcatcttccctttattttactttaccctagtggaaattcatttttaaaagtgactaggtaattagtgaagaggtttataaaagtgacaagcttggtggaaagctcttatcttaggaggaaaagctaagtatgcccgagtagtcttgatattggttggtttgaggtttcgttagttttatactaacaagcaagcttcggttcggcgaccgctcgacctagcgccttagccccagtactatagggaaggcctatgcgaagaaaaggcctgcccatcatcaaagcaagcccaagtccatgcaagaaggccctccagatctgtccaaattcaaagcccgtcaaaggcatatgaaatcatgcaaaggatccgagcccatccaaatgatgttcagcgggctaaacccaagtagctctggcccatgatccaagagacccgaaactagttaatcactccgtgccttaccttctaaccaatcggccaatcacgctatccttacctttcaaccaaccccttcgattcagtttctgcagcagtatagaatctcggacccgatggatgcctacagaaaaatgagttttccagcagtgatggcaagaatccgcgaaataatgttctttctcctttttgtgttctttctgaatggagctacgcgagggaaagctcagctttctactctgccgcaaaagggggccgctttcttcccccccaaaatgccagttccgccatcagggcctagcaagaagcataattctgttccaaagcttcgtttcattccagcaacagtagtctatggttcgaagcgccgtgttccatccggcgcgaatcctctccataactagtatagtggaggtcttacttgtattgcaataatgaaaaaatgtacgaacacaaataatgagcagaccagcccacttttatatgtgggttcatttcagaatgtttttttgttttgaataaagaagcgcgtgaacttttagtgtaaggcaggtgtttttctcggtggatggatgggataaatgcctatattgctttataatgttattgttatgttgatgttatattaaagaatgaaatctaaaaaagttgcttagtcccattctttataattgtctttctcatactgtgtaaacaaacttcaagtctgaattgtgtactgtactcaacaggaagcgtcacagccacccccgatgtcgatctgcagtattagtttgagaaagtcgtttggtttttaacctagagcgattggtttacctgtatcatgcaaatgtccaacacttaggtgctttctaagatcatcctatatgaaagatgtatgacatgtgtggataatgaatgacttgcagggtatgcaatatcttaagtacaaaaggtaagacctaaaaagagaaatgagcttagcacaacacgggatagaaagctaatcctagaaggagaaaacccatcacagaacaatcataggaaaagaagaaatgggttcagaccaagtgacagaactctctatgagttgggctacataaaagatccttttctactaaaatggatgtaggcttaactaaagcccaatgcaggttgaactctatggaatctaagcctcactacccttaccctcttagagggttacaaggaattttaggccggccccatatagattcagcttaggggtttatgagagattgattgatggacctaagctaaacaactaagattgaacctaaaccaaaacctatagactgaattaggagagcagaggtttaattcaagaccaggaaagcaagttatatcgaagcccaatgccaagcaaagccctagactacaagtgaagaaattgggttcaactaagcccttaacccaagatgaggtggagccttaacccgacacaagaggggccctgtaggatagtgggcttagtcagcccaacataggttgttaaccaaaaaggagaagttcccgtgaaaacagaaaaagacctcccccttaaccccccccttacttggcagattcacattcgtaggaaaggtctgttcttttgtctctttccctcaagcgaaggaacctattaataagataataatatctctctgcttcctagatcgataacgaatccttcggttgcttatcctgtcatccgagcccggcgttccgaacaacaatgattcggaaagataaggtctacgaaagaaaagaaaatttacaatttgccctactcctcaagaaatactgcgagcggtattgtaaaggtatgggctttttcggtcgattttgctcaagagggtggggggacttcgactttatcgaagcagcacatgagattgcccagaaggattacttttttattaacctagtgcggatgtggactccctaaaaaacctgctccactttgtacgaaaaacatagtaatgcagctaagtgggagtcttacatgaacgcgcacttgatctttgacttggtccgccgcgatccataaggaaggggttttcgttcgcaacaaggtagccgtagggaaacccctatgggctggattgaatctttcctttccttctccctctcacctgatccattaaaggaaaacagactcaaggattgggccattttccatatgtctctagaaagataggagctaatcaaaattcttattacttatgtaaatgtaactctcaaatttgatattactccatgtgtaacgccaaaggggccttgtattcaattgaaacagaggatctcccacattgatatacacatccttcacccaatctgctcaaagtattttcaactctttcatggtatcagagcactagctcttgggaaaggttcagttggttcgtgtgaagtgtggtctgaataccttcttcttaggtgttttctctttggcgctgtccaccgctctgtctctatccttctcctcagcacttagttagtatcccgtccatcgaaattgagttttccatagcgtctgtttcaattttatggaaaactaagaaaattgctttttttgaagcacaagatcttctcagtttcgttgatggaactggaaaagaaccaaagaaaggactttcttgagactgatcacaaaggtaagataatgaatcctgagtacgtcccctggagaagaacagaccgactactcaaaagtttaatgatgcacaccatgccctttcccaggcgtcgaggttgcctagccgtaatccacaggctggcttcgacagatgtcagagtgaatccgattcttcgattcaattacttttccaattccaaccccgcgcgtggatgtagaaaagtgtgtgaatggcatacgtaagattggggatggacaacatcaattcatttagtatagtcagctaggaagcactagctaggcaagtcatactgggaatgctgttccacacattggctcaattctaccttccacatccaattcttccttcattacaaggcccagcttcgctaaactcgcaccgacccttagttaaatatgcgggtagcttttcacgaaagattgttggcatgcctcccataagaagtaggataaaaaaacctatgagacccccttgttctaatctttttcctaaagagcaatcgattactatactagtgcatgcaaactgaaatcttagagaaccttgatcctattgatcagaaagagctcgggcgagaaggtctgcggggtcagaagagttcagagaaagctggatccgggaaggcttacgccgataacgaaggattttgaaaccgatcgatatgcagacgctgcaaaagcaaatgacttcgcttcctcaatcaaggtaaggtaatttgagaagctatcgaaactattccgaagttgatgatttcgttctagctagggcaatttaaaagagagaagtttacgctctccaacaaagaagcactcacctcctaatagaagagataacgtaagaaagactagcagatgcggacgatgtaagcggtcaatcaattgagactacttagagtccgctaactaggggaaagagaagcactaagatgaaaagatataactagattccccttacataatgctcctgttgaaactaaaaaaagataagaagggacttgaagcttacagtccttactcaactacaagtacatagagaaatgcttccacctattagactatgcattgacgttgcagatgttaaattgcagttggcattaggagatagagagcaaaaggaatgaatctagtatacttaaggcaatccaaaaaaagaaagcgcttagtccttatgcaactaaagcacaggcaggaaataaagctacatccacaaagaaagagatggttgcatctaagggcttcttatcttattgggtctagcttcttagaaagccatagggagagaccgaacaatctgatgatatatacttgtgatgtcagaaaaaagttccgaagagtggaggcagctttttcctctccaattttctgttggattctaataggattcaggaaaaaaataggaattcgacagagcgcaaaaagatagtcgagcaatcagcgggcaggcataggtagtcgacagcagcaatcgaccatcttgagcaacaagagaaagaaggaccaacgacgatcaaggaaagaaagactaagtaaaggcagacaacgagacgaagatagcagacttgcctcgaaacaggaacatagcataggggcatttctccggactagttaagtagttgagcccggctcccccgcttggctcctctttgctcctagtagactactagacatcttgtctactctgcttttatggaagagctcagtccaagaagggctctcaaaaaaagaaaattgtcaagctttcgaactcgccttgaagttgatgaatgattgcaaggctagcaacaagcaggctcgcttatgatctgctgaaagagtacatcaggtttttttattaatccctcacattcatgaagcagattgtcgaaaagggctttctgcaagcaggaaaacgaccttttttacgatccacagggtctagcttgatcccggtctcgggacttcccaagtcacggagtctttgatcaagttgtaaactaaaggagtataacctatccaatatatatatattttcgcttattgttagtaagaaaggtgtcactaacaaataaatccttaatcagtagtggactactagttaacgcactactaaagcagagtagccagcatgcgcacataattttttgccagaggatttttcagcgaatggaagaagcaggcagggatagatataattttttagggaaaaagtgctttgtttgatttgttcccaggtgagatccaagatctttcaacgcgttgatttcctactaaagaaactgggcttctatcaggagtttgatcattggaaagggtcgaaaactcttgctttatgcttgagaaagagccttcccggcgatctgcttcatttatggagggtttgcaaggaagacaactgaatagcgggaattaaaagagaaggatttccagaggtcaatatctggcattgagcctgcctatcctaagtatgagttgggagagcgagatagagacaaagacccaatggacgttcccctgctctctctctcgatgtggtacctttcagtctgctctgtcaaaactttctcgcaatgccgaaaggtagagcagcttcaaggtcttcggcaacgagatcaactgctgacccaagaaggtagggaagagaggaggaagggccaatccccgagtcaggggcatctatctttatttacgcaaagctattttcgatttagatatgttcattggcctgcgactgatctcatcgtccgttttccccctctttcctattcaagagttctcctccctaacggcacactgtatataatctctctagatggccaatgtgaacagttcaatcaaacttgtatgtgtgaagcatattgaaagtgacattgacaaagcaaagcacagattccctagaatgttagaactcagacatgacagagaaggtagtcaaaaacggtacgctaagctccttgcttcgtcgcttctgttttcagttattcaaagaatgatgttttaagcatctctatatgccagtcatctatctgacctgacaaggaggtcgactttgatatctcacccctgatctctacggttggttgaaggtgtcttggaagacgggtcgaaatcagatctggatagaagattcatctacgctggcaaaagggctatcagaaagagtccaatcccgaggagagttcatgtgtgaaatttctttgttgaatggaggtgagttcaagggcttctttgatcgggaaatgcacgcacttcttttgttgtcattaaggtcccttccccctgagttcaagatgtcccttccgcttctctttcactactttcctcattgggattggtcaagctccttcacttattgctcgatccgatccggaacctattgggatagcaccctttcctcctatttattagtaggtcttcttgcccgttcagttcctctactggtagtctagttgtagttttgagcgggtgaacccatgttctatctcgtagtcacctaagcggcagagtctgtaaactcaaatggtctgagagttgcctttggcttctgaacctctgaaactggactggagcaagctaccaagctcctcttcccccttcatcactctctatctccggcccttgccattagttagcttgcacttcccttgcttgccctttgagttttcaaagtcaaggtgcctttcccttttctgccttacctcttactgaagtgaaagaactgactgttgtctacctttgattctgtcttccgggtgaaggtcctgcggaggtcttttttagtgatcaaaattgattagggacagtgacccatgatgaaaggagctattgacctaagtggttttctatttgtatttgaaaagcaaggtaggtttgttaacgaaaggataaggttaggctggaatgggatatagtaagtgtgccacgagtgctcccttctaaggcttctgcttctctctaataacgagaaaatgactctttcagaaagcaaagctacaactcttcagtctaagctatctaagctagaacttaaggccgacctcttttccagggataccccacttcccggtctagcttcactaactgtattcacagctttccagatctcggaaccagatctactttctcatcggcattctctaaatgaattacgttatggtcttgaactctcgatatatcatatgtaatgaatgatcgaggttgtcttttcggaagaggtgggtgggagtggggcagggcaagaaagtaacaatcatacccgatattcagagcgccggagatagaagcggcggcagccataaagtggagaatttccatccatttgctgtctccttcgctaccgctccgtggggtcaacattacgaaattagccaggttcagttctgactatagctgcaacctatctcatatttggccgccctcgatcacaaactcgaaattttggaagataaagtaaagaaagaatttcgggctaggttcaaggtatgcccaaaggtatgccagttgattgaaaaagaaactcaactttcaagattcaagattaggtaagtgttcagtgtactaaggtacaagatcgaaaaaaaagcgcggatagcaaattccttaggctagatagagtggtggttgtaaattactaggtagccatacaacactcggcccaagcaacgcccaaaagcccatgcctttcttggtcggaccaacccaaccggcgatttccgacaagtctttctgaattggaagagcaagaagcggaacttgaagaaaactttctttctctttatggatagacagtctttttcaaattctccttctaattcatcttccccggtggatttaggtttatctctgaggtcccacgaaggttcgactagtagcactctgtcggacgccaattcgggtgatattactagcactcaagttttgagtgatatcaccgctctttttgagcaacgaatggaagtgggaaagaattcacaccagaatggagcccaatagagttctgccaagcggtttttggggaagaagcggtgaatgacctatctttattgaaagacatctattgtgatctagcggaccatggaatgctaagttggtattgggaaccagcttggggctttctaaatctcattagcaatagtccaggaatgacatagccttcctgtgcaatgggtgtcttaacgtactaagtaaggtggttttttctaaagcggcattctcccttctatctatcaacaatagaattatggaactttctccccgagctgcggaactaacgagtctgatcaatagagtccgtcattttttctattccttcctacttcttcttcctctattatgtgcttttattctatttgcctgaaactcgagaaaatagagttgtttgagaccaaatgttatagagttgggggctctctggggaggcacaccttcacttccttcttaatgaaggggttccccgggagtctgaccttgtcctttcttttaattgtcggggccgtcatgagtgccgaaacctatttcggtaagatgatgatggctccttcgggcgcatcaagctctgaagatccaaactggacggaagccctgagatcttctaaagggcagggagagacttcagaaagggaaagcacaggcacatcgtcgtccatcaacctacaaaaagaaagagcacgtccggcgcctgccccaaatgaagtagcttcccctgcccctgtcgtcccctttccatatcaagaagatgagatcatagggggcgacagtgtagaaagcatccaagagcgtttaatttgaggagaaaaacccctccttctgccgaggtcatacatcatacaacaggcccgaattgaagccgaagacctattcgaggtcaaggtcgatattttcaggggcatgtctggccttgatccagaaggagattggctgggacggggagctcgggccctcgagaatccgcgtaccgccacgggggagcattccttggagaaactccatacccttctttcggatctcgaatcgaggggagtcaattccgagtccttctctcaattaaaagggaaggtacccctgcgaaggggtggggacgaacactctaccacatagtggagtggatagctaggactactaaaatggagatcgtgtacaacaacaatcctatatttgatgtcgattcatccacacttccattccttgtagaggaaggctaactgcttgctggctgggagctgtatgagcggtaacgtccacgtacagctccgtgagaagggcggtggacagaaatggccttgttgtacctcactctcgtcttcaatggggtctgctctttcttttttgggagagtatgccaatatgatcttaatgaggtgcggggctttgcatctgacattcgttgggcttctctcttcgggagcctgcgccccggcgtttttgtgcaataaacccctccggccgaagactagtggtaggtggtcctgcggagctttcggaaaagggtagccttgtgtgtaagcacagcaatgaaccgcggcgaaccctcagacgacctatctaagattagggggggatcctcagtagtggtgaccctttcactcttccacggactgatacatgtaccgaatgctcatacgggaaagttgactcctgggtctggaacctggggggttgctccgagaaaacctttctttctcgtccactcaggggggtgcggacacacctgcgcggattacaggtgacagttacaagaatggcggggaagttaacagtacccgacgacattcagggatggatgtagacccatcgggcagggataatcattccggtcctgggagaagtggcgaccattctcaagaaccaaaaagactgagctgagggaagccctatgagtcactgaaacgacggcaggagtgccctttttctatcaatagagggagcaaaaaaggggccttgctcccctttacaatatgaagaaagaaataagggtcgaagtttagaccgctcacagtagttctacctatagaaaggatcatgaaagaggcgatcagaatggtactcgaatccatttacgatctcgagtttccagacacatcgcacttccgctcgggtcgaggcttccactccgtcctaagacggatcaaagaagagtggggaacctctcgctggtttttggaattcgacatcaggaagtgttttcacaccatcgaccgacatcgactcatcccaatctttaaggaagagatcgacgatcccaagttcttttaccccattcagaaagtcttttccgccggacgactcgtaggaggtgagaagggcccttactccgtcccacacagtgtattactatcggccctaccaggcaacatctacctacacaagctcgatcaggagatagggaggatccgacagaagtacgaaattccgattgttcagagaataagatcggttctattaagaacaggtcgtattgatgaccaagaaaactctggagaagaagcaagcttcaacgctccccaagacaacagagccatcattgtggggaggttaaagagcatccaacgcaaagcggcctttcattcccttgtttcgtcgtggcacaccccccccacaagcaccccccggctcaggggggaccagaaaacgcctttcgttttccacccttcgtcggcccttgccgccttccttaacaagccctcgagcctcctttgcgccgccttcttcatagaagccgccgggtttacccggaagtccgaattctatggtagagaacgctgtaataataattgggtcatgagagactcttttaagtattgcaaaagaaagggcccgctgatagagctgggcggggaggcgatacttgttatcaggtcagagagaggcctggcccgtaagctggcccccttaaaaacctattacttaataaggatttgttacgcgcgatatgccgacgacttactactgggaatcgtgggttccgtcgagcttctcatagaaatacaaaaacgtatcgcccacttcctacaatctggcttgaacctttgggtagactctgcaggatcaacaaccatagctgcacggagtacggtagaattcctcggtacggtcattcgggaagtccctccgagggcgactcccatacaattcttgcgagagctggagaagcgtctacgggtaaagcaccgtatccaaataactggttgccacctacgctccgccatccattccaagtttaggaacctaggtaatagtatcccgatcaaagagctgacgaaggggatgagcggaagagggagtctactggacgcggttcaactagcggagactcttggaacagctggagtaagaagtccccaagtgagcgtcttatggggggccgtcaagcacatacggcaaggatcaagggagatctcgttgttgcatagctcaggtcggagcaaggtgccatcggacgttcaacaggtagtctcacgatcgggcactcatgccccgacattgtcattgtatactcccgcgggtcggaaggcggcgggggaaggagggggacactgggcgagatctatcagcagcgaattccccatacaaatagaggcacctatcaaaaagatacttcgaaggcttcgggatcgaggtctcattagccgaagaagaccctggccaatccacgtggcctgcttgacgaacgtcagcgacggagacatcgtaaattggtccgcgggcatcgcgataagtcctctgtcctactacaggtgctgcgacaacctttaccaagtccgaacgattgtcgaccaccagatccgctggtctgcaatattcaccccggcccacaagcacaaatcctcggcgcggaatataatcctaaagtactccaaagactcaaatatagtcaatcaagaaggtggtaagacccttgcagagttccccaacagcatagagcttgggaagctcggatccggtcaagatccgaacaagaatgagcactcaactactagtaaaaagggagaaagttgactttgagaaagaaggtgcttcttgccgctttattagtaagtaagcttgttttatatctcctcaataaaggcgaaagatcactcctaaaagcaagctttctcttatatacgataccataccacagaatttcatttgccttcctgcttaaggcactagttcggatggaaaccctgatcaggcaggtggcctagctaacatagctatccgtcagaaatagcagcattccattgcaggctactatagaggcatataattttccgggtgttaagaaagatattgaatcgaaagcggacatgcttgctcactggctagatcgggctgtctgtacctttgctaactcttctgcctgtaaggaagcttgaaagagggaattctctgatctatgaccccgaaagaaagatagtcttttttcgattccgcgcattggaactgaaaagggctattcataaacagtcttccttgcttcttacctcttatcttattgtaggagataatcggagagagaaaagtcttcctatcaattccttttgaataaggctacgctcctccaagcctttgaaactattgaaaatcgaatctttgttttcaggcgggttttcttctccaccaacaaccaagacgcatgaaagcggtttccagcgctgctgggcagaaagacatgatggcatgaaactcgattacgtacgctgattgttcgtccacttcaaaggctcaaaacagaccattttccgtgtgaaatgacagggattggtttggttacttagggaatcccaagcaaagcaatctacgcaatttccgggttcagtagtaggaaagaaagggacctctcactcaattcaataacatgttctagggcatccttttctaataataatgttcgcatttgaccaggctttttggacgttccatgattaaaccgactagcggcactttcgagatgccaccttgtttctaaaaagagtcttttcaattccatttgactcggggcgtcagggaccctccaacagaaacctcgtcttttttgtcgtcgataagttctccctcagtgccctactattcataagaaagactgatttaaaagagactgatttattaaagcccggtgaggcctcaaccgacagctaagcttcgttctgcggcggttttcaagctagcacccctttcagcatatcatctcgctcgattccaaaaaaaaaaagagacgcagtttttgattatccagttctatatcgaaaacgagcagttgatcccacgaaagcaaggctggctttgttgcgggttcaactggaattgtaagaagtgaggtaaattgcctttctccccaccgcatatgcctcctctgcttatgccactggtgatgaactcactatggctattcaacgtcaaactcagagtttttctactacataggcggctaaacgaagccccagtcttttttagtaaaaccccaacccccttattagtagccgaagtaaaggccagcatgagatcaaagtcacttgccgtccgttcgctctctgttcaacaaaggcgatcgatattcccttacttctcaagttttgaattttatgagcccttcgattgtatcccataagaaaatctctctgataaacatcttgtcgatgattcgattatattatttagaatcttcgtgtgcgcttttcgcctgaggctttcggacaagactacttactccagtaggttagtaagctacctcttccgctttcaggcaagggtagctctgaagggagagttgagcggaaccaggcataaggagcaagaatcgctattgagagttcccccgctaggggaacgtcaggagggggacatgctctatgtccactgattctgtttagtacagtataggaagcccttgtttgagtgagagcttctagaatgccattcatttcgcaataagaaacttttccacatagaggtttcagctacttaaagcgagagtgcatccaaaaattcgagaagagtgctcggccttggttgaaacaattataggtgtcaatggaccgatttcactagcagagcactttctccaatgtgcgcaaacagagatgccactttcaatgatggacaccggcccttgtgttaaagtagcatcgagtttcgcttggaaaccggcaagtttctagtttccaaataagtggtaccctttctttagagtccggtaggtcaattaagttgcctaaatctcttccttatctgctgctctgtagctgccttcctcgcttcgtcttcggctttcagagttgtgaactaacctcttccttttacagccagacaactggcagataagctgggcatctaaagaacataagatccgagttgccgccaggcataaaagtcatattgtcaactagggaaattggcacaaccaggcatctcaaacattgataagggaagaatcaggctttcattaggatgatattcctttcatccgaatggcaaggcttgctagtttcctgaagtacactcgcatctgtctatctatgtcatagttgcttggaaggaaggtctcagatgtaccttcggcatgtatgagattttctttcctctatctatgtcatacttgggattcactgacagccaattccaagtagatcctccctccccctcgctccacttcgtttcgctcgttttctctttccttctgcctgcaaaaaaagtgatgagattggttttgtgtgcgttagcgatcatcaaacctgtgacatagataagattggagttcatgcagttggaatgcctgagaccactttttgccttgctgctcttgcttctctggctactgctccggctaaggctttctttccgctttgacttgccttccttatctttcaatctggacttgcatgtgttccgcatatgactatttcgagtgattgctgctatctggcttgagttagacaagcagagaaggatcttatgccaccggtgaccggcctgcctatctagtatctagtactaggactagtagagtagaggcactactgggcggggcttcctcgatcacagcttctcgcttagctaactgccagacaaggatgcaaatcaactccttatatagaatgcagatcgacacattcaatgaagcagccagtacggcagacaagctactttcttattctaggactggaagatcctctatctattagcatacccgtaccggcagttagactagcactctctccccaatcaatcgcagtaactggctgtaagagagctgactgtctactatctatgtcatgccttggcaggtgaatatgagagagaggctgtaagtgcattctctccttctccatcttctggaaagcactctttgagcatgctgacagaatgattgacactcacatctctctcatttccagtgatttcgctacagtttactagcgcattcctagactaagactacggcattgaagaagcaagctcactctcattccaggaatcagaggaaggcattctgtccggtaatgaagttagaagtttccngnnngcnntntctcttctcttgcagttggtccggccagtcaaccttgttccgggccttctcttctactctatctgcttattggattggtaggtacagtctttcttctaggcttctgattgaactttaaggtaatgggagagaaggcaatcgacagataactggtaagtaaagctatggactgggttctcactctaagccagtaccagtaatttgaaaaaacgatagacatctagcgcattcactcgttttttctttctgatcggccaactcaaagagggaaatgcaaggggcgttagcggtcttttttgcctcgcctgctactgggaagagagagccgctgtcattcttcgcttcgttcgagaatcaactgcacatgaataggctcctccttaggccttcaaggaggaagcggcttttttccaaaattcccgggaaaatgaaacttttgaaattcttttcgtaaggcaagaaagttgcctaaggaaagtagaagtctatgcacactaaccgaatctttggggaaggatggtggtgctggccttttcccttctcctttctaaagcaaaaaagaatgtcatcattctgatcgtgacttgaaaaaagaaagaagagaaggaacttggagttggcgcccacataacggattgcttgcttaccaagccatcctggcttttcgctcctctccttacagtcaagtggctttcactcctccagttctattattattgacttgacttattattaaaaaaactactcactatccaaatgaaagacgatcgattatctacccaagaagatagagagtcccacatacgagaaaaggtcacaaatagagttgaaccaagtaacattgcaaaggcataatgatagtagggtcgggatatccccgccctccgaaccggacgtgagggtctcccctcatccggctctctgcaggggaatctccactcactgcttcccctaatatcctccccttaccacatcatgggggtttacaggagatcccagaggctcgctcggaaaggctgctataccataccttttgacttaactctactctagtagtcactagactcactatagtagtccgtctggctgctcttgctgaaatcattactcttaattctcccgtgctctagcaattgcgctccctagaccactaccatgtagttaggtagggacaatcagtccgtagtgacgggaatctaggaatgaatggggatccctatcaatataaaaagaatatctaattrgakwttthttttttybmrmvsagdavgvgatatvhgagdtbcghtabdgtcbhgtgcdctvvgagatgtdtaaaagctatgggatagatggtagagggctgcctgcgcccaaaagcgatgattcacttgtccccttgtccatagggacctcgtggcatacaaccgaaacgactcccgctagatagccgcccctttctctctttttacagcctcgtggacggacgaaagaagggaagttacagaacggggcagtgaaggctcgcgaagtagacagcaagcagcaagcaacagcttctcagccccctaacctttctcttttttaataatactttttttatcaggtaagctttgaagctggctgctctgctatactatactagttgtagggcgctagcgcttgactaatataatagaaagtaaagggactctattatgatcttacgaatctaaagatctcaaaatggaagaacgagctcttttgctcgcccctatctctaaaggggcgtaagcacttcactcgctaggggatgggattcattcacttgcattcctgctagcactacaaaaagctccggtcttaacgcccctactactgctgtgcagcctttcctcgggttcgtagagtcgggtttcccgtttacccacaacggaggagccgcccccaccaggcaggcggccacgggtcataacgcactcttcgcacaacaaatccactttgaagttgacttattcgctcggccaatcgtcggaatgtgtacgagataccataagggcccaatatctcaatagcacctttgtctaaagcttcgaaggagacttcatatccgaaacgcaggaacgatctgactagaaagtcattcaaaacttgatcgaaaaaccagcgtttattgaagaagctatagagtcgattactaatagtactagtttgaaaggctcgttggaattgatccgctacgggattaacattatacgcaacataagcacctgaagtactaaacagaataggtattagtttggtaatggttggagcagcaaactcggattcggcaagaatctcattttttggtagtacgaagggggaattggcccaaaaattggatgggggtcaagacgctgtcgggcgccggcggctgactcaagtgccccccgaaccgcgcgaaatggtcgcctattacacggctcactaactctgcctggggtgtgggtacctattattcgtcggcggtccggcgcacccctactatacaaagccgcccccccaactcacttaaaggatgctggttaattacgaaggaaattctttcttaatcgagggacttccttttcgttaagcgcatcgaaccaggagtggacattatcatcatctgcagaaaaatccagattctctttcatcattagcgaaagtggaatagtatgactggctttccggaaaataagacgaaacccgctttatcgatatgataaacatgcgctcaaaaagacctcctaaacccccctgccaagcgatcgagtttagtctgaatttgctctagaagtagctcccgctccagactgacttcaaggaaagaaagggttgggcaattccgccggttctggagcttaccttattattaaggggaaagggattttttatagatgttgaggtgagtaagggggggcgtagcttgaggcttctcagccgcaggaacagggaacgaatcctccaaaaatggaatgagttcgcaattaataccacaagaaagccgccaccctcgccctttagagataggggcgcaacaaaaagtattcaaaaagggcgccggaggcctcaaactcatccggagttggagaatgaaataaaaaaaaaaagattctcaagaggaatgtatcaacaaaactgcccttccatatagatcgtcgtggcatgaactttgtcaatagattcctagcttcctattgatcttgattagttctagcttcgttttttttgttgagagttatctttctggaccggacccacttttataccgtctcctgaaacacctgcttatcctgcatgtgctttcggggcccccactcaaaaaatcacttgcttgtgattgcagccattccccgaaaagggggagggtggatgtaattcagctcgaacgaagtgagaggggtaatagactattaccgttcagttcatgtgacgaaccgaacatcgttaggtcccgaattctgcgaagcaccggatctagatcaagatctccattacgtcgtacgatatatcgatccggagaacttactttcagtttaagtcatccattctgctcctatctaaagtgatgctaggctgcttcacagaggtgcgcttcgctcgaccacatgatgaacatgttttaagctaactgcatgtcgagcgcttaagcggagcttgtggtcactcgttcctcgcttgttcgaaagagcttcagattggattctacactacatacgatattccattccggccctcactagctctttgcttgcttgtacaaagagcatgcccgagggggctactacgctcaccgcgcacttgcattaccacctgagcttcgctaccgttccgcccagctcctacgcctaccacgaacttgaatcatcacatggctgctaaagcaagctaagcttcacacggccctgaggaagccaaaagaccctctcacggccgaaggctccgcaacacgttggagagcttttagatcccgccctaaaacgcccattcccctagagttccgaagtgattctcattctcaccgcagccttcttaagccgaaagaaagccgggcaagaatctcatggtagtacgaagggggagcggaatcgtatctgggagtggttcttcggatcgatcacagattctcggccccgtcctttggcttccactccagttgacctctcttctttccatcccaccgtgagaaggtagagagcaaaaccaacccagcaaacaactatgactatgcccctattagtaaagcatgtacttcttgcaaggcttgctgagcttcttcatgtgacagacatcgcaaaagtagtccgttgaacgatcgccgatcgagggcatcgtaatagtatactatttttgaaccctgatgggtttcgcagtcgaccatttgatagccctgttcctgaatatacacagaatagggcttcgatgagccctagatgtaaaggggttcttgaacccttctaagcaattagaagagcgcggaattggacctccctcaaatagatggatctgggattgattgtggaaccgagcatagagaaccgggggcgggcaggaagataggctaggcggagtagtcgctctggagcaggttcttcgactggatcaatgcatgtatgaaccctaaaaaaatcccgaaggtctagtctagaaaaaacccggattttgttgggttagctttttggtaggaaaggcggtcacaggaagaaatgccctaccaatgaatagattagtctactaacgtcaacaatctctttcttcatatacgagaccgtctgcttttatatcctaaactatagatatgaaacaaaaaagaaagaaaggaaaacaggcagggaggtaagagcgagtaagactaggttatagcaagacaacagaggttagatagctcttaccggaggaagagggttcaggtcacccgtccccttgacccagacacgaactaatccttctctctctcgaatgtatgcccggttttcgtcgaatctttttgatcaccttcaaaaacaaaccggaattccgtcttgacatgataaatagtgatgcccacctgcagagcgtagccctccctgcagccttgaagtagactatttttcgagtctgatcttatccccaaagcctttttgcaaaaggagtaggtagcgagatagatgactaaaagctgatgatctttgcctcttactagtaaagggaaaagccctatatatctgattagtcaagcctaaaggccctttactaatataatagaaggtaagaccggctttcgcgcagctgctgcgcccttgcttcttgcccatagagagttaggatattttgtgagctccttcgcctagcggaaacctccgcttttcggccgtaatcccgtgctttaccaacgcattcaatggattccaccatgaaccgggagcgggcgaagacatgcagcttccattttcggggtacacagtcacgtgctgagcaaagaggtatatatcacactcattcacaagcgcaaggtgcggcatccgcctgaacggggagaggatttccctaaaacaaagataggcgtgtcaggaaagaatgtgaagtcacccctatttcgctgtccagggagctgttgactaatgacctaaaaaatgcgtgacgtttgggaagcatgagcaacccttcgcgcacgagatagcaatgacaggagattgaccggtcggggtcgagtgatctcaggggtttaggggtgcttctcctgctgcgactacctctctattttcaaaagtatatagaaatggtaggcactgggagtgagtgaactacccggggagaaaggggcaacctctctatagaagggaagggaaagggttctccgctcataatgattgtagagtctctcggggttggaggtctaatagtagtcacatcaagtcctccccctcttactcagaatagctagcgagaggaagactactgattatctatgaaagaaggcttttaagaatgaaaaaaatcttatcttaaggatagagagccccccgcctgcgttttcagatacgagtgagtgagcgctttttctgctatgaatgaatgacctctccatttattttcaagcttgctcttcaaaccggcctatcgctctcctctatgaaaaggttcttccgtaatcactctcaataagacatccattcccctttcaaatgaaaagagaactagacttttctcttcatcattgaaatccgccattcaatcgcagtgcggtgctctcaaaaggctcaatcctctaaggctgaaacgaataggtcaggaattcgacctgggatccgcccgttccgatccttgcctactaaacagttgcacccccggatatgtatgttgggagaaccccatgatccttccgtgtggaagggaaggaagaaagaaggcgaacacgaatactaaaaagcggttcatggggaccccccaaaaaggggatagagagcgcggaacgggctttccaagcataaaacaatccctacctatacattccatggcaacagacagaaggcagttttgtcgttgttcttaaccccaggcacatttccgttcccaataatctccatgaaaagactaccatgatttccgaacgaaccgagggagagtcgaggcatgaaaaaacttatctatgatctgcttatttccaagtacgtatcatccgctgccttatccgccgtctctgcggccgccaaaagcctaccctctctcggatattgagtgggttgaccggggaagagatccggacgaaccttccaacaagcagaatagaagttgaccacaaggccatctctgtgggaggctgctacccataaggccatctcgggcatgggaaagaaaggcggcggacaaccgacttaactggagagcctaaacggcatagaggatgagtccaccggtcgacaaacggcttctatctacaggtgctttcattatggatcggtcgacttgtcacgattgattgctcacacacaattaggttaggcaggcttggggaggtgatctgaatcgctatcgatacgatgcggggctgatttgctgaccgtaacgaacttgactctgcccctgaaaaaaaagggcgggaagacctttgacctgggctggggagggattggggtcgcttttctttaggactttagtccgtaacaaggctcgaagacctccggctggatttgaaatggatcaggtagggcatccgtttacgacgtgggtgggattagcagttttctctattttcttcaatggtaggaaatacgcatcagcgggggtatatgggaggaaaccagtctgcagtaattcaaattgctccttcggatcactaagtaaaatcttgactcacacataccgcggtgtattgttgtcaactcacatagtcgcacctaccagcaacaagacgactactccctgcacgccactaaacggcgctatttaacgcttgggttcgcccaatacaagaactacagcccaacctagcttaaggctaaagccgtggactacacccccgtgagagccctctattttactaacatactcccttttgatctcccccataccttcatatcaaagctgggaatgattgactttcggattaaaataatagcgcataatggcagtactccttcccatttcttcttttatgatcttatctacttgaaatgcttacctgtaagtgcggagaaggtacccaggggaccaaacgaaagggcactgaaaggtcttcaattaaagcttcgccagtacttgaaagactcgaaagacctacttgatgagtttccttatgagtgagttcgtaggtgcctttaagtcgagtgtagcgaagggattctcctaagagaagctttagcccttgaacctgaaacgacttttatgagctgtctcagtagtgaccgactttattttattagctgtatgattagtggcttagctcttagctgtctaaaagctacggtaaaaaaaatcccttttgaaaataaaccactaatccgccttaggtactcttttaagtccgtgtaaggcggagggaatgaagggacctgcaggaggctgaaaagccgtagtgcgctagcgctagcgagttagcgcaacaacttagtgtcttgttttcttcgctgctttttttgtccgcaggaaagcggttgctaaggcttgtagcttgcttctgtccttagtcaattttggactgaagctgttctgactgccgtatcttttttgaaccgaataccttcctctgtcatctctggtctgtctctttttgagagaagattttctaccccgcctgcctatgaagaacttcaagtctatcgggaaaggatgtggtggtaacccccgcagctttgtctagaaccgggcgtccagccgtgtaggaagactcaccctagccactatagcgaccccacccccaaccctagctgagaagcaccctyvdgccactcccdthtttccgtgtgcccaaaagcccgcccgcccggtttttgagaccctttctgattccctcacccaatctcatgagaagcaagcccagcaggccctgccttaacctgtcctcagacagccagccctcaccaggctgctggcattgctaaatgctccgccacgaagcaagctttcccgaatacgacagatgcggaagtggctaaagaagtcggaggaagaaagttgttggacaactgtatacacgagggtacattagtattctgggaattggcaacattgacagaaagggtaaggggtaggaagaaacttttttaggtcttgctctactaaagtagtcggcctaaccttcggttcccgtaaccaagtttttctttctcactccttatgtacttttttttacttcatccatacttttttactttttctgaagtgtggggcaaacggcgccctctacttctacttctaactaaaggcgaacagccggcattgcaagcaaatagaaagcccccgcccgtttgagccggaaagcgtaccggctgtttgagtcgcgaaagggccgcttgcttaatattatttatataataataatagatagataatattatattatataactatctataaagataaataaaaaactacagaaaatacttttttttttataaaattcttcattcctgggaagaggaagaagcagatagggcaaaggccttctctttccgtccgctcttcccgaagtgagcgaattgcatgtagagatccgtaggggcttatagtttaattggttgaaacgtaccgctcataacggtgatattgtaggttcgagccctactaagcctaccacccccttctcttcacctgatacaaggcagtcgaagtacccgccaccctgcagatctcaatctagcgacggcatctggaaccacactgctgccgctgcccttcgggcacgcctcctatgcttatcactcacctacgctcttgcagcatgcccccttcgggcaatacggtgtaatacgcgaagcagctgagccatagctcttcgatcgctatattcttgcggcgtggttcatcctctaagagagagtagatgcgaaggttcggatcgaagatcttcgcgagacagccccggggcaccatagcatgtcgggaataagggggacatagtgaacactcccttggttgggggctgtgactcccctatcctttcaattttttgattcccaggtcttttttattatcactgttggaatcttttttaagacgacttggtcagggcggttcacaatttctttgctgaaggcgctgttaagccctaagtttgaattcaaatttcattgcccttcttccgaaagtctaaagtccttcaaattttcaccaattccgacctacctttatttatgggatatttgaaggagagctttgtaactgtttctagaaaattctctctagctcgaagaatttgtttgattctccctataaaaatagttaaggaaaaaggggcgcttttgttaaaggactaactattgtagagaagatctccttggctcacgaggtggctttaagtgataggggattttaacctaaagacaacataggagggaggggggtcaaaagaaagtcaggatatggcaaaagcatctttttggatcgaatgggcttttgtgataaatggcggaatttgatacatggatgtttatgtaatgaagactttggagtgcttgtggatggtgtgccacatgggtactttccagcttctcgagggctgcgacaagggttccaaacctagcctgttgattttagctgaagaagtgctaagccgggacttggtatcattgaaaatgataacatcttaccatgcttcgagatcgtgcccagcactctcctactttctctttgataacgatgttctaatattatataatagccataaacggaatcttaagaagcagaaaatctttctggaaagaagtaagaagctgattgtaatgttgtaatggccaaaaggtcaatttcgataagagccagtgcttcctctcgaacagagctcctcgcagaaattccagatcattgaagaggaatcaaaaaaggtagttttcctatcaagtacctggaagttttcttgtccctcaagagaataaagagagaaccttcctctactggagaaaatgaaaaagagaatctcagattggaaaagtaaattgttgtcctccggaggtcgactaaggcttattaaacatgttatagtcttcctatgcacatgtgcaagttttttccttaattagccggcccacacttcggctactaataatgggataagaccttactactatataggatatgttaccctctctccagtgagtgcagtgaaggactctcgcctcacccgcccgtttgacttatggcatcatcgacttgcttttcaatcaaagcgatttcataaccataaagaaagacctctccttcgggatcagtcccgtccctagatgtagtagtcaatcagcgggacattcaaagaagctatgcaccttcactgaatgttaatgaaagaaagccctttcatcctaatctcatctactgaaaagggggccgggcgtagcacgttcttttttgggacacataggctattacagacgcatcaaaaaagacttttcgaagcgcggaatccctgaatggaatcattgcagaagaaaggtataacggttgggaaccggaacaggattaagcctttaagcatgcagatgagtgtttgctgtcagccccaatccttcggtttccggattggaataaggagttccatgttcatactgacgcatcactctatgccattggatgtatgttggcgcaagaagggccgcttgatcactccatctacttttaaagtatacgactttccgctttggaattatagaaccaccgaaccttctttatcatgattcgacccatacctcagacccaagatcgagcaccagagctgctcataacaaggtaccaaaaagaagaatgcgagaagttcatattctccagattcgactataaaccaggtagtgaggatgaaaaaaagcataagctacctcgttcgtgctcccgtctttctcgctgccatcttcggtggatgcgccccttcacttaaaggcggccaaaccaacccactgagccaaccttttagattgaaaaaagttactaagctagtcacctcacctctctttcttacccgcccttattagtagtaggcaacctttctttctcgcctttcttccagctttttccagataaagatctaatagagttgcgctttcttagtacattgcctttcattaccaatctgtcgttttacagcacgaagttacctgatgttcgctactactaataagggcggagagatgttaacctttcgctattagtaagcactcccctagttttgacctaatgagctttctttacgttgagttaattaacccggcgggttcgcctagatgcctagtaaagaacgagctggtgggaaagagctggagatcatgaaaaagatttccacacaaggaggcaggcgaccgggaagctttgcttctcgaatgccgactacatgggaacagatgttatataggttgattctcattcttgctgcccgctcgattccgaggaataaagggagggctttaccacaatttcccaagtaagagatagaatctcactaattggaaggaaaaggagggcttcgatccattgtgattcgctttcttggtatggagagatctctgccataaaagagagagctcctaagccttattctgcagatcaaagagcgaggtaattccccattcatccgaaatagtcttttagtaaagaagagaggcattctgggccgactactacgactacatgcccatctagtgcagtggcttggaagcaagctaccttgaccatcttccgaagttctaaataatttactgatcaaaggctgtaagggcggactgctctacattcagccacaccacagtgaccccgaagcgatcttcttctagttgcgggacgaaatccgacagccaattgctggctctgaataaccagcccagcaataagctcaattcttccataacataagggggcgggcttgcgcgcgagccgaatgacgtaggtgcacaagagtacttcgcgccacaaccatctcctttttataggttctacggaccgatgcctgctgcttcatctgggagaaaagaatcatagatatgccggtcattagaaggaagaaccgccataaaaagattcctcgtgtatcatctgtagcaaaactatgaacgggagctagcaatccggaccgtattgaaaaggttcctgagacacagcatggaaaagtaacaatattaagaaacgaggtccaagaatgaagaaggggttgaattactgaatgaatacgagctgtggctaatacccgaggcataaaagaagcattttctacgggatcccgaaaccaccagccaccccgacctaattcatgataagcccaccaacttcctggcaaaatgcctacggttaaaaaccaccgacatgtcaagatccaaattcgaattggttcctggtcctggtcagagaccactgtgttcgcgccggcggtccaacaaagaggcgaagtagtggtatctttctttccattacgaacgacacgcttcgcctgctccctccccgtgtccactagcgctcctgtccagagcgaagagaaggcgaaaaagcgccgccgaagcagcataagcaggcttctattgctacgtaacaataaagcaggatagcattttgcgcccacatgtttgaatttgagggtaaagagctcgcttgttatacgggatccgacgcatccaacagagcgaaacagtgttccattcttttcggcggcatccttccgcattggcggcgagtggagtgccacaatcccattcatcatttttgatctacataagccaaagcccatagcactggcgacgtctccggcataaatgcaaggaggatgtatagctgatataggatcttgtggaacaggatttgattctgcaagcggttcagtacaaacgaagaaatttcgaacaaaagggtcggaactcgctgataggaaaggagagaaaaacaaagcaatgccaagagctccgtcaatccgctgttcatcgatagacgaagctctctctttatcatctcgtgccagatgcaacatcctttttccttctcgcgaaccacgggagcgcctagcgcccagaggagcaaagctcattttcctttcagggtaaagcggcgcataaaaaagggctggcccgtcaaaagtccggttccttcgcgaacgaagttcagaatcaacaagggttcgtagaacgaagggagtgtataactggggcgcagccccacttttttgttcgtaacgagggagagatagaatggagttcttcacgaagttcgaaacaaaggaataaaaaaaagtttctctatggcctcctcgttttgagacattatggcttaggggtcgaccccggtaacaaagaaggaatccataaaaacttaggatccaacaccatgataaaatactaccctcatgattagaccatgtccctgagatttgataaaagaaaggtgcattagcggttaatacgttgtaattggataagttattaggaatatgacggaacgaaagaccaaggaaagaaagaagaatacaccaaaatgcaagtgctgcaccaaagactggtggttgtttcttgttgtaagtgaatgcaacgaaaagacccggaaataacgaataatgaaacaattcatatattgacatttcgtgctcatttccaaatttatgctttgttattcccatcatccggtaaccacaggatgatccacaagaaaggtggcaggattcgaacctatggccggcctgcccctgacctgctgggttgggtggccgggttagcacccctcgtcgcctctgtacccgaaacagatgcgctgcgctacccagcgcctaaccttgtctcccctactcctcttctggttgtgccattaccaatcgcgggtaacccccggtccggccgcccctgacctaagaagaactattatccttatgaccaaacaaggaccagcttacttacttctcgagcgatagttccacgatcccgaccagcaacttcttgggagtaggggcatcaaagcttgcccaacctagtaaaggggcttggggatagagggttttctgggggagagaaagtttccaggttggattttttgagatcaaatagtactagttgggtagatagaggtggtgaaatctaacctttgcatcgatcttctttagcagggcgggtcgcttgagtgtcaaaaccaagcggtggttgtttttccttggcttatcgaaccagcgtatgcccattcctcctttgatgactcccagtagagaaagcctaaattttccgatgtggattgaaaggaagttggggatggacatagatccttccgcctatccggagtgttggaaatatagcaatgttttttgtatttttgatttcccgatcattggaagcaatcttcactggcacaaggatctcctcacagcaacctccactacgatagaaaccgacaatgagtttacgaaggcttcgagtagtgcgggataggctaatcaccagactgctctggaataggttaatcgctggagacaagaacgagtgaatctagtttcgagagcatgccttactctaatagggggcgtagagtttctaagtgaaggcaagcgctactatatatgtaatatcctagctgtcagcaaggcaggtccgctataaagcctaccggccagaaagtccttaagaacgagaaagccgactaaaaggctattccataaccgactcttgttgccgagtcgagggggcttggctggtaccaggctctaaaagagttttcttcgagcgagcggtctttctatctttttgggttgcatgcccaaggcaatgctttttgtagattgagatggattgatcttcgctatcgtgcctcctccttgtaccagttgatgctggggcagtgcttaattaatatgagttttctcctgccccagacagcttcgaggttcccatcgatcgattacagaggtttctaccactgaacttgcttatgctcccctttgatcgagtgctatttctataaataagattgagtaggaaaatgttgaattggcttcaatcgagattgcctcggcttcttaggcacatgaggaaccggcctaacatcttttcaatcgaaatcccaatcaaagacaagttctaccaaggccaggatctgaaagagaggattcactttccgaaattccaagtgacatgattcctccttcagaagctaaagttgaatgatcgaagtctcctttaggttcagtcgaagagatcgaagcgaagtcatcaattcaaccattcgaatggtctccccaaagattgacctcttttccaaataaaccgaacctcgataccagattcatcaaaaagatatggccatctctctaggttgcacaacccctttagatcgttctattcgtgcttgaaaaacgaccccatcggtccgctccttttaatggacattcttagccgtcctccgagggttaacaccccatagatcagatcgtgaactctttcagacccttagtttcacttggttggggcagagtttcagcctgccttccaccgaatataaaaaaccttagagctgcctaacctgctgacatcccggcgaagagagtcattatttgtgttacatcttcgaattcgagagaaggctttcctcttatctctcaaattataggcattgaagcgatcgagagaaagtaagaaaactattgcacacgccccccattcgccctttactaatataatagaaggtaaggcaaaagcaagagtgaaactacgagctaaaagcaggcgtgcctctcttataagagaatatgataccatcccccacttttggcgcacttctttgatgagctaagcctaagcgccatagaagtcaaaagctagcctgagacctaaaaaagcaaggtcgaaatccatccctctttttcctgtatttgactagtagggctaatgaacgaccctttgatctatgtcgttccaagttcagccaggtctgattagaagttcaaaaatgagtggagcgaggggctttagagggaaaaaagggggggcgagctttaattgaagtaggggcggagctcctcatagagagttagaaagcgtcagttctcatagcgaggcttaggccgacggggtagggcgcggccccccaattctcaaccccgacctagacaagtggttttttaacccacattttgaaaagttctgttaggttcttagtagcaatcggcgaccttttcctcttttacttcacatagcttttcgtctccttgatagctggaagttctccaaaagtatgaaaagctggaggactttgtaccatccattccggtgtggttggattctgttcaacagcccaaggacttggagcacatcttttgttctttccactgcttgaagtgattgttacgaccacgaagaaacgacaaatcccaactacggatatataagagccaaaactgctaagggcattccatccagcgtaagcatctggataatctggaatgcgacgtggcatacccgaaagccctaagaaatgcataggaaagaaggtcatattaaccccgaaaaaagtgatccaaaaatggatttgacctaaagtttcagggtatgtccgaccaaagattttacctacccaatagtgaaatcctgcaaataaagcaaaaacggctcccatagaaagtacataatggaaatgtgcaaccacataataagtatcatgtagagcaatgtctagcccagaattagccagaactattccagtgagtcctcctatggtgaacaaaaagatgaaccctacagcaaataacatgggtgttttgtattgtatcgaacccccccacatggtagcgatccaactaaagattttgattccagtggggacagctatgatcatggtagctgcggtgaagtaggcacgggtatcaacgtctaagcccacagtaaacatatgatgagcccaaacaagaaatccaagaacacctatactgatcatggcataaaccatgcctagatacccgaaaaccggttttcccgaaaaagtagaaacgatatgacttatgataccggatccaggcagaatgggaatatacacctctggatgaccgaagaaccaaaagagatgctggtataatatagggtccccccctccagcgggatcagaaaaggttgtattaaagtttcgatcggttaataacatggtaattgcccctgccagtaccggaagtgataataaaagtgggaatgctgtcactagaacggaccacacaaatagaggtgatctatgcatagtcattccaggtccacgcatgttgaagatagttgttataaaattaatagaacctaaaatggatgaaacaccagatagatgaagactagaaattgctaaatcaacagctcctccagaatggctggtaataccacttaagggcggatagaccgtccacccagtgccgctacccacttctactaaggctgggcttaataggagcaagagacttggaggcaacaaccagaatgaaatattatttaatcgtggaaatgccatgtcaggcgcacctatcagaatcggaacagaccaattaccagatccacctatcatcgccggcataaccataaaaaagatcattaaaaaagcgtgagccgttattaaaacattataaagttgatgattcccaccaagaatttgatcgccgggtcgtgctaattccatacgaatcagtactgagaagcatgtgcccatcactccagcaatggcaccgaagatgaaataaagagtccctatatccttgtggttagtggagaacagccatcggaccggatttgtcgtaaaattgagattatttcgtttccttccttatcagagaggggcccgcggggcttatttattgaaaannnnnnnrggggrgkgrggggggaaggaagaatggaaagccctcactttattgatgggacattttgatccccttttcctctcatcctcccccggttctggttcaggaaagggtcaacgcaaggatcttatttcgaagcaatctctggagttttcccttatccgaacgggtcttgcaagaaaataggatttcatattgagctccaaatatacgctattgggatgggatggctcctactagctctccccccctaagaaccgcacgtgcgagttcccccgcatacggctcaagtggcgaaggccctttccttcgcgcttggtaagcgcttcgctgtagccaagcttactgctagcctatcggctagagccaagcttcgaccgcgactgctcgtcgcttctggccgccttattccgtcacccgagatccaagtcagcaccggcaaagatctcttgattcctcgcggtcgggccggcttggaagcaagctacctcttgcctatctcacctccttccttcagctgggtgagccttcgctttttggatcgtcttctgcccaatgcggtaccccccgttttttggttcccattgggtttaccttgttcacaggtcgaccccatggcagcaagaaaaggcgatcttgtgctatactccggtgatctctttcctaccgagacacgcaaactcccatcgtgtcccagatcacattccgtgaatcgaaaggggaagcctactcatctatcagctcctctcgtagatcggtgtggttttacgaagcgtctaagcacagttcactcgcgttgatcaatcaagagggttgccgccactccttaaggttatctgttgtatcatacacttcttgcattctgtcccacgcttcatacctcctctttcttcttaaggtaagataaagggccaggcatggtggggtaggagcatccagtcggcaatctttttggcttgaccaagaagtcttatgtcctccgagtcgcacggcgttttaaccgaaagaacttcttgcgcaattcatgcctttctgtttttatgaccagaaattctttctttattttcatataaaattgttctctggactttttatcaatatgaggtgatcgtaacacagtatataagactcgtgattcaggcaatccaatcttccgtgtgtaaggcggaagcccccaaaaatggttttcaaaaaatgggtgatcaaaagatcgaattactatgcctatcttggtggtcgttacttttggtggtctttctttttggctgactcctatagacgaagtgcttcgtttcagatcaattcttcgctgcaatcgcttcgatccaccccctcggtgaaaaaccgtaatacgccctgaggaattcctaccagcagacttccctgtactcaaagtgaattgtctaagtgctctcctttgtctcattgtttatctcgtaatcattcgattccgcccctaaagctagcgcctactcctcctccttctcctcctgaatcctccttggtcctttttacataacactctcggccgcccaagaggactggctatctttctctttatacgcacaatatcttgaaaggcaaagaaaaagatctaccttggcaacgaagacgtcattgactgatagtttatcttccgaaccggttaaatacctataacaaaaaaaggccaaagcccgctgaagcactggaaaaatgttgaccacgatttctaacgcttttcaaaaaccatttgcttgcaacgccttgagtggacagataattacggccactagatccttcatactcttactaaagtacacttaagactcaaccaatcttgaaagtggagtggacaactggcataccttgaatctagcctgcaatcctttcgcacttctcttatcaaatttctagttagagagagagctaaccgctgccaaaatgcagcagtttttcttatatacgatagcaccccctgccctccttgttcaagtagttcaagagtgaaagggcgtagtgaaagaagggaaagatctctttcaaagatattctacccataaaggcagttctcttatatggcaatactagattggcgagacaagagagaaagcttataaagtagtaaggtgtctatggggcttgccttacaggtagtgactataccacttacatatcgaacagatcttactctcaatggagtcatttcgatatgacctaggaacttacagaataccgaacttggataatcggtagaagaatgattggctagatcatttgcttcactgcggaagaacccctttctacgctacgttcccaataaaaagccgtcatccttctgtcgcctgttagccacaccagaccaagaaaaggcaaactaatcaaccaagactcagtcacgacctttgtaacctcacggccactttctttcctagagcttgcagccattatcttcgcttttcagatatggtgacattacttgtatggggggaagtgccagatctttacggatcataagagcttgaggtacttgatgacacagaaggagttgaaccttcgccaggatggcacacttctattccggggacgagtatgtgttcctcaggacagtgacctgtgccatgatatcttggaggaggcgcatagctcaccttttttcctgcacccagggagcacgaagatgtacaggacgatccgcccacactattggtggaaaggtatgaagagggatgtcgctgagtatgtggctaaatgcttagtgtgccagctggttaaggctgagcaccagagaccagcaggacccttacagccagttcagataccacagtggaagtgggacgagatagccatggactttgtctctggattgccgaagactgcgaggcaacatgacgccatttgggtgattattgatcggctgaccaagtcagctcacttcctgccgatcagtatgacttactctacgggcaagctagcccagatatatattgatgagatagtgcgcctacacgggataccatcatccatagtatcagacagagatccacggttcacttcagccttgtggcagagcctacagaaggctttgggtagcagagtgagtcttagcacagccttccatcctcagaccgatggccagtctaagaggaccatccagacattggaggctatgcggaggtaatcccttgattttcgaggttgttgggacagacatctacccttggtggagttcgcctataacaagagttatcaggcgagtataggcatgccaccttttgaggcactctatggacgcaagtgcaggactcccctatgctgggatgaagtaggggagagacagattcttgggccagagattgtacaggagacctcttccttcggtccggttagtacaaggttctgtcgtttaccttgcgcctatctattcctttaagcttatatcttataccattgcaatcagactcattggatatcttccttttctcttctactatcgagagtcgtacgggtgaggaggtgagctctaagcgtatacacatagataggtctgggtaagcgaccatcagcggtatgggtagcagctactatcagtacgccagtctaaggctgttcgtagaggtaggtcgtagagatctatgaagggctatatttagcataaatagcatggttaattatagaatagcgtgatggccgtaagaagatcataaataaggtaaatagtctggagtggatgtctagatcagggtgtcggcatcacacatatagcatgtgtgccgtgagtgagagggtggtcgtagatcagccctcagctcttctttcgaaattctcgaacatgatgacttatcggcttgaggcttcttttcttttcaagctgagtagaaatttcataagagaagaaaagttcacagaaggttcttcaatagtatgcctggttcacgaggttctaccactgcagggcccagttgccattcccccattactcaagtcgtccaagggacaggacccccgcactgtaaaaagtttcctttttatacaactcatgatatctttcttctgtgcatatctcggttttaataacttctgggtttataccaaatcgaccgtagagagagttcattagtatcttgtagatatataccatagctgcatcatcctttatctttgcttcttgtcttctagcgaagatgtctgatacaaagccttcgaaaggactcttctttttctcatacaagtagccccttagcgggaaaattctataacccaagtttcgggcataaaaaaattcttcgctaaaatagacgcctacgaatttacctgttgggaaggttaaagcattatgtctatccttatagggtaagaaggctttctctattgtagagaggacacactacaaaagcctcaataaagccaaagaagttatccaattccgccttttctaaattattatgccagacgggtacaccccctggcatcggataagttttcattataaatggatataaggagttcacatcgtaatagtctaaattttcaccatagggcttatagacatcggcatgtcctccataataaccacgccgaatgaagcgttcttggtttcgagttggtatatggatgggccaactctttgggtcgtaatagtgcatacgaaagattgatagagctagcgatgacaacgttattgtatcaacgatgtctattttgtacagattccaataaatctcttgtgccttcagcataacgccacctaagagacgaatatcttgtttcagataagccaacaattgttgacctatctccggaagatactcaagtcgtaatttctcatagggaatggtgcctttagaacccaatttcgggcataaatcctgggccaagttatttagcgcagcggcaaggagaaggtaggaatcccttatacggaacaataatttctttttttcatttccacgatagacttttaactcgtacattttatgcttcctcatcaccgtttggaaggagtacttgccgatctgagaaggaaaagctctcgttactataatgccatcgtatcgtgaaaagttatggaaatagaccgttcgaatttctttttcatctgataccacagccgctaaacgttctataaagtcgagcatcatacgttcacttcgttttttgaaatcagatattgagaaatccttatcttcactgaaatatgtttcaatataatattcagacttggaagcaagatcttcacccggcttaaccactaagaaccccactgcgcaaggaacatgaacatcgtcgtggagagcagcctctatatcggcaacaatgaatgggctcctttttattttattaattgctttcagtgcgggtatatgatcgggacgacgactcttcttacccatagctaccacttctacaggttcatcactcattgtcccgccatccgttaattcatcacaaagttgcttaaaaatttcctctaggctaaaagggtggacttcacggtgttcaaccctatcgaagagatagattcgaacccctactcggtctagctgcccctcttcgtatttctcagccttttcacagacttgtttcaaaatttcattatatacacgaagcgggggtacttctgcgttatcggcctttactaaaattgcatttcctgctgtaaagtcggctcgttcgttatttgtatgtatcagaccataatggatagtgaatttaatagaacgaaatccgctattgtatgcatattttattaacagtatcattaccgctaatgagataacttcaatttcgacacatttaaggtaaggttttttaaagcggaattctgctattcttattgactcaagggggctatgatatttttcctcagcgatcaacttgtagagaaatccagactggaactattgatgattctacgttagctctaaagtaaggagaccacttaaaaaccctcatcggataagaaaagatataccagatagagcttccctttgaggcatgcctgagagcaaagatagatgcactctcttccgaagcggattccgcgcttataccttctccggagacagctgactcggactccgttcctgccttctgactttcaataaccatgcgcgtactttaattaggaatgaaccaaagagttaccttagtatagagaaatggaagccagggtcttctataaataataagtatttcacctaggtgactcgttcacctatcacgaataaataggtgggtggctgcgtaatagaatagaacctgctgaaactacctcatccagggaagctgcccggatttccttaagttaagtctttttctgagctgtcttacttaaggtgttaccagtctttaccctctttgtatggcgctaaagcgactagtctatgacccaattccggatggcgtctcagggtccctgctcacctatcctatttattggaggtagcagccacaactgaacgctttcaagcacagtttcattacgtgatattgagttctttcagctctaacagagctaagacttcggtttcatcaatcctgtttcgggatcgaattcgaactggtccaatccacgtactccatcgcaactggttaaactctcatgatcgatgtaattgagagaaatgccaccagagctcatatccggcaatggaggattgaactttcaaagaactcctaattcgaataggaaatgcctggcaaaggaagaatagttcattggacaaggtcgcgtaagctgaaaggtcagcagagtcaacaactacatcggaagctttttcccgaagaggtctttaagtgctcgaacgaatgtgagaggagtgaatgtgggaagtgaaaataaatcctctaagaattccctctccttgctcgcagcaagtattacgctcgctggatagacctatttctctctttataatcagcaagggcctcagcgtattgaatggccgtcctgaggtcagggatatcatcgccaccatttcgttgcgagcccaatctttcaaccctcttatgaaatagaacactttttccttctcagttacatcatccacatgagcaagattatcaaggtactccttgatatattcttttatggtgccagtatgctttgtatcaacaaagcgcattttagcctcaaagtaagccgttttcggatagaactgcttcttaagctcacgctttcactcgccccaatccacgatagggtcggctatgccttcatcagcatccattttcaatctacgccaccatgacgctgcgccatcttgcagccaatatgtggcttgtttgattttcaagaggtcatcctctatgttttgcccctcaaagaattgctcgcatccccaacgcatcaatctctcgggcatcccttgcgcctttatatggcttgggcttgggtgcctccagcttgttttgagccacagaaatggtggtagagcctttggttaggcctagcaccgtggtcttcaaaagaccaagctcattctcagctgccgtcaaccgattcaaggcttcagtcaaatcagccctcagagagttattctcagccactaacgagttaatcctcccagtgagagattcatttccctcggtcacagttttgccaagctcttcaacagtctttcccaaggtcttcaagtcatcctccacgtcggagactcggtcttcaaccttttcctcttctttcttctcgttcttgggactctatttaggattgattgattcccgttaggtggattggttgctgcgcagctaactaccaaccccgaaattacgtacagagaaagggcttgtggaactacctttcttcatggtcaggattcactgctacggcgggtagcctggatctcatggattagccagaacagtggagaagcaaggacctgctagctacatcttcagtctgtagtgactcattcatcgggagcggagggaattgcttccccgtgggtcgtaaattgaatatgcagaaaccctgacttcctgtcttctcacagctctttatccatcatgctagcgaaaaaagtgaaagtgcgacgggctcctccatgagaaaagggattccttagtatataggatatgtcctttaagttggaagattggaaacccttgggcgtccttcggactttagttagcatcgagccctctttttaggaagaataggaaaagagtttcaatattgaaacagcattggataaaggaagtcttcgttcattcaacggcattaccgaccggcctaggctcttcgggagcagagaataggataggctgctggtaggactggcttgttgggataggtcaggcaaattcctctagtggaaggaatatgcccatagagaaaaagcctattagtaagtaagatcgaaagagcagggacagctagccctactccttctccttctcttactaatgttaaatcattcccttccttctttgctcttcgaatggcgcttgccttgcattctatgcatcttatttactactagatgtaatttccttgtccgattcaaggccatcaccagattcaatagccggggattccttctttcgatccatgtcatctggcatactagctctgacgacgagtcttctgttaattattaattaaatctctcctgcgaatccttatccttcaaaaagcttcttctcgacgcaggagattcgtgaacaagcccatctaagagcctagcaagcagcctttagtgcgacagagagagcttccaacaatacaataaaagatctatcccatctcgtgccctgtaagaaggaacttcatcagtcccagagcctattcgacgtcatcttccctgtcctcttccgattcaacctcatattactcgtacaacaactatggcaaccaagagctcggagtcgacaataggaattaaagcatcatcaaaatgaagagtgagcactttttgtgacggaattccttcgttccctttctcaaatgcaataggaagatagcctttttttcgtaatagaagaaagctctcgtcttcttctagggctgtcaggaagtctcgttctttgttctttacaattagaagctcttcctttaattacaggaccagaacaatctaagaagaagaggaaaaggggctaaggttgataggtagataggttacgtagctcaacgaaagcatatacataatatcttttcttttctcttgcctacaaagtttttggcggtatatcgtatataaagaagatcacggttttaggagtgatcttttcttttcctctcactcgaaatatcataagagaacagaaaggttttgattcgaggtttctagccgtcttcactgactggaacccaaaccaaataaagcaatggcgtctgtttacgtcagggtccgaaggaacgaagtgctcgaccggaagggaagtagtatgtccggttcactaggttctaccactgcagggctcaatcatgctagttgggctatatgcttaacacatgcaagtcgaatgacgttttcttggaaacgggagtgaacgaaggaccaacgacgatgaaggaggagttggggaagacgcggggtagaggaattggtcaactcatcaggctcatgacctgaagattgcaggttcgaatcctgtccccgcctaatcagtggaacactgttcaccgggatagaaggccggtcccaacccgtctacaaaatggggctagtgttcagtcttggttggttccacctctttgcagggtgatgacaccagtagctgtggagcacagatgaccatttcttagactattgaattccaacttagagctccttctactctaaactactgtgtgcctatttggagcttttcacagtcaaagtcaaaggtttcttggtggcaagatcggcatgccttctagttgtagttgactttaagcgcacctgaactacccatagtcgtctatttacgggcttgcactcaatagtcaatcaattcgtttttccgctttctatcgcacgcttcaactatttgtttatatagtctaactaatggaaagtgcctatgaattagttccaagaaagcgtccgttcacgtcaggaatagaggccgttaaggatgtacttgcttttccttttttgcgtcgagattgggttggtgttcagtgtaccgcttgtctagcctatgctttgcaagcctacatagggtacaagatcgaaaagaatgcattggatggatgcccgggcattgagaaggaaggacgctttcagaggcgaaaggccatggggagataccgtctgtgatccatggatctccgatcgggaaaccgtatccaagctccgtggctagtctgcgctctttggacttttcaaacttagcgaactgaaacatcttagtagctaaaggaagggaaatcaaccgagaccccgttagtagcggcgagcgagagcggattgggggtttgaagaaaaacaaagacgaagcttcgttcctcagcaaagtgttcacttctttttcgccaggtttcattcgatttgttgtggattggatgatggaaaaaccagcaagctacggcttcaaagcttaccttatttagaaaaggggaaagggcttttttatagatgttgaggttgagtaaggggggcggagcttgaagagcgaagcgagccgcgctagcctagcaacgtttttcagcagcaagctacggtctaacgaccccctaacctaggttggggcgaaaactccaaaatccaaaacgttggttagggttccaaacctttctctaagaataaggtaagctttcaagccgccgccctttaaaggagcgggcgcagtgaactgtaattgtgaaaagattggaagatctggccaaagaaggtgatagccctgtagattcgttcccatggttcgatccttcccagtaaaacgcggcgtgttcgaattctgatcgcttttacgcgagaaagggggaccaccctctaagcctaagtattcctcaatgaccgatagcgtacaagtaccgtgagggaaaggtgaaaagaaccctatttagggagtgcaatagagaacctgagatccgatgcgaacaatcagtcgaaggagcggagcttagagcctttactttatgtaaagcgcactcactctaacggcgtaccttttgcatgatgggtcagcgaggaaatgggaacagcggcttaagccattaggtgtaggcgctttccagaggtggaatcttctagttcttcctatttgacccgaaaccgatcgatctagccatgagcaggttgaagagagctctaacaggccttggaggaccgaacccacgtatgtggcaaaatacggggatgacttgtggctaggggtgaaaggccaaccaagatcggatatagctggttttccgcgaaatctatttcagtagagcgtatgatgtcgatggcccgaggtagagcactcaatgggctagggtggccccatttcgccttaccaaccccagggaaactccgaatacaggcctagatcgtttgtacagacagactttttgggtgctaagatccaaagtcgagagggaaacagcccagatcgtacgctaaggtccctaagcaatcacttagtggaaaaggaagtgatcgagcgatgacaaccaggaggtgggcttggaagcagccatcctttgaagaaagcgtaatagctcactggtctagctccatggcaccgaaaatgtatcagggctcaagtgattcaccgaagcgacgagaccttgaaagctgctttttcaagtgtcagtagcggaacgttctgtcaatcggggaaggtttttggtgacaagacctggagatatcagaagtgagaatgctgacatgagtaacgaaaaatcctgtgaaaaacacgatcgcctgccagtggaaggttttctgcgttcagtcaatctacgcagagtgaatcggtccctaaggaacccccgaaagggctgccgtccgatgggtacacgaaagtgacgaagttgctttgactacagaaccatgcctgtctgttggagcgaattggatgatcgggccgagggctgccccctcttcccctcactctcctttccctaatatgaaccttgagtcatcaaagcctttctgactcggcctggcccggtcgccctacgcgactggcgcttcaaaaggcgaaactctcggtcgtagtttggcgacctatcttcagtaggggcctttagtcttttgattagagtaggggtcgcgagagagcagagcgtaccgccctgccatagtcacgagtctgtttatagtcgcgactgttgtcatagtcaacaaggttgaaacttccaggaaaaaacttcgaattgggagggcgatcctcccggtgaactgaccgtaccccaaaccgacacaggtgaacaagtagagtatactagggcgcttgagagaaccatgtcgaaggaactcggcaaaatgaccccgtaacttcgggagaaggggtgctctcctatcttttgattaggaaagcggcacataccagggggtagcgactgtttattaaaaacacaggactctgctaagtggtaacacgatgtatagagtctgacacctgcccggtgctggaaggtcggaaggagaagtgttataagctttgaatggaagccccggtaaacggcggcagtaactctaactgtcctaaggtagcgaaattccttgtcgcataagtagcgacctgcacgaatggtgtaacgactgccccgctgtctccgacatggacccggtgaaattgaattctccgtgaagatgcggagtaccaacggctagacggtaagaccccgtgcaccttaactatagcttcgcagtgacaaccttaatcgaatgtgtaggataggtgggaggtggtgacacacaacgaccaatcctgaaagaccactctttcgtctaaggatgcctaaccgccgcaccgatcattcggggggaggcgggacactgcgaggtgggtagtttatctggggcggatgcctcctaaagagtaacggaggtgtgcgaaggtaggctcaagctaagattctgctcgtgagcgtaatggtataagcctgcctgactgtgagaccgactggtcgaacagagacgaaagtcggccatagtgatccgggagtcccgtgtggaagggctctcgctcaacggatcaaaggtacgccggggataacaggctgatgactcccaagagctcttatcgacggagtcgtttggcacctcgatgtcgactcatcacatcctggggttgaagaaggtcccaagggttcggttgttcgccgattcaagtggtacgtgagttgggtttagaacgtcgtgagacagttcggttcctatctaccgttggtgttaaagggagaactgcgaggagccaaccctagtacgagaggactgggttgggctaacctatggtgtaccggttgttatgccaatagcagcgccgggcagctaagttggtatggaagaactgctgcgccgcgggaaatccttctctatacaagttctcggacgaggtttttgaacagaacttcgataggcgagaggtgtaagcaccgcgaggtgtgaagcgatctcgtactaaacgaaacgactttcactttccataacaaaaatgaaagaaagtcaacctattcctgaaattgcggtcagtctcgctacctctttagttgccgccccctacttgctcctttctctaataataaggtagccccaacctatacaagggggtcgttagaccgccgcttactaagcgctggttctatcccggccaagcaaccaaagccggggacctggcaaaataggaagcagaaaaccgcttataccgagttccccaacagcagcttagcttagtaacaacactctttctaccggcggcgtggccctgctggatgcatttgatcaatagaacacgaagaggaggaagaagaaaagaagctttgttatgaaaaagtttccatttctttcccaaataataagaacttttggtgctgtagtcacttttgcctttggacgttttctttttttcggggcagaaagaacgatcgcgcctagctggatccttctctttctcttttgtcttatacttatgattcgggcaaaagaaagaacaagaagaaaaaggagtgtggttcattttttcgttgagttcttcctcctttttctttttctttcccttctgcgcctactcatcatggacgggatttcttcctttctaggcctgaccctgggcctgaccacttcttttgtttcttatgtttcgtctggatccaatgaaagtgggaattcggctcctgaatcagggggtcctccccctttagaatccgagtcgagttcggcgtcacttaacacctttcgaaaccagatcgctgcggataatgaagccgatatatatcggcgcatacaaattttagaaaaccaggaatactacaaccttcctccccagaacagtcctggtgactacgaaaggctggttcgcgagaacttcgattcagccataaatgtcaatcattttcggacgatttttgatagggaatactttgaccttcgagtcttagagaggaagggcgtcgtacaagaccaactccaagatctaatgcttcgggaggagaatatttcacagattctagagaaatctccttattcgaacattaggaaagaagcctattactatcttgagcacaagctcaaccccgttagcgatccacgccatgcctttcagcgagacattcttgacaccagtctcgacttctttcaacgagatttgaatctgagaggcaaagattcaaccatttacaaggagtttaagacgtattttatggacgaatgattgggaggagtagtcttcttgacataaaaagtcaagagggcgaggcccctagcaatggggggaaaggggagtgggtaagggggcccctttcacttgactgcttagttaggagtgatcttttttcatctccactctttttcctattcaataagagagcaactacgattgcgacaaccatcgcatagctattcagagttgcactcggagacttacgattcctcgaactcgctgaacactttctatatctatctgtcttcatcgaatttccgctatctgtcttgagttagacaagcacaggcctatcttagctcccggtgaccggcttcgcgagaccttttcgctccacactggagaagtcctctctcgggctaggctctattgggcggaggatcacctttctttactagaggagcaggaaagaagagacttacatacgtaattctagaggtgaaccagcttggtcggtagaattttttcgaatctagcaaaaggaaggaaatgatgcttttcttaaggcaatccataagtcagaaatagaatgaggaagagagaggaccccacggaatggtatgtgggccctcctcaagcaatcccctatgactcaacctttgttcttgtgcaaaagcgtcctccccttccttcctgtttttcgagctcactaaggcaagcggcgccccatttgtgtctgtctgcgatcgtgcctagctgggcagttcatcaggagctgctatctgggaccaagcactaagcactcttgattttctttcttaattggtttctaacaggattggcaaatgtcactgtgcgtaacacatctaattggaagtggaatgaagataatgcgcttgactctttcatttgtagctggattaccccttgttgggttgggctaacttaacttgaatctgttctgtttagtttttcactaagcctcatctgagtgctatatacatagctccttgattacttatcaaataaaatgaacattctttaagaactttttctcccgatcttattagcttagtagcatggaagtcacaatagttgtagcagagtaagctagaagatgaccaatcccgccccatcatgattggtgtcgagtccattgtgagaggcgcttaaaaggccgttaaggcattagactcaggggtgaacccacaggggaggggagaggttgcttcctatcctaaaaacaactggctttggctcgttgcctttgattccttacccatagcataagataaagggtgcgtgcttcaacatctaagtttcacacaaggaacctcctgctcttaaggataaactacgatatttgatggactgacaggtcagccacgtaatttatccctcaagctgaacgaacttgacctgctcctttatttagtttagggctatagagtttacttgcttctcactaagggcagaatcatgagcttcatcactcgactctaaaccaaattaaaaagactcggctataggatgacaatccttcactccggaagggtaggttccataccgacaagacctcctatcccagaatccgctcatttcacaccaactaaagcggaacttaatcaccaaggtagagttgtataaaaccctaatgtaactgaacgaagtggaaaacccgcaatacgagagcaaaaaccttctgtgtgtaagaagaaaagcaacatcgagttaggtaggatgtagatcgagcgcaataagctacaggagttattatttcgctttggaaggaaaaaagcatctcaaacaatttcattgcctcactcagctctcaggctgtctgggaatagctccaccagacatagaagaaaggagtataggattggtaagctttgccggaaagaagctactcgactaattcaggaggctactaccggcgaagcccgcttgcttcggagcgtgctattgcgtgaagcggaaagggacagcggaatctaagaccacaccagacagggaaaaggaggattagatatttcgtcaaccaccacttgagcgcgattcgcttatctgttgaaaagtaccatccagacagtaaacctttagggcatatgactagtaaggtaaatcaacctatcgtatcgacgagatgcaacagaatcaattaccagacggactggctttccaatttctctgtcctaacagcgttcgaagcctaacatccttgcaagctttggattctttcctatctctgaccgggaaagaggttaccaagcaagtgaaactgaagtgaaactgtactcgcctcttctccttcttgtcctcttgtacttccgttcttcttattctcgtatccggaaccggaacaagctcttctttagcagcctcgctttgttagcagtactagtttgtactctttattgacctggaacacaagctttaccagccaacccgatctgaccttcgaaactctcttctcatactcctcgttcgtcgttccaggcgtactccagttagctcttctcttacagagccttgtctgttcgattgctttcctagtcttcttcctgcttcattagataaagcgtcttcactaatagatagataggattgtttgcttcaaagtgtctttatatcaaataaaggcccttgaaaggggatgaaactcttattttaacgcccaaagataggcctctgcagccctttctaatgaagatgatgcataggaaaggtcctatcgaaaaggctgttgtcgtcatttttgctctttgcatcttccctgacccctcgtcactgctttctgatcatgtctcttttcgaatacgcgaaaggaaaggacaaagtgagggctgcttcttcgcgtcagtagttgaatatgaatgaaaacacagaaaatccaagtatggccctagcaacagttctaaaggcagttgaaagaccgtaagccaggcaagggttaggggcaagctcccataaaaaacttctaaaggagagagctccggaggcaaggcgaaaggcatgcactgggtaccgccgaaacgaatagctaacatagttatcccggtgattttgcccgaagagtttagggcagagtctgattatgctcctccaacagttcacgccaaacgttgtacttcacaaaaggtagaaaacaaagaaccaaatcctgagactagggtgatatgcccactctccagaaaaaagaagaggtggctcatgccggtgaaagaagcaaaaaaagaaaagtctgattcctgatccaaaaccggttttttgaatgaagttagaaagaagttctattgctccggaaggaaggcggtaggtgggcttagataagaaatctaggaattttttctatatatcaatccttcgataaagcaagagacgactataaaaaaaactgacttttccatttaccggaagaaacgtcgtcaaactgagcgtctgaataaaaggactcagtccccgtgaacggcctaatgtccgccgcctctagccgatgcgcactataatgagcaaaaatgctttcctttctccatacctcctaccctctgaacttcctggattgagctggtccaaagtgtttccggcaaagctaggaacgtgcgtcaaacctttcggccccgtgttaaccacataaaagagacgattcattctattccctcggttatatttgactaagacccagaggatatcctaaagtgggcattcgggctcatccctcccttcacggtcgcagtcctcttagccatagggttttcttgctcgcccgtaactcctctgttggcattggttcattttcggtatggctactgaggatttgattcaattcataaacgaagctcgcaggatctaaagtggagtctggctacaagtcgagttgaaatggaaagaaaaatggactcaacctctcaacgaaagagagacgcaggtcttttcacggcttcgttcgataaagcactcaaaccaacgagtaaggaaaggaggccttgagttgatatttaaaagaaggagttcgtcctggtgtgctgcttcctttcctgccactactttttgagtcaaaaagtcctctattggtttaattcatattcaagtttctctagcggaattagactttcatttctatttcttcaaatccagcatgacatgtgtcaagaagcgacccatcaaagaaaagttagaaaatcctgttttggcgaattcaatgtttccatatagatgaccttccctccggacaggaaatcatatattgaatagagggtactccacctctgtagaggatacaacacattgaaataaaggaattggtggatctctcccatcagacagatcaacggcaccgggcatgggatacacaggcaggagagccgatttgaccgcgcagaccaaatgagcgaaatttttttaaagcgaaagcgctgtgccaacttgcgtacaagatttatatgtggatttgatacaatagtcaaatcctcttcataagtcctttcttacaggctattcaaggtctattggctttcttgcttatgcggtacttcgaaggctaagcctcgtttatgcaccgagaaagatcgtcggtaggaaagctctgttatgcaccaacgacggccccttctctttacctttcccgtgccctacttcattcctttgctggcttgaattccatctcttttcttctttgtttgaaaatggcttcaattgatttctttcaggccctacttgaaaaggttgggttctctgtggggggtcgagccctctcctttgcattatgtaagttgggctgctccagctggattgcattagaaatcgcttttgctgtgcgtgggattgccggggaaccccccgatttggctcattctatgttgcctgggtcctctcaccaaccgcacgaacctcaagatgacgaagactcgccctcttcgagaaaaagaagaatggatgaggatcgagacggggatgtcggcccctcctcagtacgaagaagggtgggttccagagaggattgcgccaaccaaagctttgactctgagagtgagagttggcgtcaatctcacgccttgtcatcagataacaaagtagatttcgccccagaaccctccgcagcccggggcccccccttaggggaggccgaccaagagcaaggaacccccggcgccggcggcttaggcacttctgacgcgcggacggggaaagatcccttagaaagtcaacaatctttttctgcgagtgaaaaccctaaaaaaaaatgcgaagggatccttatgctcaattagttgaggacgcacaacaaaaaactatcaaaatccagggtgtaatagacgaattggaagaagaaacgtcttccatggacaatgtggatgagatcataaggaagttctcaaataagctaagaatccaaagttcctcttcctcctataaggaaggcgattcgccgacagaaccagaatgaaccgccgccgtgaaagaggtaagaaaagagtttgcaatgtcgagaatgaaacttatgatcttttagttgagggccccttcacttgagctaattccggctttccagcggaggctgcaaagcaaaggttaagatactaacccacggagcggtaggctaagcgggaaagggagagagtggagttagatccgatgccattgattctgttggaggaaggtcagcaggaaagagaattgcttttgttgaagaagcaacaataaaataagctcttgctcaccgaatccctttcaggtgcagatgaatatgctgtttagcttgggactagggcttatgatccttctcttaacggtagaacaaaaataacaaaggagctctcctaacctaagcaagccgcggagtcgtagaccattgctttaaagacgggatggaatctttctttctgatcctaagctgtgaactcatggtcaaatggcttccgaggtgggctttcccttctctatggtagtactgtgaaaacggagattgcttgtcctgctcgagccattaaggagggagctgagggagaggagtggctccttacgctgggaccccttggctctagttattggtcggcagagggtgcttgggatgaccgggattagtggattccttttttttatgcttttctttcgtttcggctttcctgcagctcttttcccgatctctttttcttcattaaatttacaagccgcagacatatagccagggagtgccatccctaaaaaagaaaaaaatcactcttttagagctatgacttacttagtttaatcctactagaagagcagtgagtgacctacattgagtaggaataaggcaatatcccctctaagcctaggagctcttggaggcattacccccatcacattggagttgacggtcccagtcttttctgtttgcgtaggagttcttcctcttgctccatcgaatgcactgagaaaagtagctgtgaggaataaagagcgtattctgtggcatttgattccattcttgctaacagctgattctatagattctcgaacagcgggtacgcaaacaagggcaccaacggatactgtcacaccggttacgagaacagctataagagtaggagggaattcaataccaattgaagttttctaagacatttgggatttgtcttgcaaacaagccttccctccctcacatctgattcaatagcactggtaattcctccaacaccatccaccgcggatacgatagatgattctatgccatcctcttcccttcttgtctatctccttcgatcagatagttctgcttccggtgccggaggaagggtagtttcagagttcgagatgtctgagcttgggggttccgcttctctaatgttataataaagctgcccagatcttgcgtcttcttttgctggctagatgcgtaagtcaaggttcacgcttgggcccttgacgagtactttgattttagttagaccataggtgctaaagggtataggaagatattacggaggagtgtcatacacatccatcggcaaatgcggatagagtagcagatcaaaatccggaagcaggggtgggaggatcatctgaccctagcatgatcctctaccggaccaagctgatagagaaggttggaccaatcgagggagggagtgaggctttcaaccggaccgggggggggtcgggtagagctgtatttgccgaggcaaggttggaccggaatcaacagagattggtgctgcgagggcgaagcgaaaataactccgtgccgcttgctgcgcgaagtcaaacttcgcgacggaagcaagaaaagaaagaaattacgacttcaccaaccacttcggcctaatcatcccacttctttcctcaatcccaataaaggatatcgatttacgataaccactttcgcccgatccaattcacctccatcgaggcagcgaactagtagatcatctttcctgaggaatggaaggatggagtggtattcgaattctccggctacacgatgagaaaaaaacatccgtgaactccttattaagactttcttctatctgctacttaattaagatgaaagccactaagaagtgcatcttgcttggacgttgccgaagaaagggctattagatgggcgattcccccctttccattgaaatagggaaagcgggatgaaagctctaagcccgcatcttcagcttctattagaggggctgtggatccaatccattcgaagggggagcagagcagcaggcaggcaaagcaggggaagagatatggattgcaccgaaagcaatgcccttcggagcgcattgcttgggctaagtcaaagttgctgatctctttttattgtattctcttccttgggaaacaaacctcccacatcatctgctgtctcgcatccatcgggatgagtcttgcgtctgtcttatcttcccctaaggtctattgtattgaaaggccatctctcgaatccgagcaatgaaaggaggaagaaccatatagatattcagtaatgaatacgatgtggatccgttccaaagcccctaattcaaaatatagtgtgaggggggcagagcttccatttccagggacaatcctccgcctcagggcgttcttttttccaggaatctgtcaatcggaggagcgcaaccaagtttcaaacctcaaagcccttcaagggatgtgaagcccttctcaatgtcttccactcgccaggaggcaaggggaatccgttgattgaatccattcctgatgatgtgccgctaacaaggcctacctattctcccaatgcaacccggctttttaggggcatggcattcaatcctatctcaatatatgctcctccaaggcctgagggtggattgaatccaatcccatccagcataggcgggtagagttcactcatccggtagttagaggatgatgaacaatgatgctatatctgctcacctttcctaatctgccttgttgtgatagggggcttaacggcccaccaaccaatctttctttctatctcgaattcttgatctttggtgccagtggagcaaaggaagcgggggacgaactcctctatttaccctagaaatgggttggatctattgaatgaaatcctggagacagggctgggaggtatgagtcgatcggatgcagggaagcccaggcaatcttttcctatcaatcattcgtcaggaagcagtggagaaagaatcgtcttttgaaatctcattgttgaaggcgtagagagggctgaaaaaaaaataggatcatttttgatagccatctcgttaatcaaaaattgtgtaattaattggacccctctgcccggcaggcaatttctgtgcaactagactttctctagtccctgctatgccagcaatagggaatccttagaaaagcggaatgcaagttgcgtgatagttttattccccacaaatgagaagtccccaagcttgacccctcccacacaggggcgactggctggggccctggtggatttctttctcagttaataaatgtctggaatcttgggttactaattggtggaatactgggcaatccgaaatttttttgaataatattcaagaaaagagtcttctagaaaaattcatagaattagaggaactcctcttcttggacgaaatgatcaaggaatactcggaaacacatctagaagagtttgggataggaatccataaagaaacgatccaattaatcaagatacaaaatgagaatcgtatacatacgattttgcacttctcgacaaatatcatctgttttattattctaagcgggtattcaattttgggtaatgaaaaacttgttattcttaactcttgggctcaggaattcctatataacttaagtgacacagtaaaagctttttctattcttttattaactgatttatgtatcggattccattcaccccacggttgggaattaatgattggctctatctataaagattttggatttgttcataatgatcaaattatatcgggtcttgtttccacctttccagtcattctcgatacaatttttaaatattggattttccgttatttaaatcgtctgtctccgtcacttgtagttatttatcattcaatgaatgactgataaaggatccgttgatattaatctaatccaattagaatgcttggtactttgtagttgtacataagcaaagtattgaaaatcgtatttactctttctatttctaaccatcggggagattcatcctatattattcctagattattccagcaaatagcagaatcgtggctagggaactatattagcgacctacccaatttattgtagaaattttcgcgatcaatgattggaccatgcaaactagaaatgctttttcttggctaaagaaacagattactcgatctatttccgtatcgctcatgatatatatcttaactcggacatccatttcaagtgcatatcctatttttgcacagcagggttatgaaaatccacgagaagcgactgggcgtattgtatgtgccaattgccatttagctaataagcccgtggagattgaggttccacaagcggtacttcccgatactgtatttgaagcagttgttcgaattccttatgataggcaagtgaaacaggttcttgctaatggtaaaaagggggggttgaacgtgggggctgttcttattttgccggaggggtttgaattagctcctcccgatcgtatttctcccgagatgaaagaaaagattggcaatttgtcttttcagagctatcgccccaataaaaaaaatattcttgtggtaggccctgtccctggtcaaaaatatagtgaaataaccttccctattctttccccggaccctgctactaagaaggatgtttacttcttaaaatatcctatatacgtaggcgggaacaggggaaggggccagatttatcccgacggcagcaagagtaacaatacagtttataatgctacagcggctggtatagtaagcaaaatcatacgaaaagaaaaagggggatatgagataaccataacggatgcgtcggatggacgtcaagtggttgatattgtccctcccggaccagagcttcttgtttccgagggcgaatctatcaaatttgatcaaccattaacgagtaatcctaatgtaggcggatttggtcagggagatgcagaaatagtacttcaagatccattacgtgtccaaggacttttgttcttcttagcatctgttattttggcacaaatctttttggttcttaaaaagaaacagttcgagaaggttcaattggccgaaatgaatttctagattcgcagatttatcgacatcaagttcgtaaaaagaaccaaattcttcttggcgattatttatgatcaaaaaaataaaattatgaaaacccctttgtcttatttatactcttcgccaaaatctacatactatgtggtacaaaggattcccagcgggaatcccgttgagttcttacgatttcatgttgacaactcaattcattcgattactacagggatgaacccaatccggaatatgaaccataaaagaaaatacctactaaaccgattacaagaataccagctacagtacctattatccaaagaggaatccttccagtagtatcggccatttaccccacttccctccagatttcatcaagtggtcatgctagagacataaacagtcatggataatttaattatgagatccttccgaatgagctaagagaatcttatttattctctttcattttcttaattgaagaaataattggaaaataaaacagcaagtacaaaaatgagtaataacccccagtagagactggtacgattcaattcaacattttgttcgttcgggtttgattgtgtcgtagctctataattcggattaagtttatcgttggatgaactgcattgctgatattgatcccaaaaaaaagacggtaggtacagctaggccgtgaacagccaaccatcgtactgtaaaaattggataggttcgatctatagtcattagggcctcctaaaacgatctactaaattcatcgagttgttccaaaggatcaaaacggccagttattaatggaattccttgtcggctctctgtaaaatactcgtttggccgagggcttccaaacacatcgtaagctaaaccggtgctgacaaataaccaacccgcaatgaatagggaaggtatagtaatgctatgaatgacccagtatcgaatactggtaataatatcagcaaacgaacgttctcctgtgcttccagacatgctgagctccacatattcttgtacagtcaaagaggatcgattccgtaaaagatgagatcagtaaatgacaattcactgaaatttaatctttgtgagatcgtcaatattgtaccgagggcgtctttagagtataccgaatcagtatagctatccttcttctgacacagcaacgcaatttgaattagtatcaaaagtaagtactaaataatttcttttttcctttacttgttgatgtaaaataatcttccattcaatagaaaattctttcaattcaacgaaagagattctaaaattcccacaatttaagtagatccgagatatagaaattttcttttcgtagttgtggaagcggttttgttgttggaatcctttttttaaagaagaggttaatggtcgagtaagaaataagagtagtagatcatattcgatgaaaggaaaaatagaataattggaatccatagttgtgatgcattgttgtggatctcgacccaaaggttctttcttgatctagctacaagggtggggcggtatggaaagataaaatgtggaacctaatagaaattactagttttagaatctagttggacaaaaaaagattttttcaagcaattgtgtgatacccttttcttcttctccatcattcaaaatattatgtgaatttatatattactgaatctaatgagttaaacttaaattaaagtaaaaagaaaaggttttataaggtaactgttcgctttaaaatcgaaaatggattcgatacaattcaacagaatctaagaaatgatcaaattcgaaagtcatttctattttgattctataaaaattaaagtttcatttttgaatgaagttagacgatacagctcttattagtttaatagtttacccaagagttactcaatgaatcggttgattggaattgcgagatagatagatgttacagatgatgaatcaatttattttatatgtctgtcactttatctttgttagtgctgtctgcctataatgatagatgaatcaaaaacttttcattcaacttattctttcaattgaaattgagatttttgcctatcctcctattttattttgcaaaaattgaaacttaggtaagtgctttttaaacatatgtataaaaagaacatatttcatttaatttagccccctcatgcttactataactagttatttcggttttctattagcggctttaactataacctcagctctatttattggtctaagcaagatacgacttatttaaactgaatatttaaaatgaagaattcataaaaataaatctttctgtgggattacgtgtattctatatttacttacgttacctattctcaatttttgttcattgtcattgagattcatggcaattcggattaatatttaggtatcaatattacttcttttttttctcctttcaaacaaataaaaatgattgaagtttttctatttggaatcgtgttaggtctaattcctattactttggctggattattcgtaactgcatatttacaatacaggcgtggtgatcagttggacctttgattaattaacatatctttttgattgacctcctcctttctttaattcacaggcacaggaggtcaaattccgattgttgtgaaagttacggaatgcatttatttggttctaattcgatctaagaagaaaaaaatcacgctctgtaggatttgaacctacgacatcgggttttggagacccacgttctaccgaactgaactaagagcgctttcttatcagaatagataagactgtaaacaaaaggattcttttcagaaccccaatacattttgtatgcatatactagaatagcgtgataaaaataaaagattatgtccagtttgaggcgatctcaattgatccctcgttactgctcaaaggagcagtaataggtagggatgacaggatttgaacccgtgacattttgtacccaaaacaaacgcgctaccaagctgcgctacatcccttcaattgttccacagtgtaattgtagagaattcctgtcttgttttccacatggttattttctccattgatatatacaaattttctgctcatttcgtctttttggtctcatttaacatataatagtaaaaggaaaagacttctcttatagacttacttacttataagcaaaaaaaagggttctaaataagaagccctttgaataagcgaggctttcccgatagaaagatttgcatgcaacagagatcccaattccgtgtatccggttaagcaagccctgcccgccagcttccacccagacaaaaaaggtgagcgcctagcgcgaaaggttgctttactaagtaagataaggcaagaagcaagggcgtagcagctgcgcgaaagccgttgcgccttagcgcatccgttttcttgctcgttagcgctcttttttgaaagaaggggcggagcttgaagaagcgaagcgagcctagagtagcagcctattacgttttttcaggcccctttgatatgttattagtcaagcgctagcgcccctttagagtaagtcttttctgttatcaatgaaaccgaaagaaagaaaaaagaccagtgcctttcgtatagatcgagacttgtagcttgattctttactcattccatactgggaagaattgcaggaaatcgttcgataacacttcttcctatttctttctcaatgatatccgacgatcaagacaattcccgtgaaactctttcatttcatagaagtgaattcttattcttacgaagcaaatagcatttcctattgatttgtcccctggactggacctattctgattctgaattatccgtcgctacgctgttcccaaggactagcaaaatcgaaatagcgaaattcttgggtcatctcaatgggttcagaaaccacacgtttctctggatcatcatagcgtacttccacatatccactcagaggaaggtcttttcgtaatggatgaccctcgaaaccataatctgttgatatacggcgtagatccggatgattgatggaagaaacaccaaacatatcccaaacttctcgctcccaccggccggctgatggaaatagactgactaccggagatattcgtgttacttcgtctgcactggtttgtacacgaatgcgtgagttataccgaatactcagtaaattatagaccacttcaaatctttgttttcgagagggataatcaactccgcaaatatcgatcgaaacttgaacccttgtataggtatgcaatttcagaaagcacaacaattgaaataggtagtccgtattggtatcagatctattcccatgttccgatctttccatttttttgacccatttcttgggtaaagtctcccaactatatttgaaaatgaattggttatccataaagagaaagaaagttttcttcaagttccgcttcttgctcttccaattcagaaagacttgtcggaaatcgccggttgggttggtccgaccaagaaaggcatgggacttttgggcattgcttgggccgagtgttgtatggctacctagtgatttacaagcaccctcactgcacactttctatatatctgtctccatccaatcaaagacgtccatgccatagagaatcaggctcggcaaaaacgagactagggaccatgctccccgctttcttcctgtggttactattagaacacaagccaaggaactcaaaaccacaacacaagcaccctttatttactagttttggagttttcgccctttgcttccggctttaatgaaggtaaatagtcaaaaaagttccccgtagaacgcgagcgttgaggctttcatcgaaacaaagagagaggcccggctggtgcttttttctgtgttagccaggtgaaaggcttgcttgactctaaatagattagtgtattaagtaaggaactactaaaacctctattcccgtttttgggctataagactcttagcttccagcgagctaggtgcataagctttttttactacaaaaacgattcctcccccggcaaaaagtggtccgccaactgaacttgccttgttgtgataggggtaccgccttttcattcccaccaaggagccgtagctttacttagatagggcttgactgccttaccttctattatattagtaaagggcctttaggcttgactttactaatataatatcaagtaaaggggcatgtatcctttttttgtaaagaaagagggctacttcacgagccgctactaataatcgaaaaggttcacagcgagttcagtctatagtgacaaagggaacgtttccgccggaggggtttgtctccatggaaaaagtattcactactgcttacagcaccttcattcactcgtcttgctacttcggaactgttcagcggacacgtggagtcgaacgtctctctacaatgttgcgtaggtagactgattattgtaggtgactgtctctagtggtttagaaagagttctgttgctaccaacttctttctttgtagtctagtagatctacatgctctagtggatctaaagtaggtttatgttcagcaacagaaagaggtgaggttctgctttcttacctgagaatatttacaagggggaagcctcgaaaggcatacgagtgcgcctctcgtagacgaataccgactcagtccgctcctactgcgcgggagtatcagccggtcggtgtcgggtcggcccctagggcactattcgccttgggagtggttcggccatcaagctactttgtggggtaggggaccagactggtgactgctgcggttgttgtctgcagggtatgtgacaccccacaagttgactagtgctgagccaggagattttcctttggatcgttacaacgctcgttgaacggttcaagtagaagtgaataggtaagaagtagaaacccccatatcaatccatctccataggagacaatatgagcaaaagacaggaatccctaaatcccgcagaaaagaactcactccgggggagtggagtgaggggggtattcaaaaaggggagccgcgggttctttctttccttgtaggaaaggtcttggtttggtatggcattagagaaaacttgttatggttatgcggctatatagaaaaggcgggtggggcttcaggcggctttttttatgaatataatcaatcaaaattccatcgattgtagctagtgattgcccgggtcggtgtgtgatcaccaaaggtgaagtaacccttcagatgctctctccgcccatgccgaatacccccggccggttccgccgggtaaggccaggagctggtttggggaatcacggggccttacttattcaggggggacttgattctgaaatggaatgattgatagaatcgagatttcatagaagaatgaccgagaccataaaatcctttcacacccgcacatgtggctgaatatataaggaagttcacacaccctggaaaaatccatcctgtatccctgacttgccagcttgatcgcttgtcttatttacccttttcttagcgggtggtttatgtctggtcctttcgggtcgcctgacctgggctgatggcgcttcgtaacggcttgtctggagtccagcggctctctaaggcttcgatgtactagtacctgccaccaaaacatcgtgaaggattcagtgaacgtcttgaaacttagtaacacaagacaattcactgaatggttgttggctctaccggaggagtctgaaatcaacaacgtgtaactgcttgggcattgagtgttccgctgcttgaggaagtatgtgagaggatcgatgttgagcagaagtggggttaaagcagccaacaacgcatccccctttacttagtagggcttgaaaggctggacagtttgttttcctttcctgtccagtattttcaatccaagccgaaataggaaaagccgcaagcaccactaggcccggtcgtcggttgaacgtcagtagggtccgatattcattccttactcaaataggaaggtggcagtctcaatctagcggcgtggtccagaacaagcctttgctgatccatggggttttcgttttggttacaagaagtgcttctttgctcgcttgcagcgcctcgactcgagtttccgctgtaggattgagtgaggtgacgagagctgaagccaaggttccttgctatgctccatagatgttcgtacgattcttgtggattttgggtgtgtttgaattcagcctctcgttaggtcttcactgaaggattgtccaccttctcaagcctctctaccatacccttagaaagtgacaacggatgacttccattactaaatggaagaacttttcaaactagttgatagttgttccctggttgcaccccacaatgggttctaatttactaaatcacatgtttctgttttcggaacatcacatgtagagttttttgggggagaatcactcggcgcggggcctcccgtgtgaggtcaggtgatggtcaacaactcaggcaggaaatgctgaaaagcggctaacgatgcaagagctcttttccccttatacgctctaaaaaaagggtatgtcgggtttttggaccctatgttgagtaagggttccaaaccttccaaaagtgataggtatgtgttctttcttggcactctctttctatattatgccaacctaaaaagagcgatggaaagtggatttcaggttcgatagtctcgagaaggtattagccaccggtgaccatactttcgtaaaagcaccattgggcggtggttcctctccttcctcttgaacctcgaacaaaaaatcgatctcgccatcagctcgactaagagttccgaatcgaaaaagtaaacttcactttacttaagacgaaggaagcgagtgccgaaaaaaaccgctttcttaaggcttcaaactactagtcattaagactactatgaatgaaaaggcaaggaagtccttttcttgacttggcctgcgtgcattatacctaaccttttaacttgatttcaatctcaacaaagaaatgaaagcataactctttgctcgcttgcagcgcctcttagtcttttattttagcctgccttgtgaagatctctcgagtgtctacggcagatccgatcagtctcgtgatgaagagaagtcttttccgatgttgaaaggtatcgtcacgacaactcaatttgtccggtaaactactcggggctccccatggtttagtaaaagggaggggagatttttgcttcatccgggggttcattcattatgaactaaaaagtggttggctgattagtgaggtcttaaaaacgtcatagaattcatgatcggccattccatttttgctttcagcaagtaggcgacgcgaatctatgctttctatctttcaatcggataccaattgcttggatgcgtttgaaagcctcgagatgacttgcagaaaaaattctttctaggtttgtcttgtgtctccgaaacaaagggtccatttattgatgggcgaacgacggggattgaacccgcgcgtggtggattcacaatccactgccttgatccacttggctacatccgcccctacccccgcacaggttgaagtctctatctacgatcagatcctttctgaactcccctatgaccgcttatcaaagagaagctttttcctatactatagtggcaagtctattgttgtgtttcggaattaggggaaacaaagcttcaacaagtagaagcttcctggcaaagcttcaaacaaagaggttgggctgttcacttcattgatttgacttcactttacttaagattaaagataggggccgggcgggcagtgaaggctcatttagtagacagcgagcgagctgcaagcacctactcctatcaaaatgaaaagctgcaagcggaacttgaacttgaagaagcgagcctctatcagagaaagccattgcgcgctagccccttgtatagggttccaaacctgcgcacccctaaactacaagctttctttgaagcccctacaacatgggatatttgaagaatcccctttctattagtaaggttgtcaaaaggctttcctttagttcctttataactagaatctaaataataggggtaggggggcgctaacgagcaaaaaaacggatgcgctaaggcgcaagggctttcgcgcagctgctacgcccttgcttcttgccttatctttgactaagaaactaatctaaatagaagcccttctttctcaaagtcaactttctcccttcttgctttagtgaaataaggggcgctaacgcgaccttccttcagctggcttcgccctatctattcatctattttctcaaatggatatttagggatctctcttgttcatagatcttgaaaccagatcaatatccatttctcaatagatctatttatcgatagaaagatctagatctctatatggatctatctccatatctaaatatggaagaaccgacacttaaagggcgtaaccaacggaaggttctcaccctgtccccgacattgttctccgacgatgtcccctgggcgaaaggagccaccattctctttctttcttcaatcgttccgatcaggacaagtgggttggttcgtttcgtcctcctatctacgcaattctctgtcttcgttcgtgatcatgttgggcgaaaggtagttgtagaggagcggctgtgaaagggcgattcccccctttccattgaagtagggagggcctccttccccaccattccggcctattattgatagggattttaccgatgctgaagatagcttgcttaccaagccgcccacttgagaagctagtcgccaggaaagaagcgaggaggaagcgaagctgtctacgaagctttgcttctccccctgtagtcgtaatactcggcttgtcgctactttgattcaaaaggtaaccgacggttcccgactttctccgctttccgcaaccgtaaccacttgtcattccgattacttcatccataaaccttttttttatttcaaaatagcgatacgctctaaaaaagtaaaggagaagcttccattctagaagcggtagcttcccgcctccctcggggtgagaagttcccttcccttttctaaaatgcctgagtggtctgctcagcaaacgtacaaagtggaccgcagtttggctgaccctcttcttcccattcgggttgggttgacccagaagtacagtaagaaggaatggaaccactggagagtcgtctgcagttcacacttgggcaaagacgactgactttggaagcggaacacgaacctatttccgctattccgggttcttattgagcgtagcgaaatcaaggttgatgataaagtcagcgaagtttccatggtcttctacctttgcgtagtctcggtccacagtggaaggctccgcacctgagcctcgttagactcagctgaagtgtaaggtgtaagtgaagaaaatagaagagatgaagtccgtcccttagcctagtctatatccacagctgacgcaactccgtaccgacgcctcactactactttcatttttcttttattttgaaattcattaacggctaagcgatttcataacctgagctttccttaaccagctgaccttacttcgtaaccttagcctccctttctttatagttttctagttcgactaagtgacttcgtaacctcaacgtactttttttcttactgtagcataggccttcgccacttcaaacggcttcaaagaagcccctcttttttttgaattagaaagagcggggtctgacttattcaggggggatgaaagacaaataaagggatcagggggctttatgatcggagaaagagagggggcgtggttggtgtgtcactgggtcggtgggggaacccgtaggaaggggggacgacccgccgaattcacatcagaaatcgccaacatgaacacaaacgaaatcttgaattgcgtatagaaacaaaacgaaccacttctattctcggagctgaggtatatgaagaatggctttttggtccctttcgtccagtggttaggacatcgtcttttcatgtcgaagacacgggttcgattcccgtaagggataggtactcattcccggccgctttcagttagtgttcattgctgagtgatcgctcgctatctggctggaaaagatggtccggaagcttcctctctcccagcaagcaagacgagatcaccacttctctcagtaatggacttcctttacttcgtaaccttagccttagatgtcctttcatagattctcgaacctccgacagacagaatctccatgcatgcgttctttctctcctcccctccgccatacatccctttttttcttttggccgtttttgttaggcattgaaccccaccttaggtgctgagtggtgtcctcccctccctaatacctaaacagagttccgtctatggagcctaaagcttaaaccatggcatggcagtaagcagtaagttggcctagtctctcgcccagccttcgccttcttcagtggccaagttgaagcgttcaacgtcggcctaccaccctttttttttcaaggttgagcttgttcaattgaagctaatgctatgctgcccttcccttgttcaagagaaagcgaggactttcttttagctaccggcccaaacaaaagagattagcctcttgatcgatcgattgattggatcgaagtacgaaggggttgattgaagtctgagatcagcccaagactaaggccgagcaactagctgctgcaggattggacgtctatctatctcaccacgctcccctactcctataaaggccggcggaaggaatgctctgctcatctttcttacggctcgttaccgcagcgctcgttcaccccttcggcttcttccattcaaaaaaaaaggtagtgtttccttggtaaatagcgtcttgaagtgaagcgaaggcattattgaaggaaagaaatggcgggtcggtcaattgcattaggtaggagatgcaggacctgtcttaaccgcaagtgcattcgctattcgattccatcctaaatcccaccgaatttggattccaaagtgtgtatctcttctttacttttaagtgacaaggggggtgacaaagggtatactttcttctctatgtcgccgtctcattaatgagcgtagattaatagccaagcctacccttttgtgcttgtcaatctgtatcccattcttcaggtatagttttcttttatcacagatcgacaggtgatccgtcctttctccccctttcgtcataaggcgtggtctgactctgagaaagaaaattcctgtgtttaggtccctactaagcagaattcgtaaactatgcaaaggctctttgaatactttttcaaaagtttttagcaaaaacaattctcaacgcccttacgaggtagtgatgagttaaactactcgtgttggcatggaagtcagcccggtaaactgattccattctgctactagggttccaaaccttcccctgagctctagaatctagaaataccttttcaactcaagaaatgctaaagctatttagagttggtatttctaactaagtcggaaggagggctttgggcaaagagcaactcgaaagtactttacttcagtcccagtactgaaagacgtgacttcaggagtggatttcggaaggaaagacttcgtttacttcctgcaaattgcttatgtaagaactagtagaaagaaaggcattttgaaaaaaaaaagaaggcagcattgacattgaatgagaatgcttgaatgggaatcatcttagcaactgactatagacatgagtctaagccgccgggagaggagagaccattttcatgagagagggacgagcaagtgacagattgggaaaaaaaagaggtaggccttatgagcggtcatttaggggtcttgttagcgacccatcattcttccctaagctgtcagagtccgatcgaagcgagcaagagatagaggaatcctcgctcatagatgtgaattgaaaaagcaagcccgaattcttttgaattaggctctatagtctggtccctgtccctggtaaggtctgattgttatccgtaagtcttgttttgaccgcgggaaggtgaactttgcaaaagtgcttatttggttgggaagaataggacttctgactccaagcctaccctacccgaaaaaaagtttccgctattgatgtagcctcttgtcgatactactagtcttctcgctacctactagaaaaatcccatcaagatagattgaatcgacgacctatacttcaactaaaggcacaagggcgtagcgagcacagaacagaggaaatgcacatgggtctccttgaagaacgaagtctagggtaaagaaagaaaggtagagtgggcgcactttgactgtgcttggattggcatggctgtccccctttgctggttgaggctcggcctttgactccgcttgcctctacttttcatgtcaagcgtacaagtctagtttagtgggatttacttctaaagacaggaattctttttcatctcccctgtcaaagtcgacgtcttaacctgacttcctgagctcagttgattcttgaagcagtagctctggatcgagagctggatgcttaccttattattatgaaatgaaaaggagaaagagctttttttatagatgttgaggtgagtaagggggggtttgctggcttgctggctagctcgtgcaatcaaggaaaaaagccttcgccttcttttttaaaaatgaaaaagtaaactaccttagtaagctagctttgtaagctaagcaagccgggcactaggctaggacgtggatcgatcatgacgagaatggacttctccgtaatgtaatgtaaatgtaatagaagaggcagagtccagttcccctcccttctcgaccagacgaaggagatatgaattccatttaggcgggtcagggcttggcttgaccctgtgttctcccgggtcggaggcgagaacttgaaagtgaatcattcagtggtggggtgttcatagaacagaaggcctcgcccaaggagtgatttggatggagtctcgctttgatgctggggagatgagatccatagatctggatagagtctcgctcatagaggaagagtacgcgcgctagcgcgctacggcttacgtagttgatcggatcagatagcccttccttcgggcaagcaaccaaacccggcacatccaattccattccgatcaagaacttggaggtatggctgagtggcttaaggcattggtttgctaaatcgacatacaagaagattgtatcatgggttcgaatcccatttcctccggtacggaaatgaaacgggcgggcgaaattacgtgagagaaagaacctcttggtggagtccagtcccccggaggacagaatagcacttcttagtgactaggagcggagagcccgttgcaccttgtttttctttgaccggcctatcttctttctataagcaagctccctccggctgtccagtccctgggcggctttcggttcttgagcatgttgggagattaggcggcagttgaaagagctgctcgaaagcttgacgaagaagcgaaaaaagcctatctattcgattttcttagtttagtaaagggcttttcccttactagtcaagtggtaaggtagggcgctattcgatgaagaaaacagactttaggaaagtggttcaggtagctcagctggttagagcaaaggactgaaaatccttgtgtcagtggttcgaatccacttctaagcaggcgaaaggtccaaaccgtagccgggagcgagccggatttggaaatgaaagtgaaagagtaagcaaaaaaatgtgagcgctcctgcactatacggacggctttttggcggtagggttggggtggcttgcttgaggcagattcaaaaaaaagcggttgattactcggattggttctcgcatccctgtgcccaaaaggatgggcgagttcggttcgagtcttcatagatcgggtagatctatatgcttcggagggtgagacgaggtgtagcgcagtctggtcagcgcatctgttttgggtacagagggccataggttcgaatcctgtcaccttgatgtggtagccttctccgtggtcggacagtaaggcaaacagcgcaaagcataaagtaaagacatgatgcctcgactaagtaaagtctttttgccccttatcggtagttccgtagcaggttgtttcgtacgttttctaggatcagatagaagcaccaccccagaatggatccttcttttcttcttacttttactaagtttgactcttgtttctcgttcaacaaaaagaaaaaggagtgtgattcttttattcctaatattttgcatctctttctttttctattttctcctgatctacttactttctcgcttagatgttcttttttttggctgatcttttctcttttgttttgcttttgagtgtggggggagggcaaggacttcctcttccgggcccttcaaactcctcatcggaagatttattcgggctccaggtcctgtcggagccttggcccccgactcacaatatagccttggagtcatcgatgataaataggatattggcaatggaaaataccaatagcatttttttgatggataaggataggggggtctattgggcagaagtaaaacattcactctaaaattcttcctcccaaaaggaatataaccaattgatcgagttcgagaatagggatcttcggatccgtgagaaaaagcattcatgctattctctttttcaacaaatacttacttcacatcctgccttggccgaaaatgccgcctacaccccccaagaagccttttgtgactttttggatgagaaacgaagtgaacttgaccaacaaggcgggaatgtattagtaaaggaccagagagaactcgaattttggaatctactgtctcgcgatatacgaacacatggccaaaactcagcctatataaatagaatactcggtggatgataatgaattggatttgcactgagaagtccctatggcgcggttgagggcagctgaacgaaaggaaagcgggtaggccgcctgggtgagacaaagcagaataatctaactggaggagtgaaagccaggatggcttggtaagcaagcaatccgttatgtgggcgccaactccaagttccctctcttctttcttttttttgtcacgatcaaaatgaaaggttgttctctgggcctgtcttttgctcccagagatgctggttcgagtccagctcgtgaaagagtttgtgagtatacctcgggatgactttttatccactactcatcctcgaaatctagtctagttcagccatagaggacttgatacttatcttcgacaaacctcaagcgggacgagtcaatagcagatgcggattttatttaatagctgcgcttacgccttcaaccccgaaaaggtcggattcgtgcaaaaaagtaacatccgagatttgtgaacagaccggcttgggacagagaaatccggatgaataccgcaaggggggggcatagggctgtgtgaacgcggctttcactaagagaaagatgtgcctacaatgaaactgttagacctttgttgatgcacatgaattatctttccagccggtgaagctaagaaaagaagcccttagaaagcagagctagacccacacaaatgcttaatcgaaagctctgtcctccttcccctcctaccagatcgaaaagaagaagcttgctcttccgacccaaaaggcttttgccgtgatattacttccccctattcgacgattcactcttcctggacttgcttgactcgtccgaaaaaagagggaaagtgctaagaccgctaatgcagctaggggagtttaaggactcatttccaaggctagaagcctagactagactagaaaggagattgctttggtcttcagtcagctctactagatgcagttgcccaggaatccaatgcactaactcctggaagctccattcatgcccacctaccgaccgaggaagacgctaccgatccctgaatcgagggactacgcgctttcaatcccttacagctgccttccaagccccgaactaccaatcgccccactatctgctagtctggttcgactcgaacttctgtcatgtcaagcttcctgacctgctttgtaccagccggtattttgtgtacttcggggcgctgactagccctgctcaacgccctacacccttctcttgagcgcttcattgagcatttctctttcctatcccgtccttaggctacgctatccataaggttgacctagccctctcttctctctctttgtccacgcgaagattccattcctttcctagcctattcaatgtggtcatgtatgtaatagaattcaatgggaagacctcctagttggacccagactgcgatggtagtgaatgtggcctcagctcccacaaatgcaggctcccaaagccttagactgagatagtaccacaaagcaggggttaacataaatgactctatggaagtcctctcccacttgaaagctaaataaggagaagaagtgccccaaatcaatgcattccattctttgcagaggttccttccatagaatccctcgaagtacttcgctcaccttcgaagagtgaaaggatcattcaaagcagactaaaggcatagggcaaaggagcttagaagggtgacggaggggagtagtaaggtatgaaatcacttagatagaagcatgttggatgacggaacgatgacttcatgcttcaattcgaaattttagatttctgaccttgagaaatgacgtaagtgatagatggaatcgttcagtaggctagtttccattttcgattgagaaagcggcgggcccagtgagctctccaatagtgcaccgaaacggggccggagagacggtaaaccttagatcggctaagatcgaattgaactgtctttgattgagcgaatcctgcccgattttgatttccgtccccgcgggagacatcgtaaatagtgaaatgtttgattcccctattgaattgaattaggaatcgattgaatgggacttgcctatcccttattcatatccgatttttctctctttctttttgatacttggttggcagggtcagggcctttctcactgggcgagcgaatccgtatttttctatgtaaatgtgaccttaacggcctttattttaagcaattattcgctccaagacgcacgacaagaccttcgatctctctctctccataattgatatggaagttggaaaaaatcaaccactcaaagctgacctcaaaatgttccaaacacgcataagtgtgaagattgaagaccttctattctatatttcatagagttgattagtgcaaaagaaaagggcactggttcacgcattacgggtagattcctcttgcctaagaaatggaagggggcacttcaccgaatgataggtaaagtatgggacgttcagtaaacaatcccttagctcaagtcctcggagatacccaaggcagctccccgtgtcctttatacccaacaggacaagagtctacaggtctgccaggggcgaataagagctcgtcgaaccgtcattctttacttccggggtcaatcaataggtagtcctcaaatttcttctcgaaagcctgtttataagaaatagcttatgccactcgtattgccccggattgacaaaataggcttggattggagattcttgtgtaaacattcaagttgacaatcgggtttctagacagccagtggactctgaaaccaataccaatgatttcgctggatctaagaataacgtagcacagaaaagcggactcaccaaggatggcgaatgggcaatacgtagagcttgctccgcttcctatggattgttttatagcggtacgattacgatgcttgctccgaatggaagagagacggctttcctttcggatgttgcaaacgcacaaacgaaagaccttagtcagcggaagaagtcactctcaatccgatctagcaagaaatgctttaccggtaaagtaaagcgagagacagtcgattctttcttagggttccaagtaattcaactagtgccaagaaaagtatccggttgtagagcgaggcagcaaaggggagttggcacaatatgtaatccctagggtatcggtgtcggagaaggggatcactcaatgctgctacaggcactcattagttcggattgggtagcgtgaaggagataatagaaggacccgccgaaagtagttccgtctttccaggtcttccggagtcaaaatttcctcatccaatagcattcttagttagtaccattcaactaagcctgtttttgacgagtgaagcggctaggctacatgcttagcctagtattcccggattggtattggataagaaagattttgctttcttcccactcatgaagaacaataaagtgaggggagggcttccgtggaaaaagggtaagtttgggatgagagggtgaacactaaaatagtagtcaccaaacccaaagaaatttgactctttttttttatgaaggcgaattgataagaaaaggtacttccatgtgtataaaagcacaagggaagggggcccctagtccaagtataatagcataggggggtgcaagggtgaagatactagagtggtttggcactcctggtcagctttctttcgttcgggctttctttcttctgcctttacgcgagccaattatgcgtggcgctgaagaggaaggcgtcacttactgtactactatcggccatacaatgatggcattgtggatctcattcgtattccagtttttttggacaaagttagagtagtcatttagggaataagtcttttttaattattctattagcatagcattaagtggtaaacatttgacactagaggttttaccatactatacatgcaaacataacaaataaaaccaaacaaagatagttagcatagataggagtctatctccagtaggcaccggagtagatctccactagaacaccagacatgaaaacaaatgtctcaagacacttatggaatttaaaccttctaaaactaaaaagagtcgacggactcttttagttttctcgggcaccaaggaagattgcctccacgatcagtgcctgctgctcctggcgtagtccctggagtctttcttctagttcccgaattctttgacggcttgcttccattcgggcttcaatagcagccgggttcacggagcgaagatgcctcaagaaaccatttaacattattcgagtatttcgaagataattttctactttttgtatttcaacgttaatttcagcaagtcgctggggaatgtcgagaatttgagcagggagggccatggcttctcgatatacactggtagaaaactcttttctcttttttgtttttttttgtagaacacgaaggcttatcgagcctctttttttagagtgtatagcaattcttccaatgcagtacgaattgcatggctggcacaatatgagtactataaccacgctgcctgtatgaaaaaacaaactttgcagaaccctttcacctaatcgatcgtggtgaagtcagcaatggattcggcggatcatacaccttacgctaggatttgggaaggacatttacgagactgaggtgagttttaagagaaagacgggggtggatttttttgctctaactggctgtgagcatgggaattgcgttgccgagcagagggcggagaggaatttggtgttgcaggtttgatgactgtgagaggggttgaaaattgattggttttttttagcaggtatattggtatttttgaacatattaaagattatagaatgtagaagaatctcgccatacggcacgagcagttgagtacagtactatcatgcctttgttttgttttgtgaagaaactaaaaaacttgcgaagcacgcacctcaatcaccctgcctgtgtgaattgaacgaacttaaaagtacaaccagcttaagctggttttccacctattttttagtgttcggccatttctagcaaagtataaaggacatattcgttgccgatttggggttctgatggaagatactgctgaggttatacaccaagtacacacgtgattctgctctggcagaagtgcacgcgcaattcagctctggaaaaactccctgaggtccagagagagatgaagtttatagtaaacctctgcctctcagatagctttcttttccaacacttctatgtggagatggatgtaatattaatatgattgatagtttcagtttactatttgcagttttccaaagtctcaaatttaggacttggttccggccttgtttcgtagtgaatttatggatttgaatacttctaagactgaattcttttttgtaaattcaacttgacttgtacctggaacagagaaaaagggtatccaattgaaatccaggcacttttttctatttttcgcttagatgtgctcggcagatgctaaagccagagcgtgatggcaagaattgatcggggagatgcccttgaagatcacttacccagctctggaaggacatgagtggagaattgtcaccggatttgatccaaaaaacacagggcggagttaccttattggtgagtcttggccgggttagtgtttaaggaagaaaaccttattgtaggttattttttatttaaagagtgccaaattcaaaaagaaaaggaaaaagatgcttgtacgcacattagatttgctaactcaattgatcctactgtgtctagatcagggttcccgtttaagaaagcttgttagctttgtattggctcccatcttacttaacggggcccttagttgaataccgatcaaaattgtttgaaattttgaaacttttccaataaagaattattcgttatgttaaataccccgaaaagccgaaacctcttattctggtccttagaaaaactacgactagtcaggaattgcgtaagagaagagacgtcgcaagtaacaatagcgcaaaagcaggcggcggagatccgcaaaggtaaccggatgcctggggcttaggacaaggggcgtccggagtctcttaagaaaggacaaagactaattaatatcatgtttacaccgatcggatttaaaaaagtgcttcgccccttatcttctcgtctatcttctattttgcatcgatggtccattcctttcctaatcctcacctctacctttttttgtgtctatcttctttatcttctgatcggatcgcctggcttctttcaagccctacttgaaaggcttgctttcttaaaaaatgctttctttattaagagtcctttaagaagctaagctccttcagatagtaagattcgcttaacttcatacctctaagcgctcgtgactatccgatgatagtcacttcgctttccttttagactgaaaaaggaaaactgaaagattgagcataaaaaaaatatagagaatgagctattacgtgcaaacaatggaaattcaataataagagtctgatcttctcccttaagaatatgcgattcctccggagtgaagttgttggggggaagagaagatgaggaagctagtttaattgaggaagccactttctttaatgtatactagctggtctacaaaagcatgacgcatgacgcttctcctttttttagtccactctcccttagaaaacggagctccttgaaagcagatttctaaattacataggtgaatgtagagatcaccggtgtcctactcgagacgaagtacttgtcgtccccaaaccaaaagggatgagggaaaaaggctcgagaaagcgtccttggaagggggaataagatcttaaaaagtgttagcggggagcccatccctctcgttcttacagaagacataagggggaatacacgacggacgaaaagcggggaaacatccttttcctgtcttctctccacagaggaaggaaagcaccgccaagccaacaagaaagcagaaactgcatgaggtaagactaagggccttgtgcgccctgcaagagattaccgggggtctcggtaccaggggggcgcgggaacaagaaactccagtaaataaaagaaagacaataggagtcctctcaatagccgagggcccacttccctatatgcgcttacggaaggggaaaagcttgattctcatagattagacaatacacatgtgcaaacaagaaaatcaaactatcttcttattgatactatatatttatcctttcccctatagatccacgtttcttcaaaataaagatatagcaactaaaagaaagctaaatcgagtcggaataggataaagaacgcacgaaggatcagagagaaagaggattctaaaagctaaaagcctagaagactagattgtcagactcggaggtagcagtaagatctctgtctccagagaaggcatgaggggtttctaaaagtctcctctcattacttatggataaagctcttaagcttaagcttttacgaacagaaagatcttcccattctaaataagaatgagagtctttcaactagatgtgctcctttggctgggtttgagagagagagcctgagatagttggtctccttactagtccaacttccttgtatctgaaagcgatgacaggatgttaggtctagtaaggagactttttggagaattgacttccacgaatagactgttaggctaagaagaataggttgggattgatcccacctttgaaagagtggttttgttctgtcaatacagcttatcgagttatcaagctgaactgccttctgtaaggagcttgaatcgttcgtttactctaagtcttattaccgacgcgatggattgctatttgaaaacactttcaatacaaaaagagctccttccggctatactctagttggacagtctttgttcagtttgagaagtcaaggaggcacgaagagctaacaaagagtctttctatttgactgtccgaaatcaagtgggagattgaattgaaaaggccccttactatagatagggtgttagcgctgttttttgaaataaggacgtttagatttgactaataagaaagaaaggggcaagccaaaacccactctgctgagttcggctttcggggctacctactttagggcttatgtaatatataaagaagaaccctcttagggcctttttgtttaagggctgctcgccttttgaatagaaggaagtgggggagcagaggttatttcggtaaaccgatgcatgagctgaggctcccatgtcccgccgaccctccgaaaaagtaagggctcatagggagtcagaagcaagcagagtaaaaggcgggtaaaactcacataagcagagggggagacacattcatgaaaagcgagaagccctgccgtgggggactgaccaactatgaatagatcttacttatgcttacgggtaagaacatatattagtccgtatcgtgggtctatttgttacaaaaggcgaacatcccctttccaaaacattaacataggtcctcaggcagacatcgaaaagggggcgaaaagagtctatttacctttacaatatttcggaatgtatcatggctctatctattcattaaaaaaaaaaagagttctgcatctctccggggctgggtgaacaaataggcgtggggaagagtgagagggggggctacgagccctctctcgttgttgttcccggaccacccatctcttccttccccttcgcctggcccggtgagatctgatttatagaacgaagtgaagtgataggaagagaagactgctggcgggaaatccctattcatgaaagccccttgttaaggttaaggggaaaacgaaagtgcgctcctgcgcaccagctgaagaaaggagctttggaagcttaccttattattatattaaaaggggaaagggttccaaacctatctgactaataagaagaaaggggcaagccaaaacctactcctaacaagttgctggatcgaagtagtacattatacatctgcccgccagcagcagagggggttcgattcccgttatacgcgatgtggcgaaaaagactgattcaacgagatatgccttgcctgcattaagatttaaaacttgtcgtctactttcaggaaatgtttggaacagagaacttacaataatacaacgccgtattctccgaagattgaggaacaagaagagatctattaagagaaagatttattctagagaaaatcttaacagttacatccaatcacaaactacacgaaagttgtcccttttttatggagatttacccatcacagagatgcacagaggaagagaacgaacttcatatatcccttttctactcaatccagaaacaagatcggacgttatcccggttcgtctccatttttgtgaaactattcctcaagcaaggcagccgataagtcatcgaagggtttgtgtgaataatggaatggttaacattactcattttaaactctcccacggtgatataatatcttttcaagaaaatgatgcgagaacccgcggtgaagaaataaagagatccttctatatcgaaatctcagttgaaaaaataataggaaaattcctggatcacccgtggagaagaaccaaaacagaatgcttccgcctactcaaaactaagaggggatgccgcctactactaaaatcccggtttttgcaacagttgcgttcttctatgcaaaaagaagacttagaaagaacaaagaagtttggatccgaaaaagtatgcttaggcagttctttcactgagcacaacagaatgaagaggaatttgtatcatttcaaatccctattcttatcgaagagaaggaacgagaaaaaccgaaatattcctactcgaacaagaagtcctatagtttacaactcttctttatatagtaattcgacctattgctccgcatccccccatcggtttactaaaaagatcaaaatcaaaaggatcgaactacctactcattattcggaggtgaatcatagaacaccaaaagctgtggtatcttatggacctaacataggtcacatacctcacgacataagattgaaagatccaaaccttcttcttcggagcggaaagggacgtggccaaaacatataaagatcggcgtagtcgctcatagggacatatctatccggatagaggatagtctaggccgattcatagatagatctctctccatatagataggtatctccgtgaatagagataaagatagggatccatctagatcttgattcactatttccatattttttcttgattctgattgattgccttttttttgacgacaagttttaaatcttaatgcaggcaaggaaagatcgtttttcaattattacttgctgggtcggagcgtagacgagcgagcagagccaaggaaagagggaagcccgtcatagagtagtcgactagaagtagaagactgctggcctgagagaaggcggcctctctcgggaaagatggcccaatttctcttctttctttttgatttcagctttcttttttttttttcaggggtccagaaggctaaaaggtgggggagaaggaagccgaacctctaatcgacctggacacataaaaaattctcggcgtcgagagagatttgagattccgtaagtaactcagtgactgctttctaagaagggcttggaagaagaaaatgaaataggaacaaccgcgctggtcgtaatagatcgactttcatgctagttcttgctccagcatgaaagttccatttcagggaaggacgacgtactatgatactttctgttttgtcgagccctgctttggtctctggtttgatggttgtacgtgctaaaaatccggtacattccgttttgtttctcatcccagtctttcgcaacacttcaggtttacttcttttgttaggtctcgacttcttcgctatgatcttcccagtagtttatataggagctatagccgtttcattcctattcgttgttatgatgttccatattcaaatagcggagattcacgaagaagtattgcgctatttaccagtgagtggtattattggacttatcttttggtgggagatgttctttattttagataatgaaagcattccattactaccaacccaaagaaatacgacctctctgagatatacggtttatgccggaaaggtacgaagttggactaatttggaaacattgggcaatttactttatacctactatttcgtctggtttttggtttctagtcttattttattagtagccatgattggggctatagtacttactatgcataggacgacgaaggtgaaaagacaggatgtatttcgacgaaatgctctggattctaggaggactataatgaggaggacgacagacccactcacgacaataaggagaagcagtggttcgaatccacatcgtgagaccaggacagtgtggagaagcatcgataaatgctattaacattgatgatacggcttagaggaattcctctcttgctgccggactgattcctttccttttgatgtggacaaatgggcatccctagaatcagctgctctccttcctgttggaggaagacaatgcgaaaaaattcataaataagtaaggcaaggtgattgttcgttgacaacattggggcgtagcggattgactattgggatctctttagctttagtatgactattactataggcgctggaggaagcttgtcatagtatgtaaactttgtggtggatacgacaacaaaaaagcctttctccccaaccgaggtgatagaccaccttatggccgatgtgattaccagccaaagggcaaaaagacggggttgaatgcgactctaccaataccaatctcctctggagcaaggaaaggcaactctgcctggtatcggtaacgattaacatattctttttttttagagaggggaacccttacttaagaacagagagtggccgagcaaaaaagcaaggcaagggataaaggagaagtacccggcccggcaaagaagggtctcccattaacaggtttttccttagtaagctagctttgtaagctaagcaagccaggttctctttcactcctggaatgagccttttggcgactctctctcaacacaaagaaagaagagatgaaaggatcttcaagtagccctgactaaggtttgaaaagattcccgggggtactacagcttgcgtggaaggctagggtggtttttagaaagcgcgaagacagaagacgtcgtagggaaccaatttctatcgctttccccctctagtggtcattcattcttttgatgactcgcagtcgaaagagttggttggcagttcaaacctcagagggagttgaagagaggcctttcagttcgttcaaaggcactagggacgagccattacagacggtctgatgcttctggagttcgctcatatcgaattgtccaaaagctcatcaacctgtccgagggatgatgaaggcgatgccacaattgagggaaccgcccttttactcttttttagataagaatgcgaaagaccctgaccctgccaaccaagcccactcagatagactaagtagactaaaaaaagtgcacaagaaagactaaggaaacaaaaccttttctcgataaggctgggccaagtagcgacacttcacccagattcgatcatcacgtcaacttgctttattcaacaaagtgatcaagcttcttagccaccggggaccggcctcgtgaacgcattcgctaaaggcactactggccggctttctcaatcttcaatctaacttcagaaatagaagaagcccacttgacgagatttgatctaattctctttctaacatttttggattgacaggaagctttcttgctgtgtgattctgccccccactctgccagcagcctatgtgtcgatctatacccagttgatctaccactattttactttgcacgttctggataggcgcgcatcctcatagagcgaggggtagaaaagatcaatgaaagactagagcgcgagctagctgatctaccgacaagtccttgatttcttatccgcgaaggcagacttggactcattgaagaaagcacttgaggtgaagactaatgagcgattgcgacaactacggaccccttaactaggttttttactaaaaaaaacgaataggctttcagaagcttttccacacaaagaggagaggaagtgcttgctgccaacttgccagacgagcggacatctgagctcagcagcgcatttactatttgatcgaagggatggctaaaaggccaaatccggctaaaaacaaaaagaagagatcaaggagagggagctagacgagcacttgcaagagagcgaccggcagatctaaaactgctatagtaaagtagaacgaaagtacctcccaaaggttctaccttttcttgtgcgttcgggaataaatagaaagtttttaaatgtatagaagactctcgattgattggttgtaatgttcacgaggttgtatataatccaatgttcagtgatatgactttcctactgactgaattgcttgaattagttgaaggtgcggagtcttcttcttttgatttgagacgaattcatttttctactgaaagtgcttttgatagggaatagggaaaagccttgccttattcaagagtaccaggaaggagaagaataagcattacctctgttgaagggagaagcccctccctttgcttatttattcttcctggtcttcgggtctcatctgaacggctcgctgcctatttagttacattttttgttttgattccagaacagaactagagatcctggccccctcccttgaaagctcctggtgctgcgactatcaccggtaagttgcgtcggatcaacatcgggattaaaataaactgcaaaagcaactaagtcaacgcctatttgctgtggatctactggcccggacgcttgaatctattccaccgcaaacaaccgaatatactactgcaggatcttctgctgcttttgttgttattgctctcacctgtcactacgccacctcagcagctgggactccctaaccttttctatctatctttagaagtagggcgagtgagtccgttcctttcccgtgaaggttttgggatatgtgaccagatgcttcctccagatctaacgtctctatcaacaaaattctcttttcttcaccggatcgatactaacttacctactcctgctcctaccggatccaagagggccgatgcccgattccccgacccattactcattccttcccgactcgatagggattgcaatctcgagagagggagcaacaattgacctccgacaataggtagatggggtgggctccgatggatacagtgaaatctatccttattccgcactccctctcaccggcctgaaacatatataaatcatgaattcttcagagcgggccggcaggccgggcgtacggggaccgtcgaagaagtgcctcaacgcgccgcagccactactttgactccttttatgcaattatgaactccacggaactttatcaattccaacgcaacttatccttttggagctgacgtaacaaactacgcgagcctcccaacgaagccaacataaatccgatccgaataaaaaaaagaaaaggaagtttgattattgtggtataccagccaccagttctggaacttccagttccaatcgaagcatatagatccgtaaatagatttgtatgtatagccacttcagtcgtgctcgtcctttctctaaagtatcttttttctgggaacatggtcaaccagaaattattatgttcgcgattcttcatccaccgatggaaaaaatgctccagttttccattctcatatgaggccggaaagtggattggcaacaggtcggcacgaagtgattcatcatgctcaaacatgagccgatcgctcgttagggacggtttatagatcatcaaattcccacaaatggaatgaaaagtgggtccatgtaaatgatcaagacctcgcaaacaacaacgctccttccccatatggagttcggaacccaaaggcaatcgttgagtgaactgtatcttttttgtgttagttgacctaagccgcacccttactgctggggtggggctcggcctccgaaccgtacgtgggacgagtttttgcctcatacagctcgggccgaagaccgggggaagtttagaagagatggggaaacctagcagctgccggtcggggcggggataagcttgcttcttcacaagcctatccccccaaaaaaaccgaccctgtagcgctagcgcttcgccttctttctattccatcccattccattccgggataggcggctaatactaaaataataagtgaagtagtcgtcgtctgaccaatcggctcggacaccagaccgcccgtgcccgcccattttgtctcgccctaaatggaatggctctcttagttacgctgcgccccgacccgagtccccacgtccgcttttctccgcccgcaacccaataagttggcaaagccaacacaagattagggccgtccccttcattctatgctgaccccggcccgggctggcttcttgggaagcccgttcccaccgcgctcacggcccggctggcctgccagcggtagtgggaattctcccgttccctggtcaaagacttggttggatgcgggatctactccacgaggagcggtacggacgtagatgatatcatcacgacccctcttttcgtaccgctagggatgcttaacgccacttcgccaactggcgttacctgcgctttcgtgtctctcagtgtggtcagcactgggtgtttccgagcagcgaggcttacacccattcgcattagttcatccaaagttccttacccttatgcacgaattattgaataagccatcttcctatcaaggttaaggagtcaactgagcatctcagcggcgggattgaatacccggatcgaatcagagttcacgccgcccgccctgaacaaataggaggcgtgggccacaggtcgcacataagccgccgggtcgcacgacagaagaacacccaacataaagatgcacactcctccatgtgaaatattcatcttcatagaagctttttgatagtagtcgtgaccaacagccatcagctctcggcttgttggtaaggtgagagcttcaagcccgatttcaggtggcgcaccctccacacaagcaccgcccgacgaaggggggacggggaaagctacaggcccaaaaccttcgacccttctttctaaatgggggtgcccgaggcacctcatcttctcatttcgtcgttgctcattccccttaggccgaagtctttggcctttccttctccgcgcccgctcaggcttcgctgacctatcgcgtggtaaaaagaagaaagtacgaaagaatagtaaacggagcacaccgcagaaagattctaaatatgagaagtcccccttggattcgagaagaaggaaatgaagaacgggaacgaaacgaaataaagcgtttctagctctagtttcggatgagcttctcctaattatgtctggtaatagaataggggggcttgctctgaccaagactccactttttgctccgtccgcggagcgtatgaatttcctggaatgtagatagaccaaaagagggaatgaagagataggaataggaattatagtaccattggaaaaaagggcacctgtgggaacatctctactgacgaaccatttcaatagtacgggtgctgccgtgccacgaggcacgaccatggaagtaatgaaaaagaaaaagttatgtagttggaccatctgttctatccgttcgagttttgcttctctagagaagatgagaggctaaaaatgaaagtgttcgcaacacataccgaaagggtactaattaagccgaccattaatgactagttaaaacaccaggagtggtctgatcccctatttgatcagaccgctctgagaaagagaaaaagcaaactctcataattcggagcccagctccaacaacttcttcgtaagtgaggtgaggtacttcctttggtttgaatagggggtcgccctttttttggttgaagtagccacgactttggtcgtagtcagtttaaccccataaacccagtccacttgcagccatgttgatcaaaatgactaagtttaatgacttgaccagtcacaagccctcgtattataagattctctcaccctgtggtcgacattccattccccttagtcgtaggtgctcgttctattttgatttgaatgggccggggctcccgaggtacatatggccgtcccttcgggtgtctcggtgatacaaagaaagaaaagacgatggtttttaacatacccttgaacaaaaggccaatccttaccaaaggaggaaatagaatagaataatctaccttcttttttccttcccgttgattccccccgacaataaagctgcacttccttctaacaagtggctgagagttagcaagcaaccttggcctcttggcaggaggttcgctgtccccctcctttccggtccggccgcagtacggcacctgaactcgaagctacgatcagatccgattggatctggtcctatccgacccaaccccggaacttagaacggccggcctgtttggacggtagaacggggagagggggagtcgtgcccattctctatccgggcacgagcaggaacataaaaaaaaaatggaaaaccgaatacatgtacatgatctaacgacatattcaaaaatacgtgatccgatttgataggctgcccgcagaaaggaaagagtttaccgaccgcataacaattcattcttgtgtgtagcgcgtgggcccatgtctctcgaacgatcatagtacggccgctcatctaatataaaatcaatgagtagatctcacctccccttccccataccatagccggaagggatagcgtatccacagaagagagagtacgggcccttgcccaacatttagtttagacgcggctcgaatgcctttatgctataggctgtgttaagcatgcttctttgacagaaaacaaactctttttccatgacaacagtcgcgactataaagggcggggcggtaagctctctatcaacaatagggggctattcatagtaaaaaactactagactatatggattccaactgaacttcaacttctacttggttgattaattcaggggcagtgctccaacataatgttggacgatctccatttccatatggtaattgaagtcaaacaggagcaaagcaggtgcaattcaatccttattcctagcacaaaaaagcaaaacctcactagaccgaggcccattgctatggggactacactatataagagaatgactaaggtaattgccaatagtttctattgaaagacaggctggctctttaaaaagggcgccctcctaatctcattttgataggaagagatattgaaaattttcccaaggaggcttactactcagctgatagatcaggtgagccagccatgatcactaaactcaccaaacctgcagcatattcaaattggaatcataggtttctatatgcttaaggaaaatgggatttgcagagtaggatacgaaagtttatttatatacaatggaaagcccctataatccatggacgaccagtggagttcataaaagaaaccaaagaaaggtccgcgacaaagctgtcccctctctccatatctctacttactggctgggtgcagataacactgtaataataacaaagccagatagagatactgttcgttcagaattgattcagatggcgaggacccacggaaaaatccaccttattcatgctccgcacagcaacttgcccggtcaatattatatgtctatgctaaacttggtgatctattttcgttgccccctttaagcgtatgtgatataatcattcttatctcagaagagaagtatgcattgtccccacttaagttattaagtattcccaaagacgaggcgatttctttttatgttgaaactttatgtcagccaggggaccctgatcataaatgggttgtttgtcccggtgaaagggacgctctcgttttaatcgctctggcgcatatgtttaatagttgttttatgcgttcatctatctttcaggagctgtcgtgtggttttcccagagatcgccgtcagttctttgccaaattaggtggagtggggaagattagaactattttcatcttgaatctagcaccctcacaaggtactattcctcataaaagaattttacgaaagctggcacccttggtgcgtgatagctacgtaatatccttagtttcatcctttttaaagatagcagtttatgaccaaaatggaattaattgttctattacggaagttgggatcccacacgctgggttaatcaaaaaggtcttatacaattttatgttggatgatttcgaccggggatttaaacagctataccctagtctttcttattatcgttacttggctgactgttacgtattatttccattgtttagtctctaaagcgagcagcagtgtgaagaagaaatgaatagtatcctcttagagttagatcttgatggggatatcacaactattctacctggtgggggtgcccatgtgactcgtgatgggcctttgattattctaagtcgagattgcagtcttcacgttgtcgaacagtcaacattctttctttagttcaatttgtagtcaatatgttttatacaaaaaggaacccatgcttagataggaaatcctttttttagagagccaatgccttaagacagaccctaatagcagttgtcgcctacttcactgagttgtggttctaaaaagaggatttttcttggtatattccatcaagagaaagccatatctatatatataaagaaaaatcgaaattgtatacaggtgcttacactctcctgaggattctaagacccgatcacccgtcaaagaaatatccttaggtcttaagtctacagctccgtagcttgtgtcgcctacatagggtagaaaagaatgctttgcataaacatctcaatgtccaagataaaaggaacgaggggaagaatcgacgaggccagtgttctcgaagagaaaatcgtgatggaaaaagcgtgaggagaattcgaaagtcgagatatgcaaaataaaaagactccctgggagatggtattctttgttttaggtcttgatagatttttctattgattgaagttattacgctggctgattaaatctcttcctaacgcctttaggggctgtgaagagagcccagttccaggccctcttttagaaagaaaaaaatggtacaaaaagagggcttgggggtatatatactataaaaattgatgatggtttatcatcatcagaactaagatcagtctaggtcgagatgaatggaagatgcttctggaactagtttttgatagggtctatcttagctcgaaggaaagaacaaccaaagttacacccccaaagaatatggattcaaatcagttagtatttgacaaagaacctaacggaatttaacaagcagtaaccggaatcaaagttttcaaaaatggtgtcaaccggtaatagaatgtagctagataactgatgccacagcatccaaaatatgtgggatggagttcatggtacactaacttaaccttcaaggtcagatagtgctacagtgaacatcaatccactatctagctcaaaattagcctcacgaactactaacactattattcgcgtagcccttttgtgtgctatttcatcataggctgtcggaacttgcttcttagcgctacgtgggaagagaatttctctattcagcccccccctattacaaactttaacttctcggtctaacttggactaatcccttagcaggcaagaaattcctactaaccagacagaaagtaagtttccactcactaccaaagcgctgtcgcacctctactattttcggcgtaacgaggttttagtctttacgagggcaccccctagccagattcaatcccaagggtcaatcaagcctttgaaactagtgaaaatagtcgtcacagtctgagttcctgctttcaacgagactttcttagcttgtcaaactttctctccttcaccaggaaagttatccggtaagcaagatctttgattgatgtgcctgaataaggttgatcaatggtagctgcttggagctttctctataccttaattgaactaccctgctctttcttagctcgggttcttgcttaatgaggcgtccttgtttgctcttggattggactaagcggcaatccttactgtggaagcagaccttgtcattcttctccttcaatgccagtggataagtacactagggctggaatgctcttttatcatgtatgtggattacttggtcgattacctgattgcactagtctcatagccatctctttagcgtcccgccattccttcttgttaacacaggaaatctaactcattctaaggtagagctcttagagtcctacttaaagttaaaggtagttctttagttaaagcaaggagagcagaaagcagctaccggccatcaggagatccacgactttaagatccgcatgcatgcaagggaagattctttatagaagattctctttattcccacctcaagctcggtcattggctgtcctcctcaatcgattagactatggcgaatcacttgtgtattggtctttgggaaagtgtaagacgctattgctcgcaactgggtcttgagtgtcgatctaacaaaaaagtaaactctagttgcttctcttgtccgatcggaaactggtcttctttttatggtgtaagggtcggcaacagctccctttggaaggaatcgatcgtcaacgtctttggttccctccacccgccgccttcggtcaactcaaacaagaggccaggaaggacattgttgaaggctcactgagtgcttataggttaaagggttgcactagactcactccacgggaactagcttttcggtttgcttaagatttggcattcattccccctccccttcctgaatttcgccttattgcttattgtctgctatgctagcctatgatgaagacctttcattttggctctgtagggctaccctatggtatgggctgttatctcaagggccaggttaggctcttcttgttggagtatcctcgctcagaggctaaaatgaatttcattctctcttttcttttgggagtgcctgaagagacctgcttactggaaggtaccattctaaaagaatggtgaaaaggttacctaccctatgatcctccttatcttacagaggtttactacgagccatacccagcgggatacatattgcccaaatggaacctaaaagatgggatgggtgatccataagatcatttggcgaggttcatccctcagcgtggggatccttctggaaataaaaacttgttttgttgaggcaatttccctcgtcgcttacccgcatttctcttggtatacccacctgtgtgcctcctaattccgtgaagtccttggagcatgtgcgatttattcaggatccttgtcaagaaagaagtcagtcccttattcttgattttatgttaaaaggtctggactcgaagagggagtcgattcacgtacttcaccatttcctgggtcgttatcgcctttccccggttcagggtatgggttctttctctattaagaaagtcccggtgtgaactcccctactgatctgactccagcggattctcgagaagccaattctctctctcgatctactttaccgacaagagctcttaatgaatgagcaatgagtttgattctaactattcaaagcagaggaaatagaatattatatagcctatagctatagggctaggctccgctcctcgctcgagctaccagctttcttagatttcattcctgttgactaatccgagtccttgagagcttagacgtcagcggggaagaactccgaaagaatttcatcggctcctcctctcttgccctcttgatggtatccagttgaaatggttgctggattgcccctagttcaagctctaagtcaggcattcacgcaccaaagacctctgactacgctcctcagcctaggaaagaaaattcccatttgcctaatacgtactactgtgcagcagatgatttagctgccgttattcctccaccagcttcttcttggcatcaagccagcccttattccttgcatcaacaggcaatcccgcataaaagaaaggctactgacttggctgattcaacaagggaaaaaggcatccattcaaactgctcccattcctatgttgacaccaaaccaagagaaagaaaccctggagccttcctctctatccattcctttttcataatcataaaggatggaaatgcttagcttactaaaccagcaacagcggagtaagctcccatatccgtgaaggactgctttccagcagaggaaaacttctcgttgctgagcttgccgttaaagagtaagatgctgattctatagcagctccgattccttcaccgagaacgagaaggaagtcttatagaacgaacaagcgctaaagaagggggtgggatctctcctaaaagaaagaattgacctcgagcctgtcctactcattctccttttcccgttcctgaccctgagtgtcgaggggttagccttgagccaggtcttgattgtttattccattttgtcagtttaagtactggaatgggagttacggatattcattcctaaactatgtcaccgattggtgacctgatcccgctaagcaagaacagctaccgacaccgactctatcttaacgaccggtaaagccctctctctaggatatggcacttcactgctcggagaggaaagaattcttctccaaatcatctcttcctttatttaagttaagaaagaagtcaattacgttcgagctttttgtcaactgattcaactcaagcaatagaaagaaaagctatctcctctaatctctaagtatgcagagttcaatcaagctaagaactagtcgacctccttacttttttaccgctagaaccttcctttcacgagtgaacccgggcacgagcctaccttgtaagaaccaaaaaaggggtaccggcgtacctaccattaccatatagggaatgaactgagttagaggcatatgcttcctttaccgatagccggtaccgaactatccgaaagccctctaaaaggctcaagaagaaggattggatgatctgcggaacggaatgagaaagagcaacaattgtctgaccaaagtcttaccctttctttccctttcgactggcattatcacaccgccatcaccagattcaatagctgctcctagcccgattccaagacctgaccaggtttgaaagttcaagcagccttgatcaactataggaaagtaccagttttccacagtgacaaggacttcttagaaagcattgattggaggtctcatggtggcaaagaaaaagaaagaggaagcgctcttgttcttgttgcgcggaccccacaataaagaaagatggaagacaagaagctcagtagcaaggccgtctcatagtcaccacttgtctgtcgtttcaagcttccaaaacaagcagaaaaacacgttgtcggttcagcagctcgaagttcatctcaataaaatgttaggtcaatcacatgactcatcctgttagtcgagcatagctaacgctaccaggacgctacgctgcgcctgcactgacgtgacttgcaaacaaggctgacgccttatagccatatacgcaacgctcgggaccacctcccttcgcttcagagtcttaggcgcagctcttctagtcagagaagagtccagttgcgaacctgtgcgctcctatcctattgttgcttctatcacgatagggaatcgtgtgattctttctatccccgtactttctcgctcttatggagttgtattccctaggttatgcagttatcttccctggcctgacagtagtcaagggaaaatcacttgagctttttcgcctttgctccttctttccggagcgcactaacggaaaacctgagataaggtatggaagcagtctgattatttccacttgagtcgacttaagtctttctctcctcgtacagtcttggctctagtaaagagaaagaatctctccttaccctactgcgggaaaaagcactttctatccccccgtgctacaaaacaaacttatctaagcactaaaagcaaagcaacaataaggaatggaatgggagaagctatagtgcagatcacttttcactttctctagagtccagaccttgtccttggttctatcagctatggagtcttcctctggttcttcccgtctctagtacagatcaaatcacaggatctctgtatgtatgcgctgaggagctatatctcccggacgaaagacttttaaaccctgatttccggaatggcagcaatcgacttctttctgtcttacagctttcttgtagtactgctctcttttcaagcgaatctctatttcaactgcattccctattgcaaagaaatcaacctcggttctttctgttgataggttagtttgattccaggtgtgagcctcttcagttgcagtgaaagttcccgactctctagtgctatcccccctttttcagcctgacattacaaaggtagacttcatccaccggacgccctggctttctttttcgttttccaatcttctgtcctttccttcattcttgcagatgcaaatcatagatgacctagtggcatttatgccagaccagagcattcttctcaagaaaagaaaagaaaggggagagggtgactgaatttcactctttatcattccttactactcctcaattcccatcaagtgttgtcttatttcccaagccactgctcaatcctccttttctgattgattgaaagtagcaaggaaagacaagcaaaaactttgttggctcaagaagcaactgaggagagacaaagagtagtaaaggaaatacaagtagcagtctcaggtcaaaggaatcaaggaagaatttcttctgatattgcggttactcttccagaatctcatcctgagacctaagtatgccattctcttcgtcaagaaagatcgagcagcatagaagccttgacttcaagcttaggtcttttttttgaaaaagggaactaaggcaacttttaggtgcagggaaagaggttcgctagccttttccctagctttttttgtcaactatctatctttccgaactagattagacggacttacttaaaatgaaaaaagggctaaaaaagaaggacgaagtaatttcgtatataaagatatggctttccgggtttagatcgaaatggaatccccgaaaaccagggctggagtcttagacttcttctgcttcgatagagggactgacagcctaagtggaataagaatcattcggccgattgctctgactcttatccttccttcgctgacagagaagagagagagcactccccaagccaaggatgagtgccaaagagaagatgggcaagctagtctatcagaaggagaaagcgagggagtgagattttcgctttcattagggtagactgaagaccaagccaatctcgattcaaaaaagaaaacttattgcaactacgaaggtgaagagatgctttctcattagactattttaaccgaaaaagtctttatgtcgaccctaggctacgattcttcttctcttatgaaatttatagttagatgaagactgctctgctgcatgacggagtgatctttccctcttatgaaaggcgctatctcactttcgaaagagagtctcgacgtggcggtctagacctagctccatagctgggctagtcactggctagaggtcgagggacctagcggaccggagggagccgagaatgttatgtaaaaaggaccaaggaggattcaggaggagaaggaggaggagtaggagctagctttaggggcggaatcgaagcgaagaaattagttcatgccacgacgatccatatggaagggcagttttgttgatgcattcctcttgagaatgaagaagaagagagatcttctttttaacaggaaaatttggtcacgtagatcttctatttcgccggaattcgttgattgctccgtacgaatttacaatggaaaaactcctgttcgttgtaagattactgaaggaaaggttggtcataaatttggagagtttgcttctacacggaaacgaagaccttcgagaacaaatattggaccgggaagaaaaagggggaaaaagtaaagtctaagcgcatatggcacgaaaaggaaatcctatttcggtaagacttgatctgaatcgtagttcagattcaagttggtttagtgagggcgaccgcgaaagtcaccgaatgggtcagtcttttagttctcccagattcgaatctcaaaggaggacgttgcagatgcccggggcggacacgacttcttcttaggctagaagaccactggaagacacccaggactatagcatgtcgtgaaagaagcacactggacgggcgtgcttcgaccgtgtctccggggcacagttgaatgtagatatcatgaacgcgaggtgcaggataccaggccgagaaacccgggcaaccattcccctatgtgccaatcgctagcgcatccagggccccggcgcccagctcagctggagaggcctagcctgatctgagaagtgctaattcggttcggatagacttcattcaagaatgccaccgccccgggaatcaataagaaaacaagtgctaagtttcagatcagtgaataaaccgaaaggaaagaagagacgtttctcgctcagcgcctaaagcgcactatgctccgcttcaacaaatgagagttttcggtggaaccggtgaaccacgcgagctggttagatgcgtgggacagagggctcgtagtacctgctagcgcggctacgcagtggaagggaaggagcctaaatcgacccccttctttttttctttgaaaaaagcagtaaggagtaaggagattaaactctcggatgagactaagcagctaccgaccgttccgacgcgcccttgacctattttgattaagaccaaaaacctatctctaaagtggagcctagtttaagctgtcaaacaagtgatgattgaatgaaagaaaaaccactagtagggatatggatggagtctcgctcagtaaagagagttgtaggattcgtaaaacaggagaagagcctttactttcaaatgacaactgcttcttcctgctgcgagggccttgcacgaaaccaaaccgccccccgcccgatcaagtaccagttgcttcgctggtaggcctacttaggttaggtttggaaccctcagttcttaccaacctccggtgtgtaatctacatctttctagctagaactaggtcgaataagaatcattgactccctctgctgtcaatttcttattcattcattgcgttcggccggtgctcctttctcatctcaaaccataactactctgaaccttagggaagataagggaagaccgcctgagcgaagcgaccgaaggaacttgacttatccgaaccgaacgatagcggcttaaagcgttgcctatcacgagcagcctcgctccttgatcggcggggaggagcatctcaaagtatggggcaaaggatgttgcgttttgactttgtctcccgggatccaccacaggttgggtttgagagccgtgtgataggtgactatccagcacggttcggagagcacttttagtctgcgctggtgaatggaagccccccctatcaagcaagaaggaagcggctcttcccacggcggagtcaccattgactctatttattattatggtaaatcagtgtatcaagatgtcaatctgagatcttatttcggttcgatacgtccacctacgagactcacctttggctttcgtctcggtaggtgtattattatacattttcccaaaagaacattcattcatttctttcttccccgtcgaccacgacgactgaaacgacgcgaaaaatccagacccgtaaaggagaagggccggtggggggcatttgggaaagtcgggccgatcgggtgtcttcattcaagcgacggtacagaagaagaacgaaacgaagtgagaggccggggggcagggaaaagagtcgagtcgatcaggctcgacgatcgggagaagcaaaacgaaatcaggatttggccgaaaaagaagcaaggctatggataccatgaccgatcaccatcgataaagaaaaatctgtctaaatcacttcgtgtcagcggggccttcaagcatccgaaatacgccgggattgaaaatgacatagccttcctgatagaaaatgacgactccttcagaaaaacaaacttattcaagttctttttcccaaagaagtcccgctccgaccgcccgacgagtcatctacttaaaaggaccctccccgcagtccgcccttccttgaattattcggtcatgcaatacttattgaatacaaagaacaaaatacatttcgaccccgtcgtagttctcaatcatttcgtggcaccgggcgtggctgaaccatctacgatggggggagctaatgcacagggaagaagcttagataaaagaatacgttcttgcatcgctttttttgtagaaagctcgaccagcgagaaaaagtgtttggccgaagccaaaaagagggtgacccactttattcgccaagcgaatgatcttcgcttcgcgggaacaacaaaaaccaccatctcgctctttcctttcttcggtgctacctttttttttccaagggatggggttggggtgtataataaccttttttttgaggatgcccgggaacaactcctaggtcaattaaggagaaaatgttggaacctcatgggtaaggataaggtaatggaattgatagagaaattcatagacctaaataggataggagaattgataaggggaatagagatgatgatagagatcatactgagaaacagaagaattccgtacgggtacaactattatttgaacgaagtgaaaaaaatgcgatctttgttgtataatagaacaaacactaataccttaattgaatcggtcaagatcaaatctgtttatcaaagtgcttctccgattgctcaagacatctcttttcaaccgaggaacaaaacaagatcatttcgttccatttttagtaaaatagtgaaggatattccattagtaatgaaaaaaggggtggaggggatccgtatatgttgttcaggtcgattagaaggtgcagaaatagctagaactgaatgcggaaagtatggaaaaacatctcgtaatgtatttaaccagaaaatagattatgctcctgcggaagtatctactcgttacggaatctcaggtgtcaaagtgtggatttcttatagtaaaaaaaaaaagggacgtgctatatccgaaacgtacgaaatatagtaaatatcgtaaaggcagatgtagtaggggttgcaaaccggacggtacacaacttggttttggaagatatggcactaaaagttgtagagctggtcgtctttcatatcgagccattgaagcagcgcgtcgtgctataatcgggcacttccatcgtgctatgagcggacaattccgaagaaatggtaagatatgggtaagagttctcgcagatatccctattaccgggaaacctacagaagtaagaatgggaagaggaaaaggaaatcctacgggttggattgctcgtgtgtccaggggacaaatcctatttgaaatggatggtgtgagtttgtcaaatgctcgacaagccgctacattagcggcgcataaactatgttcgtcaaccaagtttgttcagtggtcgtaagcttattaatctgacccaaattccccattttggtacacgccaaagccttccatttcggcggattgaaagagccatcaatgactagaatctccttttagattcgaaattcttcgtttttttctcccatgctttccgttggtcaacaaccaactaaagtgctctatacttcttcactactcgtacagggaaggtggaagaaattcagtctctcttttttttggggggagcagagcagtgaaagaatgaaccaaaccaaatgattgttctagaatggctattcctcacaattgctccttgtgatgcagcggaaccatggcaattaggatctcaagacgcagcaacacctataatgcaaggaataacagacttacatcacgatgtctttttcttcgttattctgattttggttttcgtatcatggatcttgggtcgcgctttatggcatttccactataaaaaaaatccaatcccgcaaaggattgttcatggaactactatcgagattcttcggaccatatttcctagtatcatccctatgttcattgctataccatcatttgctctgttatactcaatggacgaggtagtagtagatccagccattactataaaagctattggacatcaatggtatcggagtgcgcctcttcacgagggtgattaaagtgcaacgaaatgccttaaagttgaatatggttcgcgaagcatctggcttaccggtaatctcccattcccgccgtcgagagactttaataactatagcatgccagaaacggggagttgaggtggttagacctataccccgaaatgctcccagcataggagcctatggttccattcttgttgttgctggaggtacacatccctcttctcggtgtggaacgatatacgagaaatagatgctcagcctgcaatgtccgataacggcgctgaagtagtgaatctatcggcaccatagcagtggtatacaactttggacctaacggccggccthgtaacctttcggaatggggatccccgttggcaacaaccacggtagtagttgcggaactactgggccgggagagkacaacctcttgttcctgctcctctttcttcgcttcggggacggaggtcctacggtaggtaacagcaggcacaagcaagttgaccgaaggggaccagcgcttctactcctccaccgaggagccgttcttgcgagaagcaagggatgtcgtgaacggtgggaggtcacagagaattgacctattcatagagtgatcctatgatcgatacaggatatagactatctcattctttvttctatgcbatttctgramaaaagarrahvbcgkactcaacttctmascwagagttkgkggtkggacckcttggcataatgcacgctggaacgtgggaattcgaggtctcatgaactactactaaaaccgactttgttttgttttgtttgtggacaaacgatatccggtcaggcctatggctggatccttttagatctacaggccggccggccccggccgtttacatgagcatagggaatctatactcgagcgttccactgggcccctgacaggataggtgaggaatcactctggatcttcttttttgggctacaacttcgccgagccgactagcatccctttccactgtgcatttttcgaacaaagaagacgactataggatcgaattcgctcttcaagaaactgctcgtcccataccttctgcctgtctcatatgtgtggaacctggtcttttcggttccagcctctccctcgaatacatagggtaggtagggctgggtgataaagggttccctcttgccaataaactttccccggccttcgattaaccttactcataaagggtcttacggtcgggagaactacctaactaaagaaaaatagtgttctttctaagagtaggcgtggagagcttttgcggggaaacttgcaagtacagtttggggaggcgggcgtcgaccctaccttatgagtattcggactataacagttccgatgaacagtcactcacttttgacagttatacgattccagaagatgatccagaattgggtcaatcacgtttattagaagtcgacaatagagtggttgtaccagcaaaagttatatacgttttattgtaacatctgctgatgtacctcatagttgggctgtaccttccttaggtgtcaaatgtgatgctgtacctggtcgtttaaatcagacctctatttcggtacaacgagaaggagtttactatggtcagtgcagtgagatttgtggaactaatcatgcctttatgcctatcgtcgtagaagctgttcctaggaaagattatgggtctcgggtatccaatcaattaatcccacaaaccgcagaagcttctccagtcttcgtcggttccccaaagaagacactattcttttgggagacccgtcgtcgacgaagatgagctctacgaagcggcttaccaccccttctacgcggccaacgtagtccacatccctggggaaattgaagacccctttactctggctaaattaagtaaattaaatgggactctcctagccatagcggatctcttttcaacggccagataaggggatcgtacactaaagagctgcaacttgaattgaatgcgaccgaagaaggcgagctggcggctaagctggaagagctgcggattagggaaaagcggcgctataatttacgctagggtgagcaagcgctagctctttctcttgcggtgaaataaccgccgtatagaggcgaacagcccttatagcaatagcaaacggcctacttatagcctttcaacaggtcagtcaatatcagtaagtagggtcctcttgcctaacggagtcagcccaacatggacaatgataggcagaccaaagatttacgcagtcgttgcgtgcttgctttgcgcaccggcatagcagaattagaatccgctggctcagatgagtggctcttggcttcgtaaacatatctatgttgttgchbtccacahccacbcagbtggcagcghtggatgcttatggagatatggcttggcccaggactattggctttccgtcaagtgtcagttcagccatagacattcaattcaatctcggagatagtcaaaatgccattgtccgttctaaatgaaaggaatgagataggccgcttacacacgcttcaagtcttcttttgctgattcaataacagtctggaaattcgactgaataagtcttagtgtggttaagccggggccagggtcagaagttcttccatctcctgagataagatcagacagagcctatacgccttcttgctttgctgcagctaccgggtattcattcaaaagaatgcatttaccttttctccccttccttcggcatccctgactcgggcatccctttcaggtgcagttgacgtacaatttaggtaatttataaggactaaacgtactgatgaaagggaaaacttaggaaagaatagctaaggagaatccttcgtttgaggaaagagatgataaaataagtcatgaaaaaaacccagtttgttttaaggctctcatgaagccttagggcgaattcctctcacattggaaacttcgctcacttcctatattattcgcgcacctacctaccacaatccggttccaagtcctttattttaaaatcgaggagtagttcaacttttctctcttcgggactaagagaacttacttactaattgaaaaaaaagacaactagaacgaggtttttttacgtgatcggaaatcacccgtcggtgatgaaccagtacgcacttaggatagcacttcgggagagtgagatccaggtggcatatcaaaagacttatcaaaatcgccaccatacgagacttgcagggcatgcccgccagaaagtgaagagaggtttataagcaccccgacttaggaatcatgacccaccgaagaaaagaagactcgaggaaaactattgatccctttgatgactctcctcttcatcttcgcgggttgcagagaagaatccgaactgaggaaatgaaaaaaaaagaaaagtatctctttctctttctacgatcacctgtagcgtccttaaaagtcttagaaggagaatctaactattctcgaagagattcttgccaacaccattaggaagatgagggaaaggggaaaagaagtcaaattcgctatttccgacagctacggtagtagagaaggagagggactacttatgagaaagaggagtctctcttctactcccgggtattgaaccgggatgctttggtactagactgggcgggcgagccataatcacaggggagaaaggcgcagatcttttcatcctccgccaacaagcagagccgacaccgagctacttcgtaccttttcattcaaacgggaatgactccactctcagtcccagtgtggcttagactagtagaaggcgtaaggatgctagaccgctgctcaatactggataatccacgttcatcggtctgcagcaagcactgacttttaggggcggcaactaaagaggtagcgagactaagcgcaatttcaggaagagttggacccttgcctctaagcttccttctacccttgtgctaaaggacaggaaaaacaacttctttctttctttttttttaatatattgaataatggaataactcgaaccctactaaagagtggctttcagctcctccccttctttcattcagcgactgggtacgcacttcgccatgaaagatcttggtgatcttcatttctttcttaggaatcgaagtcaaaggtacatcgacttctctagtcttgactcagactaaatacaccttggaattactcgaactcatttgcaagactccaagccatgtcccacaccccttgcgtctggcttaaagctctctgcatacgatggtcctcctctctctgatgcaacggaatatcgtagcattgttggcgcccttcaatacctcactctcaccaccgtatatctccaggctgtaaaaggcatcttacggtatatgaagggttttcttgggcttggcctaaccatcactcagggactttaaaccaccttctttgcattctccgatgccgactgggctggctgtcccgatagcagacggtccactacttgcttctgcgtatttctcggaaacaacctactgacttgggtttcaaaaaaaaaaagaaaccgattctttccaggtctagtgccgaagcagagtacaaggcactcgctcttactacctctgaactcttatgactttcttacttactacgcgatctagcggtgccgtttcgctatcaattttcgtgcactgtgataatgctagcgctacacacttggtggccaatcctgtgttccatgtccgctctaagtacatagaagttgactaccacttcgttcgtgacctcgtcgtcgcaggcaaattgctcattcgacttgttcgtagcaacaatcaagtggcggaccttttcactaaaggattacctgaacccccttccatcattttctgctgtctcccgcctgcccttctcgaaagaatgggctcctggccgtcctatctcattgaaaaggacaaaaccatttacttttccaatcaaagaaagtgaagccaccaaaaaaaagaaaaagggtatagtaatatatatataaagtcaaagttcaatggtaacgacttcttccattgacttcaggattgcttggtttcagggaaagtctctcgctcctctccttatagcgctggcctctgtctttgatcttggctcgagctctgtcctctcctctccctatgctattgatttacgtaattggaaataaccaattaggtttacgacgaaacctagaaatcgatcatgatccaatttgagtacctctgcaggatagacctcaacagaaaactgaagagtaacggcagcaagtgattgagttcagtagttcctcatataaaattattgactctagagatatagtaatatggagaagacaaaattgtttcaagcaccgacagaaccggaagcgccccttctttcaaagagaggaggacgggttattcacatttcatttgatggtcagaggcgaattgaaagctaagcagtgggaattctaaagattccccgggggaaaaatagagatgtctcctacgttacccataatatgtggaagtatcgacgtaatttcatagagtcattcggtctgaatgctacatgaagaacataagccagatgacggaacgggaagacccaggatgtagaagatcataacatgagtgattcggcagatttggattcatatatatatccacccatgtggtacttcattctacgatatatataagatccatctgtatagatatcatcatctacatccagaaagccgtatgctttggaagaagcttgtacagtttgggaaggggttttgattgatcaaaagaagaatctacttcaaccgatatgcccttaggcacggccatacataacatagaaatcacacttggaaagggtggacaattagctagagcagcggatgagataggagcagagtcgtgaaaagagctaaaagcattctatacatacgaaagcaccaagcacatttgcttatgaaagaagagcagcttattctgtaacagattttcaacctcccttcgggaagtaagagcaattttcccttgccttgagccagttccagtcatgagatgacttttcccttactcttttcattcacaatctctctctgcccatcgctctccctgtgggtcgagcctccttttcagtcgccctctacaactaagtcagttgagctctctcggctcctagaccagctgtgatctttcctcctgttggtttgcttagttaaatatatgcatccttagagtcagtccctttttttggagaaaaattccgagccggtaagcaagacaaagcaagtcaacgtgggaaaaagctctcgatggccatagacctgaatggttggagtgtggaggatcactcctgaaactttcttcctttatataaggaatcctcttggttggtcgaagctagaagacggctggacgaactgctattttgcatagggggagtaagataggctaggtgcttttactcaactcgtgaaggttcatttctagttagcaaggataaggaagcaaaggtagagtcctttaataatatgtctgtcattacgtgcgactatctccactatagaaagaaaaaaaggaaagaacaacattttcagcacatttatacgaaaaagtctttattattatattagcataagtaggaaacattttccactagggtttttcccatacatgcaaacataaaaaagaaaagcaaacaaagataattagcatagataggagtctatctccagtaagcatcggagtagatctccactaaaaagacaaagaacaccctaaattaaaacacattactttgcgtctacagacacttatttaaaccttctaaaactaaaagagtcgacggactcttctattctagtctccctggcgaccacgggtgacagcacccacaattaggtcttcctgttttggaggagggcctgtttcctgtcttccaggacgctaatgcggtcccggatccgctgcatggctgcagccacaagtgcaggatcgatgggaggcaggtgctcccaaaggcagccagggtttgctccgattggagcttctcctcttccacttgagagatttcttgcgaaatttcttgaagtcttataaaagaatccatggctacactcaaagcttttttttgccgacttctaagttcctctccgtctccctttgccaaatagagactgaaagaagcttctatttataggcgttggaggcccttaaccctttcttattattagtaagataggttgtcttggttccgtaacatggatcatttcaaacctggcttttcatgaatatggaaccctccactagattttagtgtgctgaataattatcttcgtactccaatccgtacgaagggcccctttctttggcgggtatcgccacgtggcttaatcccggatcactccttaaggaataggacacaataatatagcgcacatcagagaagagagtacccctttattataagacaggccccacgcgtcctttcttaagagatggagcaatcgtcactcgacagctcaaagctgaccggtacaacccgcgtgcttgcctactcgtctttcaccggcctatttgtacccagctacaatctcttcccttagaaagaaaaaaggcccctcggccaatcgtcactcgacagctcgaaagcggatcagtacaaaaccatgtgatctgtacttgtttacgtactgccccttaggcctagggcttcgtcgtaccctgcttactcctctttcactttcactggcttctacttgtcttttttttttttattggcttatttagaaaatggtatcagcatttgagacgactctccccggccaatcctcagtcgtccgtccttgcttaggagaaaaccgaaccactctggtaaaatgcccgcccgtaacccagcagataaagtacattacatagtccagggattggcgacttacccattcagtgactttggcactggacgttcccaaaatggggactatcgggtaaattcaatataatagacgcctgttggcattccagccttccttctcctttcagggcctatccgaaagagaatccagtacttcttggtcgtgaatatctgaactggttgtttgctgttcaagaattcttgtttaggcagttcataccatccatacatagtgttttgatctaagatttcaattcttccgtgtttcagcagtaacatattcttccatggagctaaggtccaaaatatggaagaaacaagcgtttccacgactctaccacccagtcaattctgttccacttaatccctctttccggctaaggaatgggaaatctttctcctgttacatgaatccaattttcatttcatccgggaaaagccacctttttctcaacaatgtctttgtcatttgatccaatagcgttccgttagataggaacagatttgataaatactgaataactctcggatagagtattagaacggaaagatccattagataatgaactattggttctaagccatctctgacgattcattttaaaagtgactaggtaattagtgaagaggtttataaaagtgacaagcttggtggaaagctcttatcttaggaggaaaagctaagtatgcccgagtagtcttgatattggttggtttgaggtttcgttagttttatactaacaagcaagcttcggttcggcgaccgctcgacctagcgccttagccccagtactatagggaaggcctatgcgaagaaaaggcctgcccatcatcaaagcaagcccaagtccatgcaagaaggccctccagatctgtccaaattcaaagcccgtcaaaggcatatgaaatcatgcaaaggatccgagcccatccaaatgatgttcagcgggctaaacccaagtagctctggcccatgatccaagagacccgaaactagttaatcactccgtgccttaccttctaaccaatcggccaatcacgctatccttacctttcaaccaaccccttcgattcagtttctgcagcagtatagaatctcggacccgatggatgcctacagaaaaatgagttttccagcagtgatggcaagaatccgcgaaataatgttctttctccttttgtgttctttctgaatggagctacgcgagggaaagctcagctttctactctgccgcaaaggggccgctttcttccccaaaatgccagttccgccatcagggcctagcaagaagcataattctgttccaaagcttcgtttcattccagcaacagtagtctatggttcgaagcgccgtgttccatccggcgcgaatcctctccataactagtatagtggaggtcttacttgtattgcaataatgaaaaatgtacgaacacaaataatgagcagaccagcccacttttatatgtgggttcatttcagaatgtttttttgttttgaataaagaagcgcgtgaacttttagtgtaaggcaggtgttttctcggtggatggatgggataaatgcctatattgctttataatgttattgttatgttgatgttatattaaagaatgaaatctaaaaaagttgcttagtcccattctttataattgtctttctcatactgtgtaaacaaacttcaagtctgaattgtgtactgtactcaacaggaagcgtcacagccaccccgatgtcgatctgcagtattagtttgagaaagtcgtttggttttaacctagagcgattggtttacctgtatcatgcaaatgtccaacacttaggtgctttctaagatcatcctatatgaaagatgtatgacatgtgtggataatgaatgacttgcagggtatgcaatatcttaagtacaaaaggtaagacctaaaagagaaatgagcttagcacaacacgggatagaaagctaatcctagaaggagaaaacccatcacagaacaatcataggaaaagaagaaatgggttcagaccaagtgacagaactctctatgagttgggctacataaaagatccttttctactaaaatggatgtaggcttaactaaagcccaatgcaggttgaactctatggaatctaagcctcactacccttaccctcttagagggttacaaggaattttaggccggccccatatagattcagcttaggggtttatgagagattgattgatggacctaagctaaacaactaagattgaacctaaaccaaaacctatagactgaattaggagagcagaggtttaattcaagaccaggaaagcaagttatatcgaagcccaatgccaagcaaagccctagactacaagtgaagaaattgggttcaactaagcccttaacccaagatgaggtggagccttaacccgacacaagaggggcccwgtagratagtgbghatagtcagcccaacataggttgttaaccaaaaggagaagttcccgtgaaaacagaaaagacctccccttaacccccccttacttggcagattcacattcgtaggaaaggtctgttcttttgtctctttccctcaagcgaaggaacctattaataagataataatatctctctgcttcctagatcgataacgaatccttcggttgcttatcctgtcatccgagcccggcgttccgaacaacaatgattcggaaagataaggtctacgaaagaaaagaaaatttacaatttgccctactcctcaagaaatactgcgagcggtattgtaaaggtatgggcttttcggtcgattttgctcaagagggtgggggacttcgactttatcgaagcagcacatgagattgcccagaaggattactttttattaacctagtgcggatgtggactcctaaaaacctgctccactttgtacgaaaacatagtaatgcagctaagtgggagtcttacatgaacgcgcacttgatctttgacttggtccgccgcgatccataaggaagggttttcgttcgcaacaaggtagccgtagggaaacccctatgggctggattgaatctttcctttccttctccctctcacctgatccattaaaggaaaacagactcaaggattgggccattttccatatgtctctagaaagataggagctaatcaaaattcttattacttatgtaaatgtaactctcaaatttgatattactccatgtgtaacgccaaaggggccttgtattcaattgaaacagaggatctcccacattgatatacacatccttcacccaatctgctcaaagtattttcaactctttcatggtatcagagcactagctcttgggaaaggttcagttggttcgtgtgaagtgtggtctgaataccttcttcttaggtgttttctctttggcgctgtccaccgctctgtctctatccttctcctcagcacttagttagtatcccgtccatcgaaattgagttttccatagcgtctgtttcaattttatggaaaactaagaaaattgskwkykwgrrgsrsvagawskwchcvgttdcgbtgabggaactggaaaagaaccaaagaaaggactttcttgagactgatcacaaaggtaagataatgaatcctgagtacgtcccctggagaagaacagaccgactactcaaaagtttaatgatgcacaccatgccctttcccaggcgtcgaggttgcctagccgtaatccacaggctggcttcgacagatgtcagagtgaatccgattcttcgattcaattacttttccaattccaaccccgcgcgtggatgtagaaaagtgtgtgaatggcatacgkaagattggggatggacaacatcaattcatttagtatagtcagctaggaagcactagctaggcaagtcatactgggaatgctgttccacacattggctcaattctaccttccacatccaattcttccttcattacaaggcccagcttcgctaaactcgcaccgacccttagttaaatatgcgggtagcttttcacgaaagattgttggcatgcctcccataagaagtaggataaaaaacctatgagacccccttgttctaatcttttcctaaagagcaatcgattactatactagtgcatgcaaactgaaatcttagagaaccttgatcctattgatcagaaagagctcgggcgagaaggtctgcggggtcagaagagttcagagaaagctggatccgggaaggcttacgccgataacgaaggattttgaaaccgatcgatatgcagacgctgcaaaagcaaatgacttcgcttcctcaatcaaggtaaggtaatttgagaagctatcgaaactattccgaagttgatgatttcgttctagctagggcaatttaaagagagaagtttacgctctccaacaaagaagcactcacctcctaatagaagagataacgtaagaaagactagcagatgcggacgatgtaagcggtcaatcaattgagactacttagagtccgctaactagggaaagagaagcactaagatgaaaagatataactagattccccttacataatgctcctgttgaaactaaaaaaagataagaagggacttgaagcttacagtccttactcaactacaagtacatagagaaatgcttccacctattagactatgcattgacgttgcagatgttaaattgcagttggcattaggagatagagagcaaaaggaatgaatctagtatacttaaggcaatccaaaagaaagcgcttagtccttatgcaactaaagcacaggcaggaaataaagctacatccacaaagaaagagatggttgcatctaagggcttcttatcttattgggtctagcttcttagaaagccatagggagagaccgaacaatctgatgatatatacttgtgatgtcagaaaaaagttccgaagagtggaggcagctttttcctccaattttctgttggattctaataggattcaggaaaaaataggaattcgacagagcgcaaaagatagtcgagcaatcagcgggcaggcataggtagtcgacagcagcaatcgaccatcttgagcaacaagagaaagaaggaccaacgacgatcaaggaaagaaagactaagtaaaggcagacaacgagacgaagatagcagacttgcctcgaaacaggaacatagcataggggcatttctccggactagttaagtagttgagcccggctccccgcttggctcctctttgctcctagtagactactagacatcttgtctactctgcttttatggaagagctcagtccaagaagggctctcaaaaaaagaaaattgtcaagctttcgaactcgccttgaagttgatgaatgattgcaaggctagcaacaagcaggctcgcttatgatctgctgaaagagtacatcaggttttttattaatccctcacattcatgaagcagattgtcgaaaagggctttctgcaagcaggaaaacgaccttttacgatccacagggtctagcttgatcccggtctcaggacttcccaagtcacggagtctttgatcaagttgtaaactaaaggagtataacctatccaatatatatatattttcgcttattgttagtaagaaaggtgtcactaacaaataaatccttaatcagtagtggactactagttaacgcactactaaagcagagtagccagcatgcgcacataatttttgccagaggatttttcagcgaatggaagaagcaggcagggatagatataatttttaggaaaaagtgctttgtttgatttgttcccaggtgagatccaagatctttcaacgcgttgatttcctactaaagaaactgggcttctatcaggagtttgatcattggaaagggtcgaaaactcttgctttatgcttgagaaagagccttcccggcgatctgcttcatttatggagggtttgcaaggaagacaactgaatagcgggaattaaagagaaggatttccagaggtcaatatctggcattgagcctgcctatcctaagtatgagttgggagagcgagatagagacaaagacccaatggacgttcccctgctctctctcgatgtggtacctttcagtctgctctgtcaaaactttctcgcaatgccgaaaggtagagcagcttcaaggtcttcggcaacgagatcaactgctgacccaagaaggtagggaagagaggaggaagggccaatcccgagtcaggggcatctatctttatttacgcaaagctattttcgatttagatatgttcattggcctgcgactgatctcatcgtccgttttcccctctttcctattcaagagttctcctccctaacggcacactgtatataatctctagatggccaatgtgaacagttcaatcaaacttgtatgtgtgaagcatattgaaagtgacattgacaaagcaaagcacagattccctagaatgttagaactcagacatgacagagaaggtagtcaaaacggtacgctaagctccttgcttcgtcgcttctgttttcagttattcaaagaatgatgttttaagcatctctatatgccagtcatctatctgacctgacaaggaggtcgactttgatatctcacccctgatctctacggttggttgaaggtgtcttggaagacgggtcgaaatcagatctggatagaagattcatctacgctggcaaaagggctatcagaaagagtccaatcccgaggagagttcatgtgtgaaatttctttgttgaatggaggtgagttcaagggcttctttgatcgggaaatgcacgcacttctttgttgtcattaaggtcccttcccctgagttcaagatgtcccttccgcttctctttcactactttcctcattgggattggtcaagctccttcacttattgctcgatccgatccggaacctattgggatagcaccctttcctcctatttattagtaggtcttcttgcccgttcagttcctctactggtagtctagttgtagttttgagcgggtgaacccatgttctatctcgtagtcacctaagcggcagagtctgtaaactcaaatggtctgagagttgcctttggcttctgaacctctgaaactggactggagcaagctaccaagctcctcttccccttcatcactctctatctccggcccttgccattagttagcttgcacttcccttgcttgccctttgagttttcaaagtcaaggtgcctttcccttttctgccttacctcttactgaagtgaaagaactgactgttgtctacctttgattctgtcttccgggtgaaggtcctgcggaggtcttttttagtgatcaaaattgattagggacagtgacccatgatgaaaggagctattgacctaagtggtttctatttgtatttgaaaagcaaggtaggtttgttaacgaaaggataaggttaggctggaatgggatatagtaagtgtgccacgagtgctccttctaaggcttctgcttctctctaataacgagaaaatgactctttcagaaagcaaagctacaactcttcagtctaagctatctaagctagaacttaaggccgacctcttttcagggataccccacttcccggtctagcttcactaactgtattcacagctttccagatctcggaaccagatctactttctcatcggcattctctaaatgaattacgttatggtcttgaactctcgatatatcatatgtaatgaatgatcgaggttgtcttttcggaagaggtgggtgggagtggggcagggcaagaaagtaacaatcatacccgatattcagagcgccggagatagaagcggcggcagccataaagtggagaatttccatccatttgctgtctctttcgctaccgctccgtggggtcaacattacgaaattagccaggttcagttctgactatagctgcaacctatctcatatttggccgcccdcgatcacaaactcgaaattttggaagataaagtaaagaaagaatttcgggctaggttcaaggtatgcccaaaggtatgccagttgattgaaaagaaactcaactttcaagattcaagattaggtaagtgttcagtgtactaaggtacaagatcgaaaaaaagcgcggatagcaaattccttaggctagatagagtggtggttgtaaattactaggtagccatacaacactcggcccaagcaacgcccaaaagcccatgcctttcttggtcggaccaacccaaccggcgatttccgacaagtctttctgaattggaagagcaagaagcggaacttgaagaaaactttctttctctttatggatagacagtcttttcaaattctccttctaattcatcttccccggtggatttaggtttatctctgaggtcccacgaaggttcgactagtagcactctgtcggacgccaattcgggtgatattactagcactcaagttttgagtgatatcaccgctcttttgagcaacgaatggaagtgggaaagaattcacaccagaatggagcccaatagagttctgccaagcggttttggggaagaagcggtgaatgacctatctttattgaaagacatctattgtgatctagcggaccatggaatgctaagttggtattgggaaccagcttggggctttctaaatctcattagcaatagtccaggaatgacatagccttcctgtgcaatgggtgtcttaacgtactaagtaaggtggttttttctaaagcggcattctccttctatctatcaacaatagaattatggaactttctccccgagctgcggaactaacgagtctgatcaatagagtccgtcatttttctattccttcctacttcttcttcctctattatgtgcttttattctatttgcctgaaactcgagaaaatagagttgtttgagaccaaatgttatagagttgggggctctctgggaggcacaccttcacttccttcttaatgaaggggttcccgggagtctgaccttgtcctttcttttaattgtcggggccgtcatgagtgccgaaacctatttcggtaagatgatgatggctccttcgggcgcatcaagctctgaagatccaaactggacggaagccctgagatcttctaaagggcagggagagacttcagaaagggaaagcacaggcacatcgtcgtccatcaacctacaaaagaaagagcacgtccggcgcctgccccaaatgaagtagcttccctgcccctgtcgtcccctttccatatcaagaagatgagatcataggggcgacagtgtagaaagcatccaagagcgtttaatttgaggagaaaaccctccttctgccgaggtcatacatcatacaacaggcccgaattgaagccgaagacctattcgaggtcaaggtcgatattttcaggggcatgtctggccttgatccagaaggagattggctgggacggggagctcgggccctcgagaatccgcgtaccgccacggggagcattccttggagaaactccatacccttctttcggatctcgaatcgaggggagtcaattccgagtccttctctcaattaaagggaaggtacccctgcgaaggggtggggacgaacactctaccacatagtggagtggatagctaggactactaaaatggagatcgtgtacaacaacaatcctatatttgatgtcgattcatccacacttccattccttgtagaggaaggctaactgcttgctggctgggagctgtatgagcggtaacgtccacgtacagctccgtgagaagggcggtggacagaaatggccttgttgtacctcactctcgtcttcaatggggtctgctctttcttttttgggagagtatgccaatatgatcttaatgaggtgcggggctttgcatctgacattcgttgggcttctctcttcgggagcctgcgccccggcgttttgtgcaataaacccctccggccgaagactagtggtaggtggtcctgcggagctttcggaaaagggtagccttgtgtgtaagcacagcaatgaaccgcggcgaaccctcagacgacctatctaagattaggggatcctcagtagtggtgaccctttcactcttccacggactgatacatgtaccgaatgctcatacgggaaagttgactcctgggtctggaacctggggggttgctccgagaaaacctttctttctcgtccactcagggtgcggacacacctgcgcggattacaggtgacagttacaagaatggcgggaagttaacagtacccgacgacattcagggatggatgtagacccatcgggcagggataatcattccggtcctgggagaagtggcgaccattctcaagaaccaaaagactgagctgagggaagccctatgagtcactgaaacgacggcaggagtgcccttttctatcaatagagggagcaaaagggccttgctccctttacaatatgaagaaagaaataagggtcgaagtttagaccgctcacagtagttctacctatagaaaggatcatgaaagaggcgatcagaatggtactcgaatccatttacgatctcgagtttccagacacatcgcacttccgctcgggtcgaggcttccactccgtcctaagacggatcaaagaagagtggggaacctctcgctggttttggaattcgacatcaggaagtgttttcacaccatcgaccgacatcgactcatcccaatctttaaggaagagatcgacgatcccaagttcttttaccccattcagaaagtcttttccgccggacgactcgtaggaggtgagaagggcccttactccgtcccacacagtgtattactatcggccctaccaggcaacatctacctacacaagctcgatcaggagataggaggatccgacagaagtacgaaattccgattgttcagagaataagatcggttctattaagaacaggtcgtattgatgaccaagaaaactctggagaagaagcaagcttcaacgctccccaagacaacagagccatcattgtggggaggttaaagagcatccaacgcaaagcggcctttcattcccttgtttcgtcgtggcacaccccacaagcaccccccggctcaggggaccagaaaacgcctttcgttttccacccttcgtcggcccttgccgccttccttaacaagccctcgagcctcctttgcgccgccttcttcatagaagccgccgggtttacccggaagtccgaattctatggtagagaacgctgtaataataattgggtcatgagagactcttttaagtattgcaaagaaagggcccgctgatagagctgggcggggaggcgatacttgttatcaggtcagagaggcctggcccgtaagctggccccttaaaacctattacttaataaggatttgttacgcgcgatatgccgacgacttactactgggaatcgtgggttccgtcgagcttctcatagaaatacaaaacgtatcgcccacttcctacaatctggcttgaacctttgggtagactctgcaggatcaacaaccatagctgcacggagtacggtagaattcctcggtacggtcattcgggaagtcctccgagggcgactcccatacaattcttgcgagagctggagaagcgtctacgggtaaagcaccgtatccaaataactggttgccacctacgctccgccatccattccaagtttaggaacctaggtaatagtatcccgatcaaagagctgacgaaggggatgagcggaagagggagtctactggacgcggttcaactagcggagactcttggaacagctggagtaagaagtccccaagtgagcgtcttatggggccgtcaagcacatacggcaaggatcaagggagatctcgttgttgcatagctcaggtcggagcaaggtgccatcggacgttcaacaggtagtctcacgatcgggcactcatgccccgacattgtcattgtatactcccgcgggtcggaaggcggcggggaaggaggggacactgggcgagatctatcagcagcgaattccccatacaaatagaggcacctatcaaaagatacttcgaaggcttcgggatcgaggtctcattagccgaagaagaccctggccaatccacgtggcctgcttgacgaacgtcagcgacggagacatcgtaaattggtccgcgggcatcgcgataagtcctctgtcctactacaggtgctgcgacaacctttaccaagtccgaacgattgtcgaccaccagatccgctggtctgcaatattcaccccggcccacaagcacaaatcctcggcgcggaatataatcctaaagtactccaaagactcaaatatagtcaatcaagaaggtggtaagacccttgcagagttccccaacagcatagagcttgggaagctcggatccggtcaagatccgaacaagaatgagcactcaactactagtaaaagggagaaagttgactttgagaaagaaggtgcttcttgccgctttattagtaagtaagcttgttttatatctcctcaataaaggcgaaagatcactcctaaaagcaagctttctcttatatacgataccataccacagaatttcatttgccttcctgcttaaggcactagttcggatggaaaccctgatcaggcaggtggcctagctaacatagctatccgtcagaaatagcagcattccattgcaggctactatagaggcatataattttccgggtgttaagaaagatattgaatcgaaagcggacatgcttgctcactggctagatcgggctgtctgtacctttgctaactcttctgcctgtaaggaagcttgaaagagggaattctctgatctatgaccccgaaagaaagatagtctttttcgattccgcgcattggaactgaaaagggctattcataaacagtcttccttgcttcttacctcttatcttattgtaggagataatcgagagagaaaagtcttcctatcaattccttttgaataaggctacgctcctccaagcctttgaaactattgaaaatcgaatctttgttttcaggcgggttttcttctccaccaacaaccaagacgcatgaaagcggtttccagcgctgctgggcagaaagacatgatggcatgaaactcgattacgtacgctgattgttcgtccacttcaaaggctcaaaacagaccattttccgtgtgaaatgacagggattggtttggttacttagggaatcccaagcaaagcaatctacgcaatttccgggttcagtagtaggaaagaaagggacctctcactcaattcaataacatgttctagggcatccttttctaataataatgttcgcatttgaccaggcttttggacgttccatgattaaaccgactagcggcactttcgagatgccaccttgtttctaaaagagtcttttcaattccatttgactcggggcgtcagggaccctccaacagaaacctcgtcttttgtcgtcgataagttctccctcagtgccctactattcataagaaagactgatttaaaagagactgatttattaaagcccggtgaggcctcaaccgacagctaagcttcgttctgcggcggttttcaagctagcaccctttcagcatatcatctcgctcgattccaaaaaaaaaaagagacgcagttttgattatccagttctatatcgaaaacgagcagttgatcccacgaaagcaaggctggctttgttgcgggttcaactggaattgtaagaagtgaggtaaattgcctttctccccaccgcatatgcctcctctgcttatgccactggtgatgaactcactatggctattcaacgtcaaactcagagttttctactacataggcggctaaacgaagccccagtcttttttagtaaaaccccaaccccttattagtagccgaagtaaaggccagcatgagatcaaagtcacttgccgtccgttcgctctctgttcaacaaaggcgatcgatattcccttacttctcaagttttgaattttatgagcccttcgattgtatcccataagaaaatctctctgataaacatcttgtcgatgattcgattatattatttagaatcttcgtgtgcgcttttcgcctgaggctttcggacaagactacttactccagtaggttagtaagctacctcttccgctttcaggcaagggtagctctgaagggagagttgagcggaaccaggcataaggagcaagaatcgctattgagagttccccgctaggggaacgtcaggaggggacatgctctatgtccactgattctgtttagtacagtataggaagcccttgtttgagtgagagcttctagaatgccattcatttcgcaataagaaacttttccacatagaggtttcagctacttaaagcgagagtgcatccaaaattcgagaagagtgctcggccttggttgaaacaattataggtgtcaatggaccgatttcactagcagagcactttctccaatgtgcgcaaacagagatgccactttcaatgatggacaccggcccttgtgttaaagtagcatcgagtttcgcttggaaaccggcaagtttctagtttccaaataagtggtaccctttctttagagtccggtaggtcaattaagttgcctaaatctcttccttatctgctgctctgtagctgccttcctcgcttcgtcttcggctttcagagttgtgaactaacctcttccttttacagccagacaactggcagataagctgggcatctaaagaacataagatccgagttgccgccaggcataaaagtcatattgtcaactagggaaattggcacaaccaggcatctcaaacattgataagggaagaatcaggctttcattaggatgatattcctttcatccgaatggcaaggcttgctagtttcctgaagtacactcgcatctgtctatctatgtcatagttgcttggaaggaaggtctcagatgtaccttcggcatgtatgagattttctttcctctatctatgtcatacttgggattcactgacagccaattccaagtagatcctccctccccctcgctccacttcgtttcgctcgttttctctttccttctgcctgcaaaaaaagtgatgagattggttttgtgtgcgttagcgatcatcaaacctgtgacatagataagattggagttcatgcagttggaatgcctgagaccactttttgccttgctgctcttgcttctctggctactgctccggctaaggctttctttccgctttgacttgccttccttatctttcaatctggacttgcatgtgttccgcatatgactatttcgagtgattgctgctatctggcttgagttagacaagcagagaaggatcttatgccaccggtgaccggcctgcctatctagtatctagtactaggactagtagagtagaggcactactgggcggggcttcctcgatcacagcttctcgcttagctaactgccagacaaggatgcaaatcaactccttatatagaatgcagatcgacacattcaatgaagcagccagtacggcagacaagctactttcttattctaggactggaagatcctctatctattagcatacccgtaccggcagttagactagcactctctccccaatcaatcgcagtaactggctgtaagagagctgactgtctactatctatgtcatgccttggcaggtgaatatgagagagaggctgtaagtgcattctctccttctccatcttctggaaagcactctttgagcatgctgacagaatgattgacactcacatctctctcatttccagtgatttcgctacagtttactagcgcattcctagactaagactacggcattgaagaagcaagctcactctcattccaggaatcagaggaaggcattctgtccggtaatgaagttagaagtttccggcttgctttctctcttctcttgcagttggcagtctcagtcaaccttgttccgggccttctcttctactctatctgcttattggattggtaggtacagtctttcttctaggcttctgattgaactttaaggtaatgggagagaaggcaatcgacagataactggtaagtaaagctatggactgggttctcactctaagccagtaccagtaatttgaaaaaacgatagacatctagcgcattcactcgttttttctttctgatcggccaactcaaagagggaaatgcaaggggcgttagcggtcttttttgcctcgcctgctactgggaagagagagccgctgtcattcttcgcttcgttcgagaatcaactgcacatgaataggctcctccttaggccttcaaggaggaagcggcttttttccaaaattcccgggaaaatgaaacttttgaaattcttttcgtaaggcaagaaagttgcctaaggaaagtagaagtctmtgyacdbthbthbatghgbatgabggcadavtggttbhgvcttabtcccbtctcctytcaaawgaawaagaawgwcatcattctgatcgtgacttgaaaaaagaaagaagagaaggaacttggagttggcgcccacataacggattgcttgcttaccaagccatcctggcttttcgctcctctccttacagtcaagtggctttcactcctccagttctattattattgacttgacttattattaaaaaaactactcactatccaaatgaaagacgatcgattatctacccaagaagatagagagtcccacatacgagaaaaggtcacaaatagagttgaaccaagtaacattgcaaaggcataatgatagtagggtcgggatatccccgccctccgaaccggacgtgagggtctcccctcatccggctctctgcaggggaatctccactcactgcttcccctaatatcctccccttaccacatcatgggggtttacaggagatcccagaggctcgctcggaaaggctgctataccataccttttgacttaactctactctagtagtcactagactcactatagtagtccgtctggctgctcttgctgaaatcattactcttaattctcccgtgctctagcaattgcgctccctagaccactaccatgtagttaggtagggacaatcagtccgtagtgacgggaatctaggaatgaatggggatccctatcaatataaaaagaatatctaattagagttttctccctttctctcactcaatagatctatctggtctgatacggcacagtacaatacgagacgatggaatgctatgggatagatggtagagggctgcctgcgcccaaaagcgatgattcacttgtccccttgtccatagggacctcgtggcatacaaccgaaacgactcccgctagatagccgcccctttctctctttttacagcctcgtggacggacgaaagaagggaagttacagaacggggcagtgaaggctcgcgaagtagacagcaagcagcaagcaacagcttctcagccccctaacctttctcttttttaataatactttttttatcaggtaagctttgaagctggctgctctgctatactatactagttgtagggcgctagcgcttgactaatataatagaaagtaaagggactctattatgatcttacgaatctaaagatctcaaaatggaagaacgagctcttttgctcgcccctatctctaaaggggcgtaagcacttcactcgctaggggatgggattcattcacttgcattcctgctagcactacaaaagctccggtcttaacgccctactactgctgtgcagcctttcctcgggttcgtagagtcgggtttcccgtttacccacaacggaggagccgcccccaccaggcaggcggccacgggtcataacgcactcttcgcacaacaaatccactttgaagttgacttattcgctcggccaatcgtcggaatgtgtacgagataccataagggcccaatatctcaatagcacctttgtctaaagcttcgaaggagacttcatatccgaaacgcaggaacgatctgactagaaagtcattcaaaacttgatcgaaaaccagcgtttattgaagaagctatagagtcgattactaatagtactagtttgaaaggctcgttggaattgatccgctacgggattaacattatacgcaacataagcacctgaagtactaaacagaataggtattagtttggtaatggttggagcagcaaactcggattcggcaagaatctcattttttggtagtacgaaggggaattggcccaaaattggatggggtcaagacgctgtcgggcgccggcggctgactcaagtgcccccgaaccgcgcgaaatggtcgcctattacacggctcactaactctgcctggggtgtgggtacctattattcgtcggcggtccggcgcaccctactatacaaagccgcccccccaactcacttaaaggatgctggttaattacgaaggaaattctttcttaatcgagggacttccttttcgttaagcgcatcgaaccaggagtggacattatcatcatctgcagaaaaatccagattctctttcatcattagcgaaagtggaatagtatgactggctttccggaaaataagacgaaacccgctttatcgatatgataaacatgcgctcaaaaagacctcctaaacccccctgccaagcgatcgagtttagtctgaatttgctctagaagtagctcccgctccagactgacttcaaggaaagaaagggttgggcaattccgccggttctggagcttaccttattattaaggggaaagggattttttatagatgttgaggtgagtaagggggggcgtagcttgaggcttctcagccgcaggaacagggaacgaatcctccaaaaatggaatgagttcgcaattaataccacaagaaagccgccaccctcgccctttagagataggggcgcaacaaaaagtattcaaaaagggcgccggaggcctcaaactcatccggagttggagaatgaaataaaaaaaaaagattctcaagaggaatgtatcaacaaaactgcccttccatatagatcgtcgttgcatgaactttgtcaatagattcctagcttcctattgatcttgattagttctagcttcgttttttttgttgagagttatctttctggaccggacccacttttataccgtctcytgawacacmtgctymkmsyscatgtgctttcggggccccactcaaaaaatcacttgcttgtgattgcagccattccccgaaaggggagggtggatgtaaktcagctcgaacgaagtgagaggggtaatagactattaccgttcagttcatgtgacgaaccgaacatcgttaggtcccgaattctgcgaagcaccggatctagatcaagatctccattacgtcgtacgatatatcgatccggagaacttactttcagtttaagtcatccattctgctcctatctaaagtgatgctaggctgcttcacagaggtgcgcttcgctcgaccacatgatgaacatgttttaagctaactgcatgtcgagcgcttaagcggagcttgtggtcactcgttcctcgcttgttcgaaagagcttcagattggattctacactacatacgatattccattccggccctcactagctctttgcttgcttgtacaaagagcatgcccgaggggctactacgctcaccgcgcacttgcattaccacctgagcttcgctaccgttccgcccagctcctacgcctaccacgaacttgaatcatcacatggctgctaaagcaagctaagcttcacacggccctgmggaagccaaaagaccctckcacggccgaaggctccgcaacacgttggagagcttttagatcccgccctaaaacgcccattccctagagttccgaagtgattctcattctcaccgcagccttcttaagccgaaagaaagccgggcaagaatctcatggtagtacgaagggggagcggaatcgtatctgggagtggttcttcggatcgatcacagattctcggccccgtcctttggcttccactccagttgacctctcttctttccatcccaccgtgagaaggtagagagcaaaaccaacccagcaaacaactatgactatgcccctattagtaaagcatgtacttcttgcaaggcttgctgagcttcttcatgtgacagacatcgcaaaagtagtccgttgaacgatcgccgatcgagggcatcgtaatagtatactatttttgaaccctgatgggtctcgcdvttaavcabatghtcghvcbchbbctdctdatdcaaatctcvdadvccabvhgagccctagatrtaaagggttcttgaacccttctaagcaattagaagagcgcggaattggacctccctcaaatagatggatctgggattgattgtggaaccgagcatagagaaccgggggcgggcaggaagataggctaggcggagtagtcgctctggagcaggttcttcgactggatcaatgcatgtatgaaccctaaaaaaatcccgaaggtctagtctagaaaaacccggattttgttgggttagcttttggtaggaaaggcggtcacaggaagaaatgccctaccaatgaatagattagtctactaacgtcaacaatctctttcttcatatacgagaccgtctgcttttatatcctaaactatagatatgaaacaaaaaagaaagaaagaaaggcaggaggtaagagcgagtaagactaggttatagcaagacaacagaggttagatagctcttaccggaggaagagggttcaggtcacccgtccccttgacccagacacgaactaatccttctctctctcgaatgtatgcccggttttcgtcgaatcttttgatcaccttcaaaacaaaccggaattccgtcttgacatgataaatagtgatgcccacctgcagagcgtagccctccctgcagccttgaagtagactatttttcgagtctgatcttatccccaaagccttttgcaaaaggagtaggtagcgagatagatgactaaaagctgatgatctttgcctcttactagtaaagggaaaagccctatatatctgattagtcaagcctaaaggccctttactaatataatagaaggtaagaccggctttcgcgcagctgctgcgccttgcttcttgcccatagagagttaggatattttgtgagctccttcgcctagcggaaacctccgcttttcggccgtaatcccgtgctttaccaacgcattcaatggattccaccatgaaccgggagcgggcgaagacatgcagcttccattttcggggtacacagtcacgtgctgagcaaagaggtatatatcacactcattcacaagcgcaaggtgcggcatccgcctgaacggggagaggatttccctaaaacaaagataggcgtgtcaggaaatawwrkrrastccccctatttcgctgtccagggagctgttgactaatgacctaaaaaatgcgtgacgtttgggaagcatgagcaacccttcgcgcacgagatagcaatgacaggagattgaccggtcggggtcgagtgatctcaggggtttaggggtgcttctcctgctgcgactacctctctattttcaaaagtatatagaaatggtaggcactgggagtgagtgaactacccggggagaaaggggcaacctctctatagaagggaagggaaagggttctccgctcataatgattgtagagtctctcggggttggaggtctaatagtagtcacatcaagtcctccccctcttactcagaatagctagcgagaggaagactactgattatctatgaaagaaggcttttaagaatgaaaaaaatcttatcttaaggatagagagccccccgcctgcgttttcagatacgagtgagtgagcgctttttctgctatgaatgaatgacctctccatttattttcaagcttgctcttcaaaccggcctatcgctctcctctatgaaaaggttcttccgtaatcactctcaataagacatccattcccctttcaaatgaaaagagaactagacttttctcttcatcattgaaatccgccattcaatcgcagtgcggtgctctcaaaaggctcaatcctctaaggctgaaacgaataggtcaggaawtssmscykkswkccgcccgttccgatccttgcctactaaacagttgcaccccggatatgtatgttgggagaaccccatgatccttccgtgtggaagggaaggaagaaagaaggcgaacacgaatactaaaagcggttcatggggaccccaaaaggggatagagagcgcggaacgggctttcaagcataaaacaatccctacctatacattccatggcaacagacagaaggcagttttgtcgttgttcttaacccaggcacatttccgttcccaataatctccatgaaaagactaccatgatttccgaacgaaccgagggagagtcgaggcatgaaaaacttatctatgatctgcttatttccaagtacgtatcatccgctgccttatccgccgtctctgcggccgccaaaagcctaccctctctcggatattgagtgggttgaccggggaagagatccggacgaaccttccaacaagcagaatagaagttgaccacaaggccatctctgtgggaggctgctacccataaggccatctcgggcatgggaaagaaaggcggcggacaaccgacttaactggagagcctaaacggcatagaggatgagtccaccggtcgacaaacggcttctatctacaggtgctttcattatggatcggtcgacttgtcacgattgattgctcacacacaattaggttaggcaggcttggggaggtgatctgaatcgctatcgatacgatgcggggctgatttgctgaccgtaacgaacttgactctgcccctgaaaaaaaagggcgggaagacctttgacctgggctggggagggattggggtcgcttttctttaggactttagtccgtaacaaggctcgaagacctccggctggatttgaaatggatcaggtagggcatccgtttacgacgtgggtgggattagcagttttctctattttcttcaatggtaggaaatacgcatcagcgggggtatatgggaggaaaccagtctgcagtaattcaaattgctccttcggatcactaagtaaaatcttgactcacacataccgcggtgtattgttgtcaactcacatagtcgcacctaccagcaacaagacgactactccctgcacgccactaaacggcgctatttaacgcttgggttcgcccaatacaagaactacagcccaacctagcttaaggctaaagccgtggactacacccccgtgagagccctctattttactaacatactcccttttgatctcccccataccttcatatcaaagctgggaatgattgactttcggattaaaataatagcgcataatggcagtactccttcccatttcttcttttatgatcttatctacttgaaatgcttacctgtaagtgcggagaaggtacccaggggaccaaacgaaagggcactgaaaggtcttcaattaaagcttcgccagtacttgaaagactcgaaagacctacttgatgagtttccttatgagtgagttcgtaggtgcctttaagtcgagtgtagcgaagggattctcctaagagaagctttagcccttgaacctgaaacgacttttatgagctgtctcagtagtgaccgactttattttattagctgtatgattagtggctthgctcdtagtggttbaavagctacggtaaaaaaaatccctttgaaaataaaccactaatccgccttaggtactcttttaagtccgtgtaaggcggagggaatgaagggacctgcaggaggctgaaaagccgtagtgcgctagcgctagcgagttagcgcaacaacttagtgtcttgttttcttcgctgctttttttgtccgcaggaaagcggttgctaaggcttgtagcttgcttctgtccttagtcaattttggactgaagctgttctgactgccgtatcttttttgaaccgaataccttcctctgtcatctctggtctgtctcttttgagagaagattttctaccccgcctgcctatgaagaacttcaagtctatcgggaaaggatgtggtggtaaccccgcagctttgtctagaaccgggcgtccagccgtgtaggaagactcaccctagccactatagcgaccccacccccaaccctagctgagaagcaccctccacccacttccatttttccgtgtgcccaaagcccgcccgcccggtttttgagacccttkctgaktccctcacccaatctcatgggaagcaagcccagcaggccctgccttaacctgtcctcagacagccagccctcaccaggctgctggcattgctaaatgctccgccacgaagcaagctttcccgaatacgacagatgcggaagtggctaaagaagtcggaggaagaaagttgttggacaactgtatacacgagggtacattagtattctgggaattggcaacattgacagaaagggtaaggggtaggaagaaacttttttaggtcttgctctactaaagtagtcggcctaaccttcggttcccgtaaccaagtttttctttctcactccttatgtacttttttttacttcatccatacttttttactttttctgaagtgtggggcaaacggcgccctctacttctacttctaactaaaggcgaacagccggcattgcaagcaaatagaaagcccccgcccgtttgagccggaaagcgtaccggctgtttgagtcgcgaaagggccgcttgcttaatattatttatataataataatagatagataatattatattatataactatctataaagataaataaaaaactacagaaaatacttttttwtnnataaaattcttcattcctgggaagaggaagaagcagatagggcaaaggccttctctttccgtccgctcttcccgaagtgagcgaattgcatgtagagatccgtaggggcttatagtttaattggttgaaacgtaccgctcataacggtgatattgtaggttcgagccctactaagcctaccacccccttctcttcacctgatacaaggcckgyctcttatacacawctccgarcmcchcaadctagcgacggcatctggaaccacactgctgccgctgcccttcgggcacgcctcctatgcttatcactcacctacgctcttgcagcatgccccttcgggcaatacggtgtaatacgcgaagcagctgagccatagctcttcgatcgctatattcttgcggcgtggttcatcctcttvgcghdtadahvcgtattbbccvvcaggagactgcdgcgagadtcbhbttvdgtbaghdgcatbbcdgvdgtdtvbgggababagtgaacactcccttggttgggggctgtgactcccctatcctttcaattttttgattcccaggtcttttttattatcactgttggaatcttttttaagacgacttggtcagggcggttcacaatttctttgctgaaggcgctgttaagccctaagtttgaattcaaatttcattgcccttcttccgaaagtctaaagtccttcaaattttcaccaattccgacctacctttatttatgggatatttgaaggagagctttgtaactgtttctagaaaattctctctagctcgaagaatttgtttgattctccctataaaaatagttaaggaaaaaggggcgcttttgttaaaggactaactattgtagagaagatctccttggctcacgaggtggctttaagtgatagggattttaacctaaagacaacataggagggaggggtcaaagaaagtcaggatatggcaaaagcatcttttggatcgaatgggcttttgtgataaatggcggaatttgatacatggatgtttatgtaatgaagactttggagtgcttgtggatggtgtgccacatgggtactttccagcttctcgagggctgcgacaagggttccaaacctagcctgttgattttagctgaagaagtgctaagccgggacttggtatcattgaaaatgataacatcttaccatgcttcgagatcgtgcccagcactctcctactttctctttgataacgatgttctaatattatataatagccataaacggaatcttaagaagcagaaaatctttctggaaagaagtaagaagctgattgtaatgttgtaatggccaaaaggtcaatttcgataagagccagtgcttcctctcgaacagagctcctcgcagaaattccagatcattgaagaggaatcaaaaggtagttttcctatcaagtacctggaagttttcttgtccctcaagagaataaagagagaaccttcctctactggagaaaatgaaaagagaatctcagattggaaaagtaaattgttgtcctccggaggtcgactaaggcttattaaacatgttatagtcttcctatgcacatgtgcaagtttttccttaattagccggcccacacttcggctactaataatgggataagaccttactactatataggatatgttaccctctctccagtgagtgcagtgaaggactctcgcctcacccgcccgtttgacttatggcatcatcgacttgcttttcaatcaaagcgatttcataaccataaagaaagacctctccttcgggatcagtcccgtccctagatgtagtagtcaatcagcgggacattcaaagaagctatgcaccttcactgaatgttaatgaaagaaagccctttcatcctaatctcatctactgaaaaggggccgggcgtagcacgttcttttgggacacataggctattacagacgcatcaaaaaagacttttcgaagcgcggaatccctgaatggaatcattgcagaagaaaggtataacggttgggaaccggaacaggattaagcctttaagcatgcagatgagtgtttgctgtcagccccaatccttcggtttccggattggaataaggagttccatgttcatactgacgcatcactctatgccattggatgtatgttggcgcaagaagggccgcttgatcactccatctacttttaaagtatacgactttccgctttggaattatagaaccaccgaaccttctttatcatgattcgacccatacctcagacccaagatcgagcaccagagctgctcataacaagstaccaaaagaagaatgcgagaagttcatattctccagattcgactataaaccaggtagtgaggatgaaaaaaagcataagctacctcgttcgtgctcccgtctttctcgctgccatcttcggtggatgcgccccttcacttaaaggcggccaaaccaacccactgagccaaccttttagattgaaaaaagttactaagctagtcacctcacctctctttcttacccgcccttattagtagtaggcaacctttctttctcgcctttcttcmagctttttccagataaagatctaatagagttgcgctttcttagtacattgcctttcattaccaatctgtcgttttacagcacgaagttacctgatgttcgctactactaataagggcggagagatgttaacctttcgctattagtaagcactcccctagttttgacctaatgagctttctttacgttgagttaattaacccggcgggttcgcctagatgcctagtaaagaacgagctggtgggaaagagctggagatcatgaaaagatttccacacaaggaggcaggcgaccgggaagctttgcttctcgaatgccgactacatgggaacagatgttatataggttgattctcattcttgctgcccgctcgattccgaggaataaagggagggctttaccacaatttcccaagtaagagatagaatctcactaattggaaggaaaaggagggcttcgatccattgtgattcgctttcttggtatggagagatctctgccataaagagagagctcctaagccttattctgcagatcaaagagcgaggtaattccccattcatccgaaatagtcttttagtaaagaagagaggcattctgggccgactactacgactacatgcccatctagtgcagtggcttggaagcaagctaccttgaccatcttccgaagttctaaataatttactgatcaaaggctgtaagggcggactgctctacattcagccacaccacagtgaccccgaagcgatcttcttctagttgcgggacgaaatccgacagccaattgctggctctgaataaccagcccagcaataagctcaattcttccataacataaggggcgggcttgcgcgcgagccgaatgacgtaggtgcacaagagtacttcgcgccacaaccatctccttttataggttctacggaccgatgcctgctgcttcatctgggagaaaagaatcatagatatgccggtcattagaaggaagaaccgccataaaagattcctcgtgtatcatctgtagcaaaactatgaacgggagctagcaatccggaccgtattgaaaaggttcctgagacacagcatggaaaagtaacaatattaagaaacgaggtccaagaatgaagaaggggttgaattactgaatgaatacgagctgtggctaatacccgaggcataaagaagcattttctacgggatcccgaaaccaccagccaccccgacctaattcatgataagcccaccaacttcctggcaaaatgcctacggttaaaaccaccgacatgtcaagatccaaattcgaattggttcctggtcctggtcagagaccactgtgttcgcgccggcggtccaacaaagaggcgaagtagtggtatctttctttccattacgaacgacacgcttcgcctgctccctccccgtgtccactagcgctcctgtccagagcgaagagaaggcgaaaagcgccgccgaagcagcataagcaggcttctattgcbacgdaacaataaagcaggatagcattttgcgcccacatgtttgaatttgagggtaaagagctcgcttgttatacgggatccgacgcatccaacagagcgaaacagtgttccattcttttcggcggcatccttccgcattggcggcgagtggagtgccacaatcccattcatcatttttgatctacataagccaaagcccatagcactggcgacgtctccggcataaatgcahgdagghtgtatabctbatvbagbatcttgtgkaacaggatttgattctgcaakcggytcagtamaaacgaagaaatttcgaacaaaagggtcggaactcgctgataggaaaggagagaaaacaaagcaatgccaagagctccgtcaatccgctgttcatcgatagacgdctctctctttatcatctcgtgccagatgcaacatcctttttccttctcgcgaaccacgggagcgcctagcgcccagaggagcaaagctcattttcctttcagggtaaagcggcgcataaaaaagggctggcccgtcaaaagtccggttccttcgcgaacgaagttcagaatcaacaagggttcgtagaacgaagggagtgtataactggggcgcagccccacttttttgttcgtaacgagggagagatagaatggagttcttcacgaagttcgaaacaaaggaataaaaaaaagtttctctatggcctcctcgttttgagacattatggcttaggggtcgaccccggtaacaaagaaggaatccataaaaacttaggatccaacaccatgataaaatactaccctcatgattagaccatgtccctgagatttgataaaagaaaggtgcattagcggttaatacgttgtaattggataagttattaggaatatgacggaacgaaagaccaaggaaagaaagaagaatacaccaaaatgcaagtgctgcaccaaagactggtggttgtttcttgttgtaagtgaatgcaacgaaaagacccggaaataacgaataatgaaacaattcatatattgacatttcgtgctcatttccaaatttatgctttgttattcccatcatccggtaaccacaggatgatccacaagaaaggtggcaggattcgaacctatggccggcctgcccctgacctgctgggttgggtggccgggttagcacccctcgtcgcctctgtacccgaaacagatgcgctgcgctacccagcgcctaaccttgtctcccctactcctcttctggttgtgccattaccaatcgcgggtaaccccggtccggccgcccctgacctaagaagaactattatccttatgaccaaacaaggaccagcttacttacttctcgagcgatagttccacgatcccgaccagcaacttcttgggagtaggggcatcaaagcttgcccaacctagtaaaggggcttggggatagagggttttctggggagagaaagtttccaggttggattttttgagatcaaatagtactagttgggtagatagaggtggtgaaatctaacctttgcatcgatcttctttagcagggcgggtcgcttgagtgtcaaaaccaagcggtggttgttttccttggcttatcgaaccagcgtatgcccattcctcctttgatgactcccagtagagaaagcctaaattttccgatgtggattgaaaggaagttggggatggacatagatccttccgcctatccggagtgttggaaatatagcaatgtttttgtattttgatttcccgatcattggaagcaatcttcactggcacaaggatctcctcacagcaacctccactacgatagaaaccgacaatgagtttacgaaggcttcgagtagtgcgggataggctaatcaccagactgctctggaataggttaatcgctggagacaagaacgagtgaatctagtttcgagagcatgccttactctaataggggcgtagagtttctaagtgaaggcaagcgctactatatatgtaatatcctagctgtcagcaaggcaggtccgctataaagcctaccggccagaaagtccttaagaacgagaaagccgactaaaggcwwtyyywtarscgrcycttgttgccgagtcgaggggcttggctggtaccaggctctaaaagagttttcttcgagcgagcggtctttctatcttttgggttgcatgcccaaggcaatgcttttgtagattgagatggattgatcttcgctatcgtgcctcctccttgtaccagttgatgctggggcagtgcttaattaatatgagttttctcctgccccagacagcttcgaggttcccatcgatykattmcagaggtttctaccactgaacttgcttatgctcccctttgatcgagtgctatttctataaataagattgagtaggaaaatgttgaattggcttcaatcgagattgcctcggcttcttaggcacatgaggaaccggcctaacatcttttcaatcgaaatcccaatcaaagacaagttctaccaaggccaggatctgaaagagaggattcactttccgaaattccaagtgacatgattcctccttcagaagctaaagttgaatgatcgaagtctcctttaggttcagtcgaagagaycgaarcgaartcatcaattcaaccattcgaatggtctccccaaagattgacctcttttccaaataaaccgaacctcgataccagattcatcaaaaagatatggccatctctctaggttgcacaacccctttagatcgttctattcgtgcttgaaaacgaccccatcggtccgctccttttaatggacattcttagccgtcctccgagggttaacaccccatagatcagatcgtgaactctttcagacccttagtttcacttggttggggcagagtttcagcctgccttccaccgaatataaaaccttagagctgcctaacctgctgacatcccggcgaagagagtcattatttgtgttacatcttcgaattcgagagaaggctttcctcttatctctcaaattataggcattgaagcgatcgagagaaagtaagaaaactattgcacacgcccccattcgccctttactaatataatagaaggtaaggcaaagcaagagtgaaactacgagctaaaagcaggcgtgcctctcttataagagaatatgataccatccccacttttggcgcacttctttgatgagctaagcctaagcgccatagaagtcaaaagctagcctgagacctaaaaagcaaggtcgaaatccatccctcttttcctgtatttgactagtagggctaatgaacgaccctttgatctatgtcgttccaagttcagccaggtctgattagaagttcaaaatgagtggagcgaggggctttagagggaaaaaaggggggcgagctttaattgaagtaggggcggagctcctcatagagagttagaaagcgtcagttctcatagcgaggcttaggccgacggggtagggcgcggccccaattctcaaccccgacctagacaagtggttttaacccacattttgaaaagttctgttaggttcttagtagcaatcggcgaccttttcctcttttacttcacatagcttttcgtctccttgatagctggaagttctccaaaagtatgaaaagctggaggactttgtaccatccattccggtgtggttggattctgttcaacagcccaaggacttggagcacatcttttgttctttccactgcttgaagtgattgttacgaccacgaagaaacgacaaatcccaactacggatatataagagccaaaactgctaagggcattccatccagcgtaagcatctggataatctggaatgcgacgtggcatacccgaaagccctaagaaatgcataggaaagaaggtcatattaaccccgaaaaagtgatccaaaatggatttgacctaaagtttcagggtatgtccgaccaaagattttacctacccaatagwgaaatcctgcaaataaagcaaaaacggctcycatagaaagtacataatggaaatgtgcaaccacataataagtatcatgtagagcaatgtctagcacagaattagccagaactatgccagtgagtcchcctatggtgaacaaaaagatgaaacctaaagcaaataacatgggdgttttgtattgtatcgaaccccccacatggtagcgatccaactaaagattttgattccagtggggacagctatgatcatggtagctgcggtgaagtaggcacgggtatcaacgtctaagcccacagtaaacatatgatgagcccaaacaagaaatccaagaacacctatactgatcatggcataaaccatgcctagatacccgaaaccggttttcccgaaaagtagaaacgatatgacttatgataccggatccaggcagaatgggaatatacacctctggatgaccgaagaaccaaaagagatgctggtataatatagggtcccctccagcgggatcagaaaaggttgtattaaagtttcgatcggttaataacatggtaattgccctgccagtaccggaagtgataataaaagtgggaatgctgtcactagaacggaccacacaaatagaggtgatctatgcatagtcattccaggtccacgcatgttgaagatagttgttataaaattaatagaacctaaaatggatgaaacaccagatagatgaagactagaaattgctaaatcaacagctcctccagaatggctggtaataccacttaagggcggatagaccgtccacccagtgccgctacccacttctactaaggctgggcttaataggagcaagagacttggaggcaacaaccagaatgaaatattatttaatcgtggaaatgccatgtcaggcgcacctatcagaatcggaacagaccaattaccagatccacctatcatcgccggcataaccataaaangatcattaaaaaagcgtgagccgttattaaaacattataaagttgatgattcccaccaagaatttgatcgccgggtcgtgctaattccatacgaatcagtactgagaagcatgtgcccatcactccagcaatggcaccgaagatgaaataaagagtccctatatccttgtggttagtggagaacagccatcggaccggatttgtcgtaaaattgagattatttcgtttccttccttatcagagagggcccgcggggcttatttattgaaaaggggagtgaggggaaggaagaatggaaagccctcactttattgatgggacattttgatccccttttcctctcatcctccccggttctggttcaggaaagggtcaacgcaaggatcttatttcgaagcaatctctggagttttcccttatccgaacgggtcttgcaagaaaataggatttcatattgagctccaaatatacgctattgggatgggatggctcctactagctctccccccctaagaaccgcacgtgcgagttcccccgcatacggctcaagtggcgaaggccctttccttcgcgcttggtaagcgcttcgctgtagccaagcttactgctagcctatcggctagagccaagcttcgaccgcgactgctcgtcgcttctggccgccttattccgtcacccgagatccaagtcagcaccggcaaagatctcttgattcctcgcggtcgggccggcttggaagcaagctacctcttgcctatctcacctccttccttcagctgggtgagccttcgctttttggatcgtcttctgcccaatgcggtaccccccgttttttggttcccattgggtttaccttgttcacaggtcgaccccatggcagcaagaaaaggcgatcttgtgctatactccggtgatctctttcctaccgagacacgcaaactcccatcgtgtcccagatcacattccgtgaatcgaaaggggaagcctactcatctatcagctcctctcgtagatcggtgtggttttacgaagcgtctaagcacagttcactcgcgttgatcaatcaagagggttgccgccactccttaaggttatctgttgtatcatacacttcttgcattctgtcccacgcttcatacctcctctttcttcttaaggtaagataaagggccaggcatggtggggtaggagcatccagtcggcaatctttttggcttgaccaagaagtcttatgtcctccgagtcgcacggcgttttaaccgaaagaacttcttgcgcaaytcatgccrwgcaswaggttktrkdcgaattctttctttatbtcgagatadcvdtgdtctctggacttttatcaatatgaggtgatcgtaacacagtatataagactcgtgattcaggcaatccaatcttccgtgtgtaaggcggaagcccccaaaaatggttttcaaaaaatgggtgatcaaagatcgaattactatgcctatcttggtggtcgttacttttggtggtctttcttttggctgactcctatagacgaagtgcttcgtttcagatcaattcttcgctgcaatcgcttcgatccacccctcggtgaaaaccgtaatacgccctgaggaattcctaccagcagacttccctgtactcaaagtgaattgtctaagtgctctcctttgtctcattgtttatctcgtaatcattcgattccgcccctaaagctagcgcctactcctcctccttctcctcctgaatcctccttggtccttttacataacactctcggccgcccaagaggactggctatctttctctttatacgcacaatatcttgaaaggcaaagaaaagatctaccttggcaacgaagacgtcattgactgatagtttatcttccgaaccggttaaatacctataacaaaaaaaggccaaagcccgctgaagcactggaaaaatgttgaccacgatttctaacgcttttcaaaaccatttgcttgcaacgccttgagtggacagataattacggccactagatccttcatactcttactaaagtacacttaagactcaaccaatcttgaaagtggagtggacaactggcataccttgaatctagcctgcaatcctttcgcacttctcttatcaaatttctagttagagagagctaaccgctgccaaaatgcagcagtttttcttatatacgatagcacccctgccctccttgttcaagtagttcaagagtgaaagggcgtagtgaaagaaggaaagatctctttcaaagatattctacccataaaggcagttctcttatatggcaatactagattggcgagacaagagagaaagcttataaagtagtaaggtgtctatggggcttgccttacaggtagtgactataccacttacatatcgaacagatcttactctcaatggagtcatttcgatatgacctaggaacttacagaataccgaacttggataatcggtagaagaatgattggctagatcatttgcttcactgcggaagaacccctttctacgctacgttcccaataaaaagccgtcatccttctgtcgcctgttagccacaccagaccaagaaaaggcaaactaatcaaccaagactcagtcacgacctttgtaacctcacggccactttctttcctagagcttgcagccattatcttcgcttttcagatatggtgacattacttgtatdgggaagtgccagatctttacggatcataagagcttgaggtacttgatgacacagaaggagttgaaccttcgccaggatggcacacttctattcggggacgagtatgtgttcctcaggacagtgacctgtgccatgatatcttggaggaggcgcatagctcaccttgdgayasacccagggagcacgaagatgtacaggacgatccgcccacactattggtggaaaggtatgaagagggatgtcgctgagtatgtggctaaatgcttagtgtgccagctggttaaggctgagcaccagagaccagcaggacccttacagccagttcagataccacagtggaagtgggacgagatagccatggactttgtctctggattgccgaagactgcgaggcaacatgacgccatttgggtgattattgatcggctgaccaagtcagctcacttcctgccgatcagtatgacttactctacgggcaagctagcccagatatatattgatgagatagtgcgcctacacgggataccatcatccatagtatcagacagagatccacggttcacttcagccttgtggcagagcctacagaaggctttgggtagcagagtgagtcttagcacagccttccatcctcagaccgatggccagtctaagaggaccatccagacattggaggctatgcggaggtaatcccttgattttcgaggttgttgggacagacatctacccttggtggagttcgcctataacaagagttatcaggcgagtataggcatgccaccttttgaggcactctatggacgcaagtgcaggactcccctatgctgggatgaagtaggggagagacagattcttgggccagagattgtactttytttwtyttawkcagaagrcttagtacaaggttctgtcgtttaccttgcgcctatctattcctttaagcttatatcttataccattgcaatcagactcattggatatcttccttttctcttctactatcgagagtcgtacgggtgaggaggtgagctctaagcgtatacacatagataggtctgggtaagcgaccatcagcggtatgggtagcagctactatcagtacgccagtctaaggctgttcgtagaggtaggtcgtagagatctatgaagggctatatttagcataaatagcatggttaattatagaatagcgtgatggccgtaagaagatcataaataaggtaaatagtctggagtggatgtctagatcagggtgtcggcatcacacatatagcatgtgtgccgtgagtgagagggtggtcgtagatcagccctcagctcttctttcgaaattctcgaacatgatgacttatcggcttgaggcttcttttcttttcaagctgagtagaaatttcataagagaagaaaagttcacagaaggttcttcaatgtatgcctggttcacgaggttctactgcagggcccagtavdmsdwtmgctctaaagtaaggagaccacttaaaaaccctcatcggataagaaaagatataccagatagagcgcaaccaagtccatttttgaatgataagggtaaatcatcaccttatttgaggaagtagctatggaagattgggtctgtatggcttcctggggtcgaaagatcttccttcagccttgaaagtatgctgctgctttagcgcgaatgaaaccatttctcaaaatcaaaaggaatcctcctcttgaggttggtaacctagcccaaaaccatgctcatgggaaaaaaaagtatggggaaatgaaaagagaccttgatgtcttcgccctaagcgcatgccaggaaactcattcctctcatgattcccatgacacgaatcttactctagggatcgaaataaaaggtaaaatactccttactcgtaattaaacccactaatcatcatatcttttttaccttgttcgatttgcagaatggggatattcgaatccggtccttctgacatatctgcatccccatgtatagtaagagtctttccaacgaggaacttcactatcgtatagttgactcgactcgaatgccctcttagcaatagcatccgtaaccgcagctattgagtctgctgtgggaataagcgccgcagaataggcagctattgactccgctctaagcctaggcactctggggtgaattaccggtgcgagaagtctgatgtcaatctatctaatagtataaagattacaacgacatagccagagactgaaacttattgtttagtataggctaagcgcttacctaaacatatggtaatgcaaccaccttagtcagtgattactaagctagcgcctagcgctaaatcgttgaaagagaggtcccccatccctaagctaacgagaagggaatctctctcacaagccacgatcagcacttagcctaaaagcctcttcaacgaataatgaattaccgaaagcctcaatctcttactgcttacctggtaatgccacttttcgctccgtatactctagcaagctagtactggtcgactaagtggtctcatgcccaagtcaaatccaatgacgagttgagatcatacaagagtactttaccaatcaagggatagacctatcttgactaagtaagcaacctttctcagacctcttggaatagacctttatttaccaagtttttacccttttgtccactcactactgatcgcaacgaagattagtctcattacggtatcaccagcaaaccttctttttattaggatcacaagaaggttacgaaatcttcttttctttttgcattcttacaaatgaacattcccaatggaaataattgagactaaccatcttatttttaggtaatattgaattcccgtgcctattgtttagcctaagaatggaatggggggcaaagctgtgaatacagttagtgaagctagaccgcggaactcaagggcattctttgaggtattataaaaacatcgttccatttgatagtaaattctagcatctttgaagaatcatattgagaaaaagaaagaaggcacgaaaggagttgagcaagagctataagaagaaggtttacctcgtaaatatgtaaagtggaagacaaggcaatctcataggtgaagcttcgtttttctataagcagactttgagaaagttgaataccccaaaagtcaaagtcaaccttccgctatgaaatgaaggaagaaaacaagggctaacgcgctcatcccttgcttggttctcccgtgagggaaggggaaggtctagtatacaattatcttcttcgggaaggtctagtatacaattttcttcttcttgatcgaagctctatctctcattcagcaagcttccttcaaaaggggagtccataggcgcgaatactcggattggacttggaaccccccgcggagttgaagactgacttcggccaggagattgatagagaccatccttttgctttgattgagagagccagagccagagcccttcagtggtagaaggatctaaaattcccaatgggagagcatgcgcccagagaagagaagggcttaagcaaagaaggttgacttggaagaccgaaaagcaccttttaaaagcacctttttttgggttctatcgaagacttttagtgtggaaagcaagcctttaagccagaagtgccgctgtgccagtggaaatctaccagtacccgttgaagtgaaatccgcttcagcatcatcaagaagaaatggaaaaaatgggatttgtggactcgcctcaggatggaggggaagctactgtggaaaaaggcagttgttgagcaagtgacattggttgaagttcaatatgaatatgcatcatcaactggagaagaaagatgaagattccgctgaagatgtcgaagatttagaagaaagatacgatctaatatgattaagacgaatatgtcgagttagagcacggattgaaattgttctcttacagttcctccaccgaactgtagtacagaaggaatggaatagccgtgatgcggtctgtcgccaagcccgcctctctctctcgttgttgcgcggccattactctacagaaccagcatagctcgcagacgagcacgctaatgaggccctgagccgatagatgaagatgggaaggtcagacttctactgtctcgaaggttccgatagaaagaatgattgattgcttgaatgccgggccatctactcgcgaaatcaccccggtccgaaccctctcagctccttcctaaagaagtgaattaatgatcgatcaacggagggaaaggaatatcagaattgggacacctggactcggtctttctggttccattggttggtaggtcttaacttctgggctaggtctcgatacggaaggaatatagagggcgggcgtcgaaaccccatgctttgagagttcctttctgccagcactttctctacccgggagtcacttcatcagtacctggggctactgtcccaggatgccaaaggtatgatccacacattgaaagtgtcaacgttgactcacacgcgccaccctcaccgggtaaatccggagaaggggaacttattctaagatagaataagaataagcagaattgcttaagtaaggtagtggccataaggcttttctttttttcggtataccgctctgctcgcagagcgaatgaagataaatcttacctaatctcatgaatatccttcgccccttatctcctcatcttcctatttataagccacagcttacttcgacgttttcaatttcccatagaatctccggagctttcctagccactatagttttctttttttatcttctttgtctgaaaataggtttgatttgcttcacctatgagaatttctaccaattcttcttttattcatcaaagctcatcctaatctccgtcgagattactgccttagccctgtcctatcatctgtataatggagttcgtcatttattgacggatttttcgggatttttctttcttagaattggaagaaaaagattgaaataactgttccaaatttcacctatacctttctttgagatttaaacaaaaaattattctttttttatgaaatgtttcttattcgttgatagatctaaagcttatgccgtagaagctgacatcaggctattggccttttatctgcatcttccctcgtagagtggcgtcttttataagaaaagactttctcagtggaactaaaaaaaaaaaaaagagtttgagctcttttttttgctttacttttagccacgcgcggcggctatgcgcatgtgtcccaaagtgacgtatattttttggtaatgggtatactcgagagaaaaggtttggaattcgacctccccttatacgctctaaaaaggggtcatggactccttttttgtataggatcccctttctacattcaattatttattgagcctggtgtggaatcaccatcattacacattcattcttggtctggctgctggtctagcgagccttcctagccgcctagagtgcagcctgcctgctgaagaccgtaacgtaagtaactcagtgctccatacgggggaaatgaaagcagaattcgttcggatcctcccacatgttcaatctttttttagcggtttccccagagatctttatcattaatgcaaccttcattttgctcattcatggagttgtatttagtacctctaagaaatatgattatccaccgttagtcagtaatgtgggttggcttggattacttagtgttgcgcgcctaggagggcagcgcgctttgggatgcggaggagctattatcgtccagctccctaacctaaagcggcaccgggtttggaccgcagggaaccgtagcatggggggacgtctaatccttttgccgccgcaaggctggctaatcgtacgcagcaggctcgaatacccctggttctggaaggcacatgagtccgaacgctatgttgaatgtgcgaccgagactacactacgtaggtacccgtgcaggtgaggcgtcggtcggtcctagaaacggcggcagcggcgcgaggagttaacgaccggacgtgctgcaacctagggatcaccaggcagctctttcgctctatagggatcgggggggcatagcacaattcttcttggaggagggttgtttgcccgggtgactgatcctgccataatgtacttctacctattatagcaccggcaaccgaagtcgagcatacatacgacgatcttcatgcgtgaatagccgggaggaaagaaagggcggtagatgataatgagaaagggcgccgcgtctggacgggcggaatggatgagcgaaaggtgtcatgccatggagtggggaagagccctcgtctcatgtaagacaactaaatgcacctcgaggtgctgccgaggaactgagggaccttctcgagcacaggataggtaattgagagatagagctagcctattcgttatgggaaatcaatgctccgggccaaatagagcttacctacggcacctggctttctccggcgagctttctatcgtaaagccaaagacgccccaagacaaggtacaactgttgggaaggggacatgatcaatagaacctggctggatccgggctgggatagtggcgcccattcttaaccagttccgagagggttcgctcatgctggagggagcatccccacttagtgatcggtccgctagttcacgcaaatccgaagaagttatcacggacgagccacatgcagggaaacttgcacgtgtggttctggccgggctttcctgaggtatctaataaccttgcttctgctcgccgctggcgcacctctcctaactattgcccatttattctggaataatctttttaggagggacaattttacatatttctgccaaatccttctattattaagtacggctggtaccatttcgatgtgtttcaattctttcgaacaagagaggtttgatgcttttgaatccattgtattaattccacttcctactcgcggtatgctctttatgatctcggcttatgattcaattgccatgtatttagctattgagcctcaaagtttatgtttttatgtgatcgcagcatcaaaaagaaagtctgaattttctacggaagccggctcgaaatatttgatcttaggtgcatttccctctggaatattattgtttgggtacgaccggacaactaccgatatctattaatatcttttcttagaatgttctttagaaatatatatctatctatctatatcgtaaactatcggatcgggtattacttagatgtgaaacttgcagacctcataggttgtaagatttttcttacggggggaacgaaatcaaagaatatatagactagtagagaccctctatgtagtttctatctagggcgatcgatctacatctttccccatagccctggggctgtgtctcgatctcctatgtgctaaatataagggactagttcctatagagattccccttggtctaattccacgccttatgacgaaaggggagtcggcgtggcgtaaagtgaagattggggggagtagaaaaaattcccttatggggtattccgaaggtgtaacctaggcaacgaaaaaggggcccgatacttcaactagaggagcgaccagttggttcaccaaaccccgacccagcgtcacacattctccaggtccgaagggatccagtgcccaactaccgactcctcccggaattgcgttatcggagccgagccaggaatggccgttagtggacacccaccacttttcaccggttagagaggccctctttaatacattaagaaaagatgttcacaggggccagaaagactcggtcataggaatttagaacacctacgtgctggtaaacgaaaaccacctcgaccggatcagagtaaacaacaatgtcgaatcaggccgccctttgccttgaaagaattcacacgcggccgccagctttcccaaaataaggggagatctgctgcttactgctcacggaaacatccgacctatactatagtcaagtcgttcgcctatctttctgatctcctttccttctattcatcatcttttttgctttgacccagtgaaaaatggggttgatggtgttggctaaaaaagggggagagaggagagccttagggtacgctcacttctgcatttttgtttaggttctcgagattctcaatcgttctttttagtggggaggaatagtacgtgaatggcggttctcagacgagggaatcattcctctataaataaaaaaaagctagaatctttctattgatagagctttcacgtctgcgcatagaatccttttttgcccttccattctgttcttacggtagttgggtcggaatccgtgtgatggttcgaaagtcgtttcaaatattcttcgcatccccagagagatagattgttgccattgtgccttggtcgtcaaaaggggcacgaacagccttaaagtactgttccatgtcccagaggtcttcgagccttggcatttcgaatcccgttgaatggctgtggttccgggactcaagtctggagtcgccaggtgagacattcggttcacgaaccggaaacctatctccacagcaagctcctcaatttgacccggtccgtcacgctttggacatcgccaccgggatcgttgaggccccatgaagacggctctacttcacagggaagacgcggtactcattagcgagcgtctggtgaccaaggattccggattcccctgcctttccgctatagtctacacttgtccgtccaaatggtcgaccttgccatcaagttaagttgggtcactcgatccttgagtgtttccttaacaacagccgccgctgacagcactccactgctatcgtcatgtacatggtacaacaagaagagaattagcagaaatcgaaaggtttttacccaaaactccgctctgatacctcctaaagcgaaataggcacgcgcacgggtagagagtctgcctgagtcgtgcggccccaggtaacgcctagtttagtgtagcacctgggttccgccttctccttgccgagttttgcttctgatctctctctgagtctctagttcgttaccttctactaccgatcttctccctctgctgctactggatatcgacctaagagatactagaccaggtgcgagaggaagggatgctgctattgatggaccggtgctacctctggatctaagaatcatggaagacgtaattgaaatatgcacctggaattgaatcacattggtataaagagccggaaaggaaaaagaggaggaaagaagcaagggactgagcgacgaagcgaggtttggaacccttcaattacaaagtggaagatgcctctcacaatgggtaggattactgcatttcttatatttgactcttctatttgataatatagggagttggggcaggttgaaggggaggggaagtcaatttaaacatagtgccaccataaccctaagaaaacgagattgggtttgtgtgtgtagactatccttggaagtgtctattctaccaaaccacgggacgcagccgtagatcgagccctggaagtcctctcctcgcggctccctgcgttgatattcgaggaagtagctctcgacacgagggatatacaagaaagacctgctctagatccccaagtctccatggtcgttctttttaacatctctttctattcttctaatgtaatgctatcagtcacctcgtactaccccccattgcgcatcctgtgtaacatcaaggaaagggaaggctcatactaccccggcgggaggtcgtctcccaacacattccccctatagtagatctgccacagattgaggcatatcttttggagatggtcacgtcagcggcggcaagtggatcattcatgcgaagacttaactgaaaaagaaagattcccttttgttaccgaccttcttcccttgactggtgttttaggtcttcttatccaagaggacactttaatcttgctttagaggccgaatgcttatcattcttgccttctaaacttctttatatcgagggatgaggaaccatattatcctgcattccttaaacctatgtagtgagtcgtgtaggtggcgtgtttaaattaggaccatacattgggattcttttcccctcatcgctagccagtcgggatgctatctctcttctccttcgtcactcaaccatcaaaatatggtatataataatctcttttttttatatttacttaaaactatactgaaccacctatctattcgttttttggcgctgtcccgacactgatgagcatcacttaggccttcattcatgagactctgctaggatctgcagcgcttcagtaggccctaggcactgatgtgaggttaaagttttaaccaatgcttaatactatccataaacattgtactcccataataataataaggcaagaaagcggaaaatttcaaaaaaaaagtaaaatggaaaaagtgcccccttttgattagccagtttccaagagggagaaggtcttatggcaatctcaggcatactcaaaatcggttatttggcctgatcgagcaacctatgaacagttgtcgcctacataacctacctcccagaccaagggaagaaggtatcagatcacttttgagagccctttagttaaaccagttcctttactctttttgaatgaattacagtcagtaaagtaatctggtggaaggggtccatagaataaaaattggcttctttttcttttttctattttgagttttagaatagagaaagagtcgaaactaagggtacgctctctagaagatttgctcggagctttttttttcacttggtcgcctggtatcttgaaacctctttgcttgcgggggcaggagtggaaagagcgcttcgcgaaagaatcgtgtggcgcggtgaaaggtttcccgttggggtttccgaccctccaggtctccacctacttgtggaataggggggggttccttgatattaaggtgtcaaggcggtcgaagaaggccacaggtggaagcaaccgatgctttgatcattcaattgactccttgctgccagtccgtgcttgctgtcatgctggcaaaagcaggggttgcggtcggttttacctactattggatttgaaccaatgactctcgccgtatgaaagcgatactctaaccgctgagtcaagtaggtcaagctgagtcaagtcaccctataagagaaagccgcgcaaccaaagtagcccttactatacaaggggggcagagcgctaagaaagagaaagccttatcactatacgaaatgaagcagcggttagcacgctaagctaagatcaaccaatgttcgaacgcggagcctttctttctcggtcctctgtcttaataagtggattccgattcatgcagtcgttctctgctgcattggtcttttcactccccactctccaccataacaaaatgtttccactatatctcaggagtagtcaaaggaagtacggcgggtccgagtaggaataaattgactaagaagtagggcatacaacaatggatcaattcattcaacaagatctgttcggatcagaccaggatgaatgggattggtctgacctctcgctcggatgtaagactcccgccgctgacagatgtcccatgccacctttcgtgaacagctatgcccgagaatgaatgaattgtgatatagcgccgaataagccacagctctattcccgactcgaaatccataaaggactttaagggagataaaatagggggccctataccatacatcctgctgccttgggacgactgcacgttacatcatagcagcacgaccaaatggaggtggaaagcccttgtataggttgggcgctagctagcgccttccttatactaatcaaaaatgttgggccttccccttatttattagtcttagtaaagttgctcgaggacttctactgggaatgaaagttccttattataggatccctagtaaagccaatttaatgatggccgcttatctgagtaagaagacgatggctcctattattggtgagcgatctcctctacacgttatctttgggcgttttactctctttcaaagagatgactattcaaacctcagagtattcggatgcacgtgctttgttaaaattccatctcctgcacaagacaaactgagccctacatctcactctatgtgttttcttgagtgaggttggggtacccctctctcaaaagggctacaagtcttaatgatccttctacacgacgattccacctttctcgacatgtcacctttttcgaacatgtgccttactacggagctcggggctttgagattccctgtgatggtgggccattatgttcccttgtctccccttagaggggaggggtggaactattgaggagtttatgtgagacagcatcagaattctccgatttaatagagtcagcaagatccgggtgaccagagtgatcagcagcttgatcagcttaaggggaagtttcgcaggtttgtgaagacagattctcgtcactcagttttcagagctgagccaactgattcagtggtctccctctctccctatacttcgaaccaagactcttcttcagacttaggttctctagcttctattctcggggtacgtagatccacccgtcttcgttttcctattcataggtttgtatcaactaagtctctgtctacttcccacgagtcttttttgcaatttcatccatcttttttaacctgatacctttgcagaggccatatctcaaccctgctggcagctctatgcagaaagagatcgtagcactagaatggtttgctacttgggattgagtctctcttcctctagggaaatctatagtgggctactagtgggtctataaagtaaacaaaaagctgatggagcagttgaggggttgaaggctagattggtggccaaaggatacacacaagagtattgagtcgaacccctttagagataggggaaagatttgccccagcttggcgaatcgcatccccgcgcaacgaattgcattgccaacctcttgattgtcttcttatcattctccgttgcatgttagggatacgtttggtcttcaatatattccctgatgtcagtaaaccatggtttaccgttgggtgccctttcaatggccaaaagatcactattgaacatgccgggagtcaactcaaaaatttctattagtttgcaatacaccgggctgcttctttgttctatcatgattgggcggactttccctcaggaatgtttatcatggaggccagtgttgccaatacatccgcgaacttattttttctctgggtagtggagagaaacttattttcttgaattgctcagtgagcttttcaagataagcatggtatgtcaaatttcatatttatttggtttttcatttcttttgagtttggcagatgataagcgtcgaatccctaaatacttcgatttcttatattcccagggtcaacgcagtctttaatccatggatacatgcttcatcttctgtggtattcttagttccttaaaagtggagcttaatggcaatgggggtgtgcgattcatcaggtgcaatcagcaatgcccctactccgtacccattttgattagtcgtgccatcaaagtcaaatttccatgccctcctcttctgtgacagctatttcctcgtctgggaagcaatccttaaactcatgttcctccttgatagggtgcaaggtgttctgctatcgcccttcctttttggttacatacgtgatgtcgaattcagacagaagcagtaaccatcttgcggtccttcccgttacgttaaggcgggtttttcgaacaaatactttttttgtaggtccatggaagctattaaatgtactgggtaagacagcatgtaatgcctcaatttccgccttacccaaaccaaagccaagcaggttttctccaaattggtatacctggtcttgtagtcagtaattttcttactaaggtagtatatggccctttacttccgtctgtcttcatcgtattaagccaacatagaccccatagtggtttcagtgactgataggtatagtaataaaggcttcctggcgttgtaggcactagaatggaggtattcctgtattttgtcaaaagctttctggcgggcttcatcccattttcctgctaaattttgatttcgaaatttgtgtatcggctcgcaagtggttatacaagagaaagtcaaagtctgatgggactattgatcgctacaaggctcgcgtggtagccaaaggctacaaccagcaatagggtatagactatgatgagacattcagtccagttatcaagatggcatcaagggcgattaggtgttacttgcttgataagggaaagagaagacgtccctcaaagccccattaacgcaaaagaagtcgattcctacgtttttaaattaccagaagctcttagctactcagctatactataggctctaaaggcattacttgactgaaagagtgcttatattatgggggcttccctttccaacatctgacttatatacaggtcaacatcgacttaaaaagcacgaaaaaaaaaagtagctacctcgggagagggatgagactagtctttttccaataggctagctgcctattgcaggagttcctgacctgaaaggacaccagcaagctgctactgaatgtgaacaaagtcaaggagatggaatcaactcaatagaattaggttttttttatgactgctgaagcgaccgaacgaaattaaggattgattcaataccgaatcccagatctctatagacgactaatggtaggggctgcatttttcggaaagaaagatagtggcaaaaggaagactgttaatcaagaaccgacgtctcatgccgaccccgtctgcagttgctactacactgttacatccggataaagtgatccgtactggtggaataattgcaatgcgactataccgtctgctgataaagggaagacagtataccaagcttgtcccagcagtcaggtttggtcctccgggcagcaacccggccggtatacactccacagagcaaattgggctgtgaggtgagtaactatattcaacaatcatttgccaacatcgttcctaagccctactaagtaaagggggatgtgttcaatcccaagcatcttcgtcaatactccatctgccccccgccgggggggttaagggggaggatgtcaaaaccttacccataaaaaaaagtacatagacctgctcacaaagagctacaagacagccaaaaaaattacagctaataaaatgaaagtgaacaaagccaaatcaatatgatattcaataagcccacttttttgagagaaaaaacctgaatttgttgaggaagatcagctgtagaggaaaacctatagtcaaactgagaatcgcagccgaagtttgctaaagagtctgccactttgttgttttctctaaatgtatagacgattttgaaatggccagccgagaatttggatgaaatgaagctccaccatgagtctaggtatgggtaattttaggggcttctttattttcattgaagcaatcaacaatgattttggagtcaattgcgagtttacgagcttgatgaatgtagagcgcatccagaagaatagaatcagtaaacgtccaagatgatctgatgtcaagaagctgagaacagtctttcagccagtccgtaatttgttgaataatagcagccggttgagatattgggctttctaatttactgctattgccttccttccagagttcccaaactgaaaaaatagtaagcatagacgtgacgtagccaacttgggatttcctgcgagatctgttaaaccgccgggactgaatggaatccgtttggaaggatcttatattgaaaaggcgatcaaaatggttccaaacctccatagcaagctcactcttgatgaagaggtgatcaatactttatttatcatgctccgaacagcacaagcatttgcttgctaatcttatacctttcgtttgaatttattcccttaactgattctgaaatccccgcatacaaagtaaaataagagcttccacgcaaaaatgcttcgatatcattgaaaaagcagtttccatgtgcgtcaagcacatctatgattttggagaaataactagtaaaggagttggcctggtcaataagagggagtcatactttggactgcttttttcaaaagaaactatctgaaagcccctatggtttgctgcttccaaacctggttgtcaggacttggagtgaaatcagttctattttcaggcaaccccaccaatacttaagggctaaaaatggtggattggaaatggagctagcactgatttctggttccacccctggctctctgatattcttctcattgaaagtacccccctcttattgaccaggtaaacttcatacgaaaagcttttgaaagctcttgaaaatgtcttgtagtaggaggacccaaagccccttcctgaataggtaggcacatagtatcaaaaaatatccagtgaagctttcttttgtcttcatcaccgcctcaccaaaagttagctaacattttttcctactggtcaagaactccctttgaaactggaatccctgcaagaaggtgtataggcatcgagaaaagaacatgtttgcaaaataagccgccctccactggataacaatgctttcatctcctaccactttattttagactctatccagaagatgagcaattttttttttaagatttaaatagaggtagtcctagataaaaatattaggaatcaaagcaaggaaagttgcattgatggaacgggggatcgcaccttcagcgaagaaataaggtgaccagctggaagtttttgaaatcccaacaagattttctatataaaaagaatccggaaagccatcaggctttaaaggataggggagacctttttttgggttagtgcgcgccgacatgctaaaaatgaccttttgaacttcttccatattaggagggctcgtaagcatcttattatcttcctctgtgactagagaggggatggtctcaaggatctcatcttcaagcaccgaaccttgagaagaaagtaatgtatgaaataaattgagagcttcctgtcatacagagacaagttctgaatttggttcaaggtgcttattctctatctttcttcgtaaagcagaagtttttcaaggttactcttggccgaatctaactccattttcttatcagcagaccaactctgttcaagagcaaattggccttcttcgttttcggcatttctatattctgaaatagttcgccaattcagtgctttatttgtcgagtcaatcttcctggagaagacttgaaaaggatttcccgagcatggttgagatcaatgtgaaaataagaatgccgaatccacattctttggaaacgaaagaccccaggcctgcgagtattagaatcttctaagaagattactagaggagagtgatcagaggatactctaggcaaatggtcaactctggtggaagcaaaacggcttttatatagaagcgggcagtccccattcaaaaggattctatctagtctggcccagatacaatgttgaccgctttgattattgctccaagtcaatttgctgtcattgaaagcccaatcaaataatccaaacgagaaaatcatatcttcaaagctcatcacttcaataaaggcattgaagtcaggaggccgacccccaagttttttctaatggatccgcaattacattaaagttccccctactagccacgccacgggaagttaatgcaagtcgataggtccttcaatcatcgagtacactatcgacttcccacacttatcatgacaacatcaccgatctttggcgcttatggggggccctatcatacacatgcaccaccagagtcttcataagaactctggggcgagggccaaggtgaacccggattaacgatgagaagcggtcaaatcagtagcaaaggcaccaggacggacggttggttgaaccgggcgatagcttcgcgatcgatagctcagtgaggtacgccacccgccctacttctaatgatagatagaaaaggtgggagaggtgctgagggacggcaaaggtacaaaaacaaaaactacatgacatacgtacgttaaatggtaggcccattacgaacaatcattaaggcggtctccaatctcgctcggctcggggcgatcacttgaacagggcgggattgatcgatctacatcaaaaattctgccttcccttcccaggagcgcatctacagaataaagagagcacgcaccacactcctactataccagggcctttagctttcactgagaagaagagattacttccagctagcttttttccctaaccctaaccaatgaatgataggccggcttaggataatcgaaaacgaattcactttcagtaatcggaggcaggtcaggggccggcgggcacgcccccagcttcttaagtttgggaattgtgcatgacctatgcaaggagcttccggaatccaatggaatcttcgtaaagtcgatcattacgagtgttacgattcattcgattggcaggtccaatcgttcatagcctctcgagcacaacccatattcatgcaaggattggtgattgaggatccatacagagttttatgaaatatcttagagatcaaggaacagatgctttcttcaggaaatatgaatactttttggtagggacaagaaattttttggccttgaatcgggtcaggaagaacaacttgttccagctccggggaaaagattcatcttccaattttcccttccttccaatattttggattttagcttccctcattccttttattgagcataatgatgcgaatcgggcttgttgtatttagtatacagcgtcaagcagttccgctttcccctaccgatgatgtgccgagaagtgcattgttggaactgggttggaacttaagaccataagctctagattcgggggtttacgctatagccgaacacaagggaaagatcatttttttaccggaaaagatcgttttatcaggtaatggatacactataagcattcctttggttatgtataagctttccaacaaagagaaagacttgtatgcatcaggttcataggggtaaatacattcaaaagggaaaaattttagcggctcatatttcaaataaagatcgccgcgtggaaaactcgtttttttggggggttgtccccactggtttgcgaaagcaatgggagacttgctccatagaacccccccccagagactttcgtccccagtattctctatgggcaaaggcgctcaggtgcgcttaaagtcttattgcctatatcttatcttaagacgaggttgccaccccgcctgctttagtctcaaatagggcgcaaattgaggtgaacagactggaccgaacctccctacgtcaagagcttttggctcttcacaagaaagcaccaggtcgtaacaccggaagactgcgccgttattagttattattaaaatgatataatttttttgtatggttagtcaccagtggcacaacctacgggctaagtagcgcctcaatgggagtatttttttcctccgcgatagtgtaataccaagaccagtaagagagaatggacttcatccattcggacaaaacccatgcccccctaaccagtcgtactctgaccaggcttcgaaaaacttcgagatcaccgagtttctcgggaatcgaggggtcaagagcctaatcaggtcccctcaccataccttgttgataagaggttaagtgtttaccagtggttgcgcttaaccagatccaaaaggggagaggacacacaccgttcggtgagtgaaagacgaggaaatgccgattccagtgtctcctaggaggcgccgtgcgtcgagtatacacccggtacccagcttcccgtaaacgatacgacaatgtaagatccttatacataagagccctcattacaggaacaagggatatggaactaactaaggatcttaacatgtgacaggagacaggaaaaaagtccttagtcactccgcgtacgaagaaccgcttagcaaactccaaagcaccaactgacgagactaacgatttctctaacgaaaatggaacattcagtggcgaaattagctcgcgataacgctcagccacccgctcatctccgatgacgatatcgtcgccgaggatagcctagcgtgtaaaaggaactcctggatatacttgggctgctacgaaccaaatcaccaaatggtgagttaatgcgaaagcaggccaagctccgtaaaagcccaacggggctcctgttacaaaacgaactctacctcgaggaagccgacgacgagaatttcgaatcgtcagaaaagagtagtaggcatactttcacaatagtcttgtccacaagcaaatcaatgttcggcagcggaaaatcatctttgggaacatgctttattgagatttcaaaaatagatgcatacgcgaacacgtccatccctcttgggcatggggacgatgttcgaaatccaatcagaataatctactgccttaatgaaatcagtataatagtaacaagacagctgaagagaggatgacgtagacaagaatcaacctcttcccggtgaggttttgatgtatcgcagaatccgaaaagcagcttctaagtgagatgatctcggcttgtccatataaaaatcggctgatcactccctcctatgttgtaagtgtaagcaatgtctgggcgataattagtcaggtagaaaagagtcccaacaagtctccttgcaagtagatgggtcatccaatagctctcctgcatctaaggctaattttagatcttattccggtttgcatgcagaaagaccagcttttgacaataaatccaatgaatacttgcactgggttccaaaactctttgtgacctcatcactttaatctccagaagagactttgagtctcctaaatctttcatatcaaactgggttcttaatcttctcttaagctcatttatcgaagctaagtcattactagagaaagcaatgtcatccacataaagcagaagaaggacaatacctgatgtcgacctccttataaacattgaatgatccgatttacttatttgaaaaccggctccttcctctactcctatttcggctcttatacatgctgctgtcacctttcaaaccaagctcttggtgcctgctttagcttgccggaggccgtaacataaatcgctttcttgagcttgcataccaagttaggattcctaggagaagagaagcctggagttggaggaggctgaatagaaacttattcttgcccccttcccttatgttgttgaaaggcattctattcttcacgtcaaattgaaataaggccaccttttgattgcagccaaggcaagaatgccacgaatggtgtttagcaacctgaagcaaatggtttccctatctctaaaggggttcgactcaatattcttgaaggaatcctttagctactaatctagccttgtatctatctaccgagccatctgctttatgcttgatcttgtaaatccacttgcagccaatggcttctttccctgcaggcaatgagactaagtcttattattattatttttttcctgggcattgatttcttcctgtatagcatctctccagcaagaatgattggaggcttcagcaaatgattcaggttcatgagaagattgaactgagatgaggtaagctcgatcttttggggaaaacgattcataagccttcaacaggataagaaacttgagagggtcgacgaagctgagagcgggatccagaatttgaggaagcgactggaagggaagcaactgggctagactgctgatcttctggagtagcctgaccctgggaaagagactgtaatcgccgccgagaataaacatgctgtgccgggtgacaggaatcctctgaggtcagctgaacaggctgacaatcggcagaaaatgctgagcaaagctgctggcctgaagagtgaggctaatccgtaacatcaactgcagaagaatgaggttcgagttgatgaacaggagaaggccgcaatacatctccatcatcattctcccccggggctgattaattaggttaaggaaaatatgaggcgaccctattaaagagagcattaaggatacatcgactctcttggatttcacgtcatagcatatatatacccggactgagcatatccaagaaagacacaagtggttgccttggggacaatttttctcttaactgcgcaggaatatgaacaaaacacgtgcatccaaacactcgcaaatgcctattatagtactgccccagtaagaagttcgtgaggtgccgctgcagcttggattatcgtagaataagaggagccgtcttaggaaatgacttaacttaaaagacagatgccgccgctgcgaggcgagggagcaacttgtctggtcttgcggtgcactcattcccgttacgagaatgaaatgaggccccagcttgactcgagaccaagactccttacaactcgcaccaatagcggcactgagcggccggagattgattgaaaaggcaggcccagccgaccctctccccccctaaccgcctatctactcgtgttcgtagctcgatcggaggtcaagactgtggtccggcggaaaaacagaagtcgtccgtatcaagtgatacgtgaattgctcagtagtgcttcgccactaccctagctggcggaaatagcttaatggtagagcatagccttgccaaggctgaggttgagggttcaagtccctccttccgctcctggcttcgtcgtttagtggtaacaagtggggtgcataagccactttagagataggggcgagcagcaagcagccccttgtatagggttccaaacctatctgactaataagtaagaggaaaggggcaagccaaaactgactcctaacaagttgctggcttttcatcagccgttgcgcgctagcgcgctagccttttcccaacctagtaaaggggctgctagttgtagcgcgcagtgtactagtgaataggaaaagcgaattgagattactaatgacggatggaggttgagggtagaacatgttcggtgcctcgcccttgtctccttcgccgtagactgaaaatgatgggaatcctatcgataaagaagaggcataagcatcgcctctcgatccaatccatcttccctggcctccccagcacactcttgatacgaaagaaacctcccgccatagagaagagatcgaaagtctgggtcccctcgatcaccctcccttgaacctgaactggtcgagagagatgaacccgcaccacattttctcgaatcgaaacccccaactagagatggaattccagaacctaaacaactcagttgagagctccgtgactggttcaagggaaggtcaaccaatgattgataggccattccctccctatccgtctcttgatccctcattccactaatccgttgttactgattcattcaaggcatagactctccatttctttgtcttattagcgcaggtgttcgtcaacgatgaaagccgctgaacttcagactcgagtggagaaagagggctaggcccccggagggctttcagggactggggaagacgggtggattatagaactagggtaggggcaaatcgaaggttttgcccatcgggattgggcatggacgagcctcgactgggccagcattgatgaaaaaagaaaaacttcccccatcgcatcattaaccggtgtaggattcaagatcaggtccaggattcgagtcaaatcgaccttccctctcatctcagggtgaggcaaggaattgtttcaaatgttcgttgttgggacgggttcaaactggactgaagggaggaggataaaaagagtcctctcttcctggggattcatcactggctagggctttcgaatcaaagcatgggcatccgctattaagagggagcagtagatcgtcgattgaagagccaggtcagtcaacttctattgggacttctattgattattaattcgactctagggactcctagcagcaaactagtataaaaaaaggggccccatagagatgcaggagccgccagccggatcgaccaagaaatgataggccagagagatgggctcattcgactaatcagtgatccctgggcctacctaacacagatgtccctgaaataggggattggttgatcggaaagctcaggcaggagtaggacattccatacaaatctttctgatccgctagctggtggtcctctcaaatcccattttttcatcgacaggtagggtgaattctaaggttccttattccggttgtaaagcggaagaagagggagaatgggcacagccccactagcagcccgcgtttccgacccgaaaggaatggaaaatgaaagaagaatctgtgtgcactatctatggagtggagtgactatcctgaatctcctcttccctatctcccccttttttgccttcggctattaccggctggcaaggcttggcccaacattggatttgtttgaaaactaccaaggtggcattcattcaatcaaatcttttatgcctatgccagcccaaactaattgactttttttggaaaggaaggaatgcagggaagaagtctttcctttccactggttcttgaaagctatcaatccccgcttctccctctcgcatcggttctgcatcagatgatgagcccatgcgaaaactttctcttttattggcgcccgataggtaggctattagattgagtcgaaagcctaccaacgcataaaagttccgattcgagcgagagcccaaacgggtgaggcgagaagatcttgatcgaaagctccactgttctgaatagtgagaaagatttttggaaattcgatcaaatcgatcgagaatctcatcatctgttaggtgggccaaccgaccgaccgagttgggctgggcgtccatgtcacagaacctttctctagccaagaatcccattattgatcgaatcggggcggatccaattcattggcaaatgaaaaatctatcgttttaacactcagaaaaaaaacctagaaaagaggaagagtcactaagacaagagagctataggtaagcaagcaagaaggataggtgcaaaaaggcgaggcaaggggctctccatctctaggaagattgtgtccaggatctggtaatctaagccttgtttcttctggtcggctcgtattagcctgtgctttattacaggtagtcattcccccgttcctttagtcttttcaagggtacttttttcttaagtcgcggtcatgtcttgcccccccagtatagtgaccgcttccatgttttccccgaatttcatcagttccaggctcaagtgcctgttcatccatcttcattccaaacaaaggcgaacatctccattgagtgactgtaactgctatggtttacagtcaatagttcttaaccaaccctttcttttttgaattattaattaattaattcattacattattatattatgtctttctttctgaagggcttgcggtttattacaccaaaggctttcagtgaactattgaagctatcgagagagtaccaaatgctgacggtgacgaaggttaccgactttcggtggacgcggagccaacaagttcagtcgaacagcgtaacgagtctaaggttacagaagccttcgccaactttgatagttatagcattgcaagcaaatagagcagagagcttaccctttctttctattagagtcgcgagcttgttgtagtcggtcctaaggggagaaccttgctgcttacttgctatatccccgcgtccttgcacggctcggctcgttcttcgagccctgcttctcccttccccctctccccgttcctaccgtccaaaacaggtctatggagtatagccaagtggtaaggcatcggtttttggtaccggcatgcaaaggttcgaatccttttactccagattatgaacacccgatcggatctgtcaagaacgagctgacgactacaagggaagcagctgactgcagtccctgagcccgcaagccaaaagtttgacttgaacctacctttgctaagagaagagagagaagggaaagacagatggcagaaataaatccttccaaccgcggaattgaacacaagactgacttcggccaggttcttttatcaatctcctggtccttgcttaactccttgttccgtaaaccggtcgctggtagatctgatcggatcccggacacgcgagagcccagcccgggaggaatgcatggttccctggcgcttcatgggacggacgttcgcagtcctcctccatctaatctaaccctacctcgttcgcccaggcctgccggcacaataagagaatgagggagctaatctgcttgcttgtgcaggcgaggaccgctcggctagggcgcgccagaggagcttcgagtgacttttttctttgctcttcgacagccctaacaagtcacttgaagctctgccctttgctttgccccgtgctgtcttcctccagttgcccccacccaatagccaataggccgaaaaaggttgcagtcaattgcccttcccgttatcatcaaacaaaagactaccatacacgctgccggcaagctaccctcgcctacctcatctataggcatttctatccgcccgcgcgcgagatcagatcgactactctactaccatcattccgaaggtttttttattcaaaaggacggagaatgaatagcttattcataatcttataggccccgcaccgcttcattcaattgctctgtcataaagaaagggaaggaaatctttttttgatcaatcgcctgaacctgcctttctttctttgccaggaggggtggcccaatcactaatagatctctcaacgggagcctcattctgtctagaggaaatagcttcggtggatccggttgattaagtcgttgtgtctgtcgatacccacctgctcggagtgcgggtaagggctcacctgttgattgtgtcgttgcatgctttttggtagagcccccacctcccacggctacagccagcaccaggagcctagaaaggtataggcacccgttcattcagtcaatgaagctgcagtcggttctgatgattatgccgtttcaagtggatgttcagttggttcagcgatagatgtagtcgatggggtagagggtctgcagatactcgtctagctcctcattgccccaaccttccctgtaggctccctgctccgccagcgcgacaactgtccaaatcatttgacgcttcttctcactgagcagcccctcgacttccacttcaggttcggggagctccggcagggggacttgagtctcagcagaaccttcccttttcttctctctcctttccctcatctcccgggcctcaaccgaatttgctccattttgctcagttggggagcggaggtaccctcgagcggtgtatgggctgtgatatttgtggtagcgggggtagaactcggaaggctggccaaggttgtgtccttccgagcggacgaggtcggctcggtgaccgagggcttgcgtggaggcggcattgcgaccacgggcttggacgtcacttcaacatttctctgcttttttgaggcccgagtgaaggcatatatgtcgaacggattcacaataaacaaaggcgattgaaaaacataaaaaaaagaaagggggcttactcgtgacgatgtcgggcagggtgtcatagaaagatgtttggggtagtggctgtaagttcgaaggcttttgtgttattcgagtgaggatgtgaataagtagaaaaggaaataattaggctttgaacttaccttctctggatggaaggggtgaccggggtaagtgatgtgcgaaaagcgatatgctttacacgtccgcttccaggacgtcacgcccacgcgtctcctgactgtaatggttgggcttggctctgctcgccggttgtgctgcgtgagccttcagatgcctccaagcaagcgaaggttttcggggtaatcgccgcgcgtccttcccatgctccgtgacaacggcggtaccccgaaacaaaggggccagtcttcgtcgtgccggggtatcccgatccggatgccacgaaaatttagggaagcctttttcttaaaagactttctgcgaccggtgagaaagcggacgactttagggcttaaaggaacacctttctctttcatattgagtcctcagaggtgcggcccacttggtgtcggatcagctcgacaggtcactcaatagtctttcgcggagtatcccccgttttagtgaaccctgggagttgtcggcggctcgacgatctttattccaaaggtttaccgaggtgaagcttttgacaggtattcttttatttgtaggtttctctacttcaggctcttccgagggcctttgtttgaggtgaggttctatagtttgatggttacttatgttctcctctccccttccccggtagctaggaaagatttctaaatatatttccttccttccgttcaggggcactctaaaggctttgcaaccttcagagctggttgacagccgtctagtcagtccctctcgctctttgatagacatctttcggttctcggtctcatccgacgaacaacttgaggtctttattctgtgtcctatccttccttgcggattcccggtttctgaaggagtagcggcctgtgtctccggctctgggagaactttacctatagctaacctagagagctttactttaagatagctcgggcaggcactcttcttcggaaagaggagttgcttgccttaccacaccaaccaccttagcgctggaagttctagcaatgggcagctaggcaaaggaatattatatagcaatttcatattcattagataagagattgtggatctgttcttagtgaggacaaccggattgggacgatcaggtcggttgagggcagcagcacaccaataggtggattgccattcttgtactgtttgggtaaagggcaggagcgctctttccctctcaccagtacttactataaggggtggggcaaccggttaaaaccaaatatccaacagccgctttccttaatggctacccgctttcgagtgaactgaactcttggactggctgaaagggaaaggggaaactgtacaaggtctttttcactcgtttacgggaccagtgtcaaaggaaaggattgttgcactctcttgcttgaatgaatcgacatttgtggatgcttgttcattcgggattcttctatctatatttagaactactggatcaactactccggcttttagcctttggaacctgtggaaccctaaagtcactcgcccgttcaaactcttctgtccatcccatctaaaacccttgaatcagtgaatccggggacagagacctagcccctgctttatttaaacagctaagataaggtctaagaccgtttcttcttttccacatcctccttcctccttctttccggatacttaagcttctaatgctacggaacctgctttcccaatcaatcaattcaaattaatgtgtaggaacctgccctcatcgaactgaatgtctacccttcccgcatttgaagacagactaatgtttaagacctcctgctttcatggagatcctttcttctctgaccgccggagattacccatatatggatgaataaccgtgaagttcgacaatcttttgagggaggggagtcgactgactgacaaggaactgacagaaggggaaaagaggagtgaaaccattcgacggagttggaaaggacttcgctaatcataataaggttggtctcaccttcgtccggggactcgaacgaggagatcgctgatgccgaccaccctctgtgtctttgtcagtgaagtaaatcaccccgaggctaagcgatccgcagtgttcaatggttgcctaagcacccgactttaatagtaggagaaaggaaagcgctcgatccatggaatccgtcatcggatctccccattgacagatagagtagaagaatcaattagcccgggatttaagatttagatcttcaactacttccgagagggtctcatgctacgatacgagtagaatacataggggtatagttcgggtaaagcaaatcagattttgacgtataccttttattggaaacctacaaagtcgcaatcctggcagacctttttgagattccttcttgcatcccagtctaactcccctttctgtctgtcactggatctacactacttgacttgcgacttgagctagcagactgagctttagcttgagcgagaacgaaggcagacatctcttttttggacttttctgcttgagctggagctttggactcgacgaggtattttgtgcttgccctattgagagtctcttccattctctcttcaccagacagatagacaaataggcaatccgatagatagattatggcttcctcactatcagcaagctcccacaggcgatgaactgcttccgacttcttcattcggtttgtagccataccgtatagagtgaaaaattccttttaatgggagtagctatattcaagcaagcattccagcgaaacgatcctttgacaatgggctctgcccaacactgggactgactttatacagagagaggaaaatcagcaaaaaaagctctttttgaatcgaatattggataggctaagctaggtgtagcccgctctctctacggttttgcttgaacttgtcaagcccgggtgcctatgcgattattaaggcagggtgctattgtaccagtggtggagtggcttgaatcaaatcgtttgtctagagagggtgtagcgataaccaaagtggactctactagaaagtcaagatgctgtataggcaactggccttagagtagtgtatcgaactaaaggacaggagcgacccataatcattgacgaagaggaaggcttggaaagggatcaaacatattgaggaggagctttcacaaaggccaatagccgatagctgatgtcactagccttaacttctttatctacttgaaagctgatgggagtacggctttcttcaaggaagtgtcccatatgatattatattagtaaagagcccttgatcctagataagtaagcagatatgcctatggctggaaagatagcgagcgctattctcaacttagtctctcagaggccagctcgttgtaaccctaaaacacggcgttagcggggttgggctccccctgcagaaatacaacaaacatgggacagccgggaacgatgacccttctcaagcctgaggcctaagttggactttctctttctgcaacttgccactccgaagtttaggatttcgtttcgaaccgatgggatttttcgaatggtaatgaagcttgccattctgtttatttggccgaatccgactctgggcctgcccttttgctagctttttcattatgctggttcaactactgcttatgcttgaaatatctaaacacctgaaatccactctcaatagatgctgccccttaaacagtgtgaaagggtggtaggtagaactaagggaataatcttctttggttcggtaatggaatcaatagctttcccgaacagggatataggaagaagccaatagcctacaggcttgccagcggacttgcttgacctattgaaatgccagtatagacttctggcacatggtcggctagctaaaggtcagcttcggttctaggcaaagatccgccagtagcagttcctatcccagttcccattcaacattcattcaaagtattctccccttgccatgcttcaaccagctgctttgcggactgctcttgctcttactgctactgctctttcctatgcttcctgcttctgactactatttaaaatagtttagaaagctattcctacaaggaaaggcctcctttctttcatctaaaagctggctggtctcttttcatattcaaaaaaggaagccccattccattctatcataagataagggggaatgaatctcttcaaagaaaagaaggaaactatcctgacatcctaagagctaccccagtctggagcacagctaaggctatacttccgattctgaaggtaatcccattttttctttcttttccggaaccccccgaaaacctaagtgagagcgaaaactacataccctaagatctcgtcccttactcttctttagaggaagcgaccttacctatattccaaaaagaggataggagcgaaactgcctcttcaagtccactccttttcctatgcttcacacagggctcgaagaatcatcttatagcctagaggttaagcttaaggttaaggttaaggttaaggaccttccagtcttcctcgagttcgtgccttctatcccgccaagctatagctatagctagtgtcagtgagttcaacctcccactcgtgtggatttgctttctgttctaatcccctactagacctccttgcaaaagaaaagagaaggcttacttcttagcttctctaagattctttatttacctttgattcaatcctttcgcttctctcacattcccatcccatggtagtcttttgccctcttctagtcattctcttttcctccctcagaaggtgaaggagaaggagaagggacctagaaaagcctcaaagaggtatgccgagtcctctatcttaaaacttcctctaatgtcccatcccgtcgatgttgatttcacacaggatgatcgattggataccttgataccgctctttcgccttgattgatcctattactcgacacatctactcttatgatatgaaattttaccacattgaccgctttctgaagcgaatcacatttgcggatggaatgtcctaaacctccacctactcctgtggaaaggcttccccttcggcttggggataaagcaaaagggagaatttactttctgcagctaccagcacacgatcccacttttggcctgggctacaagccaaaagtcaaatactaaatcagtagaaaaggagagtcagaagagcgctggaacagggttgactcctaaaaagccgcacgagtacatgcctacgccaccgcccaactatgtctcctttccgatccacatgccgctacgagacccctgtaaaccacccttagccaagaaagacaagtccgtcccgtccatagaaagtccacacccaaatgtctctatccctagtcccacagtactctcgactgctgaacaggcattattatcctgatctttcttgtctgttcttgagtgaggacggtcagcttgatgcagaccccgagtctgagtctagttcgtcaagcacggcggaggaggtacggagagaaggagacgtcgagatggattaagtaggggtgactctgaaccactcgcgctcgaaggaagaaaatggagacaggaatcactagccttagctagaagcccgaaaggcactctagtcttcgttgactctgagaccttcgatctagtggaattagtggacgactctgaatgcggagtaagaaagtacgggtttctttgatcgacaacttgctagtcgacagaaggattttcaaactcgatagcctactggtttaactagtttctggaactctgatagcactatccttcgccttccaaagtctttagtagggcactcaagacttcaatcgcgaattctcagttggaatcttctttggaagagaggtagtataccgggctagcaggactgaatgcttagtaagctacccggatagagggatgtggtaaggaagcgtagcagttcaatttcaaaggttaggtaagtgctagctcgatcatcataagatccaccagcaactctcttatctacccaattggaaaatctttatgttaagattatatagtgaagtagatcgctcgctctttccttctactttggacttacattcagcttgccttccgtggagctaacagaccgtgccactattatacctccctccccttactcgtccattcactatgtcagttgctttagctgctccttctgtaataggctgctgcttgatctatatcattaactgcagaatccccatgagtgtacttacagctagcaaaagactacttcttggactgtggccgacaccagagaagactatttcgagatttgctaagcgaacgagggactgtcttgactcactggatcgcaagcacctattcgttcagctgaatcgacatagcaagcatgggcgagaaacttatttctttattaaaccactggacaagaggacaatatgtgtaaagcatatacttggctgtccccgcttcttccccccctttctattagaccggtacgccaaggaacaagtccataggtcatgtcaaacttaacacttgatgtcttcaagtccatgtgataggacccaacccggacatggtcgtacgtcctctaccttcggtgcacataggggaaaacgtggaatactgttataaggacaccttatcttttccaagaccttaccatctctttccttgtctctctgtgctctctttgtactttagggtataggagagagaaggagtgcatacgagggggttgaaagggcaacgaatgaatataggcaggctgatgctgcccaagcagacgctttatctgatacaactcagacctccgggtttggttaagtaatctgtctattcatcagtcagttcggacaagatctctatctcttgaggacaatcagatgctttcgaagaatcggaccaaagaggatatccattggaaaatcaggcagatcgcaggagagctccgttacacggaaagtccttttttactgatggagatcctctagcgggatcagaccttccacaagatagcatcccgtaacaagagaccttctctcaagaatattggttgcggagaagagagtgtgtcaagccgtaaaggggcagagtaccagccacgtggcatcttgacaaggaaatcgaatgcttaacgcgagcaattccaagatcggattctgctacggaatcggataatgtttgtgataccacatccgctgtctcctaatcttcttctgacagagagtctgccgttggaaaatcaactgcctcggttcggttatcttatataagatagcgcattgatgttcgcggatggtgttcgtagacagcaggagtttagtcagagttatcgcaaataagataagagtttggtaggtagaatgcctccctcttgagaggatgcatttttagaacccgcctcttttactcaagtcgaattccccctcatccatgttgtagtatcccttgcccaaagcatcaggcaagacagacacgatagaatatccgatgttgttcgtagggaatccgagagggtccttctattcttcccatagaagtcagacgatcctaagcttacgtacttagttccggaaaccgatctccagaaagtcatcgaggctagtaaacaagacatccaagcgtcccaaggcgaatgcaaagaattggccctaaggaaagaatggcatacctacctcatttcttcaaagggggggtacgaggaatggaatgagggacaaaaaggagtgaaaagctatcagcgcttaccacgattctctcaaaaaaaggaaggagatgaatctgcctaagtaaggagcccctccggggcttagtgtgagtcacttcactcgggaaagaacaaagaaggggcaatcaattgtttaagctgtcaagaatttctttaaattagtaatttgactgcggaaaagcctactaaggtccgctcgaggttatcttcttcctgattcaatcaatagcagctccttcctttcttgctaacagggcaagggcattcgatgcatctgattcaattcctgatccgccctctctttcacagcctaggagtacacatcgatgagcttaagtaagcctttttgactaaaaaactttgttgatgcaaggaactctttctattccacgagcagaacaccagagatgcacagcacgtgggccttgtctaacgaacgacgactttcgattcttaatcgacataggtttctctttttgtgtaattgaattggatgggcttgcaacccttaggcctgcctctgtcactgcaagaagctcgaagggatgaaattgctcctttaatcaacaataagagggaagcgcttgagcgaaaggagaaggcagaaaaaaagatgcacaaaggaaaaagggctaaaaaagaaggacgaagtaatttcgtatataaagatatggctttccgggtttagatcgaaatggaatccccgaaaaccagggctggagtcttagacttcttctgcttcgatagagggactgacagcctaagtggaataagaatcattcggccgattgctctgactcttatccttccttcgctgacagagaagagagagagcactccccaagccaaggatgagtgccaaagagaagatgggcaagcaatgcccactcccatgctttccgttggtcaacaaccaaccaaagtgctctatacttcttcactactcgtacaggcttgacggagttaagctgtattgagggaatcgttttgtctcaatcaatcaatatgtttccgaaaattccacgtatctttttctttgatgaagagagtctaaattccagtgctacatcctctcaaactccgagtcaatccacgacaactattagcgattttagtcttcaatcgtccgatactcaaggttcttctaatggtatttttgaggatcatccaggtcttaacccttccagtgaacgtatagtagagcttcaatgttgtatacgcgaaagattcgaagagttgctgcctaacaacaatgccgaagcccaagcccaagaggctctggtagcggccgaagttttacatggcgaaagcaacgatatcgccgagctggaacaccttttgacagatttgaatcttcacggagtactaagtgaagcctttctagaggcgatgcatctagtgaaggagctcaccagcccccccaacccacctaccgtccccagcccacttgaacaatttgaaataatcccattgattcctatgaaaataggaaacttatatttctcattcacaaatccatctttgtttatgctactaactctcagtttggtcctacttttggtttattttgttactaaaaagggaggaggaaactcagtaccaaatgcttggcaatccttggtagagcttatttatgatttcgtgctgaacccggtaaacgaacaaataggtggtctttccggaaatgttaaacaaaagttttcccctcgcatctcggtcacttttactttttcgttattttgtaatccccagggtatgataccttatagcttcacagttacaagtcattttctcattactttgggtctctcattttcgatttttattggcattactatagtgggatttcaaaaaaatgggcttcattttttaagcttcttattacctgcaggagtcccactgccattagcaccctttttagtactccttgagctaatcccttattgttttcgagcattaagctcaggaatacgtttatttgctaatatgatggccggtcatagttcagtaaagattttaagtgggttcgcttggactatgctatgtatgaatgatcttttatatttcataggggatcttggtcctttatttatagttcttgcattaaccggtctggaattaggtgtagctatatcacaagctcatgtttctacgatcttaatctgtatttacttgaatgatgctataaatcttcatcaaagtgcttatttttttataattgaacaaaagcgagtctgaatgggtatacttagtcgtggagcattccgagtatttgctttagggatcgttcctgcgcatctccttactttatagcagttattgctccggttccagaaggtatagctcttggctcagctttttcttagaaattggagactgttccaatttcctactgagataggcaagcggagggagaactagacgtatcttgctaggcaaagacaggttagaatggatagctcgcgggtgggattgacgggatagatcactattgcagaaggaggtagaaccgggggaagaattatggctataaaggtcctcgccctcttaggcacatggttctaaagattcaatctcaaagcggtactaaagattaggcagaagcagaactagaactagaattcttcgcccctccccttgtaccaagaagcaagttcagaacataaggataatgggctcgtctattagaagttattagtttacggagctatctcagatatctcgagtaaggagacggggcgggtttgatagttagagttctatttctaggaaggaagagactatcgggaagctcactctcggccgggctcgaagcagaaggtagaacgtaatatctcttgttggttcagctcatcaagctattacaaaagagtccagcggagacaaagaaagaagccatttttacggtattttcgcttccagtccgtaattagatcttcaagcttagtccagtccggatccatcctaaaccaaagagcggggctaagcgaggggcatagcgatacagtgttcatactcgagttgctcaaatccagtaggaatatcaggaatagtaggatctagtaggagcttgccttggaatgcagtgagggagcccggagctattgaattctttcataacccaaggagaagaataggactctttaccagtatcataacctctcgatgggaaatggaacttagatcacgatgtgaacctacttatgagtggaatttcgttgacaagcaaattccccgggaaaacgaacttttctccaattgagatgctttcttcatttatggattctatgcgagattcggttagtgtgaagtgtgatcctggctcagaaggaagagctatatgcttaacacatagagttcgatgtaggtaaggatgtgctccaaagttttcaattccaccttatcaacctgaaaagagctaatacgggcttagcctgccttttatcttatccttctattctaggcgaggaggtttatttttaaatagtaaatagccccataaaaaacaacaaactagtcaaaggacagcctgccttattcttctcccgttcgggacccctattttctcggagatagcctggtctgagctagaacagcagattcgtgagcaagagcgtatttcacagctgattcaacaacagccattttttctggggaactttcatatgagtctgttctttcttttaatccactataaaggttcttaattttctctttaatatgaaggagaattacattcttgaaaggatcaagggctctaccctctcgcataaagtcttacgctcttatcgtcaaccttcgtggctttttgctcctttggtctcgctatttcattcctggttctctctttcaagcttctttccatcctggggatttcttctcattccgtccgttctgctagctggtgtcgccttctctcttacttatctattcccatccatctttacctctcctactccactacttccctccttcaaagcgtgattaatgcgccttaaacctctctcttgaaaaagagcattttttagtggagccttagcacgtgaacccataggaacagggcccttcttctttgcaaaaaagcttctgaattatcatcacatcagtaggcgcagaaagcaaatcttggtattgacttattgaaaatctctttgagattgcttagacaaatctttttgtgtgaggccgctgttccccacctttcttaccttgttttttgggcttaaaattctgtgactcataagccctccatatctaaagatagatggctaaagggcgggttccgcagttaactaagaaggcgatcgattggcttggagaggaaacgaaacccgggactgaaaacaaaaaggataggaatgaattgaataaagaaagaatatatagaaccttgagcattttctcttctcggcaatggttgagagtaaaaaaggggtatccgcatagaaggattgctggtataccgggtagatgtttatcttttcgacttcagcgaaaatgtaaaaagcacaaatttcgtaaattttctttctgtcgaaagggaagaggacagggtcttacttacttaaaagtaaaaaaaaaaaatggaagtttcctgtcttagtttcacttccttgaactggctactaccgcgcaacgtgcccttgcttggtgggtcgttaattaatcagttttaaaaagagggatggatttcgaccttgctttgagtcgtcaggctagtaaagcgctacttctaaaacgatcgttaaggtcattcactcgattccctcggtggctctgctaccgatggatcaagatatgctgcctgcctatcatgccaaaggcgctgctggtggatatgccaaagatgtcctggctctgaaccgggtacttgaaatgctaaaggtacttcttatggtcctgcttcaaccacccttccttctctacctttttcttcaaaaacttaagctacttagactgatgctggcgatctcgaagggagatatctggacctggagctactcatcttgatctttattatattaggatgcgaggaaagggaaagaaggtgataagcaagaagaggaaagaagaatgttaaagaagtccctataagtacttcacttagcctttctatagtctgtctttcttcccctcttccctcaaagcgcgctctttcatccatgcgcatggttcttactttcatttcccccctcctcacgtaggagcgcatcttgttttcaaagatgagttgtagatgagtcggttcgatcaccccacatatcgacggttttttaatgccttatcctaagcccatctagttgatcgagggatagacgagtataaagaagggatggagaatcttttatttgatcttgatttgatgtatatgttacgatgccttcgtattcaggaggattgggggtacggcagataagaagagcgacccaaaaacggaaagaagagtatgaggggcagcggctcaccgataataagaagaactcacattctcgtcctgacagatgaccaacctgttaaggcatctttctcaatgaccatcctctcccattccagttcttttctctttttttagggacaagttcattttcattccctcgatatggccaggtgtgaagcaacttcacgatccaatgaattccctaaaatcggatgacacaaggcgaactagaataggctgatttatccacaagaatgtcataaaggttttctccggtcttcctcaaaaagacagctttagagcgcaagtcaaactcatgataggcgagaaatcacgcgcacatggtttagcggtttgctgtgctctgtgatcttattcttctccaagacccgatgcttcatctgcttctttagtttagtaggacttctttcacgctattgcgtgaaacatttgtttggtctcccactgctactgctatctatgctaacttgaaaggtatggctactctcttgtttcctgctgaacctccttcccaatacaggcttcgcagccatccctgcttgcattttttaaaaaagtttggtaggggctgccaagcttgactaatagaataggggtccccttaaaaggagaatgcctgccctgtgccaccttggtagcacaaacaaaggtcctgtgtaccagggatgtacgaatcatagtaataaactttacaaactttattagttgcaaggcgactttgctgtaaagtttattatactcttaaagtatattctaaagtaaaagtcttcttagtattcaaatttttgactatgaatattcctacccttgcagtgctaatatattcattagtctgagtcttagtctactaaaagcataggaaaggaagagtcaactcttatgttgcaaggttccaccccaaccaagtaataagcactaaactgaactctataaggatagacggggtgatttctcactacaaagaaaaaggctgaggatttgaaatagatagaaaggagtccaatctaagcaagcgtagtggaggaaaaaaatcctaaaagtaagcaagtagttgaattagtccctgctagtattggttggtcttactttattatacaaaggattgtggcaagcaacagaaagtcaagtgagtgttatggtgcagcggaaggccccctcgaatcttccttgagttgacgtcactgggacatctaccgcttggatcctgccttgttagtcatccgtagagctaaagggaattttttgaagccattcccattcccacacaccaataccaaccagggtggctgttcagtaagtcctacccctaatagaaaggataaattgcttgcgcgcttcgtcaagtaagagagaggatcttaggccgaacagatcaccggctccgaaggcctgcaatcgtgactttagttccggtggttcgctttgctgccggggtgcaacagccttttgtgacacttcgaatggagtggtccgtacgcccctccccctcgccaagcctgaagaaaggagcaacttagatacctctttgttaactagattcctggtttgctaaaagggtccttgggcccaatcaatctctatactcttgatgcaatggactccccaaagccactaaaccgctctcttccacccgatttgaacagaacctcgttctagtgagattttatcccttttttaaacggaaactcagttgcctatctgatccttggtctaattgggcctttctctatagctcgaatcgaatagctgggctaccccttcccttggcttggttggttatataagagaatcccaggagaaagcaagttagaccttacttagggcgaaagattttttggatggttcattccagtctgaagtcagtcaagtcatggaattggcagaagttcccccttaaccaaccctaagagggaattcttctattcattaagatgaagccattcagtcagctctgaatctgaactcaatgattgcttttcaagaagggcatgaagctttggctcagtacagtagcatttgactttgggaaagagaatcgatagaatcgatcgcttaccttgctttggcatgccagaagcatttcgctgtggttctcattgattgagtcgatcccgagacaaagcaaagggagttccgtgggttcagtttgcttagaggcagaaagcctagaagaggcctagaagtcataaggaataggcaatgtaccggcaactctaaggtttggctttttcttttattgacttttttgagtcaatgtcgcatttcgcgtgcttggttagatctcctaacctaatgtaatgaaggagaaggcagaaaaaaaagatgcctttatccctagagatgcaggagcttgccttaggacagaaatgatatccgaatggcgtacggagctgcttaccctaagacttcaactccatcttacatcgaagtcagttcggctggatcgagagaatctggataggcatgatcgaaagagggggcaactctgtctccgcctctgctcgtgcactcgttaaagtcatggcctagcctagttggtgaaggagcctacaagtggtaaccgctctgtatccgtcatctctttgaagaagcagttgggctacaagcggcgctttcaaaatcccgtgactctcagtcatctatcttcttttcacctgaaaattttggattgggggaagcagagaatcaaaaaaaaaaaaagaaagtcatgcttactataagaaggaagcgggcggagacccgtgcgtgcagcaggtgtagagtcagtcgaactagtcctgcgaatatgcgaaaatgttctttatgaatggagaccagacacaattgctttagcggggactgaaatcgtgactatgtgttcatgctttcgaaaagaaaacaaccatctacacggggcgctatttgtctacttattgcattagtcacgtctattttgaagtcttatttaactcgttcgatgtgaagcccttccacacctgtatgaagcatctcctctcgggattcaccggacttcgtagcttgaaacaacctgtccttttccctatgctgaggcagcaccaacaaatcaatccatcgaagttcctattgacatacataaaaatatagggatgcccttgatgattcggatcatctcaatcaattgattgggaagagattacttatgagcaaaaggggaggacgaagtcgcaggagattaggtattatttaaactgtcaaaataagggatatcgttgactggtacaagaatagaattccttgcttacactttctttctactggttggcttaccctgtatttcaagagtaaataccgcagtgaggaatagcggttcctctctttgtttggtctaataaaaagattattcatcaccgcaaccactctcgcttagctaccacttgtctttgcttgcttacttctaaagcaaaccagactgaagacagtagagaaagactttttattacgttatccagaatgcgatgccccaaggcaagaaagtagcaatcggctttcaatcctatgattttactcgaatagctaatatcagagtagcagatatggttttagcggaagctgctttccccggatgcggaattgaaagaaccatgccttttttcttataaaagcctcctcatcaactctctatctttcgaacccacctcaccgagcttaacgccctgtggacttttttacgaaggcctaacttgacaggcccggacggccgattcataagggtctgagccttggtcggctgccctactaggtaaggcaagcgctcaccgatttctttacgtcttttcgatcgtgctttccgtgaattgaaaggggggaattaattatccagcagagatggcatccattagcttattgtcggctctcactctggctcatcatccagaggcgggttgagccccttgcacagctttttagcagatgattccaggcaagacaagatcagggtcaatgaagtgtttaaggacaatcaatggcactgggattgtctgcacactcaacctccagactttgtgaagaacatcatctcctctatgcagcttacactcagtccagatgaagatgatttggcaattttgtctccaactgcatcaggtaaattctctcttgcttcagcctggaatatgcttaaacataaaaaaggggtgtcctttttagattcaaagatatggcataaggatgtgccttttaaaatggcatttcttacctggagagcagtccatgataaactcccaactgatgggagagtgtccaggtttggtcattctctttcccctaaatgttattgctgtgttgactctactgtgaactcaagcttagaatctgttgagcatctcttttgctctggtgtttttgctcaactggtttgggaacatcaattgttgaatgctacttcttaattggtggaaccacaaggtccttaatcctgtggcttcatatattactaaggtcatgcctcctttggtttgctgggagctgtggaggtccagatgcagcaataaatatggttctgagaaaccatcactcaatagatccaaggcattgatcacatactccttatctcacctgctgcattctcagtttggcaaggttagagtaggtgagagctgggagagtatctgtcatctgtgtgatgcttcaatgacttagaaatctgtggctttggttaggtggatcaagccaccactgctttttgtcaagcttaatagtgatggtagctgtagagatggtatttgtggaggtggtggtgttgtcagagatagtatgggtgctcttattatggcttactccattcccttgggtgctggaaccagcaactgggcagaagcaaaggccatgctttttggccttaaatggtgcattgaaagaaggtacaggttggtgataggggagactgattccttattgctgtcaagctgcatttcaggagaagtgaagtgatccccacccgggaatcacgaacgggaatctaaatagaaaaagaaggccctggcaaagcctctcctaggcacctaagggcggataatagcagcggatatatcgctttctgtttccgctctatctgccaaggggaaatcccggtaaagggaaccccgaccccgagaagaccgtactcatgtgcaactaattcaataggaccggttatgaacccaagagaagagcggataggagtactcatactcaaggacaggaagctctcacagcgtgaaggcaaagaataactcctattggaagaagagcgtttacgatcagagctggaagagtgggagggaatgaaatagcaatagccgctacttctgtctgcggctatcttctcctattgattaagcccttcaaaggaatttcttctatttcttctttctaaaggcaaggctaagccatccgcccttcattgctgggtaaaaggggagacggttcccaaggggtggctagttcgagtaagagagacggatacagataaggtccttttttctgagagacccgctcttgacttttatcatacccactagtaagcgcagtggatgctccttcatacagggacagagaggcgagtgatgggcactactcatcataagaaagcagtcatgcagatagaaagagtaaaacaatgactctgactaagtaaagagatgaggttttttttctcatctattttccataccacagctctagacatgcgccccgattcaaactatgtttcaatcataccacccttgtggggtgttcgcaattcacattaaagaccctttccaaaggttgagtaccttggctcgggtaggtggtgctgggttccgtgtccttggcaggctcgaccatcggagatccgttcattacgaacgttttttctcgatgtggaccaagctccgacttcctttttagctttggctcggaagaggccggcctttgagcccgtattggaaggggatcttggtttctttttttagaaaagaaaccccaagagttacgtcttattcccgaggagatgtttgatctccctagtctagggacttcttgtaagggccccttatttatggaatgggtaatgtgttaaaggatagcttaggtactgcagtaggtttggaattagactaccttaatatcagacatcaaagacaacacagaatccaagtccaagacttgagtgataatgctagagaacgtatccttcttggcaaggcaaacaacctttgccaaggttccgaaggaaagatagatctgaactaacacaatcactataatcatccctcttgtatgtatataagtttttcgatgaaaagaggggattatcctacgataccctaggagcgtgtcagaaagatgggtacgcgaagtgagtaatggtgaaattctccgccacaagccctctgaagcgaggatgcacactgctttaaatagaaagcgcaatgcaacatccccgaacgtcgggccgtcctcattaccgtaagagcaaacaggtaagctccaatacagaactccttagtaagaccgtcagcggctatcaagatcgctttgttaagcagtgaccttaagaaccgagagtcttctaaaactctctgccacaaactaaagaattgaattaccttgcgccggtatcatttcgcttgagccgggaactcctgtttaccttgcgacaggtattccttcttatagataccaccgaaaaagcggaagactaagaagacttttctttgtctcgtccacacccaggaaagaaaagatcagatcagcaacggctttcgagtagaggatttttttgcttttaattattccctcggagttgagttagagttagcagatgggatctaattcattagaggaagggatggtgattaactgatagaacctcttctcttctttcaaatcgcatctctcaagtgagaagaaaaggccccccacggagcggtgggaaagcaagggcgtagcaggaagaagaagtatgaaagcagcaaatctttcctcctcgggctgggatcacgaacgggaatctaaatagaaaagaaggcccaggtcgagagttcgctccctctctctcagctaaggaaagagatagagaattcatgtacatcgctatttcctgcggatctatcgtatccttacttctctctgattgtgatttcccttgtgccgtactataccgctaaggaaaacaaacaagaaccaggctaggctactcctcttcccctttctgaatcaacttgtccttgcgcttaccacttcttaaaacttgcgagcgagtgtcgatcgctcctttgcctgggcaagatctgacgactcctgcccaaggcgggttacgaattcagattagctactgccaaagaggccaggaacgagcttccgctttatctaaagaaaaaacctcttcctttctctcttcctgatcagcggattcagagtgatcaggtgaagccccccttctcgttggatgaccggccctttcttagacttggtgaactcctgtcgcgatgaattaaactccgttccatgccccgctgcttgtcaatcacatcggaaagtcgttgggtcggcggagacctctttcggcaaagaattatatcacaaagaaagccccaactagggactaccacttataggagtcttctttgctagtagaatgccccccacgagaagaaagaatagtgggatgctcacgctctcgttggacgtgacagtcagttacagtgggtaaactaacgaagggaagaattttatttcatcacagaattgaatcgggtctcatcccttcgattcctcgctgcatacttcaatgagaaaggaaaagagctttgttgcgtgcttcttcgggtgtggttgcaagatctcgctttcagttcgaaaatgtgtacgtagcttccttgtacaatagctctctctctctgagagagtgatcgggaagcattctctcttcccctccgtatctgaccctgacccacgctctagccctctttcgtcgtccaagtcgcatacctcctaaacagtctatttggtttttaaacgcgatctatttaactgattaactgtgaactaggtgggacttgattctttttttgctgaaaagagaaggtacgtaggcagctctcctaaaaaagagtgaagttccgcccgcgtttgaaggctagctcctgcttcggagcttcatccccacatctcacatattggaaaaggcaaacaaaaaaggggaactcagtcaatagacaaagaaaaaaacggatatgttacacaaaaacaatccaatctttgtctttctaaggattgatttttcttgtcgtagttcatattcatattcaagttggaaaaattcttctttttcttcttattgtggaaacggagggaaggcaaaggtccgtaggaggacaactatcaatattagctgacaggtgacgaggatcatatagtttgagagctggatcgagtttgaaagcgtggttatggcggaatggaatgtgccctatcccgcgaaggagaggaacgaagtaactcgacaaaaagtagaggaacctgtcatgtgaggaacttaggtcaaaactacgctctttcagccggtttagtatagtagtagtttcaaatcaatgcaagccaatggaaacccccccttcacccccaaaacctatactcattcgtcttttacttgtgcgtttacaacatccattgcttctgactatgtcgatgaaatgggaccgcgaagacaacccaccactagagcttgctttgctctcgctccgctcgctcccacctgtcttctttcccactatagtgaaagatctttcacttcaccatagcaggaacctcgctaaccttctcggccagttactctaatctaaccacagggatcccctatgagaactctgtcaagccctcgctaagaggtagaattggctaaaagcatcgtacttcttcccatagctaaggatgtatcattatcagaatcttggtcttccgtctacggcttgtagaagtagttttaggatgaggttagacctcgagcttgctgacataactacttccctaaatctagctcttgagggaacgagcgaaatgaaatgaagcgagtgataaccaaaaggaacgagcggaattctgtagcgatagggacatgtagctaagggagcgcggggtgctggttctaatcccttcttccgactgttatagatgctaaatgctaaagaagaggagttctaaatttatatggcatcctttgtgacagacgattcccactctttcttatactattatatctggccatctatctctacttctcttatatactcgcctttcggtaactcgttatactagttagacttacttcaaacgaacggaataaatgagttgaacgaatagctcttcgagctattcgttcaactcatttcgtttattccactcgcttcatcggatagtgttctaattccaaggctagtgtggcctgccttacctgaatctatctcttcgggtcgttgcaatctttctgttgaaaagtatccttcttcgggtattattgatattggcatagaacagagcttcaggtcgaactagtgggttgggtggcaaggagactattagggaaaacatacattcgttggataggtagctggatttaatctaattgctgattccgacggaagccataggagttgtattcgagtaagagcgcgggaacccgaagagaaatacggatgagtgcaaaaagggcaaacgaagggtacgagtgaaatgaaattcaatgcccgtagcgagtcaaaaagcaggggccgaagacttggttcttagccgtgaaaaaataggcgaataagcatcctttgcggcgcttgcccttaggaaagtctattcagttcgattccgcgatgaggccatgcatataaaaacaaagcaagagaagctacagaaagcgaattctttaataatattttagaccggcgtaacaagaacaagctgaagaatagaatttagatctttcctccgcttcggattcattcattagaaagagttccctacgccgcctagtcgctataggagacacgtgtacaccgccgcgtctgaaatcaaagaacggaataccttctgcggctatcatggctagggtaataattcgtatatggaaacgccgcttcctctttatcctttattcgatttaaggatagaagaaggatagggaatacggccttgaaggcgatgaaaaaagatgataatataggaacgcggcaaactctttcaagaaattagcatcctcagctacagtggtaaaatctctataggcaagtagcccatgattttccaattatagctcgggccgaatgccctatagctttggagtttccacccttctctgaaggtggtgatttggctgtagaagcctaggctaatgaattggggaggtacgcaagcgagggaaaaagctttgatgaagcaaagtgtaaagctgaggcatatttttaaaacttgcaattccgactcttctctcaaagggtcttggtctcggtccggtcttttcttccttggtctgacgcttgcgtcttcctttcagcgaagaacatccatccttggggaggtcacctctaaaggcctataggtccgtctatcgataggcagtctttcttttctttctcttacgggtcggcaaagtctgattctattggaaaaaagggccggtctcttcggcgagggcttgacgccatctgaagcgtcagacgatgcttggcattcctgaaatctatctctttgggtgatgatgctaaaagcacaggtctatacttcggcacagacctcttttgagatttaatgtaggaaagtaaagtgctagtatttcttagagcttggctttctccacaaccagtcttctattggggcaccatatagaggttctagaggaaagaagggagctaaaggagtacgaagtccgatcagcgtcttcaagagcatgattctataggaaagcatttaagagggcaaaaggtctgatgaagttgtgcaactgacctctatcctttgagaacgatgtcaaggccttgaaaggccctttatggctaatgctgcatccgaagctaggaaaagggcgcccttgactacgtcttttctttatttctcattgccatcttccgcgtctgaaataagacaataatccttggaaaggtcacaagtccccaagggaaggaagtcgtgggatattcaagaaaagcatcctaagcgaattcattgtctagggaagtttctctttgggggctgcctatcggtactcccatgaactgaacacatacctattcgatctaatggtgcgaggtcaaaagtcgataaaggcaggggtaggagaaggagagagaggtgcgctttaccctttgagatatccaagaagtttcgactttcaagagattgaaagattttagtcttatttcataggctgcaacaagggattattaaaagaatgccgtgctttcatctattagagaagtatgcccctagggaagggagaactgatcttttcaaacgaaagccttagagttggaagggactatcctaaacttttattaataatcttcttttggcccttgattggacttagagttggggatagaagacccgccgctttaccttgaaattggaatcggaaagggcgtaatcgaagaaatttcaatcacaagaaagaaagactttcggaacaaaagacaaagcttcaattaaacactccttttagctacaggaactcctattacatttgaattcaaaatatcttctataagggtatgactttttctcaaggatgggaagccctcacttgacataatatcttagtgggaaggtaaaagacttagctgaacgttagcgaagcgctggtacaatgagattcttcatagaaaagaaagaaggaatgcaccgagagcccttcctcttccacggattccattagagccattttgaatggtatggccttagaccaatgcgctttcaggtcgggtaaatctagccgtaacagtcagttcaataggacttagaaaaaaaagcgaaaacgaaagccttcattcagctccggcataagaaggagcgagaagccactccgactaaaaggaaaggatcacttagggagcgggtaaagcaaagagtggaaagggcaagcttcacaaatcatgctttcaaacttgccgaagttcttctaaaaaaataatttatagtaaaccaagggaatcgtatcatccatggcgagtgctatcgtatactttcgaatgcttgctcagagtcttcgttctaggttagggttactttcactcgctttcgagaacctaatctctttcatggtgaaaattgcccgagtgcatcaaacaactcttggaggagaacaaagacatcatgccggacgagttgcccatgcgtctaccactgaggcgggagatagaccatcaaattgagttggaacctggtacgaaaccacccgcctttgcaccatataggatggcacccccggaatttgaagagttgaggaagcaactcaaagagttacttgagtccgggcagattcgaccatccaaagcaccttttggcgccccagtactcttccaaacaaaagaagcatgatggatcattacgactgtgcatcgactatcgcgcactaaaaaagataactgtgaagaaaaaatatcctattcccttgatcgccgacttgttcgatagattggggaaagccaagttcttcacgaaggtagatttgcgcaaaggatattatattaccaagtgcgcatagccgaaggagatgagcccaagaccacgtgcctaacaaggtatggagcgttcgagtggctcgtgatgccgttcgggttaactaacgcaccagccacgttttgcactcttatgaataagattttccagccataccttgatgagttcgtggtggtatacttggatgacatagtcatttttagtaaaaccctggaggagcacgtggagcatctacgtaaagtcttccaactactaagggagaatgaactttacatcaagaaagagaagtgctcgttcgctaaggaggaggtacacttcttggggcatgtcataagccaaatcaagatggacgaggccaaggtgtctgccataagggagtgggaggtgcctacttccgtgaccgagttgcggtcatttctggggctcgtgaactactatcgtcgatttagaaaggggtattccgccattgctgcacccctaaccgacttgttgaagaagaaccgtccttgggagtggacggagagcagccaaagagcctttgaagagttgaaggccgcctctatgtgccaaaatgggggaacttaaggcgcactcttataaagcagtgtcatgatacaaagtgggctggtcatccggggcaacaacgcacgcgagcactcttggagtcggcatattattggccgcaaatgagagacgagatcgaaggctacgtgcggacttgtcttatttgccaacaagacaaagtggagaacaaggagcccggtggacttttggaacctctaccagtggcggagcgaccatgggatagtgtcacgatggacttcatcacggcactaccattgtccgaagggtatggttccactatggtcgtggttgatagattctcgaagtatgcaaccttcattcccgcaccaccggattgcaaggccgaagaagcagctcgtttgttccttaagaacgtggtaaagtattggggactaaaacggactatcataagtgaccgagacccgcgcttcacgggtaagttttggacggagctgtttcaactcttgggttcggagttgcacttctccacgagtttccacccacagacagatggccaaaccgagagggtaaatgccatacttgagtcttacttgaggcactttgtgagtgcaaaccagcgggattgggctaggcttcttgatgtggcacaattctcctagaacttgcaaaggagcgaagctacggggcgtacaccgttcgagttagcaacggggcaacaaccacatactcccctttggtgagttcttacaaaggaagaagtcccggagcatatcgcttggcaaagacttgggaagaatataccgacaccgcccgctcatacttatagaaggccgcatacaagatgaggaagttcgcggataagaagaggcgccccgtggactacaaggtaggagactttgtgatggtgaagcttaataggacacaattcaagacacttcgaaaacatcacaaagggctcttacggaggtacgaaggaccattcgagatcgtggcaaaagttggtaagatcccttatcgactcaaatagccaccacacttaaaggtccaccctgtcttccatgcaagtcttttcaaaccttatcatgaagacaaggaggatccaagccgagggttgtcatcgcgcgcacctatggccgtaaccgcatcatatgacaaggacattgaagccatcattgacaagagggtcgtccgttcaagtggcaagaagccaagcacggagtacttggtcgtatggaaggggttgccggcgcgagaagctacttgggagaaagaaagagactattggcaattccgagaccaagtccaagcatacttggggagtacttgcgccgaggacgtcgcaacaataggtgggggagagtgtcacaacccgctcaaaacaccccaattttccgaccaacacaatgtgccaaagatagccgacgggagcgcgacttatgtccgtggccgtatgcccgaccatgccgaggtgagcacggatggcatggaacatgttcacaaggatcttggcatgatggaaggcctaggagtatcgtgggagcacgagggtgcatgtggaagagtggccaagacaatgccaagaacactagaggccatggaagcacaatgttgcgctatggaaggttctagaatggcctagcgtggccttgcccttgggcaataggggctgcccaatgccccaccgacttaggggcctattccaccgactttaaggcttcaagaactctcctataaaaagaaggatagacaaagaaaagagaaagggattctatcctcgtccaaccaagataatatcgattgctcgcccgacatcagcctcttcacccaccggggtggaacgactcttaacgaggttgatggacttgactttttctttagcctctcggcttcgagaagccgtgggcccagtagtgctttcttaaagccggtaacctgatcgacgtaagaaccgatctcaagctggatgagaaggcaaataaagactagtgagaatagccgtaattcaactaggccttgaatcagtggtttacagagagaattagtcatctgcttacggctaatctgctcttcgaatcttatcttagaataggttggaactttttaaacatgagaggcttcttcagaaagtacgcatttcttgctctaagtccgctgggttggatcgaactagttggtttggcaggaagataatggcataaaagaagcattccacttttggaaagagaagagtcagtctgattctagatccctctgtcttgcattgggttaactggagcttagataaagcgataggcagaagagagagaattagtatgtctttatagactgactttcctcgcatcaaagctttccagttctcttcctttatgaagaaaggaaaggcttgttatcgacgaagaagatctttatactgttcatcctaagaaaagaagttttcttttcactcggtacaactattcttattctatgctagcatagcatgcttctacttatgttgcaaattccggatcaggaagaatcctttcttattcgttgatgccagtctaaaaatccgtacttgttgactaaaaggctttcggctttctttctagcttgaagcttaagggctaagggaaattcatccttggatcaatgaaatagttgaattagctaagatgcaagaaggaacctcttctcttattgaaattactttagctttaggaagtgccaaagctttctccttcgatccgatcctttctgtgacccatggtctgtaaatgaacttattctctcttcgtctcttgcctttgaatcggatattccgatgaaagcggattctctttccgtccctcgtcatcgagaggaagagtcgctatctatctatccatatacctatcaacaaatgtggttccagggatcggtcgattgcccctcaccagcagctagaggaggagaaaggaatgatgtcccggcctgggcacctatcagccaactattccttttaggaatggaaagaagaaaggatggtcgtagatcactgatgtcgaattcaggaaaaagatcatatgtgaaagaatcgtcagattatgggttcccggagtagacggttttgaatggagaatgaatgaaatagaatagtctgggagaatcgtatgatagggaaagtgcggagcctcccacttgtctgggttaccaggctggctaaagtgactatgaatttatatcaatgtcgggatagacagaggtctaggatagtacgctgtcggagtgagaccggggtagagtaaggaagttagaccgaaatgaacgactcaattcctctagaagaaaggagagagaaagaagaaccaattcaatgaaagaatatcttatttactagaatcggttgctactagtccgggttacctcagagatagagccattaggggagaaaaaagaacctagttagtgcacgaaatgtcctgctaacataggagcactcctactaagaaatggaagagcaaatttctttctttggggtcaaagggctattctattacaaaaaaagttatggactcggatatgatccttctaatgagagttccttggggatatatgaattagtggacatatacaagaacgacccattttcttacacaagcatttctgtactcagatcggtaggtatggaggtctttcctaacctctttagttagacaatcagttatatacggacattcaacaagataaccccgaaaggaggcaaccccgttcactccgacaagaaaggtgtcaagtctgaaagccaagccctcgtaccagagcgctctcataagtcaaataaagtattcattccttcatttatccatatattaaacaccctgtctttgaagcttcttgcaaaaagtcgttcgacgacacaatgcctcacctgccctctgctacacatctctttcgttcgccctagacccacccaccaaagggaactctgcccttttcaaccaaggaacgagcaagaacgctttgctcctggggctcgtctacaccacatcgactagcgcttaggcttctctttatgttccaacgcggcctttgattgattcgtaaacctttccccgatcgagggcttcctatctcctcagacggtgggaaaaggcgattctctttagtcaaagaggccttctcgtggatttcgccttttttgatggctatctcgtgcctctcaattcccactgcaagcttgggaagtgccttgctttctcgatcagccaagcccttgcttttgaatagcaggaattcgaaaggggaaagaccttgctaataccttttaggcactagacagaggctgctaggaagattacataaaaaagtgccgagttggcagctctggaagcgctgatagcttttcactccctttccctcatagctgaatagtaggtaataaaacctagtaactgaaataccaagtaatctcaggcctaaagggtactcagttaagggaaattacataagtaggaatataagccgaaacatccccgattgagtttcaactattggtaaggcggtcatacttccttcacctaaactagaacctaatttagcggctctttccaaaaggcgtgaatgcaaataaaaaacatctcctggataagcttcacgcccgggcggtcttcgtaatagaagagacatttggcgataagcttgtgcttgtttggagggatcatcataaatgattaaagtgtgtcgttcacgatacataaaatattcagccagagctgctcctgtataaggagcaaggtattgtaatgtagcaggggaatctgccgcttcggctaccacaatagtgtattccatcgctcccctttcctgtaaagtagttactacctgggccacagaagatgctttttgcccaatagctacataaacacatattacattttgaccttgttgattgagaatcgtatctgtggctactgctgttttaccggtctgtctgtccccaataattaattctcgctgaccacgtcctatagggatcatcgaatcaatagcaataagcccggtttgaagaggctcatatacggaacggcgcgaaataataccgggggcggcagattcaattaatcgaaattcggaagctggaatttcacctctaccatcaataggtttagccagcgcatttacaacacgacccaaataggcctcactcacggggatctgtgtcggggattgaatataggaagaccaatagtggaattgaatcggattctcgctcaaagcctattctcgaggcagtcttttctcttctagcggaattccccttcacttccattgagattacgacagattacacactgccactgacctgagccatgtaaaatattgcaataaagatttgcatacgctccacaattatggcaacgatggggatcgcgttgtatcatctgaggcccaggtgacatctcccttccagtggaaactaatgcaccaaagcccaaacttggaatatttgcaagttttttctgtttcaacaccttgtgagcggagaatagaacatttggagattccgtagcaggtgtccaatcttcagtagcatcagaactttggtgatgcagctcgacagacccatttgaaaaatggggaggtgatgatgtgggcagagatgaagccgacgaataggcaagaggctgaggggtggctggagaagttctgaatggcacggcagcaggttggagcggcgacgaaaatacaggaggaccaggtggagtgctgagatgaggtgcagggcttccagttctaactccattagccggtgatggtaaattgggggtcttgatggacggagaaggaatctggttcggttgtacaattggtggaggaaatatgggacctgttgatgacgggaaaggaggaggactaaatactgtttctgggcgaggtgactgagtcccttgctgagagggtggaatggtgacagagtacccaactgaggattcaggttgcttcgccatcaaaatggcatcaaacaccagcttttcaagaatttcaaaaaaaaaaacgaaaaataaagccaagaacctagaggattgaaaattggaaagaggcgaagccctcagcagtcacatccaagatctcctcggagactcagaatcgatcgcacccaagtcagaattaatcgagatgggcctttgctccaggatgattaatctgatgacaaataatgaaagggaaagcttatattttggcatcaaaaaagtgaagatcgccctgaattggatcctttgagggtctcagagagagggcaagtacaagaggaactcaaagtaaaaactagactttgtcttgcaaactgacttcagccatagtgaataggggaagctgctcactttgatagccctaccctagtgtatgcactcaagcagagtagacggcacgcgtcaccaagcataccgcccgaggttaagggttcatcagcgaatggagttaggcccatttcctagcctagttttaagcagaacagcaccatcctagtccagagcagtacttctcttatgggctcgaggcaagacaagcagcccgcttcgcttcctcaattgctcaaggaacaagatgaaataatgcttttgtggaacgtcttcaggcgaggctttgggattaaaccaatatctttctatttgaagcagtgtgcggtatgccttcaattcaacaagcatacgctggccagaatagtactgagatttccgtctctctttagctgactcgctcgggatatcctcgcatcattccggcatttcaccgtaagaggatccttaaaggtgattccaaaagtgatttgctagtggtacttgtcgcttttctccgaaggctattgaattagctaaaccacgtgggtggcggttgtccatggatgtcccttgggcctattcttcatcggatacgagagcaggaagagcttctattccatcaacacaagttattccagcaacagctcttactctaacagaactaggaccgtcaactccaactgtccttatagataggcgaaagccacctccttgacagattacggagctacccagcttctcttaatgccaagtagtagaaaaaccgctttcccgagctggctttatcgagttaacgaggtaacaagcggaaccttgcgcaaagacatacccggcatactaagatgaatcatctaagttccccgccgtcttgattgatgagctcgaacagccggttgatggcaatgaatgggtgaagcagggaaggctctgactttgaagcccgggctcaggcaataaagataaagaggcgatcaagaaagtcacgactgtctgtcccttcctcaaagcaaggagcggaaccctatgatgactcactttaggttgaacctgatctgagatctctcccgtcttcaaaaaacaagcaatgaagacaactctcaccttcgattgatagatgaagagccccgccaaaccaatgaaagttgagaaagatttggcatcttgaaaggcagctaagagcgcatctggtcttccacaacacactggggatattctcatggacgccagctggagaggttcttaatagtttgttccgagatgtcagtctgcaaagcatcatcttcatctctttcatcgcacgtaggctcaacatccaagttagcgtaacgaggcccaaactattctggttggatgaaccaacttgagatgttaaaatattccatcggcatccctggtatagtgatagaataatattaggcacatcaagcctaactaggcttgcttctatctttatagatcggtgtatgacaaagatatatatggtctaacagctccctcaagcttcgtgtagttcctccccttcagcttggaccgaagaggacttagcagaagataaagccttggtttggtaaagacatctgccaattggtacatgctggaaacatagcatacccgaacttcaccacgcgacactctcaccgggtaaatccggagaaggggaacttattctaagatagaataagaataagcagaattgcttaagtaaggtagtggccataaggcttttctttttttcggtatgccgctccgcgagcaaggagtgccacgcacgagcggagcaaaaagaaagcaaggggaattcttctcttttttggggagaaatcctttgattgcgtattgaatatggatccatgtctttcttgttccactagctaagaccaaattctcacatgtccctttccttattacaaccttcttttttgatgtcaaagaccagaagctacgcgcaaattctcattggatctcggttgttcttaacagcgatggctattcatttaagtcttcgggtagcaccactagatcttcaacaaggtggaaattctcgtattccgtatgtacatgttcctgcggctcggatgagtattcttgtttatatcgttacggctataaacacttttttgttcctattaacaaaacatcccctttttcttcgctcttccggaaccggtacagaaataggtgctttttctacgttgtttaccttagttactggggggtttcggggaagacctatgtggggcaccttttgggtgtgggatgctcgtttaacctctgtattcatcttgttccttatttacctgggtgcactgcgttttcaaaagctttctgtcgaaccggctcctatttcaatccgtgctggaccgatcgatataccaataatcaagtcttcagtcaactggtggaatacattgcatcaacctgggagcattagccgatctggtacatcaatacatgttcctatgcccattccaatcttgtctaactttgctaactcccccttctcaacccgtatcttgttcgttctggaaacacgtcttcctattccatcttttctcgaatctcctttaacggaagaaatagaagctcgagaaggaataccaaaacctatttcactcgctgagtctttttgcatccatggctgaatggttaaagcacctttcctagtaaaggggcaaattcgtaggttcgattcctgctggatgtttttataggatcgggaaagaatatacatgagagtcagtgtgaggagaaagagctttccctttttttgttcttctagaccttgccttttcagctatcacttcttagatggagctctgacgggagacctatgaacgccttggctctaagccgtacgaaccccctttcaatgccgtattaagccaggcggaaactttctttcatgctatagcgtgcttttgagcgcattcattgctttgagggattggttgtgataagcaaacaaggaagcgttgagttgggcgcgtatgggttcccggccttgattgctttttaccttaaaaaaaaaagaaatattcgtttataccattgacattgataattatagaaagttggatagtatgctttgatgaatagcaatggtagttaaaagcattcctttcctagggtcaagataggtctcttcccctcttcccttattcctgctcttcccgcttcagttgatggaaaagcattgaataaggcaaggaaggggtcgagacagtgttagctacaatctctgcccttagcttagctaaaaggataaagtgaagctctataactcgaacgcttggattcgtctatcttagagtaggttggcttgttagatctatatgaactaggagtcatttagttggcttctccgtcgttagagctttctgtccgaactttcttactcttgtaagctcgtcttgtcctatctatgctcactacctcgttgtctgacaagcagtttccctcatctttctctttcagaagagcctactttcgcccatggttcgcgtcgctatcgtgcttggtccgttcgctactctcttttcagccattattgtatgcgtgtagcctaagtctacccttcgattggactttctccagatcctttgacacccgctcatcttacttcccattctggtaggttggtgcgtgatgattcgtggagtacaaggctctctctggttgggtacgtaggctggtcctgcagmttgtggaggtgaccagcgctgcatgcccgaatggaatattgactatcccgtagaactgacctagtcgctcgtsaaggagctggtcattatggaatatactatatgtaggcgcaggtcttcctagagcgaacctccatgtgttttatattaaacatataaaaatcaacagtggaagaggcactggttgtgcgagatcattatgactggaggaagcccattcgacaaccataataggctctataaccggatcacgcacgctaagaacacagcggattagaggggacaagaggttccactcatcaaagtgtgagacgcaaggcttctgcctggaagtaagctaccctctttgccactttcaaatcaataataacgatgtcatcgatattccaatccgatcttttctttcttcacccaagtaggtaaggtgctctataggtatccccccgtagccctaaaatcgaaaaaagcccatggttgagtgagcatagagctctgcccttttctttccttttgaagccgctttcctcctttccagctttagtgttttgctatacattttaatgtgttaagcatagtggcatgctctgtagccggagtaagaaagattcaaggagcgcagggggatctgcttttacgagtgatctctctcgctttcttaaggaatttctagagtcatatggcatggctatggtttccactcttgtgagttccaattttttctttggttcgctttcccttgggctcggttgcccttctttctatttgctgcagtaaatgagactgggagttggatttcctttatgactttcgctccgctcttcccacggatatttcaaagaccggtaattcccttgcatcggattcctcgttctattcctccaaggctcaaagacctcacagctgattctcaagaacttgctatttcatattctcttagataggctatcttccgattcaatgccatcaaaatgtacttagcatgcctacttttccttattagttcaaatagccctagctagattctcaagctcggattcacccgcaaagcaaagatcaaaaagctctttttcaagctgcttattcgaaaacagtaagagcttttgagtgcacaacttattctttcactcctgttctacgattaccagtggtctcagcgctaactggcaaaggcaaacttctttcagggcatcttagttccttcccttaggtctaggctaagccttaacaatcccttcttgaagaaaaacgattctgtaacaactcaacctaagagctgatatgtctccaaccgcggatacgagacctctaagaacggttatttcagttattcccaaagctaattcaattgcaaagagaacagcggcaacagatatggcaacaagaggatgataaaccttctccccttaaccgctggactcgaaccctaactctacaccgtcgccttcaactggcacaaaaggaataggaaagtcatgacctgacaaaaatggaaagacttttcttctttatcgccagactcgatcacaagcaggggaggttcaattgatctatctacgtaaagggagctaattcaatattcctcggtgagaggaaagaagcctcggacaacattagcctttcttgtctttcttcactgcaagatatccaaataagtttatcgctcgttcgtgtggggagccactcaataacgcggctagggcaatcttcaacgatcagcccggtgcttcaggatatggatcacggatacccgttccccttcaagaagattaggatatgtcgtctaggcctccaggatgcaaggagggggataggaatggattaagagttcgagaatgcctctcattacgactatgatcaagtttgtacctcttattgtgtcgcggaacagcaagagtcatccgactcttaggaacctccatacgaggatgctaaaaaaaagtcctattgaggtaagccaatataaggatcccatacttagcaaccaagaacaaacagacttcggtcaggagtcggcggatgatgccggatatgcctcgaggacggcggccaacctacagtagacgaatttaaagaaagaaagatgggcgatgagactgaccagcgacctatattcatcgcgaaggctctccccgatagagtatcagaaagccctaagctaagtagaagaaagaaatgaggttagagctgaaccggaaacatcttacactacactaggtaccccatatagagtgccaaggagaaaaggattgagaaaggcagtgatcatcatcaattccaaatttctttcaatggcccttcttcctaaacgaaaccttgctttttagaccaaagatgttggataatctgagctgcttatcgagggtttttctttaattcccttttcgccccttttttatattatataggatattcaaaaatgagttcaaataagactcatacctatctcctcgctctctttctttatctgtcttaaaagtggtaaattttagctatttggggagagtccagtcccgctggaagaggtagtagcatccccgtgctatgaacaacaaatgaatctcaatgaataaagttgagtacgttgacaaaaaatccactttaatagctggactctacgccaaccttatcttacgatctgtctttctcctatctacgtaattacatattttgtttggtccaggagtagttcgtgagacatggaaagccttctttggccccatacgcgtgaatcatagcgatagggaagctgggtactgcttcgctttcaattacgactcgaggtcgggtgcaaaggccgtgggcaagatacatacctcgctagttgaacgaaatatagaatttcttatctaaataaaaaggagttcaaacttttgagaggcggaatcgatcctgcaccttagtctacaggtgggtcaaaatctgaccttgttttcgccttaaacccccgcgctccatctatcattgatgctatcaaaaactagatttccaatatccaaaatttccatagaaagagttttgcttcccttgtgtgtgaaaatgaagaatccatactagtaagagctccgtcgtatcctgccaagacaggactcccctttactcgtaaatagttcaatgcctttttttaagaagattctaaaggcgccgctatagcttaatacaaagaaatccattcacatagtaaatggaagatgcctctgtaactctacaatgcttggggcttcaaagcttagtgcgaatggtgggaaaattcatagctttttaaaatcaaaccaagagtactcagtccgccctcggtcaggagaattttgcgaaatcaatgctcggagaaaactaccgaatgaaggttcagcttaaattgagagggaaggaggtgctgatcaaggctacttggatcttgagagtagtaaagtactctgcttaccgctaaaagtacgttagttttcggacttaatctgaatgcacagcgtgctgttggtgccattcatgcagcttcttcctcttattcttcccgaataggacggaaacgagaaaatgttagacccaggacgaggctactgccactgggaaggttaaatatatggatagtcttcttattaatgaggagtgatcgacttggtgattataatagatgccactacttattattctttttgcggacacttgcaaaaccttcgataaacagcgcctatggactttgagacatggagcgcaggaaagaaggacaggagtggttccactagccgatgcttaagcgtcagcccttgcttccacttcaatgttgctaaaccgctagccgcttcctatgctgcattgctcactttgacagagttccctcgtgcttttcctcaacgggaagcacatcgagatctctgtggttgcactctttaaaaaattctttttttgtttagaatgtcccacagttactctctctcaaatttgtgatttgagttgctgtaccatacagtctttccgcttaaagaattctattttctctagctacgtcacagtgtcctttcctttcgcgtactcctctgtctttttcctatcctctctcttcaattaccgagacccgtacatactaagatctaggtagctcatctccttctaagaagtcagatctccttcctatattctaaaaagaataagagccctttttaacccttcaattgtaaagaaaggcctcatttaggagcgctgttttcatccaactatcaatctcgtaagagaataaagcgtggaaaagaaaggttttgattcgctttataaagaagaaagctttttccggttctaacaggctaattaaattagaaagcgtctgttcacgtcagggtccgaaggagatgtacttgcttttccttttttgcgtcgagattgggttggtgttcagtgtaccgcttgtctagcctatgctttgcatgaacatctcaatgtccaagataaaaagaacgaggggaagaatcgacgaggccagtgttctcgaagagaaaatcgtgatggaaaaagcgtgaggagaattcgaaagtcgatatgttagaaggtgtcacaaatgaagaatgcgttggaggttggttgaagatgatcttacgcggcgttcagaaccagtcttgaagtgaatgaagaaaagaagcgttgttatgaaaaagtttccatttctttcccaaataataagaacttttggtgctgtagtcacttttgcctttggacgttttctttttttcggggcagaaagaacgatcgcgcctagctggatccttctctttctcttttgtcttatatttatgattcgggcaaaagaaagaacaagaagaaaaaggagtgtggttcattttttcgttgaattcttcctcctttttctttttctttcccttctgcgcctactcatcatggactggatttcttcctttctaggcctgaccctgggcctgtccactgcttttgtttcttatgtttcgtctggatccaatgaaagtgggaattcggctcctgaatcagggggtcctccccctttagaatccgagtcgagttcggcgtcacttaacacctttcgaaaccagatcgctgcggataatgaagccgatatatatcggcgcatacaaattttagaaaaccaggaatactacaaccttcctccccagaacagtcctggtgactacgaaaggctggttcgcgagaacttcgattcagccataaatgtcaatcattttcggacgatttttgatagggaatactttgaccttcgagtcttagagaggaagggcgtcgtacaagaccaactccaagatctaatgcttcgggaggagaatatttcacagattctagagaaatctccttattcgaacattaggaaagaagcctattactatcttgagcacaagctcaaccccgttagcgatccacgccatgcctttcagcgagacattcttgacaccagtctcgacttctttcaacgagatttgaatctgagaggcaaagattcaaccatttacaaggaatttaagacgtattttatggacgaatgattgggaggagtagttctacctatagacaagaccatcagagaggagacaacccatttatgattccagccgagaagactagtaaaaggaaggatcaagaatgttatatatttcaggagctagattagttggcgatgaacaagtaagaattgcctcaaccaaaattgatggaattggacctaaaaaagccattcaggttcgttatcgattaggtatcagtggaaagataaagataaaagaattaactaagtatcaaatcgaccaaattgaacaaatgataggtcaagatcatgttgttcattgggaattgaagaggggagaacgagcagacatcgaacgattaatttcgatttcttgttatcgtggaattcgtcatcaagatggatcgcccttacgcggtcaacgaactcatactaatgctaggacttgtcgcaagctaattcggaaatgaaagaagtctaccgaaagcccttggtacttgtctgatcaatcacactgatagcttcaatagttcactgaaattttgtgtagtttgctatttcaccggttactaatccagtatacgtatagtaggcctccttcgccacgacattagtggcttagcccttcgcgcttcccttcgcccgcctatcgtatcggctcggcttcgtcctcgaagctactgcttccgcctctctaggcatgagagatagctcatgactggtatatggatctctctatgtagtggtcggccttctagaagcttcgccagaagcgactagtcgcttcccgaatgcctctttactttagtatagtctaatttctttttgcctccttccttgccgccaacgtacgctactaggaaagtaagcaagctagcttgcttgcattctcgaaacggtagcttccgctaccttcctgcctactgaaatttatgtgaatgatcgtgacagctcttcaaatcctattcagtctgattagatatgtcactgaaacaaagtgattccgttctgtctctgttttcttttcggattccgaggatgagccggccgatcctaacatcatttatgaggagccggacgacgaagcctcctcctcagataaagatgtctccgacgctactctcccggcaagaacaactttttcaattgtgatttttttggcgagttcggtcaggagggacaaaagagagatgctttctatcagtcaaaagcggatatcgccccccatgctcccacggtccgcttaccgaggaatagaagggaaggacccggggccagagcaagttgggttggggtatagagccgtaagcgcggtggggggtgacagaggacgtgctcgtacggttcatagaaggatatgaaaaagtacttatttgttgggaactttcactcctctatattcgaaatatgcctttctaggagcattacgatctgcagctcaaatggtcccttatgaagtctctattggtcttattcttattgtgcgccttgtgagcgcgtttggatccgcgaaggcaatcgctcggatgttcccctaacccaacccgggaacggaccggagggaaccgcagcatggggaatgtccgcgtctcgtcgcaaggctcattttgagttgtgggtcataaggcgggcagctttatctgagcaagggccggggcacaagggtcctggtactatccaggtgcgaagaaccccggaggtgactgcaatgagcagaaatctcactcacgggcctaaacgacgagcaaacactcgaacgtgagagcaagggatcacccaacgaatggacgagctcaaaggggggagggaggcaagaaccatgctttcagagacctaacccaacccggtccgaatcttatctgaactgcgagaataactgactaagccgtgccataaggggtcattctccaaacgggacggggccaagcctttaggttgtttaagtaggttgggtgacagatcggccataggagtactccgggatataaaccagggcaacaaaagtggagcatacgacgatgccgcccgttttcatttcgtggaagtgcccggcagaggaaagggctgtaggtgatggcgcgttctgcttcttatctagagaggggcgtcgaaatcctttctattggttcttgcgtggcagctggtatagatgatgaaaggcgggccgctttttcgggacctattctcttaataggcggcaaagcgaaataggaaaggggccgagctgactgatgagtgcctttttagcctttattttaaaggctctcatgtggagctaacatggctggctacatacaagtatagccaaatcaagatgagatgggacggccgttcagaggccgcagcgggactaccattggaaagcccgcccccttctcccatgctgagtcacaggcagcgcctcggaaagcacggacgagccacatgcagggaaacttgcacgtgtggttctggccggggaccccggtatactgtactaatatgtgtaggttcccgtaattcgagtgagattgtcatggcgcaaaagcagatatggtccggtattcccttgttccctgtattggttatgttctttatatctcgtctagcagaaactaatcgagctccgtttgatctcccagaagcggaagctgaatcagttgcaggctataatgtagaatatgcgcgggatgcgatccttaatagttcactgttggcggaagccaatgtcccggggtctcggggactcattctgactgaaacaaggggcgggtctttaccaacttccaaatattcgattttagggaagccaaaaaaggtgagcgcctagcgcgaaaggttgctttactaagtaagataaggcaagaagcaagggcgcagcagctgcacgaaagcccttgcttcttagcgcatccgttttcttgctcgttagcgcttgactaataagatagaaagagcctttcttgcttgtttagtaaagtctcgctttttgataggagtaggtgcttgctagggcggggcacttttcattcttcattcgaaactaacaagtgtcgggtcggggatttctgccttgttatcaaaaagggagttgggtaaagcaaactctctccttggaggagcacgggcttagtcaagtagaaccgggttgcgctgcttgatgctccgatcgaaaacaaatcagtggggccatgccggtacgactgaatatgcgttagaaaggtcaatccctcccctacgacaccaaaaaaaccgggccgaacttctaacccgcccgcttccatagaacaatatcgtggcaacgtagatctaagtggtcatattggatccttgggaaccatcacaagtacggccggcctatatatatttgaacgaaaatgccgtgtcgtccagcggagcctagaagaaggtgactcgcgcagacagctgactccttttcaatagaaaagaatagccaaaccaacccagctggctggtcaatctcagagatcttatcggccggcaaaccggagacggacgaccacggtcccggccttaccagcaccggaggtgtactaatcaatgaacccacgaaaccaactttcttttatgacaaaataaaccaagcctaagcggtcacgacatcttgttgatattgattgagttggagggactttcgctgactgaatccatccataaacctagaccgcggtaaccttcgtaaccaaagcgtcacgacaacatccaaaggtgacctttggattcttaagtaggggggcaaggaggagcacgtaggaatgccgaccactacataagccactagtggctgagagaaagcgagcagcaccttgtataggttgggcggagcttaaagaagcaagcccctatcagagaaagccattgcgcgctagcctagctagctaacgtttttctttcagctggctgttatgttagttgtagcgcgccttccctccttctctcactttggaaagatttttcagtattttcttatgatgacctggtcgagagagtacgatacatcggtgtaaaagattgacttttttctgtgagcttgaccgaagggtgcagtagaacctgaaggagaggaataaaaacctggtctataattttgacaaaaggaggatcactattgggaaatatcttcctcctcttggtcgtcatcaaagaagttgacgtccggggcttcctctttccctttaaaaccggtgaagtccatcctaaagttccaaatctacatccttaaccagaggttcctggtgagaacaaattgtaaggcgttgaaagaaactaaagaaagaaaatatttgaaactcgggaaaggagaataagcctctctaagggaagaagacctagcccagctttctttccgagccatcaataactgccggctttcaacgggtccggctatcctttcaccggtcggtaagtgcatcctattcctattaagtggggcggcagttgctaaataaaaaggtggcgccattcccgctaataaagaaaaagcaattcttcatccaatctctgttccagattctggtcttaccaagtcacctttctctaaggctaaatagctaaatatccccgtactttttttcctattttctttattctttcatgtcgagctttcgaaagccactggggagggagaatgaacgatcgactgctaaagatcttgaataaagcattgatagctttgcagaggagaaaaactttgattcttcccgaaggtcttccttgcatgctgaagtgaacaggggcggtaccaactacgactagaaagcggtcactcctgtcaatgaataccattcatagttgtctatgttagtaacatagccataacgactttgttttactgcttgaggtggtgatagcttttatatatttactaaattataagcttgcatagtgctcttcctatttgttttctcggctttcttctgccgaaccgaacgaagacagtttctcgtacctctgtacctattgcactgatatcttctctttcactctctttcttcattcaggaaaggtgaagattgaatcgggaaccgaaaacgaagcaggaacagacttgtcctttggtcgaaaagtcttgtacggttcctcagtccgggggcactgcaagaacccctatgacacttggagattgcttgcctatgtcacttgtacagtcctctaacatggtaagtgtgccatatccatcttggcttcaaagtctgattctgaagagagagacaccgaccctagtcagtctaaatgatgtagacagaacccgctccgggcttgattaccaccgaaaatttcccgagacggtagaatgtaaactctagggtgaagaagaaagcattgcatagaaagcatttttgtataaggttcccacatccaatagataagggatcttgccctataacctagtgaagagggaaaataagataaaaatatatgacttttttaacttctaaatctatttccaaataccctgaaagcagcaaagaaagcagcaagtgaagagataaggcctctcatttccattagggcggatgcattccattcccattgtaacggcggcggagggtgcctccgggtcgcagcggttcttccatgtcaacttaattgaaaagcatcctagagattgattggcttttccagtactaggcttttgctttcttgtagttcttctctttacatctaccttcaaaacaaacaaaaaggacgacgaaattactatatctatatatagaaagatgtggactggagagtttggattgagatccatatgcttaacacatcgtagttggacagcttatcgaagagaggagaaaaaaactatgttttgtcggcatcacacatatagcatgtgtgccgtgccgtgagtgagaagtcaatcactttcagcttttctttaaaaattctacaacatgatgaagaactcttttcggctcgaaccttctttttgagctcggtcaaaatatcaagaggaaagatcgtagcgtagaaaagaaaggagaaatcgttttgattcgaggccgatcccttccttaaacaagtaagcaagtaaactacccccttttttttctttacgggttgagtaaacaaaagaaaaaaaaagctttttcgtaatttttaactctaatgacaaagcgtccgttcacgtcaagaatagaggccgttaaggatgtacttgcttttccttttttgcgtcgagattgggttggtgttcagtgtacccctgaagaatttcaagtaactgtctttagtacgaagtgagttgatcgagaaagcggcaggaccgtaaagcaacgccttgagttggactgtggtcccgcgaagctggtatcctcagaccgcctaagagactttccgactgtcgaaagaagtgaacataaattgactagtttatttaattgacttaaagatctttcttctatgcctgtgagattggcgtaataccttttcactaaaagtgatccttattatcattctaattatctaatatatattattaatctcaaataattaaagttggaatttgtttaagtaattcgattaaatctttccaagctaaattgagaatgaaatttcattcaattaagaacaaagatcaatatggaacgctttggcgtcatcgttccccattaccattactttgttaagacgattcgctttaatcattattttgttcagacgatcgatatggaataataaatattatctaataagagtcgctttttccctaacggtcgagtgacttcttacctctccaaccactcttagctacgcccctcttctcgtaacttcgtacctttctgtgtctaaagacgctcataagcgattctttgacttgtgaacccatttgccttgagtgtatagaatgaatagataagaaggggtggagctagttagaccattaccgatatatgacaactcttacttaaagaagtagtccgtatcgaatctattttctattttggaacgaacaacgaccaactaacactttgactttactttattagattcagaaacattaattgcaataatatctcgaatgagaagaaaaaaagtatcgcgcgatcgctcgaagaaatcaaacctttatttcggtctaacccgattctaagactagtcattcctatgttcttttccttttaggttatttcacgatggtgtttttcgtagcagtctaaggggttggtttacttttggacatacttcatttgcttttcttattcggacacatttggcatggtgctagaatcttgttcagaggtgtttttgctggtagtgacccagattttcaagtatataaaaaaacatggatccaacagatttattcattactactacataaagcactacattacataaacaaccacatatgccttttactagagctttaaaagcattaggcctactacattactaaacttattttcgaaacataaagataggccttaacaagtagaaagtcactatttttataattttttttctagtggttttccgggacaccgaaggtggcaacccgcacaacgagttcttccttctccgtccgcagcgcttgcagcctcctctccaaatcgcttatgtcctctctggcagcggcaatgcgcgcttcttttcttgcaggatcctgtgttctaacacttagcaaaagcgcgtttagcgttctacggcgcccttgaattgcattttgcaggttactcatttggacatcaatttgagaaatcctgtttatatcagctatatccatacgtgctattactcaatttctttgctttgatatttgatgaagtgaagaagcctctatttatagagtggtagagtaatctcgccatgcagtacgaattgcatggctggcacaatatgagtactataaccacgctgcctgtaacaaactttgcggaaccctttcacctaatcgatcgtggtgaggattcggcggatcatccacgtcacgctaggatttgggaaggacattcacgagattgaggtgggaattgcgttgcagagaggaatctcgccatgcgtcaccgaatttgatggcaggcacaattcttactagttctccgcacaacttttctgcagttgaagactatcatgcctatttagtgaaaaactggctggctctggctaccacaaaagatccccaaatcacactgcctgtatgaacaaacaaaccttgcacaaccagcttacgtagaaaagattccatattctatgccaatagactcgtgacatccatgtactgagtcgtcaaatgagccacgttaagaaagcccaagcttatacgcattggcccacagggtgccccaataggccccgaatgaaagacccaagcctacatgaaccatccaagaaagtcctacaaatgaagacttgtgcgtgcctgtttcgatgaaagcaggcttacatgcttatcaaaaatgtaatcattttaagggtttgggatgtattttacgtgaaactgaatctatttcccacattctcaagatcctgatccagccttcttcgctaacgctcaacctcgcatcgcatccttaccttaggctatcgagcttcgaaaggactatattaatattaatttctaatattaataggtaagattgcctttaagggaatgtgactctctttccacgggcattttctgactcttgaaagaatgtgattcaaagaattgacggtaaccaaggtgcctactcttcctaacgagcctgcttattaagcatggtcggtcaatcaggtaataccccaaaggctgtctccagagatataacatttcttgagatccaaaactaccccgagaaatgctctagatcaaacgaaaaggggaccagaaaaggaatcccacatgaggaaattacttaaaaaaacttattgctaataaagatgctaattggtatcctggaagccatctttacatagaccaaggtacatgttcctcgacgcttagggcatccttattttgctttgttagagcgcttatttcctagtttagtcagtcagtagacctacgtccaccggtgaagctccactatggagatcacaagattagacaacaaaccttccacaagtaagaaaacccctgatcagacgttggtggattgtgtaatcaagctcccatttcctccaaatctccttccactctgaaagatccctcttttacacctccggaagacctacccgatcgcaaatcaatcaacttgactccacccttgcaaacacagaagactaatggaggaccgcccatcccatcgactatatctccccactcccagagtctacctccgctacaaaaccgccctcttccttttcctagccttcattgatatcgtatgcggtttatcggaatcagaaagatcatatattcaattacttaatccgtgaacggaacctttggcttaccctcattttccagggaatggaccatcattcaatgcatattgatttagaatctgtgttggatcgcgaaccttctcttctctcaggtccagaggggaactcctagttaagtccctcatgatgcctatcggtaagaggaaactcgggattcgtgccatgtatgtggcacacaactggttttatcgatgtgaatcaacaaatcacaggaaaatttggtcacatagatcttctttcctacagtagcagattcggctagtgatcagtaccctctctttattcccatagaaagactcttatcttaaacaaactctcggattggctgagctttcaaagattgaagaggacaagaaagggatcgaactcatgtaactaagaaaagaaatccttagctttagtgcagtgacccaatgaaaacgaggagaagaaggccaagggtaagaataaccctacaggctaagatctctcctgggctttcctcacaataattctgctgttgggataggtgaatcaatgggctcatttcctttttacgggatgaagagatgatatagcgtgtgtgccacaagtgcgtagtctcattgaagttcagttcgataagcaggtctttttcgtaggctagaaggtaagtaagcagggttagagaatccgatagcataagatagactcctcagattatcattatctaaggttgtagccgtaaatcatgctctctactcttggaaatatgtctttgcctaagatggtaatagcgtatgaaattatataggtccctttctagtaggagtaacttatctcttccttttcttcttcagaaccgctgacactccgttcaggcggaacaatcagcgagagaccgtctttcacctacacactgggcagtccattgctaaggactcggtgctcaaccgtgcccatatgctagttgaaaccaatcttaccttaccttatttacgataaaccccgaagacactgctcagtctatgtcctccaacgttaggtagtatcttgcgcttaaatggactggcccttcttttagggaaactatatgcttgtcttcccttagatctgagggcggcaatgttgagagggcgaaagcacacaaagggggggcacgtcagccaaaagaagggtatggagtcggaaatcgaaccccttgttgttgacctgtgacagcctcaatgctcttatggcagggcagtagcaagaacacgatctctcggaaaagaaaaaaaaagactaaaccctatccaagatgccccaccaatcaaataaggcactgcagagccaggccccaaagtacgcttttgctcgctccgcaagtaagtacgaaccaggcaaagaagcaatgtcgaccacccctaaaggtaaaaaaacctgatgcatgggacaagggcggagagtataaagactataaacgcacgcagccctcaggcaaacctctaaccaggctgatgaaacctaaccaaaatgttaaatcaattacgtcggtcgttgtgatccttctttcccttccagctcatcttgactattcctcaaaagaaagaaaggaaagaactcgatcacactgcacggaaagaaaggcttcattatatcaaaaggggcgagcgtatcgattgcagaaaggctggctgtacccgagagtcgttattctcccttacttcgtccttgctgctattgtagcagtagtgccttttggaattgtatcagaacagaagtccctggcttcttaatactactctaagtcatttcgtcccttgaatgctgatctaagcgagcgcgaatagggtccagctagtaggttgtagttgcatagttcctaggccatccatcctgccttgtcccttctcgcgtaaaccgctgtattaaaggaggtgagtaagtaagccagttagaaagcatgataaaatagccccttaaatatccctttcttttatcgagctagccttttagtatgattaccaggagtgaaagaaagctacgaaaactctgaagttaaggagaagagtgaaccccttttactacccgtaaaaatacgagtacctgttgcaaatgaatcaaccccgcttgttttttctgttgataggttagattctcggttgaacgttaggaaaccctaccaaaaatggagtctttcccctatatcccagtgcctcgactagtgcttttcctaagtggtggatattttttttaggcttttagtcatatgtattcccctctttgagtgtgctagtaataagctgggaaagtcaaatccatcaaggcgaggaaaaactagtttgaaagtagtcctccttgaagttccttttaattgaatgtggtaaggataaatagaaatgcaatctctgaatctcttacatcccgcctagtacctttttgaatcgagggggcgaaagcttaatatcaagtaggagttctggattgaggtccagttggttggataaaggttggagttctaagggcatcatctcgaaaaattgcctttcctggagtttctttttaagtcttttctttcttcttctatatctgctttctctccgctccgggcaagtcctaagctttgcctttccccccgtctccttaccgccctactcgcaacttgattttgaccatatcccgttcggggctctctggtctaaatgctcgaaatgagcgatattcactcggaacctagagattcaaacaggcacaggtcaaccaaaagcatattgccgagctaaggtggaagataaaaaagctatatttaaaataataaagagaatctcttcaaattcatattcaaaaatgggattctcaactatacttgactggaaaaaccagccaatctactctcctttttttggtctcccccctgtaactttataaatcataagagaagaagaaatcgttgcgtagaaagtcgtgcttactatctcctccatctaagttatgtaagaggaaaagagcgaaaagcttacttttaggtagtggcctaagcgctaagaagctccaatcatgctactcagactatatgcttaacacatgcaagtcgaaccttggttttcggagttcgaaagagaaggggaagaagcggggtagaggaattggtcgactcatcaggctcatgacctgaagactgcaggttcgaatcctgtccccgcctaatccatctgaggcccggcctcaagatttgagattccgtaagtaactcagtgactgctttctaagaagggcttggaagaagaaaatgaaataggaacaaccgcgctggtcgtaatagatcgactttcatgctagttcttgctccagcatgaaagttccatttcagggaaggacgacgtactatgatactttctgttttatcaatctccgctgggttgattcttcttcgatatccatagattttagatatgcttacttatgttgtaacaaacattcaaaatagcaggttcctgatagacggcaatccacagttacattcggagttgaagtacatcttagtctcgctttgcctttatttttttgtttattcattcgttacaatgagaagatgtcattggtattatttttagaagaacacaagtaatattctaaaaaaaagtgctttctgctttgcttttccttttctattgataacggcattcgccccttcagtagccttttgcgcagatcctgcgcctgcgcttccagaccagacctcaacgagattccagtaggcctttctcctgctgaaatagcccaattgcatcgggagactgaagagaatgccgcccagtgtgggtgtggcaggctcttgcaagaaatctgtgtgcgggcaaaagaagttgcccgtcaggcaggagtgcaggacgaactcaagctggaaaaactcgtcgacgccgtcaagtttcttgccgacgtggacgagttggacgaagaggaccgaatccccactctcattgagttcagggccaaaatcgagaataaagactcgacaattttgtttcatatagataaagaaatgaagaggtggggtggccgtggtctatgatgcattttttttcttagatagaatgaatggaaaaggggtgcttgtgttgtggttttcgtagttgcaagaattttcttttcgagaaaaggtcccctccttcaatatcatgattgggtcgaccaggctagatcatgagtgaatagaaaatcgaaaatgtacatagctgttccagctgaaatacttggaataattctaccacttctactaggagtagcctttttagtgctagctgaacgtaaagtaatggcttttgtgcaacgtcgaaagggtcctgatgtagtgggatcgtttggattgttacaacctctagcagatggtttgaaattgattctaaaagaacctatttcaccaagtagtgctaatttctccctttttagaatggctccagtggctacatttatgttaagtctggtcgctcgggccgttgtaccttttgattatggtatggtattgtcagatccgaacatagggctactttatttgtttgccatatcttcgctaggtgtttatggaattattatagcaggttggtctagtaattagggggcggccgttcggtcgcctatgatactaggaccaataggttcaaaatgggtttgtgccgcaggtgttgaacgatctactctacacaggtgtgggcttacagggctagggctcataaaccccttctttcatttatcaatagggccccggtcggtcacttttctggaccgggatcgataagtggaagtcataaaaaagagatctttctcttcgcacctcagatcaagaggaagggttgcttgtcaagctggcctatatataatataataataataaatagaaagaaatttctttctatttattattattatataatagattatataagaaaaatggaaagattcgctttcttttaaccggctccttcttctttgtcaacgctactaaggacctataggtttgcctactttacttatcaaagataatgataatggcttattcaaacaaaaaggaaaaggccctacttagtttcgcaagcctttgtcattgtcagtcaactaagtagggcctgaggccccctgcgaatccgtaaatctgaggagcatgccgcaacaaaaggatggtcccctatgcatatgcatttcattttttccttaaggaaaaaaaaagtaccccccatcatagtgaacctctccttgtgatcgggatgaggtagatgcctcccagccggggggcggatcgaatcggagtttccttaggtagccaccgacctacagttatccttaaacttccgtgcttggtggagaagaagcgaacaaaagtacgctcgcttgctgtcttgttctctgtcgcgaactgggatcgctcgccagctaggtcagattggagcaagattttatgagaacatattccccatattcggggacaaggggcggaacgacctctcgatctacttactgcagcccaggaagaaaaacgtcgtctaggcgttccctgttgctccgatctaccctacgcctaggacgttgtctgggccaagagccatagttagttgctgtttccatttggttgtttcttcctcgttgttgataccggcaagacccagccagatgatgtccgctggttggtagtgagaggactcttagtacctgcatacccaaaagagggcgctggttaaaaaacaatcatttgattttgtttcttgctctcccttagcagcgggaaaggagtctatctatctgcctagctttggtagatttcccccaacgcaatccacagaaattccacgaatcccttggtggataagtccgacgactcagcagcagtgcggaattgagtttcttgtctggtggatctgatctatagttagggggcaatacataccaaaaggttcgaagaaggaaggcgcataagagtatataaccaacctacccttctgtataacctattcacattagtgaagcggttggatgcataagggaagtgcacgtttgtgagaccttagtcgggatgcataggtgagtcaacctacgagcacggaagagcgtggtaccgctacccctctctaagtaaaggtaagattcttagccctgtagatgactccatctaaaatacaatagggacagccgttttcggctgctcgtttcgtatcttgaagaaagagtaggcttaagtaataggggtcaggtcaataatagctatgctattgccctagtgatttaaggcctccgcccgatcccgaatgcacattttttcgggttcatcttcaattgatgttttcttaacctttcgaagaccttgcgtaaattttcgatgtggtcggttctttcttttgaaaagactaccaaatcgtccacgtaaggctcgcatatgttatgtaggaggtcaatgagaatttgtgtcatcgctctttgatatgttgcactttctttttctttttttggggcatatcgtagtaaggaaaggaagtgagggcactcattcgaatcgaatagctgaaactactataactcctatttttctgctttaagagaagccttctagctcgttttaaagcgttgaagagagagataggacattctaaagatagttgttgaggaagcatctgatttctaactacgagtccgttttcaagctaactgaatgcctatctgctgctagttctgttccactatctgctgttactgctctcgttgccggtgtgacagtctgagtagacggtgctctctttcctgtagtttttggggttcataaccggtgctattgaatctgcagttaagggaatatcactagttcttggaataagagctctgggacttcatggctttgagggagggttagcctagccctaagccttttcggaatagaatgccccgttagaatgggcagggacagtcgatcatcggcttaatttcctgggttttgggactctagtatcaaaaattcccggtatttcgtcgtgaaagtgtcacatttagattgaacttattaaaggaaagagccgaatagacaaagggtttacatgaccgctcgctttggacaagatgccatagtctaagaagaaggcctttgtttgcaaagatgactttcccgctttcctttgtgagggaggtttgtgcacatgaattaatagtcaaagtataaggaagatggcatagagcatagaatgagattgatgcttcgaatgccctgttttcaggggttgtgatagaaggagctgtggcactttcggaagggggaatcagactaggctgtcactgttctagaagaggaagcgtagctggcacgttgaaccatgtctgtcaacggtgaaagatagccctaaagtgagggccccggagatagtatttctcaactgtcgatcgacgtgacaatcatgcctgcttgacaaatcctttttcattcagtctcccaataaacgaaaaaggatttctggtgacacgaaagctgtgctcgacgctctctttcctattccactgtgctaagtggtctttccctttattgctggatgactactatggaaaaagatgacgactactcccagtctctggtcaatccatgctgatgcatgaagagctattcccgccgcccacccgaaagagacgaggaagactaaccgccatcctgctcgaacctttgctgcctgagttatatagctgactgcgagaaggaaggttcaagctatggctgccccatgggatgctcatttgaaacctttgtccggtcaatgcgagaaagagagaagtgatgtaaacataagaatggaaggtttgcttgtcagctgtcgggccaatgatgctcttctagctttacctacacggcaagggaaagatcaaaggcgaggtgggaaatgccccgcacgaactatctgatcaagttttctttttcctatcacaggcagctggcaaagccgtgtttgatcgtcgcgtacatgctccgttacagcttcgttcatgcgccaatcaattgacagtgaagcagagaaggaagagttttgatcaccgtgtgggtagtctctattagggtttccgtttcatgtgcactaaaaaggaaggaagactggtgcgactatagtaatgccaagcatacgagcaaaggactctacctaccccatactgacgaatgaaagaagctcatcgcggatgataggacaagcgatagcggttccattcttgctcttcctattccataccataaacagacacctttgattcatcgacattggcgcgtcaggctctacccccaccccccagccctttatggagttagcggaccaagagaaagaattccccgatataataaagaaagtaagaagggttccaaaccattgaaacagaaagcactaaagactgatatgacgtggcagagatgatcaccgtcaagcacaagattcaaagctggaatcttcctactcttcttagttgggacagagcatcctatcttgttgattctcctttcccaccgcctcgagctctcgctttcagggtagatacgcaagaaattcactaggaaaattgacatgacacaatccctgaagagtatgatgtgcccggccttgcttctcttgatccccacccacctcccgtagaggcgggccaatatcaatatctataccagagattgcttttagctttctcttttcagagacaggagaattccttctgtacttacaagaatgctacttagggagaagaatctcttgactcaggagcacctgaatctattctttctgtgtcccacatccgcctatgttaaagcatccgcccattcctcagtgaaaggaaatgctactcagggatcaaaaaagaaagctggtgccttgtcagaaagacttggttcgtagagtagaggcctttccccaagatattggttttaagctcctctccttacagtcaagtggctttccgctcctgcgggttactttttgtcttacgacacggcatggtaattgatcgagtgcgctttcctttctcctactcccacttcgggaagggaagtgctaaagggcgggcatgctcgactgcctaaaagaaaagaaagaaagcccggtatggatattcattccgctagagcaaaggcatgaagtgaaggaggccgctaaggttgagccttacaaattttaaagagtcatattcaatcacccggaaatatccgcatctgcgaatagaagctgtggagggagatccatgcaatggcatttcatcaacagataccacttcttcttccctgcttgggcatttggaactcttagcagttgaggacgaacttcaggctttctatgagtagaaatcctattagcgaaccctctttcgtacctccgcctttcccttctaggtcatggtcaccattttgtgatcaccgctacagactacttcaccaagtgggttgaagcaataccaatagccttaacattggaaagtcgcttttaagcccaagtgcaaccaaactagcaggaaatgaaagaagaaatggatctgtgtcactgtctgtatgcttgtcttcataaaggtttgagtttgattgtttgttgccaaagagaaaagttcattgtttaggtcctactctgggtctgtagctgacagcggcagttattttcttttcgatttttgtcgattaataatacccaaaaacggtagcgagtagaataaagaagttgcttctagaatgccgattgctaggtaaatcgcccactatatatagcacctatcggtgtagaaggttcaagcaagggatgtggattgagtccaagttctggagaaagagggggcctttttttttcatctttcctaaatcgatcgatcaaattcttcatatccgaagcgcaggaaggatctgactagaaagtcgtcttgctgatgcaatagtcctctgggtatggccacattcgtctcgacaataggatagggaaagaaaatccatagacgagaccaacagggaccgaacccttctatcttcttctttctctttttgttcccgcctgccgaggacctatctttcaataacgatgaagggctactagaagggaaagggcttcaggagagatacttagattggatgggcctattcccatttatgggacagtatcccaagcagtaaggctctgtagagctagtctcccttgagacctgctgccgcaaaagctctttctgctgctccttcgcctgcggattaagctgtagaaggcaagcaagcaaaccttggcaactggcaatttcaaggatcaggggaggtatgaaatggttatctcggctgggaatcaagccccaacacaaagagctgtgggccaggttgctttgctttatcggatcaatcagtgtgcagtgggcaagctctttcccaagtcgctgagctgtttaacagagggaaggtcaaagagctgtggggctaggagtgttctcaatcttagcattccgagacaaagcctgggtcgtcgaactaaagaatctcagcattggccataaaaacgcgtttgaaggcctgtttctgggactgatagggaggggtctaaaacttgaatttctgctatatcaaccttccaaaccaaaaggggattctgctcctaccgctaaagcattgtttcggcccctgcttccagaagagttggtgcaaaagtcattgtagtccaaatagcgtatttccggttaggggcctaagactcactaaagcaattgtagctattcactccttctagttctagtgaatttcgctccaaatagcataaaaagaagcttgagttcaattaggggggaaccctctgtagtcaacctgctcccaatgaagaggtaaggggcgtagcgatgaagtcgaacagggttggtaaattcaccgggtgactcgaaagcaggctcttaaagaccactcctagcgcgtcagtcatttcgctcccaaagagctccctaaaaacgttgccaatatcgacagcagctcctgttcaagctcttgtttcggttcccgcaaaagaaattgttgcagtctcaactggataaatgaacagcttcgcatctatttcctattgtaatgacaaaggtttttctactgatccagtgtcagataattgggaattcgctttcagctcttaatcttcttcgggagacatggaaaaaggcaaggctcgagagacctagcgctaaagcaattgtagcggcccttgcgtacagaattgtagcgactccttctagcattcatttaacaccttcgggtattctggtatcgaaaactggagaaaggaaggaagtctttgcccgagaaaggaaagaggttgactcactcgcttggcgaactcataggtcagtagctcccgttaaagctaaagctattgttgggccccctgcgtacaaaaagaaaaaagacatctttcccccctcagcactcgaaatctcattaagagaagtaacgtagaaaagaggacatgaaaaatggcttagattgtaagagcaggtgtaagcttataggcggtagctaagaagttctttcttgcactttgcttaacacatgaaattcgagcagtgatccactaacagacacgcgtcaaaaccaaatgactcagggcatctccaatcggtggcgttgggagctcctggtcgaggtgtggagttttctgcttcctgccctgcggaagtctaaggctgatccctgctgctagtgtaatttattctaaggctcttcgagtttattcactctctggtaatcccttacgagtctcaagactcttcggtcaccggaaagtagttgttttctatccttctcgatagggctggcccgctatagagaggtattgtcggcttatgggggtataggatatgacttaagaatccaccttccctttctctttgtctgagcacaagtgttaagggtacggtgattacgcagcaagatcttttccccactagatctctgagggacaactccttcacttggaaagcggatggagaggatggcgtagctttcaaacttagcctagccgatttgctttttgggtttgttgtcttcctccctaagactttcgttcagtgacatcacaagggttggtttgagcgcttagggccattgggagggggctttccgatagggcttccttcgctaggaaatcggactattctaccgctactgactgactggacttacaaaaagggagttcattatctaggtgagctctttgctcctggtagaccggttggtgttcatcagtcagtttgcttctttttttgactgacgtaattgatttgcccttccttccgattcggatggagatgcggaatcttcttctctgtattaaccacccttcttcacagaaaaagagagctcagaagacctcgtctattacgacggtacggaaaaatcaatggcaccgggggaaactcagtccagagaagaaaatgtcagttaggaaagagtagtcagacgcagaccagcgcaggtgggcgccacagctgtcttcctccatatgatatcacgcaagaggcgaaagaatccctttaccttatttacaaaataagaacccggtcgatcggagtacccttcctcctttttgaggcttttaggcctccggtcagtcaggggttgacatgagaccggattttttggggaatccattctttgccctactgtctgtggtaagtcagtctgctttgccttctcgctcgaattcttttcaatgtaattgaattcaatagtatgacttctatttcattgggaacttgatgagtcgatccgcctacacgtcttgcttttactgctatatcgggtcttactccacgtattgcttgacgtaaaagagagagtggatttctttctgtcttttgttgaatcgctcgatagagaatttgataagccagtatccgcggtaagttccaatgcttgatagagtaaagtaaagaaagggctttttttaaagagtaagtcagtccccttgaaagatgcatccaaatctgcactcggggtacgcataaggcttcagaacagggttggaaacgaaattagatgttatagatagttatcgggaaagaaagacttgatgacggctgcacatactcaaagggttccttagctctttacagagaatctcccagtatgctaaacagtgacatctctcgttatatcgagaatgtgcatcccgttatggatgatgcagcttctcggtttggcgaagtgttctgtagcggagtcgccgccacacctgccggggcgggtaagctacgactgttcatcataggtaactatgtgaagcagaggctgttgaagccttatcacgactgggcgatgtcagttttgcgtcgcttagattgtgatggtacttacaatcaaacaaaaccccctagagcgggttggtccgctttccaatttattcttctctttttctatatttctaggtcgaaggaatcggggcagagaaggtttttatccctaaaaaaagcctttttccgttgctcgactcgaagcaaccacgagctctaacttaaagtaggtctagaaccactgagattaagttgttttctattttctctccaggctatgaaagatctgggatttcgttccaggaaatccgtatattgttttaacatatctaatagggagaggaggagacagacagtaaggtatggcgagatcacatctcccgttactatagtagagcctatacggggaataagatatagtgatgccgacaattcaataactaatcaagaaagtaactcactgaactgaaccagctcccactaaacaaaacaagcttaaaatggggcttattcttgaacaaaccttactgtagaaaaaaggagattttctttctcggcttgactaaactttctttttcttatactcccctttgagaagagaaggaatagaaatagagaaagagatattcgtgggccgttaaacgaccacctatgaacctttttaataagcttttcctcgcgggaattacatgaataaagaatcatccttttcgtatacatttcatagacctccctattagcctactaataaagaaagtaaagcactaatgggtttccgatgaaaagaaggaacaaggaagttccgagttaagcgatagaaattggtccacagtgagaaactcaagcgaagcaagagagaagatgcccggccgagaggaagttcaagtcgctgaggtaatttcagatagagctacgttccgggtattcctaccatcttttcttataggttactctttgaactcttaattaaagcactggaagagaatcgctatcgtctttctaaaggacggggatttacgtgtattgcttatgcccgatttgctgacgctagcttgacttcactcacttcagagacggaaaaaaagaataagaaaggggcgtagcagccggaaagagggagaaatcccctcttccgcttaaggcaccgaagtcccacagctaatatcaatagctgttgattaaagggaagttctttctagagcagtaagagcctattctgtcttgctttctgattcaattccgctgctagggcgagctaactccaaaaaaccgtcctcagttcggattgcgggctgcaactcgcctgcatgaagccggaatcgctagtaatcgccggtcagccatacggctgtgaattcgttccaggatctctcgctcgccctcaaagaccaactcttctggaaagagttctatctccctaggttttaattccttccggagataagcaaccatcttccctttaagataggggttaagaggatttcccctccctaaccaatattctaaaggtagttgctgtgaaccgtggggtttgccagcagccgctttcagtcgttcccatcgctttgtttggattgacatcaagcgagaccgaacgcgatagcctgcacctgctaagggttgtaaaacagacatcttttggatgccatatttacaagccagctggcacaaaccaatggtcgacctacaacctgttaaagcacgaagagatattggggacaaatccttttgcatgtccttagtccagtacctcttcgcgaactcgagagtaccattctctgaaataatggattttgacagagaaatagtaactccgagtctttccagtaacaggctatactctctggctaccaactcatcggcgataagaatatcatcgccaaggagagcgtagtcatagaaaggggtggccctctgcgggtaggccttcttcgctgccaaccataccagataatggtgtgacagggcgaaaagcgaccaagagccgtagtaacccaaaggctgtccagtcaagaaagccacttcacttatccctttaacaaaaggttttgttaaaaggaaagtgttaagaccaagagtactgttgacgattgatgatgccaaagtacttccccacatacaagacatgagggagtctatgacactcaatggccaacagtccgtagcagacttcaagtcaaaggaagaaagtttcctcaatttcttgacccgaagcctatgtaaatgtaaggctttctcttggttgaaggtaccgtccttccgtattggtttcctcttggactccggcgtaatcccgagcctgtaaggtgtctttttaaaccggatggtaagattgttccaatccacccggaagtgacttaccacctctactacttttatacgagatggatcggcgtactgggactcaaaccagtctgtatcggcccaagctttagcgggacccttgaacttgactacaggctcggcctcccctttaggttggtaccaagaggctttcggtgctaaaaatagacctttctctattttgtcttcaagcttaaacttacctaagacagaaggagaaaccagctcgtcagggagtggatgaccaagcacaacagagtcggtgtcggtatagtaacacttcttattacggataatggggtccatatgcatcctagcgtaggcagcagccgctgccgccatctggaccgcagcgttcctcagggggcgccatttttctatggtcgggccagtgtagctagggtaggtagcgaggttggtgttttctttaagctctacaccgtgcaggaactcctcatgggagtgaatcaattctttccagcgtgcattatcgcagatctcggcagtcgtgctttctgggctaataccgaatctgccgtagagggcattcatcaggatctttaacacataggctatcgcctcattaccttcttcgcgcgccctcagcctactctcagagagagagctaacaaagtctttaaatgggcttctttcgcccttctcaaagaggtagccctgggttgggactacagtgtaccccagggttctagcatactttaactcctcgctaaagtagacccctataaacctcccggtagggaagacccagaggtccaccccgcgatcgataaggcagaaagggcttcttgatagtcttggggcactccacatatgcctcgataaagccaaagaggctatctaagtcctcgccacccagatcctcacgccagacaggcttcccggcgggcatggggcgctccgccattacaaagggatagagtgagttcacatcgtagtagtataggtccttacctattggtatgtaggcatccacatgaccaccgtagtagccacgccttataaacctctcttcattcgtgttggggatgtggatccgccctttagcgggatcgtggaacttcatacgaaagaggtacattgccaatgaggaaatgggaattttgtttactatgtcaacctcgtatacctcccaaaatatctcctgcgccctttgcatcacaccgccaaggagaaggacgtccttcttcagatagtctatcaactcctctctcatactgctaagattctcgagagtcactctctcatgatcaatagaccccttattcccaagttcggggcatagactacgcgaaagtgaatcaagcgaacccaggagtagagccatagagtctctgaagcggaataagagcctcccccgctcggaatagaggcttagctcgtaaagcctattccctctcgacagcggtcttatcctgcccggccacttaccggccaggtgctctagcaagagaattccatcgaatctctgaaggttatgaaagtagacggttatagacgacctatgcttgatagctatatcatttatcctggatactaaatcgctaagtaccttagtactcctttcatcaaattcttttaaggtcctgtactcctcactgaagtaggtttcaaccttattatatttgaccggctcgccggggcgaacaatcattagacctgcagcataagtcttttgaaccccatcccttattactgtctcgaggtccgctacaatgaaaggtttccgcgccccgggacgtggtttggccgctgtcatatagacgggggggctacgcccatgatgtttgatcgcccttgctggggtggggccgcccctaattaatcgggtgccgatacggagggccgattgttgtaagtcatttctctcatcaaaagacggggctggcccttccgccctagactcccccatatagactcgtatgttgagtcgaactagctcggcgttcttgtactcttcgcaacgatctacaatagcttgatatattttagggtagactacacccatcgggagtggcttaccgtcattttcggttaatggaatagcggggcccgcggtaaatattagaacatccacagcgggtggtcgccgcgcctcaaagccaatcgtgaactttccgacgcccgctagagcggggtaagcaaaccggcataataggtccacgaccgcgagactgagtagctcagtctcgcccaaaagaggcgaggggggtgtgaaagtcatggacgcagcgaccaacttagtatccttactatccttcttccttttcttattcttattattacttataacgtgcagcacggcttccccaatcctcccataatactcgtccagcactcggctgccagtttttaatcctccttgatttttcatgggtgcacgctccaatttatcaccccctcatcagaggccccctcaagggtaggggcaagctggccccggaagactttccaccttaagaaatgcatttcataatcctagttagggccgcatacctcaccagtataggcctcatacgccttaaccaggttttggatccttccagaccaatctttcatcaatttccggttaaccgtgccaggtataccctcatgtaagcactccgccaggtccgtactagaaaagacccggtcaaggtcaaaagcaccggcgcggcgccatgacgggccggtgtccctactaaacaggccggcgggcctaccaaggaccggactaatcacattttcgtatatgaactggttgatgaccctaagtggagggtccaagcgcgaaaaggaaagggtataaagaccagggagcatccagctatggtgagctgtacttacaaagttgtcgtgtacagtgtatataggtgcatcgcgctgccgcatttcctttaccacactcatagcaatataggcgtccttctgatggatgaagttggcgaagctagccacttctgccttcctacgatctctcttatcggtaggaactttgagagtgatttgccgtctttcaatgcctgtgccccaaaagagggctaggttcaagggtaggcacctagtagctgcgagcctaagatcaaaggcagttccaaaaaggagttccctatttccagcttgataaagtaaagtctcagtgccagttgtaaggttaggaaagccaggtatgatgaaatcctcttttcgaataggaattgattcgatcttattattattatatgaagatgaaactgaatatactctttttcaagaaggaatcgccatcaccagtggaagttgaacccggcgatctcttcctcctgaagtatggaaaaaggaagaaaaagcagtcaaccacagggaaggaaggaggtatagctcaactttcttgcctcttcctcaatccagtagcgaggtttcaacgagttctttgtacgcgtgtaacgaaaagtatatatactttttctcccgaattccctattactctcggtccttgttcttggtctctgtgaaagatccagtcgatgggaatgaatccatgttcaaatcttattaccgggttcgattacattgctcgatgtaattgagtcttaaaggggaattgcataaggaatctcttttcttatgagaactacgaatcatcctcatgaataagctctactctaccttaaggagatgtggaggcaataggtcccgtgcagctttaactaactcgactcctccatacgcctatcctttagtttagtgggccaggtcctccagccttccattagctttcgatttagtttgcattcaaagtcttggaatgcgagcttatgtgctttcaggtataggcatcctattccccgttttgactttcttttggaatcgtcttcttttaaataagatcttctcccttgttcttccctctgcctatgatcttgacctgctaagtgatttccgaaagctcccactatgactaaaaagctcccaataggccacgtagcagcttaagcttatattataataaagtaagtaggaaggagcgaaagctactcgaccagacgggagaggcgaccaaaggaagctggttcaccttctctcctccgttacaacataggtcgttccaatcccggatgaaaatattccaaaacggaagtcaaggaggaaagttccatcctgtccttcaaagatcgactcgaaggtagccatacttatcttacgatataagtggactacccgcgatatcgaaaaccatgagagataaagcagaaccggtcagcctttgcatcacgacgtcgaatcatctttcgatgaaaggacggtatgatgcgaggaagccccggcctggtattttgaccggctgaagcagcggcagaagctgaacccgaaccaaaccctaagcaaagaagggatgtgccttagttcagtctcgaggacgggataataggggcgtagcaccgaatatgtcggagtagtcccacccagtagatggacaagccagtagtaccaatcaaggaagcctttcactgtagagctttctttcctgatggggactaagaaaaggagacgaatatagctaaacagctgcagcagaaagaacgaaaagccaaaagtcaaggtgcatagcggtctattcaagaataggggagtacagaataaggggtttgcaagacaaaagagaatccgctggaactacggacaaggatattttactcaattcccctcttactatttaaaaaagcggaaaaaaatgaaattccaccagtgtgtatgtaagacaaccttaattctctatgttcaacgctttgggcaagccagagcaagacttctctgtgggaatacccggctatctcctactttaaatagagaaaatccctggagtcaaagagttatcacccgctgtatcattgacgcggacggggctttctttcctgcggtttccgatattgcaatggcaagcaaacagaaggtttccctctttcgggtataggctttcccgattgattggaaagattttatactgccagagaaaaaaaagctatctaaccctgatatccttggtactgtccctgctgagaaagatcctaatttcccagagagtgcttttccggtgcggtgtaaccaacaactcaaggctatcaagggaaggagttgcaggaccggagttctatctcggatccacagaatgacctgtttttgtctcgaaaaccgctcttagggcaggttccacgtgggattggatatcgaaggttccttccgagcattttggatatggaatctgtattgccggaaaggttctccctgtcccgggcaacctctcttcttataggattcatagagtggagtttacctttaaggttggattctgattgagaagccgcatcggatagagaacacgagatcttgcccccattgttgaagatttgctcttctcaggcgtctccagggagatgaagtatttgtctttgtcgattccactagatctgagcatgctacgtgtcatcgggccagtgcgatcacgttcaacggacgcaacagcgtagatattgttgcatgggatgttgttgctcttccttgaggccatcacagcagttggctccagagtctgcagatctgatttgtgagagaaagagatgaagggcagagttggtcccaccgggcgtgccagaaatttgttcgtgacaaaaatggaatatagaaaataaataactgcaatcacaaaacaaatatgagaaaaaatcatttttttgataaatgtttgagtacaactccaagtatcccctgattcttgtctccaagttgttcgccttgattcgagggctgaagcagcgtgtttctcgaatgaaggatgatgtggacctcctcgtgatgtatttgatctccgagaaagtcgggcagcacttcgggttgatcttgaggaagaacttctcttgatcacttcacccttgctagagaactttgagaaagacgatgtagtcgatgtcttgatctccttgtgaatcttccaagatgttatggaattttcaagatgcctccaaagagaatatgtagcccctttatataggcatggattaggcttttagggtagcctccaagtaatcctaatggacccttgggcttgaaatatgtgggtgggccattttgtagaggcccaacctagcccaatgtagttggatttgacttaagtcatgcaattttgacttaaataatgaatccggctttattaacccaaaatgttgacttgggtcaatatgtcttgaatttagaacttagtccaaattttgtatggacttaatcccataaaattttgcatgtctacacttaccaaactaggtaagctagtcatatagcttgcttagcacaaagtttagcttgcttgctcctttaaattactcgtagcgtaagcgagcgtagaggaacgaacggagcatctctcgtagcaccgtaaggcaacgaagttgctgcattgcatagaggtcgctaagattgctggtaagaatcgctattgcaagtctatcgaagcctacgctacttattgattatcaaaaagcgaaccccccggcccttcccacctggggctacccctaccctaagataagacggttcccgccctcaggtcagggaatagagctaactgcatcggaaaaaatagcaattcctagtccgaatcctggacctggttcacgcttgaaagcagcaattcttcttccaatttcgtacatcaaattgtgtatataaagaagagttcgtccttcttcaaagagataaagtcacgcggcccttcaagatagaggcttcagtcatcgttagaatcccggggcgggccaaattacataaagaaaggagacttatttcaaagtggttcaggtagctcagctggactgaaaatccttgtgtggttcgaatccacatccacttcacagcaaagaaagagaatgcggggtagaggaattggtcaactcatcaggctcatgacctgaagatggtgcaccatctatccatgggagtagcgaaagatacctccttcagggcaatgaatgccatggtttctaatgaactttatccagaaggagctgcagcgattgagcggccagctggttaaagaatttttattctccgctccgactctcaagaaaccccatatctcccttactggtcgcggtctcggaagagacacagcgctgccgaccttctgagctacgcaaagccttctaatatcagggtggctgtacacgcaattgagagtacttcttgctacttcatcgtccgtcaaaaccatcagctattggccggagaacctaacagaacttttttttctttcaggagttggttggtggcatggttttcttatttatagtatttgtttgtttgctggcacaggtagtctagtcattatcagtagcagatgtagaatctgaaaggtgggattaccggtttcatttaaacctagcttacaatcactagtgaaagagtgcccattgacccaactagcgaatctgtttagaaccaggttcagaaagatagctgaaagtgctagcataaggaagagattctatggttttcggcattcaaagtcaaacgattcttttcattcaaggaaatcgtctctattgaactatggaaagcactttctagtagcgacacggattcaccatttcgccaatggggcaaacgaaggctaacccgttctggttgttatgaaatcagtaggttctttcagtcttgctttccttcttacagagataagagagataagtaagtataagtaatgatccatccaaggaatgagcttccccagagtccaatcccgtggactaagaacctcgcccggcaacagcagatggttaacctttcattcgatgcttctgattcaaaccaaggtacagagattaggtcgaggtacgaagtctctgcggggctaccgcagaggtacgaagtgactcgaccaaagggagaggggctaccgctcgtttcactatgttacctatgttcagtttcacatagtgaaacgaatcgttacactctcatttcgtaccttttccctgcgagcagaagctctccgctcgtgcttcattggagcgagacagtcgcttccacacagaatacttggctacctacctagctcgcatttgtttatcctctcgtgggttgatgacatagcaaggggataagcggtgtggggcgaagtgagcttggccgctctgagtagaagtgctctctagcagcctagatctagctcagcttgagactttcgtactgaaaggatgacttcgctagtcgcgagtaagcacccgtacgggaacggctttcggcagacaagttgcagcagcaaagagtgcgccctttcgtttcaatgtagattctcctctcagagaactagaagaaggggcctaagcacggtacacttgagtggaactcaactcgaccaaaggtacgaccaacgtacgaagttgctagagattcgttgaacatagttcaactcattcgactgaaaggagaggggagaggaattcccggaaatccttcttgacgacgcatccagcaggaatcgaacctacgaatttgggcgctttaaccattcagccatggatgcaaagagactcagcgagtgaactaggttttggtattccttctcgagcttctatttcttccgttaaaggagattcgagaaaagatgaaataggaagacgtgtttccagaacgaaaaagatacggggagttagcaaagttagacaagattggaatgggcataggaacatgtattggtatatcgatcggtccagcccaggcttgtgcggttaaggttgttgtacacgatggaagctgttacgtgtgggattcggtgtcgccatcggatcggagccaaagcatacgctgctttaaagcagttactgttgtggcgtccccgctcacaactccatcccttagtcgcaataggttctccagggaatcctcgcccgttaaggtacgaggattcgcgagcgcccaggcaccccgtcccatccaatccccatctgggtgaagacccgccatgacccgacagatatctaccttggcctcgaagaggtcttcggcgtcaatccgggccatttgaatggcatgggcggagggaaagggggatccccccaaaagcctccgctgaatggattccacacaatccccccctatcaattcattatggggatagggataggggactggggctgcttgattagcagctgcttcctgcataacaggaagagcagcttgttcccccggaagcggctgattgaccgttgaggtacttccagaacgctgggaatcctccaacatatcggttgtataagtaaacaactccgtgctggtggatccgtgaggaatcatgctgctcccgatggagagacccccatcggcggcactgaatagtgctcgcaccaggcacccaatggcccaggcaagtccacccgtgaggcccaaccctctaagagcaaaggagagggcccgacccaaccataaatatgaaatcaaggatgcaaatgattgacccaaggttgtattaaagtttcgatcggttaataacaagcttgctyrsammtygctttatattgaaagaggtcttcctccttgagaaggyagcctttctatcatttagtggataactccttgctccattccgcttaaggtggcgcgccttagtcccataagcttatgcctatacctgctttcccttgaaataaacatagtaaaccactttaaactcgcagttagtcttggcccaactctgcccgggggttggccttttaaggcttatttcacttctttttttatttttctcttattgctaattggaactccggctccggtaacctcctgaaccttatccattacgtcaacccttcttcaacaaggggaagataggagggaattccctttttcaaggcccctaacctagtcctggtttggttctccagtggaaagatttgagataccttctcctaccctataaagtaagggagactgacactttatgctttatagaaagcgaaatagtgataaggagttgcggaaaagtcccgaaaaaaggaagcgacttttcccggaagagcaggggacagtctttagcccaggtaaaataaaacctggcctccccttccaccaaattggactattctctcatatggagtctaagaaagagatatccttgcgcaaggcgaaagatcgatgtccttcagaattctaaaagatcaagattgcgtgcctttagatccgtctttcttgattcataatcaagacagaaaggtcggatgtacttgttcaggtcaaggtctacttttggtcattcttctctctgaaaaatagaatattgctcaaagaaggtgactcatgtagtcccttttcgagtattatcttcgctgtggatgatcagtcggtgtgcgtatgaacgaacggattccacctctttatgggctgtatatgccctgcttgtccccatacccctttcagcaagggttgacgtggtctcaagaatcttcttccgacctctgaggtggtcgtcaagtcctctagcctaggagtgagtcaataaaaggcaggattctcgtcttttttttttttttctgagagagatgtcgtccttcagttcctgatgaattgagtccgccatctatttcatagtaatcacgaacaagccctatgtgtcacaaagcaccacgggttctttacttttttggtgggggtggaggcttttgtgcattatagcacagccgtgactacctttaccttgattgttgctgcatatcgcccgcttgttctatagaaactaagtgcctatcaattggttcaaagcggccggggtctaactagaacttcatttctcgatattgttggaattggtctcgaagaagcgattgcccgcgaagccggtagccccttaagcttaggggaatcggccttctttagtaaaagctttttcttgcttaatgctttcctatctcgactgattccccgtgatccacctatgagatcgtttgcaccggctttggattcaagaagatcggccatagaataaggaatgggaagaggcgagactctcgattcgctgctctacatttcgataaagtggaataagaaaggccgtagtaccctaggcccgacagaataatgaagaaagaggccgattggagaagttttgtttgagaggctaagggactagacccatcaaaagcagaaagaaaatgcgtgactaagaaggagtaaccctagaacaagttgtcaagacttgacccctgaagaactggccaaaacgcaggacattccggaagttggtcggtcaagacgggcactcccttcgctcctttcgacctgatctcccacaaaaccaatacaaagaaggtggaagtgggtcaccccatataagtaatatgggcaaagtacgcgagatatgaccaatagttttttttttcaacagagtccttctttcagcaaaatcaaagctccttagtgcaatcgatttcagtatgccagtttaatttgaagagaaagagggcagaaatccttacaatctcagaaccaaaaggagagaaggtggcgaaggatccggattcactttttttatttgattcatacccgcgtaaaggcttttcctgattaaggaagaagcctgaaggaaactctgaactaagcccaaaggctagatcccatccacttcgaactttatgtttcaagcacgttggcatttgattttcaccataaagaggaaccccggtaaaaaaaaaggcttgcttctttcttgatggttgaacggaatcaagcccaagggcaatagctgacattgttgaattagctgacagaagaagcgaaaggtattctgatttaagttcatactcctaagcccttattcttgaaaaaataggcatatgggtgatctttttataagcaaggagctatctataggaagatacttctttgccaggtcagtctggtcggaaagaagcttgcttacaccttgctttatattgaaagaggtcttcctccttgagaaggtagcctttctatcatttagtggataactccttgctccattccgcttaaggtggcgcgccttagtcccataagcttatgcctatacctgctttcccttgaaataaacatagtaaaccactttaaactcgcagttagtcttggcccaactctgcccgggggttggccttttaaggcttatttcacttctttttttatttttctcttattgctaattggaactccggctccggtaacctcctgaaccttatccattacgtcaacccttcttcaacaaggggaagataggagggaattccctttttcaaggcccctaacctagtcctggtttggttctccagtggaaagatttgagataccttctcctaccctataaagtaagggagactgacactatgctttatagaaagcgaaatagtgataaggagttgcggaaaagtccccgaaaaaaggaagcgacttttcccggaagagcagaggggacagtctttggcccaggtaaaataaaacctggcctccccttccacccaagtggactattctctccttatggagtctaagaaaagagagatatccttgcgcaaggcgaaagatcgatgtccttcagaattctaaaaagatcaagaattgcgtgcctttagatcccgtctttcttgattcataatcaagacgaaaggtcggatgtacttgttcaggtcaggtctacttttggtcattcttctctctgaaaaatagaatattgctcaaagaaggtgactcgtagtcccttttcgagtattatcttcgctgtggatgatccagtcggtgtgcgtatgaacgaacggattccacctctttatgggctatatgccctgcttgtcccccatacccctttcagcaagggttgacgtggtctccaagaatcttcttccgacctctgaggtggtccgtcaagtcctctagcctagggtagtcaaaataaaggcaggattctctcgtcttttatttcccttttttctgagagagatgtcgtccttccagttcctgatgaattgagtccgccatctatttcatagtaatcacgaaaagcaagccctatgtgtcacaagcaggcaccacgggttctttactttttggtggggtggagggcttttgtgcattatagcacaggccgtgactacctttttaccttgattgttgctgcatatcgcccgcttgttctatagaaaactaagtgcctatcaattagttccaagaaagcggccggggtctaactagaacttcattccaatctcgatattgttggaattggtctcgaagaagcgattgcccgcgaaagccgtagccctttaattgcttaggggaatcggccttctttagtaaaagctttttcttgcttaatgctttcctatctcgactgattccccgtgatccacctatgagatcgtttgcaccggctttggattcaagaagatcggccatagaataaggaatgggaagagagcgagagactctcgattcgctgctctacatttcgataaagtggaataagaaaggccgtagtaccctaggcccgacagaataatgagaagaaagaggccgattggagaagttttgtttgagaggctaagggactagacccatcaaaaagcagaaagaaaatgcgtgactaagaaaggtaaccctagaacaagttgtcaaaagacttgacccctgaagaactgacccaagcaaggacattccggaagttggtcggtcaagacgggcactttcccttcgctcctttcgacctgatctcccacaaaaaccaatacaaagaaggtggaagtgggtcaccccatataagtaatatgggcaagtacgcgagatgtaaccaatagatttccatttttcaacgaagtccttctttcagcaaaatcgaagctccttagtgcaatcgatttcagtatgccggtttaatttgaagagaaagagggcagaaatccttacaatctcagaaccaaggagagaaggtggcgaaggatccggattcacttttttttatttgattcatacccgcgtaaaggcttttcctgattaaggaagaagcctagaaggcagaactctgaactaagcccaaaggctagatcccatcccacttcgaactttatgtttcaagcacgttggcatttgattttcaccataaagagggaaccccggtaaaaaaaaaaggcttgcttctttcttgatggttgaacggaatcaagcccaagggcaatagctgacattgttgaattagctgacagaagaagcgaaaggtattctgatttaagttcacccaatactctaagcccttattcttgaaaaataggcatatgggtgataaggaacttgaaacaggcatggacagaagtatgcccctccttttgatggtgaatgtcggaaatcctcttcccggatcacctttgatggacattcaaaaggatctgctaggctgtcttacatgtcccaaaaagcaagcaaaagggctcctttccttccccatgtggaagaagtgtacacacagggggcctctcgacctcagtatgaaaagcatgacggaatcgacggtggtcaatcttccttcttctttggcatctcgactggggagcatgaaaacaagactggaagagggctcaggtatcaacgtccttagcccgcattgatcaatatcaataagaatagcagtcgtataggtataggttagcgcttccttgcttgcatcctttcctctctttcttaatgaaatagatatagatgtctcgactgccgaatccttatcctgcaaacaactcgattctgttgattcactgtccatttgtccttaaaccggatgtttggtcaacgactttgacagcctttccttcacacaaggtttttaatccttctcccccgcttaggacagaaaggggaagtagcgagattacgattccttggtgggaaatcaacgaaggcagtcgctccagcagctttagtacttagttaaggccccagcccttcgcccggttcttctccggctccaccagcagcctttatcagctgctatggttcccttcccgcaatgcgaatctctatctctttgcggctacagcctattctaataggacccatattcaatcttttaagtgacttctgaagactagctagctctggacctacctatattagccatgagcgatcaccaagcggagttgaaagaaaagagacttgacatgccaaaacttcgctcgcgagctcggaacgaacggagcggaagggatcaaaagttccagggagaaaaaaaagacgagcactttgggccacggagccaacgtttaagacaaggctaaaggaggccatacgtgtagtaaactcctctcgttgtgaagagagtgagtctatagagcctacgagccggccgatccactgtagtggaatcttgtaggctagcgggcggtcccgcgcggtttgcattagaggggcccgctttcatcatccttccccagatctcttctattctgtgatctgggatgattagatgaggtttccatgtgtgtgtcttcgggagcatcttctcctgtgggatcatagccagtttttcactgcgagtggttatctaaagtaaaggtaaaggagggtgacagatcgatgagggcgctcctgcttatcggttatacccttcgacccctgttttagcagctagcgaaaaggcttcgttctgctgttccccgtgagtggtctaaatcagctgcggtagttaaggtttggaacaaatgagcctaagggaacgaagttgtgagcctttagtaatatatgaataagagatattcgaaataatcaaacctgatggttcctgtcctgaaacgaaggatgcgaagaaagtactgccgcctgtcatcatgctcaatcagtaataagttggcttcacctccggggatcagtccagccttgtgaagggagaggactctgttatcttgctttcctcattcgcatgagagacagacacattgtgcactcaagatgatgaatgccacaagagagatagaagaaagaagatctgtctcgattctatctctatctttcgacatctcatctctataatagagataatagtgggtggagaatccttgtgtattctactggtatagaatctttgtggaaggcgggaaacttccgtctagcggtcatgggaaagccaaaacttgtatataataagtcaatactgggtcggtcgagactctttcttagtgaagtgggaagacagcaccgaatcagacgggcacagaagaagaagtggtttcatccgaccggcgagataattcgatttctagtcagctaactgagaatccaatagagaaaattgcttttctaatgatttctcgatagaacgatttcttgtgagccacgaaacagataatccaagtcgtaagtacgaaccactcaatggagaatctcaggccaataagctacgactacgaaacgaattggatcgggttcagcgcttgaaagctatcgaagaagagtcaattcaatgctcaagtcaaaggggggagtccacttattcaatagaagagaagcctatatctgccgaccctacttcacttccaactagtgccttgcctactgtctttgaataatgcttcattccagggcgtaaaagaaagcttagtatagcaattgaattgaccttttgtactgaggacgacctatgagatggtttgaaccggttctcaaacctactactatacgaacagtcttcttcggctaaggctggcaaatccaactattttttgttaaaaagagatctcggatcaagggctatcgacccgacagtgctccgttggtccatttagtggatcctccccccaaaaacaagatcatattgagcagcaacttcgaggaagatagcattgggacatgctattacctatgtatggtgacgggtgtcatgccagagtctgtccgggtgggctcaagctaaagcaggagaagagagttagctttctgctgagtgagcccgaacaggagcggacgcacactagatcagagcaagtttagctggcccaatggcgcagacacctactaggatgaggcatagcgggaatggaacccacatctcgttgagctgctccagcaagcacccctttcggaagctcaatttgtaggaccggggagaacactcgcaggcgtgcaggcgttttgagagagcgcaaaactctaacttgagtaagtgccagccaggcaaaagggttagcctgaagtggtggtttagccaaagggagaacgtgcaacggttggattcagcacgctcttagaatagctgttccaatccgaacgcctatcccaacacggagagcttatccactacatctacataaggaatagtctagtccaatatttcttgtccttaaaatagaatatatgcaccgctgctgatcctttctaaatccagcttcaaccgagcatacgtctgccgcgggaacaggaagaacggaaattgacttttatgttgaagtctttccccttggaaggctggggggcgccttgcacgtcttggaaaaataatgctttgtatctgaagttattggcccatggtcctcagtgaggaaaggacctagaacagagaagagggccgataggaagttaaaagcaattcttatttcttctttctcgaaaacctgatgtgagggggcccactgggatgtccataattgaagcatttttcttcatcgactgtcggttttttactaggtggccgatgtctttgatgctttggttttcgcaggaaagggtaaggagctttagcccttagcgtgtgagctttgatgaagacttgcatcactattcgtttcctcgtggctcgattgctcatttgcttcttcctttgggcatgaagtgtttggtgaggcctttcttcgcctgttgaaaagctagcccttgctcaaagatcttttttatttagcactagagggagccctccaatcttaaaaaaccgatggaatgcgatctcataggcaatttgctatgagggctggaccccctgcatctgtagaagaaaggggaaactcaatcatgaaactgaatttccaagcggaaggatgagaaaaaaaaaatccactattgcaaaaaatctttccttcttttttagtaagggtgtcagccgcaagtatgagggggcattccccatcatagagaaagtaggacaagttgcctaaaaacttcagcttctttccaagctaaagatccaccctgtcttccatgtggggtgtctaaagacataccatccagacatggaagaccctacaagaggcgttcccaagaggccaccggaaaggatgacgactttcttgtcgaaggaatatgtgatggcggaacgcaaagttaatcgacgtggtgtcccagcttaaacttttgacttggtaaagtagaaggttctaccgaagcagggaagctctagggttttgctaaccagtgtgaagttgagttctatctttccctagttcatgcaaggctaaccttcgggtttttgctttctggaaaaacctcttaccagatggttgttcgctacagcctttaagtctcgcctagcctctcccgccgttctccaggaaactagcggctcgcagctgttcagccgcttctctaggagataggagatgtgccgctgactgggttcaggacacaaccatcgtccgaaccgtctgctaccaagtccatgggttggaacccataagaaactgaaaaagcacttctgccggtcgacgaatgcgtgctccggttgtagcagtgttgaatgaacggctgatttggaaccagaccgggtaactttaaaggtggtcccgatgttagattctgaagaaccgacggttctattggtgacccattcaaaagaagctggccgctttgactttgattagccaatcgagtgcggagggtgctgtgctcctcttcatttgttcccgttaacgaccacaaagcccttaactgctcctgctcgctacttgcccacttgcccttttttactactttgactagcgcccggcaaaggaatgattttttcccaaagccgacttcctttatcgagcggctctctctgttgacgataaaagcgatggtccgggctgggctgtctgaaataagcggtaattttggtcagtcctaatcctaataaataccacgtgaagcgcgtgatcacccagattcctaatgccttaattatcttatatatataataacttatcgacgtcagcccccttcctactccagctaatggaaaaatgcctttgaatggtcgtaatcgtcgacaacccaaccgacgtccaccataggctcggcgagctgtcctcctagatttcccgaaggtaatgccagggccttttcagtactgacgactcttgatgccaagaaggagaccaactagacgagacagaccattgttcataggttggttataagcccggagatcgaatcttattcttcccctttgagagggattctcgtgccaaccataggaagaagaactcggttactcatcttggatcggattggattaatagctttgtgctgatctacgaacgagccttctatttgatttatactatacttcttcaagtctccatcatcccgatctctctttccgggtttgcctgtccaaagaaaacagaacctcttctagttcaaggtcgaaatcctcaaaccaatcaaaatatgatttctagttcactattcttatgaatagaagttatgtctcattcatgtgatgagaaagctgagaatgaaaattagcaaatttcacatctacggcagattctgtgccccaaatcatttagacttattaaactaagcgggcggggaaggtatgacccctcccccattgaacaaaggggatccgtagggcgggctcactcacatactggataggtgactcggaattatagtgctagttccgttccctcggggaagagaaagcacgaatctattacaatcttagtagagaacagaggaggaataaaaacgttggttcttcgttccgtccttgacctatgatatgatcaatggcttaatccatccactggaccacctggaattcttaattaaacctttacccgaaaaaggaaattggattttctttttaaatcttcttttcttagattaagatatcatcagaccggtaagtttaagaaggaatgcattgattttgtgatttcttctttccgctcttcgcttagctacaccggcttacagatgcccatgtccttcatggatctaggagttcatacgaataatggctagcgggatttcgcattcaatcggagttgccttagttggtttccgaagggaaggcactcaagactctatatagtggtttatgcccttatttggcttcaagaagcattagaatcccttatttaacttgcggggcaatcaaggaatagaagctaccatcctagggggaggatctattatctctctacccagctcctcgtctagcagccaagaacaagagagctacaacactcaggttgttgaatgatttaggatcagatgagaaaaccaaccctaggagagaggctcaataagataagttaatcggagttcccggaaggaggtcccaccatttacttgactcttagaacctttgttggttttgggcaacggggatcaacttccaggacaggaaagggcgatccatctatttatttgactgaacctagttcacgagaaagagtcctagggatagacccctttgttttgcaccgagaagaaatcaatagaatcgtctaacgaatcgtctgatactagatgaagaggtaccccggaaagcaggaatagaggaggcacaggcctgccattagaagaaaccaaaggcaattagttcatctttgaataggtagcccggttaaccagacaagctggagggacttcctgccatacaggaaaggaaagacctgggacctgtactccccaacttgggaactcagcttatagcgaagggaaggagccgctttgtatgcgacactactatggtgaagagtgaaccgagactctttttattgagatttcccccgggtttctgcttcattcaagtcttaattcaagtaaggacaagtccttatcatcccgatcgggatagacgggcctgcctcgctgcgggtcagcacctcgggctctctttctgctttctgtctgtctacaagcggaaggcgttaatgaaaatgttcaagtaaaatagccatcaaatgcgaattgatgttgagatggagtccttacggaggtacttctattatcagatgaggcagaatcagaacctggagatcaaccccaaggactgactgcgggagcaaggattggattggagactgcatgacttgattcctctgataagatccatccatttagcagcaccttaggatggcatagccttaaaagtgaagggcgaggttcaaacgaggaaaggcttacggtggatacctaggcacccagagacgaggaagggcgtagtaatcgacgaaatgcttcggggagttgaaaataagcatagatccggagattcccgaatagggcaacctttcgaactgctgctgaatccatgggcaggcaagagacaacctggcgaactgaaacatcttagtagccagaggaaaagaaagcaaaagcgattcccgtagtagcggcgagcgaaatgggagcagcctaaaccgtgaaaacggggttgtgggagagcaatacaagcgtcgtgctgctaggcgaagcagcctgaatgctgcaccctagatggcgaaagtccagtagccgaaagcatcactagcttacgctctgacccgagtagcatggggcacgtggaatcccgtgtgaatcagcaaggaccaccttgcaaggctaaatactcctgggtgaccgatagcgaagtagtaccgtgagggaagggtgaaaagaacccccatcggggagtgaaatagaacatgaaaccgtaagctcccaagcagtgggaggagccagggctctgaccgcgtgcctgttgaagaatgagccggcgactcataggcagtggcttggttaagggaacccaccggagccgtagcgaaagcgagtcttcatagggcaattgtcactgcttatggacccgaacctgggtgatctatccatgaccaggatgaagcttgggtgaaactaagtggaggtccgaaccgactgatgttgaagaatcagcggatgagttgtggttaggggtgaaatgccactcgaacccagagctagctggttctccccgaaatgcgttgaggcgcagcagttgactggacatctaggggtaaagcactgtttcggtgcgggccgcgagagcggtaccaaatcgaggcaaactctgaatactagatatgacctcaaaataacaggggtcaaggtcggctagtgagacgatgggggataagcttcatcgtcgagagggaaacagcccggatcaccagctaaggcccctaaatgaccgctcagtgataaaggaggtaggggtgcagagacagccaggaggtttgcctagaagcagccacccttgaaagagtgcgtaatagctcactgatcgagcgctcttgcgccgaagatgaacggggctaagcgatctgccgaagctgtgggatgtcwactcttttctttgcagtatttttattgtgattatttttgagtattctattttacgcgtcacagcaattaggaattgagaatctatatctttagatcaaagaagggtctagctgttggaataatggtatccattgctatttgatcccttgttgttagtaaaattggtgaattaagcgaaggtacggaaagagagggattcgaaccctcggtaaacaaaagcctacatagcagttccaatgctacgccttcaaccactcggccatctctcctacataatgattatgaccccaaaaccgagtgaatagcgagtcagtcataatccatattccattattggataggtacgaccaatccattttaactttaactgaaaatttttcatcaaagtcaaagcaaagaacgatttttctttccttcgaggctccggtatatatcctccttccttggattagtactgggacgcatatatcaaaagctcagtgtgaaatttgaatgagatatatctttcttttttcaaattcaaaatttgagtaatagaggttacacaaaatcggagccagaaaaggaaaaagtggaatctggaaaagtattctctaagggtaatgtaattgagtgaaattcattttgtatcgtacaagaaaggaattccatttgtgtatgtgctcccgataaaaagaaataaggtactctattccattacatacatggatcgggttgaaaaaccagacccagtctctcttggaatcctgaatatgccaataaataattaattgtactaatccacatatgtctctctcccatcaatcggtactagttgaagtaatgaaaaaatcccctatttgtttgatgagaaatgcgaaacgaaaaagaaaaaaaaaaaagatcccccgttgggaatgaaattatgctccctgtcccccttttcacagaaaatggagagatgaattgatatatttattgaatccgtcgggactgacggggctcgaacccgcagcttccgccttgacagggcggtgctctgaccgattgaactacaatcccaggaaaattaggtgtacagcctaaaatcaatttagattcgaaccatttagtttcgctgtgttgtaacagagacacgaatgatatacttttttattattattatctaattatatataattattagatatataaaatatagtagactcatagtgggctaattcatgaattgaatcaaatggggccttttaatttaacaaatttgaacttaattaaactaaagagccacgctctttaaacgccctataagaagaagaaagaggcttaagtcatcgcttccaatccgataaagggcttttttattttccacgaaagtccgtcccttaaatttaagcagaggatataaatatgaatatgaaaaaaaaaggtaaccgcctggagagtcgttttttagtttttaagtggaatgttcattatcataataagtagtcgattaggagaacagctatctcactacagagtatactcttcctcatctttcattattcatattttatgtcctgggacatagatattctagatacccccttctattatgaatcgccaaagtcttcctacttctccattgttacaatcagatccgaaaaatgagaaatcaatcaaaatggacctgaattgaatcatgactatataagctattctgatattaagagattgaatatagatttcattcgtggaagcggacttttgatttccttggaccacgtaagaattcgtcgtccgattgaatctgctttttcctggatgctctataggaatccatcgctattcctttcctccaccgataaaggttcatcccgagtcacaagagcaatctcttttttttttttgaattcttttttcttttcgttatggtaatgcaatgcaagaggtcggaaatctggttgtttctgatgatgaaaagagcttttatcttatgtgaaatttatgaaaacccgaaatgtcggtaatgttagaagacgacctacggcatctgatggtcagatgcctacggtcggtatatctttgaaagctcagacggagagaataaacggactcctcgagggctacttaagccactttagtgcaaaccagaaggactggagctgttggatgttgctcagtcctgctataacttaacaaccaaaaagctctgcgtcgaacttcagccccttcgagttggccacggggtaacagcctctgacgccccacaccattgcgacaggagggggcttgcccatcagcctactttaccaagaggtggcaggagcgcaacgaccttagcccaaacctacttaaacaacctaaaggcttggcccggtctgaaagtagaccttgtagaaaagcggataggaaaggtagcctatagactcaagcgaccagctcggtgaaaacgaaccccgtattccatgtgagtcagttgacttcgattagaccagaccgccccagagaggaacgtgcccacgagggcaccaccagatgttgtagataaacctactaaagaagaagttgattatatcatagctgaccgcaccatgggctagcccatagacccactgcacgagtggaatactacttagtcaagtagaaaggccaacctgagagcgaggcaagccgggaacgggctgagacttacgattcgaagaccaagtcagagactactagacgtctcgcagagcgactctcaacgaggacgttgagactgttcgaaaaaaaaaagattttttggcttaatccgcctttactaaagaaaaaagagtacacttgtactccggctaataagggaaaggtttttttttcaaatccaagtttgactctgattagatccttagcgcaagcgctaagtaagcaagctaccttatgtaaaaaccgaggaaaataaagaaggtcaagtagaaaggaacaaggtcttacggcacgatcactatatcttttctttttctttctctctcctctatggaaagaggggatgatacgtggcgtggtatacctgatcgtttagtcaacaagacgtacgtaagtcgacatagctccatgtatatgttctttggagctagaaccaatcaatagaatgaaatgaaataatggtaagcctagggcgacgaacatggctcaagagtgtctatacaaagcccctctcttcttcactcaaagaggcaatgcaccctttgtttgaatggtacttgattcataaagaatgattcttttgaagttctacggactttctaaaaaaaaatgccacgcggagcgtgtcacgagatatatcgctctcggacttcttacggtaaggccaatgcaccagccagccagtgtggtggcgaacacgctgtgctctaagctaagctgtttaccttgtagacggaggagatatagaaagtgtgccgtgcttgattcataagattctataatcaatagcaccagtatattattttacttagcctgcctctcccatgactttccggaccaaccaacccggatctgccttcgcgagtctctctgcattttgggagcagagcatgcagcaaaatcgagcaatggatcttagaagaattcaactttgaagcacgactctttctatttctgtgctggcatttgacttgtctcccttcctctttcaatcgaaagactcgacgcagatagctccggtggcccccgtttctgcctctatcaggcggcgacagcccccccctccacacccacagcatagaggagctgctccttaatccgcactacaaccaatccaaattctctccagagcgatatatgatgctaaaccgagaccgagatatagagagggctgtccttttgttttgttgtctcgaagagagaaaagcactcatatgaatggtgctaattcccatgttctttctagtctcgtttggtttcgagagcctccctctccccgtcccttactcgtcttttgaaagccgtcatcctggatttgatttccgtatgccggggaaagtaccccaccctcacctttctacatttattattatatagaatttcctcgggtctctataaaacagaatgaaaagcccgggtggaagcacaaacaaaaggagagagaaaaagtcgaaaagaaaggggggaagaagtctagtgctagttcttactaacacttctttatctaactttcatttttgagtgctttctttgttctcttatttggattgaaagaaagaaaaaacttccctttctttctcttctttatttttgttttatcccttcgacgaatttcggctatgaccaatgccccactagctaaataggcgtaagaaaaagctacctgaaaaaagagcaaggtgcaccttgaattgaactcgacgaattgcgttttgccagagagatttttttagaaagattctccattggtaattcaaaaatagaaagaatataaataaaggcgcatacgcgggaaggggcccccactacttcttcattcaggggggagggggggagactagcctcattacttcccactgggcgagaggtgcacctaacccacctacccactcatcaatcacggtgttcagctgacttgcactgatagacccctattgtattggaatttggcgcccatctttttactgttgtcaatgaatctcttccatgttcgattctactctatgttagaacatttctgtgaatgctattctgatctaagtggtcttattctttgtcccgtgctaggaagcattactcctcttttcattccaaattcaagaatacgaccgatacgattaattggtctgtgcgcctctcttattacttttttgtatccccctgttcttcggatacaattcgatccttctacggccaaatctcaatttgtggaaagccttcgatggcttccttatgaaaacatcaatttttatttgggtatagacggtatctctttattcttcgtgatattgaccacatttctgatccctatttgcatttcagtgggttggtctggtatgagaagttatgggaaagagtatattacagcatttctaattcgtgaatttataatgatcgccgtgttctgcatgctggatcttctactattctatgttcttcccgaaagtgtgctaatccctatgttgtgcggagctgagtatcttctattcgctgggataaagcctttcctctgcaggggccttgtgcagtaaaccccctacgggcggtcgtccgtcgtcctaaagtagtccccgcgaagctttcgggaagaggggtagtcttgtgtgtaagcatagcatttctggtcgaacccgcccaacccaactaagaagaaccgaacctgacagacacatctttttccttttgggagggtactccgagtagtgggtacctcgtaggacctcgacccgcctactcgggtcttgtatggatatgcaggaaggggtgctcctaggtgtgtgtaggggttgtgtttgttcgcgagaaaggattcctcgtcaagtaagtttggggggtgtggacacacttgcgcgaattcgggtaacggctacaagggagaaatcgaaaggaaactgtacccgaccagggatggacgtaaactcgtaagctaccgaaggtagggataatcgtccaggtcttattgtgaaagaaaaaagccgccccgccacagcagacgggttgcttcctctgtcgtcgccggggagctcttggcgaggagaccttaggataagttgctaaaacaaaggggatgggaggatcgacccgttcagataattccgaagaaagactgttggcagcaggtagagagatttttttttcctcttcaaaacacaaggaaatgcgggcagggtagagctcggcagagggttcgagaatagggtagggtcctgtccttaagattcagataagaaaagagttccaaacctttatgcatgcacctccgtacaagtgctgcatacaagttccggccaggatgattgagaaagattcaaccaatttgaaccgctcacatcacaatagtagtagcgtaaaggccgtaagtcggggggcggccataacataaggctattactttcacacctctctctctatctatagatagagagagatccgctgcgtgagcaacccgactgtgccttacatgtgctctacaggccgcactccatctttcttcccaacgagccctttttttgatttggaagacgggcattgcgttcggttcgaaaggcatggttttcagtatgtctccagatagggcccccactagtccggctagctagtgagcggttctttcgggcgggaagcaggccgggccctacgggcgggcatctcccgcaacgcaagcaccattgttcgacaccacccgagaagcaaaagattctagagtccaggctgaaaatacatgcatagatagtggtttaatgccaaggccgacgacggaagctcgggacggagccgtatgaggcggaagtctcacgtacggttctctgagaagggagtggctacctactggagcttcgaccaagcaccaccggtcaattccgctttggggccacccctgactctaccattattataggggtatggggttcgagacaaagaaagatcaaggcagcatatcagttgttcctttatactttacttggatctgtttttatgctattagctattctgttgattcttctccaaacaggaacaaccgatttacaaatctcattaaccacagaatttagtgagcggcgccaaatctttctatggattgcttctttcgcctctttcgccgtcaaagtgcctatggtaccagttcatatttggttacccgaagctcatgtagaggcacctacggcaggatccgtcatcttggcaggaattgctttaaaattgggaacctacgggtttttaagattttcaatacccatgtttcccgaagcgacactttgttccactcctttcatttatactttaagcgcgattgctataatatatacttcctcgaccactttaaggcagatcgatcttaagaagatcattgcttactcctcagtagctcatatgaatctggtgactattggtatgtttagtcgggcggcggccgttaggtcacctattttgagttatggacacacaaggccaaaacatgtgtgccgggcgcgcgacccatcaacctactagcaatgggggagaaagcatagcatgtcgcaataaaagcttgattcgaggcgtcagcaaaacactgccgtctgttccaaaaacaaaagccccttagcgccccgggacgggagtgggggacggccctacgcgcaggcaacagcagcaccggctctacgaagtcagaatcgaatctttctgttggctttcccaattcattcgtgaataataattcaagggcgtgaagcgagtacttctagctgcttcgcctgcttcttattatggcggctatgttttcgtggcgaaaatgaacgaaaagcgagatgagcgtgctattttcaaatcgattgatagatagcctgatctgttctgatagatcgaaagagatagagagggaatctctcaagaataaggggaaatctcctatttctatctattgatgagacaactatctattcttgatccatcagaaagaaatcgatatgtatctgatggagtctacatcgtacgtagagcgcccaagcttaggccggctcagttctcttatccatcggtccaatgcactgggctcatctcatggaaggaaaagccaaaatgtagttgtcttgttcgccgcctcgacgcattcccttctctccccggtatcgtcccacacagaaagaaagagcgcagagccccggcccgacctgtaggtccgctaacgtaaagcgaggagttgagcctgaactggcgaaccgaagtcactttcggaaccatacttcctacagctaacatgtgtccagtccagcgggaacgcgcagcgcaaacgaacctgagctgctataccgaatcccccgctgaccatcggggaccgagtggtaaggccatgatccgcaggggaacagatcactcattcttccattggggacaggtgcacgaacgacaactccaaacgtcacacatccgccgcctacctaccgtttaggtggcaccagcgagatccagctaaggtaaggaacttcgtgtcgcggctgctccactccgctgcgctgcggtctcatgaactgaacttcgttgccttcccgcgcgcgaagcgaatgggcgctgtgccgtgggtcagtttcggggtggggagcgaagagagaccagaagaatgattcatttggatcgacgagctttttcagcccaaaaactaagaatcaatggaatgtccgtctatccatgaacatctattctatctgtatatctaggggatctctctatacatatagattttttttatggaatgatatgatcggctagccgtagccgcatatcagctacgctcaatgcgggatttctgttggatcagatcttttgggaagcttttggacctagcgaaaagggctctaagccttcacgcaagcaagcgcgagaggagcggagcacgaagctaccgcttcccccgaccgactaaaatacaacagtcgcgacctactttgattcaaaagaaaggcgaagggttaggcaacaagcaaacggctttctatcatagttgcaagggttccaaaccttaactacttaagtaccaaaggctgctttcggttggtttcataatggggctgttcactacaagctatcagcgctcagcgctgtcttagattgaacgttgacttatcttattgccgttcaatctctaaggcgggtttccgctgagaacggaatagtgttcgtgtccaaaggtgaacaaagccctagcttctagagttcgctgcttttcccaggccggagaagggcttatactgctcgcctttgtttgatatgttcattcagtaccaatacaaactaaaactacaccaaagtggaagggccagtatagaagctagaagtagctagcctatagtagtcggcctaaccaaagcctcacgacaacataaaattagccttatgaattgaatcttaagtagggggcttagcccgcccgcctaccaatcaaagaggctgagagtaagcgtaagctcacccggaagctcgaagagcttcccttcattcgcttcgcgggagccgcacagcacatagctggaagtcagagggcccatactacctgcctaacccctcgctccgagggaccgtagatcggaaagcgccttctaaaccaccccattcatccaaaagagaagggaaggggcctatgtatttgcatgacccctgcagatttaaccctatctatacccggagccactcccctagcggtcctgccaccacgccgcagaacgggagctcgtgtggaaccttttattctggcgtaacagcggtagaacgtaacaaaatattacggccgcctaacataggggacggaggtacggtaaactcggccaaaatatgagacccgaagggcccggcgcgcacaatcctatcctatccgaggccgagtttaccccttgcacttcggacagccgtccgtagcatcataaggaggacccccctttcgaggtacaaaaagagtacggtacataggaggttggtctttctcaacgtggtgtatagcacgaaaaacctttcgatacaagatagggccgttcacatgaaagaaaaaaatgaatcctttcttatcttctttcccgagagggaaagagaaagagggtcttatggagggaggggaaaggcttgggcctacctatcccgataggaccccataaaagaacgggagctgttgagaggttccatattgccgagacgaaggacagcacttctgtacgtgatcgtagtatgtcacctcgtctcgtccccgctgcatcgaagagtacctatgcactatgttccggttcactgataaggaagatagcgttggggtgggggtctacgatgtgatactaaagtatgaccgggggagatacatgctaactatgggtaggaagcaggaaccattatgtaaaaaatttcggggggttacagatctcttatactaccatcgatcgacagagcggaacgaccagaaaaagaagttaagttagaaagccgtatgataggtggtaactatcttgtacggttcggggggtaatcggcgtactccgatcagtgggggggaatctttggctctatcgaacatacagggaattggaggtagcattctaccgatgtcaagtcatggactggtttcttcagccctttttctatgtgttggtgttctatatgaccgacataagactcgacttgttagatattacggaggttcagtgagcaccatgccgaatctctctaccattttcttctcttccactttggccaatatgagttcacctggtactagcagctttatcggggaatttctcatcttagtaggagctttccaaagaaatagcttagtagccacattagcagcgcttgggatgattttaggcgcggcctattccctttggctatataatcgtgcggtttctgggaatttaaaacccgatttcctccataaattctccgatccaaatggcagagaagtttccatatttataccttttcttgttggaggggcgaccgtacgttaaactaccaaagaaactagggtaaaccaatgtgatcatgacattgtaggtgcttgcgatgggacggatgcgacttccctcagttggtttgggtggcatagcccgttgcataagtccccccctttttttttttccatttttttagtctttagggagccaaagcttgactttactaaactaataaataaggctcgcgctaggcgcttaccttttttggctgagccctatcttgctgggtgagactgatagaaagaaaggacggggggaaaccatgcatggtacttctcgaccctgtctccgagggacagttgaactagcgactcatgaatgctgccgggttggacgagccaataactcgaaggcgttcggtctgttttttgagcaagaatcacagccttaccttatcttcaccaggatacggactccaagttcttatggcagagcacgaggagatttatcatcaatatgatgattggaatggaaaccagaagcacgactggggtcttcgtggtccaagataatcaaaccatcaataagagtaacgtaagcatgagactttttggtagtaccggtgaaccggatggccgcggcgatggaatctgggacggaggacttgtagtatctctctagatctggcaaaagcgaaagaccccctaacataattcgaatggaggctgaccgctgagcccactctggcctcgcggggcgggcccctgtggttgcgagctggagctgccatagcttatggctatagcaatgggagggccccagcagagagaaaagtcaggataacgagcgctccgcccgccaagcgggcggcaggagcagcgggcaagtgcttggtaagccaacagcccagtgaaccgggcggggcactcgaagaaaggggggcacactgagcaagtacgagaaattggccccgctccgctttcttaaaagcaaggaccactacgggaggtcaaaccaaggatctatggaagtgggggctcgtccccggtcaatattggatcaaacaatagggggccgtaacactgacctcttttttttttttgattcaatacaataggggaaaagatcgtacagttccctaccgagacaaactctcaacggatcctccgcgcgctgggaatacctcttccgtgcgtctttctcgtggcgggaacagaacaacagggaaagacccggcccagggcgagctttatttatttaagagagaatggggagtgaatcgaaaggcttccgtttccgttctttgggggctttcgggcccctctcgatctttttcgtagttgagaagggggaaggagtctaaatcaatggacattaatgaaccatcattgatggacgttgcacatgacacgatcaattcgactcaaggtccggcgctaatagaagttgcttactttcctagtagcgaaggaaagggcagggcttttttcgtagtaatagtgggcgggtctcatgagatctatgccggccgtcggaatcaaacgaaggtcgaaggaccattcgattcattaaggggcatagcggcgccctcgcctggcgccatttccgggcctagcagcagacgggcgggccgtgcctgaattcagaccggaccagactcttctttgtttgagctgctcccaggcacgcagaccgaagatctcacttgtcctggacaagtacgtagagatcttcgtgggaccgtggagggagtctcaatcgatcttttctaggattccttatcacgccacacatggagatctttccattgatagatcagagggtccccccttgaacaaattcttaaaggttaggttactacctgcttctacggaagaggtttactttataccgcccggaggtcatatagatcggaatccggagcgataagaacgaaagggttggtgtggccacagctacaactactggcgcttcaaaaggcttagattctaagggcgctactgaaagcctttttttaggtcctgtaatagggaggtgtaagcctcgaaagcctttggtacttcggtagggcgagcagcccttaaaccaaaaaaaaagggttggaacccttcccctattttttttatgcatttcattctctatttggcccgcttcaaacaaaatgagaaaaaagggtccggtcaatagcatagctctttctttccccggtctcctttcgaaggagaggccttcgcattcctaatccggtagggtcggacggctttctttgccccagcttggcgaatcgcatccccgcacaacgacattctttgtttgtgcgccccttaccgttctcgctcagtctttcaacggctgggaaggcagtcgtagaaaggaagcctatcgccacgccgaccatcaaatacgagattgggccccttctcaaagatttgatggaatggcccaccccacccaagagcgcttatgtcataggggaactcatggctggaaacaatccttatggtttgttttgatatccggtaggaataataaaaaaaaagtccaggttggttggtgagcctagtgataggagactatctagcttggttcggagagcacttgttgggttaaatattttttggttgctaaatgttacggcctaaatgctgaactattgaccctacttgttcggatgggtgttcaccccaaagtgttcccggaccgcatgcatacatccgtaagtaacttagtgcaacatggaaaatttcattgagaggaatcagcaaagaaaagaaaaacgggtcaacaacatcaacatgtgtatttgagagattgtcctcgggctgaggagtgtccacatgagttcgttgaggtgtttacacaggcctgtggtcctcttttctattctgtcgagagttcggattgctccacctaagtagaacgaaaagaaggaattggaaaagaaaggggggagctattgtgaagcctagtaaaggcggaagcggcaaatcgcttataccgagttccccaacagcagcttagcttagtagcaacactctttctactggcgtggcgctgctggatgcttctgatcaatagaacacgaagaggaggaaaaaaaaagcttatgatgagcatctatttgagtcgatcatttccaagatctaattccagttttttcttatgtagtggaaacgccttacaatctgaagttttacgcttaagggaagaaatgttcttggtggatgcaggacttgggacccccagaatttgtatgcaagatgagcctacaggagtgccaatcaaccgagccaccaggtttgagaataaggtgggattcctggatctagtggccggtgaatcactgatcaaagagaagattttggagagattcttcatcgatctagtggccggtgaatcactgatcaaagagcgagcagccgccaggtttaatgatttggtgggatctacagatgtagtggctggtgaaccgcttcttcttcttccacgaagattcagacaaaaccgagcttggatggaactgaacaagatttggcgaacgaatacaaaggtcaaaggctttattattgagaaagtaaaaggaggttattcagtagccatcgcaggtttcattacttttcttccattccgtcgcagaaggaaaaggatatcgaatgatcgattcaccattgagaacattaaccccaaaaagacgaatattgtggtgttctaacagcggcagatcaaacaagaactggatgagcgaaatccgctgacaaaaaaaaagagaactttttgaattccgatgcctagcgtcccctgataacctaggattagtggtaatagggctgatgtggtatctcggaaactgggatttgatggtatctgtagagcggatcccatgggcttctcgggtggaggttggttgaagatgatgtgatgcaagtgaacgtctacgaaaaagctgtcgtaaagtttcgttcttcgttccgtcgtcgatcaatctatcactcaatcacaggccgctctgtcattgtctgatttttggttgtctgatcacactcgaaattatgtatctacttatcgtatttttacccctgctcggtagttttgtagcaggttgtttcggacgttttctaggaaaagaaggaaccgctataataaccactacgtgcgtttcattctcttcgatcttctctttgattgctttttatgaagtcgcaccgggagctagtgcttgctatctaagaattgctccatggatctcatcggaaatgtttgatgcttcttggggcttctttggcgaccgtgaagtcaccggatgaattgccgagtcaatagatcagatccggacgcggctgttgctccgcggcgatacggactcgacccgctcctacccactccggggtaccatagcatgtcgggaataaggggggacatactggacgtaaccactcccttggttgggggctgtgccgccctgcctttcgatcgatacacagttgaggaggccgatcacgaacgctacaggtgtgggagcgatcctggtcagggaaggctaagvcgvhdcntcgtatatgggtagcaagagggcgcttatgccccgacggtgdgdchctcttggatttbttgvaatatgagahggvatdccadddbbcytctckkgtcgtgvtctgtatcgwctgwatmacwcwtttggtctagtcggtggaaccggtgaaccacgcgagctggttagatgcgtggggcagagggctcgtagtaccccctttgattgatccagccttttcttcgcttcggtagtgaatcacctactaaaggggcaggcctgcacgccttatttgagactactaaggcaggcggtggactctttcattaggtaagggaagaaggggcctaagcacggcagatgccgtacacttgagtggcaaaggaaagcgagaccttaccttttttccaggcctgttcggacatacggttcccgcggaagatcaagttggtgagccgtgtgatgggaaaccttcccgcacggttcggagagcactgaattagaatgagaggtttaccaccacatcattgcatgcaaggggagctcgctcgattcgcagattggtccgactcgtaattcacttctgaccccgtgttcgatagcccgaccgtagtgatgttaattgtggttacattcataagtagcttggtccatctttattccatttcatatatgtctgaggatccgcatagccctcgatttatgtgttatttatccattcctactttttttatgccaatgttggtgactggagataactctcttcaattattcctgggatgggagggagtaggtcttgcttcatatttgttaattcatttctggtttacacgacttcaggcagataaagcagctataaaagctatgcttgtcaatcgagtaggtgattttggattagctcctgggattttgggttgttttactctatttcaaacagtagacttttgagccanttttactacttyttttttycarbrsagtctcyscywtrwratwwkcymaagtrtsrcrtggtmkccgatatgtaattanactttttattggtgctgttgggaaatctgcacagataggatcgcatacttggtcacctgatgctatggagggtcccactccagtatccgctttgattcatgcagctactatggtaacagctggcgttttcatgatagcaaggtgctcccctttatttgaatacccacctacggctttgattgttattacttttgcaggagctatgacgtcattccttgcggcaaccactggaatattacagaatgatctaaagagggtcatagcttattcaacttgcagtcaattaggctatatgatctttgcttcgnraatcwggcgatsntckgataygktgdbbccchtaatganthacgccttttcaaagcattactattcctgagtgcaggttcggtgattcatgccatgtcggatgagcaagatatgcggaagatggggggcttgcctcctcgttccctttacctatgccatgatgctcatgggcagcttatctctaattggatttccttttctaactggattttattccaaagatgtgatcttagagctcgcttacactaagtataccatcagtgggaactttgctttctggttgggaagtgtctctgtccttttcacttcttattactcctttcgttcactttttctaacatttctagtaccaactaattcattcgggcgagacatcttacgatgtcatgatgcgccattcctatggccattcctttaatacttctggctctcaggagtctctttgtaggatacttggccaaagtgtgacctgttagcccataagtaagtactgtgacgaagcggctgttgctcacccgacacgatcgtacgaggtcacaattcacccgacacgatcatccggggtgaacaagaattggggatcggatgcgggcgaaattcccgccaatggctgagatgttcagtcgactccctcccctttgtggggtcccgaccctacgagtgagcagaaagggaggaggaaagaggccctggtgaaccgtcataattagtgaacaagtgtaagcttcgctgcccgacagtatggagtactgaccacaccgagggacaggccctgaagcgaaggacgggaacgagcggaatcaatgtgttccaatttctggccttgcaccgaccatccaatggaccatggactaaacggccactgcctgaaaggactatgtccaggggaccgccgccccacaaggtacatctcgcgcctatgggccgctataactatcaagaagacactcgaaactggaaggataaacaaacccacccggtggactgccgagctacaagtcctacgacacaggagcgggattctctaaaagccaaggtcgtgggtggccaagagggcccacttggagacttgggatctcagcaggaaatgcgaaggttgcttaaagccggccggccaaagagaatcaactagtttagttctgatctgagtaggctcataatagggaataccctaaccctgggaaccggggcctggccatccttcgtttgcggtcgacgttccggctttgtccgtcgacagctgaatgtttcgatctggttcgattcatgatcgcatctgcaaaccttatcccgtgggctttagcggacgttttcattcttcacccggtccttagtagcctttccaaagtcaacctaaccggttacctttggaaaggcgctaaataaaccttcgcctttacgcctttctatataattgaagaaaattagatagttgtatatagaattagccagatcgtctgaagcatgaacagaatcgcctttgttctgaaggcctagcgagttccttttttttcaaaggcggtccttttctttcctcggaccgatgactcgcttgttcagtactgctaactattataggaggatgccgcccctcaggactaccagtagcttcggttgttgaatctcgtgcaagttaggttgtggttgtattggctgcaagcggaacgtaggcgctttaggtgtgtgttgaccatgcactctcgcttcgtgtaatgtcgtatgtatgatagaggtagtgtggtgattgacctcaatgctaatggtgatccccaaggttcaacgaatgaatgaagctatgatcgtacccggatagagatgatggtcttcctctgatgtctccaagccggccataatagaatagataggcgaagcagtcaatagcagtctgttctcgcctatcgatagatagcaggttgcttccaagctcaaaccatttgaaagggaattgctacttttttcttgttattgatagagtggtattctccgcccctgtcaaataaagtagaggggagaactggaagagaaaggaaaagagcaaaggattgacaagtctaatggggaagaatggctgacacgttgactgccttcgatactagaaaaaaaccaagcggtctaacctaaccccagggcggaccccaaccgaaaggcgctagacggactaagggcaagcgagataaagaaagcagctggccctatgtgtaaaaccttgccgcgggagagtctttctccaatgagaataaagaaagttttgggcaagacaagaaaggaactcgccctttgacaccaagggataagagctgattgctggcgatgacttggtaaagggaatctatgagagaaggttctcgaaccgggttacgaccgaatagagcgcggaaccaacgagttcagtcgaacaaggtaacgagtctaagggaaggatcaagcttgaaaggaatggacgggcgtaggcttaatagtgaacgcagaccccctgcttatagatatgagatcaatgacttaaaaaaaagaaagatgcaggaaaggaaaatgaaagaagaaatccaaatttgctttgggagtgtgagataggcagacggggagtacgcagccgaacaaccgctggggtttccagcagtgatagctgaactaatcagatgggccgccccaaacctggagctgacatttaaatcggaaatcaacatcgggtcccggctatccgaaaacgcagactgaagcggaagatcacaaaatgcaacacaacaaggggtcgttagaccgtagcttgcgcgaaggaagaagctaatcaatcagaattgagacagggaggagaaagagattttcgagcctgcaagcagcaagcaacaacggcttttcagcccttgcgcgctagcttgtagtttaggggtatagtagggtgcccctttctcaaacttttctataatataaggtaatttggaaccctagttttggagttttccccaaccaacctataccttactaataaaaggggcttccctttttcagctgcattgcactgccgcataaacaatggatccgctgggctggatgagcaaccttctatctggcctctgtaccaatagtcgagtggcttgcaactttcaatcagaaaaggaagattgagcaaggcaaaggagaaagaagttgtcccctcttctctggtaacccgccgccgcatatgtagaaaagaaggagcggagaaggaagaacaaccctttgactttggcacatgaggtggcgggtttggctaggtaacataatggaaatgtatcggactgcaaatcctggaatgacggttcgaccccgtccttggcctcgaggagtggtgagcagcacggaactttaatcaatcaaatggcatagtattagggtaggaggctttcctttgttatagaaatccacagacaacattctggaacttccaaaccaaagaaatgcaagatgagaaggagcttttaccttacgcttcaatagaatgaattcggtaagggtagaataggccctatggtcgatcgaaggtgctgtgccacttgaactcaaatctatctgaccttcaatccatctttgtccagccagctcataacaaaatgttagaccaatctcagggctgacacaaccgaattggttggggaaaaggaaaccccagcgaccaagcactcccgcccccaaaagcggagaccgaagaaccgccaggttgtcgaggacccgtctgaagaggaggcgggcgcccbctaagdbbavcrcsmtwcccgywwrysgtctkyykcttrwacamawaaccvhvhctayvmkaaawagayavcgctyathnnncbccttcadhbtvcaatvadaaaggttggggatggctggaaccaatcagaagtgcaaatcgcgcaagcgaagccgggaaacggaccgcagcgcaacgactaggactcgtgtcggaggagttttgagcgtgagctaacactcatgcagcggcaaggacccgcaactctcgaaggggccaccaaccgcccgaatcactgtagcaaaccctctctttactcaatggatagcgcttattctctttcaattaacaaaatgtgaaatgggrasaaagaaaaaaaagaggtctttatttaagaggctttgcaccggaaatagghmtaatgcagatccagaagaatggtctgggctttagaaaagatgaagatggaaggggtaaagagacagtcttttgaacaaccaagctgacataaggattctagctcgcgcccacttagagcagatggagattctcggacggggaaaagcggcactcgacatctattaaacaagaccaagaacaaagccataccatgccctcgggagaaagtagtgatgattgccatgaatgctgccctcgaggacgtgtacaagaaggtctttgccgattcctatcaacatggtgcatctcttagtagaggggcgtgaaaagtggagactttgaccgaatgaatagggatcaattgatagccattttcttgaggaagagaatccaggatgaacgctttttcattcgctatgcgctgactggatgcgtactcgcgtgatcaatcgatggacggggaattgcgtgaatgatgagaccggcctaacctaaagtcaaggctcttccctctcttgatggcgaatcttgattgactgacactagaaaccgattcggagaaagaagaagcatggcatgagataggcggcggatcaatttccgatagcgaattacttgactcgatggatggatggaggagagccctccaactcaagcacgaaatcaatgttgagtcaacaatcatcgagagggtaccaccaagcgagatcgagaccagccccttgtataggtatagggttccaaacctgcccttcttcaaatatcccataaatctaaataaagtagggacttcaaagcttgactaacaagcgagaaagttgactttgagaaagaaaggggcgccctagctgcaatcaaaagagcgctaacgagcaagaaagggcccttactatagatagggcgttagcgctttactaataacatatatagggcttacttttttcagcttgatcggaatcgattctatgattgaatagcagaagtgctacttagtagtagaaactcggagagacagacagagaggggactctttcatacctgctaactcctaggatgagaagtaggtcccttgtttttggcaggaagagttccagcctttgttgcccctcggtagagtgagtctacttagcgaactggcaggacgcggagatctattgatcaatatgaatctcgagagtggatggttgatcgccgcctccttgtcctggaggctctccggccggggaggggcttgctatcgtaaccttttctcccggtgtatgtgaaaaagagtgacgaactcatttttcttcggtcataggttggtccaaagaacgagagtcggcttccttaattaagtccgttgttcctcagtagctcagtggtagagcggtcggctgttaaccgattggtcgtaggttcgaatcctacttggggagatttttgagttatcgcttttctgacctagcgacccctgtccttctccttagtttctaaactagcagaatcgtgggacatcaaaagcggtaagttgattgttggtttttattcctcactctcgtataggttaacttggttcgttccattcttagggataaaaaggatccactggaaagactggagtagtatcttcattagccggaaggaattagtctccactagcgtcattcgaagaacgaacaagaaaagggttacagtttaggtaggatagatggatgtggcccaatggctaaagctctgccagcttcttgtagactgaactctctttaggctccgagttcttttttggggggatggtctaatttactagtggcaacgaagttcttggtaattagcaagggggaaggaggatctccactcatttcattcattcagtgcctgcggtgaggcgcgacccacaacaaacgaagggggaaagcttgctttgcttgctgtagccctattttagtagattaggcttggtaagcgtaagctatatttaagtaggctcgcagcttcgctcagcagaagagcctgactttttattatattagtaaagcgctagcgcccaacctatacaagggctttgaagggataggggaagaaaagaaaacaaagagggtcattttcttttaggaacatggctcgttcattcacttgctcatgaactcgcagcttcgccagaagcgacgagggggggctggggaaggccgacgactacatgagggggaagctttcgtagaagctttaccccttgctttacagagatagttatgaactgactaaatgactagattctcccggaacgctagctaagctaatcgtcttagttcccttcaattaaatcaataaggctttttgattgattcagggcgacgccccccttcttagaattagaacccattgaggggggcctcggcccgggaaggggagagtggccgagtggtcaaaagcggcagactgtaaatctgttgaagtttttctacgtaggttcgaatcctgcctctcccacttgtttgttgtagacttcagagaagagaaaagaggcattcgtcagcgtaggaaggccaaccgagcgaagctctttcttttttttggccgtgccgtgaagtgaaattgtatcgtatgttagttagagaggttggcgaactactacgatctatagatttcccatctatatccaatcccaacgagaatagaagcgagtcgcttccggcctgtcttgtagtcgtagtcttttagcttatgtagtcgtcggccttcctacacgcgtgcgtccgccagaatgcctccttggttcgggacgaagccaagccgatacatacgataggcgaaggaaagacccccatttcatagcgcctggggaacgcaagtttgatcgaggattggagaggagaggtggaagaaagggctcgggatggatttaggagtctttgtgcgagccgtatgcggtgagagtcgcacgtacggtaacgaggggggttcgcgtctatacgtgtagtgtggtgcttaggcctacccaccctatttgttccatgatctatgggtctactggagctacccacttcgatcaattagccaagattttgaccggatacgaaatcactggtgctcgatctagtggtatttttatggggattctatttatcgctgtaggatccctattcaagatcactgcagttccttttcgggcggctgtaggacggacggccgcctataggtggtagggtagggtgggtggtaccgctcagattgcggccaatcttcctaaccgcgcgcgggccgggcttagagcgcgtgaaactcatcactacctcgtaagggcgttgagaccatagcatgttacacgaaagcgccgctttctctgtagtgttgtcacacagctgcccgcctagaagagcaactcgctctgtagtgttgtcacacaagataagcacgccgcccgcctgctggccgggcgaatcgaagttatcttccggtcaactgtccacccagtcaagtgcaaaaaacacagtagaatcacgcaacgcacgctgctggtgtgcttcctgctcgcgaggaaagaaagaagagcgacagggttcagttcagatttgactgtttgcagcatgggagcagattccccaaaaaatccctgggaacaatgaaaaaaaaaagatatctcggtaacgaaaactatagggggctgtattggcgagatccaacggtgaacagctgcccaaaagaaagaccgcctggaagtccgaggacctttagtactgtactctacccccgaaccagcagccttcgcgccaagcaagaccgcccttgtccctttcctttctccattccgcctccttctttgctttgttccaatagagtctaaggctaagtggttcgtatgcctactttacctacttgacgaaagggaacgaactttgtttcatttccgggtttatggattggattcagtcagcctcacgacataatcagagtgaggctttggttaccggcaaacgcttctccaaaggcgaccctctcgagtttccggctctttcctagattgaagtagcctttcgtcgccctaccaaacgaaagaagtaactatcaaacagctcgccctattgaagtaccaaaggtgcgctcagcctggtgactaggaaatgggtttgcccttgaattgaagtgatgaggtcggaaagagggaagtagggctcctattgactaaaggttggttcttcgctttcctttagaatgaaagttgctatgaagcccctactacttactttgtttgattcaaaaggcgaacagcccccccaactagttgtatggggtggggtgcttgtgaaaagctgctttggatatgagtaattcctaaaaaaaggcaaagtccggtatttgacgaagatctttctatcaatagataggaatgagtgttcgatataggggataggatccatctgctctttatctctccattttttttagagagagcagatataacgatagaaaaaagaatcgggagatgataaaggatagatagacatctaaagggatgtctattctattcctctttttttttttagaaatatatatatatatcgtttatctatctcttgtctatctatcattgattctcaagtcaaaagacttcgtttttgggttccccgaagccccgaatggaatggatcgtttctgccaacgaaatgaacgcggagcccgttccgaatgcttctacgatccggaagttctcgcgaagagaataagatgctgctccccttccctctttcttttcccgctttgctaatcttcccctctaacgcgggccgggcggcgacgggcgcgggaggaagaaacctaagagaagacgctcgtctcttaggtcctttttttcagtgcaacacaggaaagcgccctctttttgtcatccctgcagctttccagattttgtattgaacgcatggcgtagctaggacccttccaattctgtttgagcctatgttcaagccaaaaccacccccaatttgactaaggctggaaagaatgcccaccaagttcagataagggaatgctttccccaaccattaaaggaaaggctcgacgaagggagggaggtgcggcgggggaaggaaaacgctttcggagatcaagatttttttttcatcgaaaacgaagaaggccgaggatggcctacggtgcgtcttatctgaagggaacacgcttttttgaccgccgtggtatgattgccgggccctctcctcgttccgcccttcctattgggatagcagccttcgggctttgcctgccctttataataaaaaattccggctcggcccgggaaagcgctggcaacaacagaaaggaaggggtccatgtagctgctgtgtccgcccccttcttagtcaatggggcacagcaggttcggcatctactacaaaagagagaatccacttcagataaccacgtctctgctaggcagcgtgtggaatggccgagagcggacctttttggatatataatccaagtcgagagtagagttagaggaaaagccgtctgatggaaaactactttcacgttcggttcagagagcacttttttcgttgagaattcctcgttccctttcgtgtgaattccccagcggcgaattcaaaacttgtggggccctatctattccatctctcgagccccgaagaaaaccccctacccttcggactccatatatcttttgactctatatatgtgggcacctgatatctatgagggttcacccaccccggttacagcattcctttctattgcgcctaaaatctctatttctgctaatatttcacgtgtttctatttatggttcttatggagctacattgcaacaaatcttctttttctgcagcattgcttctatgatcttaggagcactggccgccatggcccaaacgaaagtaaaaagacttctagctcatagttcaattggacatgtaggttatattcgtactggtttctcatgtggaaccatagaaggaattcaatcactactaattggtatctttatttatgcatcaatgacgatagatgcattcgccatagttttagcattacggcaaacccgtgtcaaatatatagcagatttgggcgctctagccaaaacgaatcctattttggctattaccttctccattactatgttctcatacgcaggaatacccccgttagccggcttttgtagcaaattctatttgttcttcgccgctttgggttgtggggcttacttcctagccccagtgggagtagtgactagcgttataggttgttgggcggccggaaggttgccacgagtaagtaagtttgggggaccgaaggcagttctccgtgcaccggacacgtagcttaccgaatcagttgcgacacggatgggaatgcatgctacgaaagatagggtcgagtctgatacatcaaccgtctactcaatatccttgtacgagtccacaatgactacacgagatgaaccttggtttggtgaattgaagttggccttaggtgtaataggactcccagttactgcgcgcgatcgtatactgaggtgctccccgccggttgttggaacgacgcgagccgggccgggtctcgattcagaaagatgaagggcccaaaagtctaaatagggggttacaaattccccatctcattgggggcggaaaacgaatcgacatctcgatgtgatacagccctttcgattttagttgggaaagaacggcgaagtccatccgaaccgtccaatgaagaataagaggagagcaaagcgccaatggcgcgcgaagcgcatgcggaacgggcacggagaaaaagaagtgtggaggagaagcagccgagctcattcccttcgcttcctgggcccaaagcagtgcagtctttcctggccaaatcaaggatttggggcttcttgctacgctacttaactatataaatccattttttttagtaatatatatgaatagaaagatagatccatccatctatcctatccgatttcgattttgatatctaaaaaagaatcgatttcattcaacgtttgattcaaagaactgcgcttagcccccccgctcatgaaacggctctgctgcaatggatggcagagggtccgtagtacccgaagcactggagtgatccagtagccgggaaggggcctagaagtgcctactactacaccacactacacttggctctacacatttacagagctaacccctgtccagtgcctggcagagctaagggggcttcaatccttactctttatccccatcttcgcccaggctaacggggccttacttattcaggggggagagtggagcctcgaaaagcactgttgagaggaagatccttggcccctcttcattctctacagggttccaaccctttcttcaacataggtgacaacgagccaggcagagatggaagagatcaaagacgggaataagaagcaagctcgccttcctttttgatcattttgatagagggggatgaagaaagtggacaaaacagactcgcatttctcatcgaacaaatacaggaaaggaatcatattgaaaacgctcctaacccaaccccttccttcgtagagcccgtgtattgtaagtgatccgaacctgcccggagcgagcctcccatagaggcaagtgaagttggtgagccgtatgatgggcaactatctcctgcggttcggagaggactcagctgttagttagtacccccttggtttcggggtggaccttttcactctattttattatatacgcttagcgaaaagaatgttttttgatacacctaggacatggattctatatgaaccaatggatcgtgacaagtcgttactactagcaatgacttcctctttcattacttcattctttccatatccctctcctttgttctcagttactcatcaaatggcactcagttcatatctttaagttcgatcattgacaaggttcaaagaaagggtgggccattgataaagaatcgattccaaaccacaatgctagcagatggcgggcctccgcttttcttttcattaatgaaacccgccagttattcttattaggaactcaaataaaaggactttcacttagagtttgattagcataaagtgccagcccagctaggctgagttccgttccattgctttcccaataagtgaagtagcgaaacctccctctgaatgaacagaagcggaatgcaactcaaaaaaagttctaggatcacaatgaggtcccacgaaaaaatgagctgaaacggagcaaaagggaaagcccgcgcgcgggaagcaaagtaccatcgtgcacactcatcaaaccaatgatcgctgccaaaaagacggtgagttcgaagccacttcctatatccgatatccgaggagatggaattgtgaagaacctgacgaagatgatgatgtccaaaacccggtagaactaaggtagttcagttctccgaggtttaatctcctaccttgcttccattctttaatggcattctgcagttcaatgtcggcgaagccttgcattgaataggttgttataagcctgacttggctctagaaagcagattcattattatagccttataatctaagaaggtcaggcattgtgctgtggcataagctttgtcttcctctacctttggattgagagttcatctggactgagtaagcactttaaagaaaggaagtaaaagattcaatcagatcagaagaagactgacttcagctttgacttcctcccgagcgagagcgatcaaaggactggcggagggaaagcaaaatcagaaagaaaaaggatcgagacaggactctcttagcataggctttcagccatttcttcctatagtaagtggaagtcataaatcctatccatcttgctcaaaccctttgcacgagtcagaaagcagtctacttatggcatcggaaccactaatgccgcatctctcggtgagaaggaatcaaggaaagaagagaaacttcttccttctttgatcttctgccccggaaattggaaacgtaaaagtaggctgtgggactgattcttttccttctttcaggcaaaataagcgtctgccagcggtcagagtgtcaatttgtactcatgattgcacatcgcagtcgttgcgtgcttgctttgcgcaccggcacagcagaattcgaatccgctggcttagatgagtggctcttggcttactgagaagggctttctgtaactaagaaatgagaattgttgatccatatgatctcaggcaactttcgttgatgaaactgacaatttaacacttagagattgagctactcagtcttgcttccatggatatcttaaacaagtttgcttacccatcgttatctggcgggaagtgagccacctagcctaccttctctctttctcttaagcaatttcatgtcaccttaactctgcccttgggaaacttctctcccttaaggtagcattcatagttttgagtcaacaagactttgattttctccatcgcctctgaagttcaggtcaaaatcagaactggaatttgaaatccagtaggaaaaagaaatgcagactttttcttgacttttgaatctattagaaagagagtctctgaagcctttgctttcgaccctactaggataggacttagaaagcctccttgaactacggtttacagttcactaagatcattctggccttttctcttctagcctggttagttacttctatttaccaagaagtggaattagatagaggagaccgagcatagaaatagaaaaggattggatttgacttcgaatggatggttctcgctaatccccatttctcagattgtgcttcgtggggggagtcggatattggtccgtaaaagggtcaataaccgagctgggtttatgctccgtttttccaagaacggatctagtaaggcgaaaggtattccccaatgcaaaggagtctaatcaaagcaatcctcgagtaagaaaagagaaggcgctacttagcgctattaaataaagaatgaagctccgtgcgacacccggctcccaaagaaggaaatgctaaccacagtttcaatggtaacgggaatacgcctgacggcgaaacacagagagtgacgcttccatcgcttagatttagggcgatagggcgccccacagatacgaactagaaagcaccattgcatagggaaggcttgctctgacaatgagtaggctacactagtctacgggtacctagtctttaaagtgggcgaggctaaccctatactttcttctcaaaaagaggtcgatcttccgctctagatctttcaaacaattgatttccatattggtatggtaccctttcttcatagaaagggcatttggcttcctttagtatactcctaacaacgaaaacaaggaaaaggtaagtgaaaaataggacagagattctgaaagagggcactaagagaagaagaatgaataactgttaccgaggcccaaggagatgcagcctagcccttacttcaccagattcaatagcagctcctattgcgatgtggtaaggctatggcatcggtttacacattcttgacttgaaaagagttagaaggattttcgccatataggaagggtctgagaacaagagccattcgtggtcacatgaaagcggcaatagagaatcctcctactgctaggctaagggcaaagatcacagcagtacttgctaaagtcccctatcctgaacgtgtgctatgtagaaagtagttagctaggcatcataatagccatcaaccgtcagccttcgaaattagcactcgattagccggcaaaagcgctcttctttccattttatgtgattttaagatggatatagatagaactcgatcgaactaaatgctattgtggcaaactcgtgggaaaagagatcgggggtatcgatgtggatgaaaggcagagatgagagcgacagaagaggagtggaacaactaccttcccagtctatcgggacctttttggtttatttttgccctgggctgaactccctgaatcccgggactcgctccttcgctctccggacttcttccttcaacaaaacaaggtttttctgatgagcatctttcgggactttctcttgttgttttcggggagctggctgggaactcccactcaaaatcaaaacaaaaaaatccttactacccctttaattttcaaggagcctccaacctacgaactctgaattcggataacataactatatttagctgaactccctttcgctttagagaagacagttcgagcagaatcataagaagaaggtaagggacaaggtgccaatctattaatctcaagcctgcaaaagtcaaagtcactcttcttcagaagaaattttccttgtagccttagaggctaaacttcagtttcatacgttctattagtaggtctcttgaaagcagtttcagcatatcgtctaaatgtatcctttttttacctcttccctagtactgatctcaatccttatgtcatctaatgcggctttttcactggctagcttgctggatggattgcacctctgaaaagaactaactatagggtctaatcctgaaaaacttctacttatacggggtcgggtttgtgaactactgctactggtacactaaaacgaaatttagggactctcataatccatcaagttcttttttaggccatccgcctatttagccacattacacgctctcttacaagcccttacataagacataaggaacaataagtgtcttcttcatcaaattcaaatcaaagaaattgagtactactatggatgctgcaaacaggctttctttctagttaagttcttagaagagcgattggtgtaggctcgggaggcatacgaacatggtgcacttcgctttggtttaaaagcgcttaaactagatagctgggaatgcgttaggttatggtaatttatatagaatataggctgaaaaagtatctattaccttgaattctcagttttaaaatgtcttaattaataaaataaaaggtaggcccttagacagactgttagcgcttgttaggaaggggaagtcttgcattgcaagcaacctaattcctatgttatagccttcgttcccttctctgtcggtgtgctccgacagtgaacccgagatatctggttcataaggttgccaatggggctagcggcgtccccgcctcatgaaagggaagcgatatcattttgtcgcccgatggaagtcaataagagagaaagcacgaactaggatcgacctgcatgtgaggcaagtaaaagctgcgagtgaggaaagctggttgtcaaagaagttatggtgtgcccttcattaagagtaagagcgcaaacttggcatttccggtccggaaaactctcttattttttagaagtttgccaggaggtgaggtttaaataggcttccaactgtgttggagtttcagactcactactaacgaatgggcttcgaacagctcttttttttccaacaggctgcaaatcataaggataagcctgaacctaaagctcaaggagcatagttccaattcaaactacctagagagaaacctatcatagtcctagctataaggggttttcagcgaaagcgcgtgttcttagattcgtaagaatatgaatcgtcaaaaggaagatgctggtctttcattcctttatcattgaaggccttacccataggataggaatcccggagcccataatagtcatcgtaggcccagaactatagttcagaggaaaccgccggaagactttgtttaggaaaagaaagacgaagaacgccattcctttgccctatgcccttcatttacctgctcaaaggaagaaactaaactataagatcagagaaagcaagagccttcgatttaactacatcagtagaaccggccttaactttctttccatttgaagaattcctgatgatggttgataaaggctttccttccacttaccgtagttctatcaaagtcagccttaaattaaagcttcttgcgaaggccctgcctttttaatttgattttttatttgatcgaaaatctagctaaactaaagagcttcttttaaagattccccgctagagcacggaaacctagagaatagctagcggattcgccaacatcgaaagcaatcagacttggtttggaaatctccgcgcttgctatgttatatcaatctcaattgccgattcactgatattggcaactttcagatcatctagttattatccttcaaggcatagggccgtgaggtacttacttttagcgcagccgggattgattaaggtagttgttcagccgagggaaagaatcattcaatgctagtgaaagaggaagctgttcccttcgttgattaccgtggtggcttctgtatcatgatacagagaagacagaagcagcactcttgtcgaccgttcatggctagcttcgaacaaaagaaaggctaggcgaagaatccatcccttaccgaaggaagattgcatcgctagttgactcctcctcgtcgacagctagcagtttccggactcgcttttgttgccttaaggcttcctcctaaaggggaagacctgctaaggcactaataagagcaacagtagcaacagcgacccccctatctcttaaagcttctgccttcagacgggatgatggctaaacaatcatttggtaagtagggtgggtggactggtgagccgcttacgctttaagcgaggagacaggagctatcaagcttaaagtagtccctagaccagacagaggttctagggggggtccggatagaggattcctttaagcggtctgcccgcagatgtaggataggaaggcggcctgcctgctaaccgaactgcgtaactaaagcgactccttcttggtgtaagataggtcttggtccgattcacctatgtcagttcgaacctgacgggtcgttcgtgtggagaatctctctccttactcaggatttctttatcttcgaggcgaggcatattcatatatatgtcgaagaaggaggaagtgtctccatattctatttatgctcatagaacccgaaaaaaaagaatataccgtcgtttaagggccaaggatacgatgtgagaagcgtaggtcggagtagcaggagtatgcgacaagcagttgcatgttcgatgtgggagatcttctgcacttaatacacactctttcgtgccttggttcgccatcatttggttaaacaagaccacatggggtgattgaagttggaaacccttgtcggtggaactaacgaagcaaagcgtgcttggttatcctagcctaggtggaatggaattagggacgcttgcttgtgcgcctaagactcctagttaaagagcctttttctgatgaacctttaatggggatttctagcaaatttttaggctatcccttcggggatctagcatggttcccctagtccgaaatctagactctgtctttaaccttcgctcgagcgatggaaagagtctttacacaggactggtattctaagttttcttcgttctctgatatcttactatagaaggctcgaagagctatgcttgataagaagagttagcaggcgagacatcatctcgtgttaacaataactcgtaaagactagtttcataagctagctttgaataagagaaatcgtagcctagaaagtcttgccaacggaaagaacagcagactcaatagccgctctagacgccctaaagggaagtttggcgctagcttcctaaacaggattttctatgaggtagaggcccggccgcgcaaagcaagaggaaataggtataggctggatcaataaaagaaagataaggaaagtgtacaagattccaatcttrctgtacagcaattggggcattggtctttgcagcgttaatgctttttgctggttggtttcattaccataaagcggcgccaaaattggcttggtttcaagatgtagaatctatgctgaatcaccatttggcagggctactaggacttgggtctctctcttgggcggggcatcaagtacatgtatctttaccgattaaccaatttctaaacgctggagtagatcctaaagagataccacttcctcatgaatttatcttgaatcgagatcttttggctcaactttatccaagttttgccgagggagcaaccccatttttcaccttgaattggtcaaaatatgcggaatttcttacttttcgtggagggttagatccagtaacggggggtctgtggctgactgatattgcccatcaccatttagctattgcaattcttttcctgatagcgggtcacatgtataggaccaactggggtattggtcatggactaaaagatattttagaagctcataaaggtccatttacaggtcagggccataaaggcctatatgagatcctaacaacgtcatggcatgctcaattatctcttaacttagctatgttaggctctttaaccatcccttactatgaagggattaagccactatcaaagcaggaaagagaacaactaggatgaaaggtattactaatattgatatagtgacacaggatgatagaatgtaactaggataagcgtccggttagaaccatgggaagattagaatgacctcactaggaacctcattaaagatagatagctaccttagagagcttacacagtcaattgatctatcctaggttgaggaatcagggaagaaggctttcaagtcaagaagagattcgctcctaaggaggaaataagggactcatatcgaaagggcttacaggactaaaacctatatctgagagcttgaaccgacagcagccccatgggagaacctttcatcttcatctctctcacttaaaaaaggcttagcttgggccttagcctaaaaaagagaatcaatggctgcagatcgtgcctttcttgcagctttggctactgaacttatgaacagaggacagagccttaagttaagccgcagagagaactctttgttccgtctttcgggttgtagggcgtagggagtaggcgagtcagtctatagagctagttaaagtcgaaaacacgttcagctccagtgtcttagggaaatccatcttgtcgctagttgagttacgggtgccagtattcttggtctcgtcgtagaaagtctttttttgctgtccggtagtcgtagtccaattcttctttctcgggctttttttaagatttgaatctgaaggttcgtaaaccaaagctctttacgatccaaaagaatctttctcttcccttatccgcgattccggttctcgatcgaaggccgggctttgaatcgttttattttagtacacaacactcgcaacaaaaggcttatagccgaactgaggcagcaagcggattagaaaagatagagtttccttgattgggaaggaaggaaggaactagtaatccattcaagaggaccttacctttgagttctcgagtgaaagggtccaagccataggaaaatatccagtttatctcgcaacatatctagtttatcctgaagcagcatttctcgaagtagcattcccataagtagaggatgaaacccttgcttctttatcccgacgagggtttatgaatcactcaaacgagcctttctagccgcatctgaatcggcatccctatccatatgtttatgcgcaggggcatccaaatccgaatctgtagaatctattggggaatccccatccgcacccgaattggctaaatctagtatagtgggtcttgttccgatgcgggaaaaaatctttttaaaaggcatctcggcgaaagaggactgagaaccataaggcgagcgccaaaacgctagcacaaactgctcccacagacacgcatgataagggggtgtggggacaaccaggccaccacttttaccagatatgggtccggacgacccaagagcccgccactagaacccaacccttaagaggctaaggtccaaggggctaccgcaggaagtcagcttcacctgtaaccttaaggaatacagaaagttacccggaattcctagcaaggactttgcctgctattcattcctaaatccctttcacccttaactagctaactcgatgggacgtcaacagcgggaatgccaaatgcaagacctggacctggttcacgcagtcaagcagcaaagacctctttctcttcgggagctttcgtaacggctataaagaatgggtctttcccctcgtgaaaggctattgggatcgatcccttcaaccctccttggcgtggaaggtcgcaagagaaaagaaaactattcttcttagctgctttttcaacctacccgaggtaaggaagtaaagcaaccaatagcctttttacctactatgcctttcaccgggtgagcaaaaagtagttacctttagccgggtcttccttattaattattgataaggcacaggggaagcattatccttataagactgttgctaaacaaaagcaattctttttcacattcaaccatgagagggcaacttgagcaatcaaagctaccccctcttccactgctgactatgaacagttgacagctaatgatttctactttactaagccagttcggtaagttaaggtccatgcttgaaacgataaaaaagaggaaggggaaggggtcgcccaaagctgtggagataaggtggaagataaaaaagctatatttaaaataataaagagaatctcttcaaattcatattcaaaaatgggattctcaactatacttgactggaaaaaccagccaatctactctcctttttttggtctcccccctgtaactttataaatcataagagaagaagaaatcgttgcgtagaaagtcgtgcttactatctcctccatctaagttatgtaagaggaaaagagcgaaaagcttacttttaggtagtggcctaagcgctaagaagctccaatcatgctactcagactatatgcttaacacatgcaagtcgaaccttggttttcggagttcgaaagagaaggggaagaagcggggtagaggaattggtcgactcatcaggctcatgacctgaagactgcaggttcgaatcctgtccccgcctaatccatctgaggcccggcctcaagatttgagattccgtaagtaactcagtgactgctttctaagaagggcttggaagaagaaaatgaaataggaacaaccgcgctggtcgtagagctaatgaagagaaatcttacctaatatgaggatcctttttgctctttctcggctctgtgttcgtggtaatagtgttacttatctttcgaaagtccctacaggtcatagtagttcgcgtctccttgatcttggttatacttgtgaattagcagctagtaagtttttgattttgcttcttttttggaagcaaagaatgttgcgacgatttcccgtcttaaagaaaatatcgcccaagatgtatatatcgatatgccttttcatttatctaattttccttaaagtaggagtatcgcttggatacctcttgatggacgagcttcaaagggctgtcgctccatttcttcatgcatcgggggggggaatgtctgggtctgaaggaaacctggggggtagcagtggaggccccggttggccgtccttcggtgtaggcctatttgcggataatagtagttgttattcaaatgacgaagagttcgcccagccaaacccccaaaacgcccctaatgcagtggaggcagtccttccagaaccggatatggattctgtgaggggtgtcatcaagcagaggttacttgtgcaccgcttgggtcagaaaaatttctcggtttccgagaaagaaattgaccaaatcgtggagctcaagaacgacattctaaatagaatgggcgaactggaccccgaccccttctggactagccatcgaaggaggctcattcgggactacatacgaccgcacatgggcggggagtatagaataaaggttttgactaaaaatttaaacttattattgggggaaagtccaaccagctccttgatttataaccaactgatgaaagagaaagactggttctttttagatgctccatttcaaggccctagatagagctgaatcatatgtggttggtctgttccgatcggtccggagggtggagggtggaggttggaggttggttgaagatgatgtgatgcaagtgaacgtctacgaaaaagctgtcgtaaagtttcgttcttcgttccgtcgtcgatcttcctttcctatttcttccggtatgccgctccgccaacaaggagcgaaagaaccaagttttctgtggtgatgtcagaatttgcacctatttgtatctatttagtgatcagtccgctagtttctttgatcccactcggtcttccttttctattttcttccaatagttcgacctatccagaaaaattgtcggcctacgaatgtggtttcgatccttccggtgatgccagaagtcgttttgatataagattttatcttgtttccattttatttattattcctgatccggaagtaaccttttcctttccttgggcagtacctcccaacaagattgatccgtttggatcttggtccatgatggcctttttattgattttgacgattggatctctctatgaatggaaaaggggtgcttcggatcgggagtaaccactagtgagagggcaaaaataggggggaaggacaaaggaaagagcgatgcctacactaaatcaattgattcgtcatggtagagaagaaaaacggcgcacggaccgtactcgagctttggatcaatgtccccagaagcaaggagtatgcccgcgtgtttcaacgagaacaccgaaaaaacctaattcagctccacgtaagatagccaaagtacggttgagcaatcgacatgatatatttgctcacattccaggcgaaggtcataatttgcaggaacattctatggtcttaataagaggaggtagagtgaaagattcgccaggtgtgaaatcccattgtattcgaggagtcaaggatttgctgggaattccggatcgaagaagaggcagatcaaaatatggtgcggaaaaacccaaatcgatatgaatggaagatgcctctggaacttgtttttctcggtaaggataggtacgaagtcactcgactgaaaggagagggaacaaccacaacgttacaccccaaaactatacggagcccttccgaatgacctagaatatagtctactaaactagccaagaaagagtctagtagactatattcgcccgtggaggtgagtggaggaagctgtgaagcttctaactctaattaccaactcgggactaaattagtaaaaagcggcattatccctttactcaatcccccctcgcttaccacctttcccgatcaattggtttttaattatttaataagaaagatggcaaatcctaccattgtatttccttttttcatttggatcctatcaacttttagagtgtctagattaagacacttctcgtattcggactatcaagatcgactaaatgagagtgtggctgacatggtaaaagaagaaataagccacacttttctggacccctttttctctttacaacgtcttactaccacagctattccactctggtagatacgaatagtccaaacacgtatcttcgggcgaatagcctttaattaagcaagggcgagaccaaagcacttaactatagaaattacttagaatagtgaaaatcggcactactcaagccttcttatccgcgagtgctactcgcccaaggaagtctctagcggttcaattcaattaggtgaaaactgtctcggatgccccttcctcctcaacccgggagaagaccgggctttagccgcttgagcgcactcgtctctctctttaggggcctttgggaatcttgttcaatggggaattctgcatccactttccagccggttgacgatgtggcatttcttcctaaaccttcagtcttgtcctaagcgaaaggggaatcggattcttgcacaagccattctaagaactgattctagcaagacctattcgtgcacaagggaatctgtccatttacagcaagcaagccgcaaaaccaaaagagtaagacatggtaattgctacgctactctagccagtcgaatgataaaggggagtggaaatggaattgatttaaaaaaaacagctagttccgcatcaagaccgctttcacctgaggaaggagcaaaataagacatacttttattaacctttctgtgctattattcacttgcccaagaaagggctatgcaaaatgaaatggtactggcacttcgtcaaaccttccatgagcagcagattcaatagcaattgcagctacttctatcatccttatttgatttagctgcggttacgtcgacgcgcacggcaaaaacgctttcagtcaagtgtcagttccttgtctgattcttggcatctagatcgattaccaacagtggaaagctagtagcctttgacagaagatcttgatttctttctcacccccgtcctatgttcttgtcgtctactcaggaagaacccaaccaatacagttcgctgggccttcccaacttgactagtgagcactgctcgactataagagcgtcgcaatgctatctatacaaagcgtcatagcgtagtcgttcttgttcgttgtcgtagtgagctggttgggctccgttacgcttgctttcgagccttcttgctattagaaaggagcgtcctaagacctaagacgaggataaggaagtttcatatggggccggggatatacctacgaatgagtggttcagtccagtcctgaaataattggactaaccttcaataatgacttccgcaacatcgacatgatggtgacaccttttacataaggaatgcaccctaaggtgtcaatctaaggtctcgtgttaatccttccattaatttcgttatcatttgaatttctcatacctatctctttgatcatgggctatcaagatacactcatacccacctaagaaaggtggtattctatctcccaccagactgcctatccagattaccatactcactaagagacttgattgcttactctccctttcttgcttgttctttttctacatttgcttcctccgcactcaatgaacaatcagatgcgggattacctgttgattgcggtgtgcttgtcttggttgatttcgcatatctctttcttgtttttgggcaagctgctcttgctcaagtggaatcagttgcagttggcatatataaagaagtctaatatcctgtcttcttttattaaggaatttctagagaggaatcccctggccttagctcatctagccgtagctcattgggcggattgctttgaatagccaaagtcttttgaaagagaagaatcaacattcttggattaggctggtgctatctcttatttaagagaaataataaggagaaaggctgccttaggtttaggagtttcgagttttctctgctttcataggctatcgcttcttggtgcctagccttctgcttctgatcccgggagaataataagaatggccgttgttgaatcagctgtgaaagacgctcttgcctcagtttttgttggtggaatagaccctacgggagccccgtgaaggctaatttctctgtccggctatcccccctatgtcaccaattgttgcaacgagggtgacgtcattgaggccctcaaggacatgcttagcaaaggtatgataaaatgtcgccagttctataaagtcaagggctggagagtcgaagagcgcactttgggactgaaaaagttccacccttcatcaatgcttcaaatacgttgatgagaagggggtatttgccgacaagaagcccttttttaaaggagtctaggcatactttctgtacggatgcgcgtctttacaacgacggcccagcccagacagtgatggatgacaaaagcccgccagcgaaagccgaagcacaggttcgtagacctctccgaatcccaaagtcgaaagctaagggattgacggtcaacgctatctcaaagagcatgaccccgttgacgaaatctctaaactggggctgagggagaattacttcaactctcggtaaagatgccacttcctgcattacagcaaccttctcaggcagaggtgtttataaaactggagcgacattcgtcctctcaatggaaggttttttcctcatctttcacagggtagcccggaagtattcttctacgttggaaagaatcgtcaccgtcaccgatggtgagataagaaagagaaagtacagtccgattgcaaagaagcgaaggacatgggctatatgaccttgaggagcctgtcgggctgaagtgaagaacggtcgaggcagaaaagtacccctcgagccgcatctaagtgaagaagaaagggaagcttggctagccggccagtacgtcgatctcagaaaacataggcttgggctacctgccaactccgctccctgcgccaaaaactttgtctgacgccgaaagttctggagatctttctttcagatctcttccaattgtctataaactctgtctccgtaaaacaaagagcaaagagacgagagtaagttcaagaataggatgtagagcctgtgccccctacagaggacgaggtcaagtaaatggatctcgggactgttgacaatcctcgccctgtattcctaagtgcaagcttctcaaatgaaagagatttgacagtacatggatctactcagagaattcttttatgttttcgcttggagctacgccgaactggactagaccgaaagataaatgagttagctcaggctcagggcgtgaaagaaaatagataagaaaggcgattcctgatctgaagagtttagttgctatagtggaatctgttgaatttgggaaggctcaggtttggtggtatatccttacatatataagtagttttgatcccggctccggtcaaatggatttaggaaagcttccacgtgacatcctcaagttagtcttctgcttgaactgtcttatcgaaagctaaaggtagttaacctaggggaagaatccgactaagctttgccttgaacttggcaccttaccttctaatcctttgcttgggaattcgattcaataaagaggaatcactgattggacagtggcactggaatgatagcaagcatcccttcttctctttcttggtatgagaagttggttatgtaggctgacaacctttcctaggttgtttcgatcaggccaaataatctattttgagtatgcctgagattgccagaagaacttccccctcttgaaaactgactaatcaaacaaagggggtaacttttttttatgagggtagggagtttgggttggtgttcagtgtaccgcactttgggtacaagatcggaaattccattctcttttttaccatccaaaatcgaagaaaagaaagaagggcgagataaacaaataaagagctaactttctttaaactttctttattattatgtaagattagaaagttcaaaatgaatcggcgcaggagctgctacaattgcttcagcgggagctgctgccggtattggaaatgttttcagttccttaattctgttgcgagaaatcattcattggcaaaacaattttttggttatgctattttgggatttgctttaaccgaagctattgccttgttttccttaatgatggccttcttaatcctccttgtcttttagaaaaaaaaaaaagaaaagagtggaagcgggctagtccccgaaaatgcccggtactttagcgttggggacaagtaagattattatctggtttatccgccatcgttatcacaaattgaatatcctgttaatgtgccagccctagcccgtcttgctcttccaattccatttcgagagtcatcatagctcttttggacttatacatgcagcacccttttatctttcggcatagacccttcttcctccttgcgatgcaaaggcaatgtcagggagggcgagaggagagaaggagagcacgtatgggtggtatgaaagccataagcggaggcatgggtctttctcacgaagatgcgaagcctagagatgagtctattcaaaattgactgaaaaatccggggtaggaggcttgatgacaggtgataaggtgaggaaaagcgaagtcaagcctgacctaagaaaagactggttctcaaccacagcagaatgaggttttttcctttaccgatacctatttttgcgtctttcttcctcgtctaagaagcagaatcagccttctcctccttatagaatctcattcatctatggaaggaaggaataatcgttgggtaccctgaacgggtgagagatcctggaaaagggagtcttctggttgcgggatctccggcataagctttcttcccttgtcggccctccaattttcatgcccgatagtcaaagtaaagcacgcacttcaagtggcgcgatttatgtcgttgcgcagggatgctcttcccgtagtgccccttcttcctccttctctctttctctgcggcctgcgtgggactgatccggactgataacccgaacccttcgtagactgaactctcttctctttaggctcgcgtaggttagggaactcgcctccttcactgcttccactccaactcgaactaaaaacctcttcctcatcttgactcatggcgtcttcatcagtgagtaaatcctcatcatcatcctccgtaagataaaagaacctaactcctgggcctgtgcagactcttggtgaggctgttccaagtgtgtaggccccacatgttgctcatctccccctgttggtggtcttacagtagcaatggacgtagaaggaattctttgcatggcttttaacgtttgggttcaataacattcaccttagtgggaccccccagcaccatctttccttagtaaatactagatggattccctattgctatgctagcttccttgggaatactaccttgcactggtttaggcggtatccgggcccttttagaggcaacagttgacttctccttatttattgtggtcccaagaggcgtaataacctaaaagttgtccagtcctaaacaagacaggaaaacctttaggcttcttcagaaaaggaacatcaaacgtttacttggaaaacacgttatacacgtatgatccaagtaaacgtccaaacatcctttctagcatacccgtccgaagagtcaaaggccatctatcagtggccgactttaaatcaatcatacgagtatgctatctcactacccgtcaatctgagttctcgaaagcgactgaaccagccacccagatgagactcccgctgaaaaacattctttttccgacaaaacctgccactaagctttgacaagtcgctaacttgctcattttgtaatagggcccagtcacctcccttcttcccaacctctggcagtcaaaagggagacgtgcttcggtctttccatcgatagaagcagtaggtatataacgcatgcagctagtaggtgataggaggatgtaagccctggtggcagtggtactttggcgaatcaggcgtcgcttctatttcgtttttgattattatttttgaccctacaatggcagaacctagaaagctgctcttttttccctgtcccgtgatttgataccgtctagcctctagctaggaagtcttggattcgtataccatgtaggtgagaaaatcgtccgtgactagctatccttattctcctcccagggatgtttaggaatatgggtgcgggaggctgagggacgaccacgatgagtacgcgtttttatataggatcaaacggtttttgttcgatcgaaagttagcttgactcaagtcgacaagcgagagagaaggttgggtgagggtacaaggcatcatgtgggatctacgatcgactgtgcccgttgttggctttgcagatgctttcaaatactctagcagtatattccattcattgtatatatccctttttcgtgtcattgacatcagagattgcattcaatcgaatggtttgacataagaaatgttctagtctatctgtagtagttctctttgtttatagtagagtaatgagggtggcgactcacaagaggagtgtagaccagagcaagagggagccaagccagctactgtggttgtgccatttggtgggccaaagtagtctagtggcggtgaaaagacgatagtagaccagacggggacaccaccagaacacccgaacaaggatctattttctttttaagctatagtacatatgcactttatacgtctgtcttactaataatattccttagcgtacatctgtactataaccctcccctctgggaggtgttttcaagggaaggcggactccgcagctgcggaccgggcactatcactatactatgcgatgctttttaccaaaaaaatggaaactgtcaagattagcgtactaaacgattcgatctatcacctacgtcatttctactttgaataaatccatacttgttgcactcagtcatcgttccgtcatccaacatgcttctatctaagtgatttcataacatatggatatgtaaggaataagctaaagaaggccgcacctccctattcattacatcacaatatccgcaccatttgcttaaaacacagtttttgcatttgtgtagcttactcacttgccaagaaaaattcatcacatacttcgtggctttatgcttcgaactgtgatcagaacgagaggagtgggcaccgaagatgccaaagaagctagccactatcattgtatatatttttaaaacaaacctgacttctgtggtttgaaacctgtgcctagcctttctggcttgccttttgaatgggcgtgccaatattcaatatatttacccttttcctgcttcatcgctttggcctattgaatccgcagctgtctcagtaggagtagcacgttttcgaccaggcttggcttattctatagcatttgtgccatctatatctataagagactcctctctgcatttacaggtaaaaactcacatgctttcctttcttgctttcctaagtccctttctccatatggattgaaaaagagttattcggcccgtcatggaaagaaactacacctggctcgctagatcaaggaaagggctcgcgtagatcaattacctgaatcatgcttttcccaagctgagttctaagaccctttcgtttcggaagcaaaacccaaagcaaagaaagcagcaagagtggagagaacaagctcttcaagctcagcttcggcaacagcaactcgagaaagcaattcagtttgtgaggaaccgtccacttatttatatacgtcgccctttgacgatctgtctgttcaggcaggtgccacggaagtgagtacggaatcagataatggggaacgtaaaagactgagggaatttagttccgagactcatctaagttcccatcggccgtttgaagccacgggatggggaaaggagcgtttacactcgacaagaggtctcagagcaacccctatggtatggctaagctccgttcatagcctgaaaaacactgacgatctgtcctcatcgtggtcttttggtgatagaaccaggatggaaagaactgaaaaacataactcttcttttccgaattttctagcctggcccatagtcatggtaaactataaggattccctagcccgctttctggattttcggctttatccgaagactttggtagatgtgcggggtcagggggcaggatggtcgaaatggatttcaaggatcagtaaaattcgccaaaaggaggggaattttctcgatcctttggtaaaccgaattcagttcggaaaggtgggaaagcagttcttcgggtgagcagtttcaaaggatcaaggaataataaaaggtaccctagctggatagctaagacactaagaaggcttaggccgaatgcttaccttatgcttacgtaccggccgtagagaaggtaggtaggaatagatgggctgacggattaggggaatggaccactggcaagactgaaaactcaaagaagaagcaaaaaaaaaaaaagaaactaagaaagagaacccttttagctacggcaaatgctgcccaattcacattcactcgatctacgtcgagcaaaaagccttgaaactgactgacacgctaccgaaatgccaagccaaaggatttgaattcagtttagcaaggtacctgatacgattagaaggatagctaagagagaagtcaactaaaggttgcttgcttccttacactaagaccactatcaggcttagagccaaggggccactgcttgcacggacataggggcatacgaacataggggtagagtagaggtttttccaacgcaggacggaatggattagatggacagctagcactgccccctcacttcccacttccaagagaggaccgaatcgaggactcgaagacttagacggaaacccctttatatcgctcctgcaacagaaagactcaatcaacagccgtataatcaagcaaaaaagaaagagaaatattcgagggaggaagatgctctcccttacggtcgagttactttgttccttcctctcgcttcgctcgagcatcttcaaacctcactccggcgaatgggtacctaggcttctcttgccaatgtatacaaatagacagacctggcgaactatctttccaaagccccctgcaagtataatgattagacgaagaagaggccgtcagaccagaaagaaagctaccctttgaagctagattgagatttaggtaatgggctgtcagacagagactgagcgcagacgcacccgaggagtttgatttctacgcttcttcttcctttctgaagggcactttctttctcttgaaagatttgatgcgccacacgacttacccaatagcttttcgattgttggcgccgacttcccctttcaaagtaagatagtttcgaacaacatatatgatattgtaacttcactcttttcatccaactcgaaatatcgtaagagaagcacttttacgcccaaaaagccccatgtctttccggaccaaccaccggcgatttccgacaagtctttccccgggggagcagaaaaagaaaagaaaatgaatcaaaggaatggacttgctaatttaagaatacatcacatctctagggttaaccctgtctatcgcccttcttgtggcttttagggctggacaggccagaaatctaaattccattaatatggagaataagctcaatcaattgagtatagacacgctaaaagaaagaatcgtatccaaagtagaaatgcttgtacgggtttctaaagaaactaccccaggtttggactttgagctgcctcccatagaacctattgctcagcagatcctttttacagaggaaagtattccctatcttaattccctatatacgagtctcattgagaacgggacccaaggggaatacttggaaaaagtattcactttggcttccatgatccacaagatccatatagatatggtttagccagtgaatgttgtcgacgctaaaaagaacacgttcagatacaccatggaaatcgaccgctgctggtaagtcaccatctcccgtaggagtagtgtccctatagactttatatacaatatacagttgatcaaccactttttctttaacaacatctactgcaacttttgttagagcagtttccatattgatactatttaaagttgggagaatttgaccagcactaacggccaccagaatagctacaggcaaaggcaaagccattttcaatatgaaatcagcaactagttcacccattccatacataataccgagtcttagattccagttttcttagaccggcaactcctatcccgaatatacaagacaagtaagcgcccggtcctcttgcgtcgaagtgaagtgtagtgtggtgaggttttgcctcacagaaggcgtgggaaattggggaaaaagccgaaactgattcggccagtacaatactgagtcttattgaggccatgaagacggacagcacttggtttagagctgaccaacgaaaaaagactccaattcattccgttggtcaacaaccaaccagtgatttcaatagctgtttattcgttccctcaatcctctgatgtaaacctgagactagtgaaagaaaataagtgacttgttctcctctctttcttcattcaatatctgtctagcctactaacgacgccctttcttatctacgctatttacccttcattacttccccagctttgagttcagttcctttatttgatcttgtctcctagtggtaccatctctgcttactctttcttctttccatctactaagtttgcggaaaagagagagcagacggttctcggcatcatgatgcaagaatgacatctgagatcgctcattccattgctttacagtcatgatgggaatgattctatttactagaaagagacaacaccctattcttagcatcgaagagggaattttgtgtagactgctttttgaaagtgaaatagagactttcactaaagagtgagattgaggagtgaaagaacccggtattcacataagaaagtggcagtagtctaggcggacaccttttcttttgccttacccgcaacgccccctttctaagtagcagcttagggtttgacaaaccttaattcaaaagctggaaactcatatgctagtacacttgccctgtatgccccatctccatgaaagtcttagccagtgcttctttccgccttccaacttaatagattctctctatctctatttcactttcaggggtgagtattaaaacgccataggaaaaaaaaggggttagctcttagctcgctggtagtactgatacaatcaatatgtacacacatattaggaaactaaaaagcagaaagatcctttcaaaagggggttggatactaaaactcgggaacttctcccaatctctcttcaaacttaccttttcataaaggttagaaccttcctaaaattcaggagagctatgccgcactctcaaatccactcataaaagcatagcgagagatagcagcttctgattccggagattctatctaggttctagttaaactcccaaactccctggttataggggcttataatagtactggaaagaaaaaggagtattgtataacgtatcctaatacaggaaaaaaatatattataaggaaagattctatgttagtactccaggtactttcttattcgagacgagaataggcccaactcgcctgcatcgacagcaaaggaaactggcagggaaatagatgccattttttctcaatggcaactggtacttaaactagatatccctcagccagagactctgggatgaaatgactcttatgatagtcagatggcgaagacttagaacgtggctaatccgctttctcccatttctctctactctatctattaaggctatgaaggaattcgttcatagaatgcgattgcactactttttgaaaacaaccgtacgggatatagtcggccgaggtaccaaagccttttacggatccggctctgtccttaggaagcttacccaactcattttttaactcccaagaaaggaagacaaccccagtaaatcgtgcataatggaagaggaaagacctgttaacaacaggataagggaatagcaaaagttaggaaccaagggatatgagaatgtgaaaagcgatacgataagacagtcatctcacacgctaggcccaaaacctattccggatctgattttttctttcctgggtgtggaaaagacaaagtcttcttagtcttccgctttttcggtgatatctataagaaggaatacccttctcaaggtaaacaggagttcccggctcaagcgaaatgataccggcgcaaggtcagtcaattctttctttaggatagattcctagtgctatcgatttagctcttggaagaagggaagtttcattttgaagagtaggcataagaggtcttggagtcggcattagccccgttgttgtaggagagatgaaagccataactctgccctaagcattgagcttacgcgaaccaagccccccggtctttcatcaggctacccccactccttggtcttcttctttacgcttttctctgtcttctatagtaagttcccccacgggtgcagagatgcgaatccctagtttattaatagaatagcaggtattaggtcctagcgggcgtaacctctttgtcctctactgcctttcccacatttaaagatgcaggaagcgcccacagagatgttagctctttcaactctttatccggactggaaagcaactctatagaaattggatgcttgtaaagctgctcattctgatgaagctgggaactgcttgctttaaactcaatcacacagtccggtcgggctgccctttgcccgcattcctaactcccctggtaactcaatagaattctctcccggaaggggcttacaccaaaatagtaactgggaaagatcaattattccttactcttcctacgggttcaaagaagatagggacaaagctccatagcgggataaagtgttattgtgcccgtaaggcctttgtctgcattgcctcccaattgtgtattggaagagattctaagggcatagtaagaaattctataggataagggcctaacttccccatgaatcccaggtcatttgaatttcatatgggtaaagacccagtcctctaacttctaaccagataaagagcagccagcgggaagaggattaggatcagatgacctaaaagggcttttcctcatcagtatgttgttccccgtgaatcacagggaagagtcagatcttaggctttcgggtccttagtctctctttgccgctaaagtctaagaatccattcaactgcaactgcggactcaagagaagatgccctctaacttacaatcaattcctaactttcggcttgcacaacaatagacagaggatgctccgctttttctcaatcaatgggcagaggcaggttaatccccgagggttattggattgatttctcttcggtagttaattgttatagttaaaagggcgattaggagaaccaaaggttctttgaagttcttagtccccgctttcctgaaagagttctctctgctcgggcttctgtctggacttacgtccttttcaatcacaggaagagcggtgtaaaacgaaatcataatattctgccttcaatggctttgcctgcgacgtatcatcttacctcagtctgttacgggcctacctgtcatagcctaccagatcatcagctggaggaggatgggattgaaagaactaaagagaactagttttcccgggctcttctaagtattaactgtccgatagcgtagttaagtgacttctggggtcagacagataggaatccacaccaagcttttcatatgtaatttcgccagtaaataaagaaagacttcttgaactcggtgttccggtgaagaggctttccgtctgttcgctgctaaagtctcatcagaaagattcgtacttgacttcctcttctttctaacttacaggcctagcagaaaagtcggttttatagactgacaaagctgggtaatgcaccctaatatcaatacttcctggctgatcaattttaggaagctggggaaaggacagacttgctttcttcagactgacttcagggtatcaaaatattatgattcatacttttgcccacctttaaagagaagggatgggattgtaccaacaatagatcgatctaaagaacgggcttttaccaacctagaaatactaattcattctaattctggtcggacgtttaagtcaaagccgcatctcttttatcacaaagttaccatttagcaataaaggataagctccgattgaaaggatcttcttctctttaaggcattttctcctgctttgtctatttaatttctactttgaagtcaagattagcctactgcaggaagggcttcattcacctcaagcactaattcttttcgaactcttattacggactctaatgcaataccaagagatagagtaattcaatcctccgctcgtgggaactcaatctaaacacactaactcctcaagcactaagtccatacatcaatcctcaagagaatgcctttcaacggcagcatttactctagcttctacttccgaagtcagttccgggaaagaggcagaaattgcttatatagtagttcagtggggaagacccgtgagggaatagtaaaagaattacagggtttcggaattgattaacagggatggggaactccgccttcaaaggtcgtagtgctttcctaatcaaatgacttgtttacggctctaagatgccatgctttaactatttcccgtgtaaatatcatgagttcttgcttgattcattctcaggacgtaatgctactgctttctcagactttgcagagaataaagagacttgcaaggatagattcccctacttcagatacttcttagggctttcaatactgactacaaggaagtctgggaacacagtcgaaatctattcccctatcaagaaaagaaagagtcgaaagctagagctgacaaaggaaagaaagcctctaacttctaactcaacttcctccgagagggctgcgtcagtctttaaagttgctttcgtagttgctaccttcttttaggcctaaggaatgaaatcctggaagagtcagagaatatcgaaatcaaactacgcacctcgggttaagacttccaagagcctacaggggaatctaagggaatagctcaagagagatcctgatcttggtccctagaggaagtaaataaatacatgaattaggattttatttcccggggaacttcttaatggggagtttgcagatctgggtgtaggggattcggaagtaaatactgactagacttccctcctggggataaagactgagaatctgtaagtcttgaagctctaactctttataagactaggccagcccgtcaacctttagagttgcatttatgcccttgcttttggttggaagttcagaagctgtcagatcccctacggctctgttagcagataatggacttgattcaattcaatggcatttcatcacaggcattagacttccagactttccttgctttttagcaatgaactccgaaacttcagatactgcttacgcctgatcaactcataaggttgggattgtattgaaatagtaggcatctcttccggacaggcgtgtaacaacaaaagattaatcgtaaactgcttttctttcctacgtaatttcccagtgaagaagcgggagttgatatgatcttctttacctaactgcccgggaaagacagcataattaggaattgaatcaatgggcatagtaatttcatcatcgggattatctcaaatagacccaaaggtaagcaataaagactacaaagactacaaggaattcaatccttgcactacgcatctacgggaaatttagaagtcaagattgaaacgaaatcaaggacttcatctacggattatgcctctactttttatatgatatttttcttgcttttttcctattctctttcggatgcagctttgactctagcagagctaaagtaactgattccactcaactacactaattgaggaagaggatgaaaatctaggggaatatcctactgcaaaagacttagatcaatgaagctcagccggccttgttgtatggcgtattggtcctatttgccccttgtattagtataagtaggcctttttcctcaatctaacaaggactcattaggaccactacacactaaccataggcctgatcccgtagatgaaccgctaagttaagtttaggattatgagttagatcttagggtttaagccgcccataaaggcagagaatcgtcttcgccctgacttccgggaggcgaggtagtttaaagcagtggaaatctcatatgattgggtttcgactctgtcccgcagtcttgactaaaattgtttgtccctgcagctgaaactgctagatactgacttgagtttaaaacctcagatataggaggaatgacaatctaaaaccatggaagttcttatgaatggtaggcttattgagttaccggggaaagacttagttaggaaagcatcatatcttcccctctactcactggaaagtctgactgatgaaatgcaggagtagaatgaagtcaaggacttttctttctttatggctttagtcgagccgtaagtagttgaattcagtaatggagagagtgatagttgtctagggtaaagttagtgcgtagttagacaggctttctagatctaaggaaagcaacgtctttgctgttgtgattcctcattgctggagtaattcatgctttctccagagcgggatcaagctttctaatgaaagcctatgttcacacaatggttaactcattcgatttggggattgggttagtgttctaggagtgaattgtagtgcccctggtggcttattgcgtagttaactctttatatacgaccttactactcctcaattcccatcaagtgttgtcttatttcccaagccactgctcaatcctccttttctgattgattgaaagtagcaaggaaagacaagcaaaaactttgttggctcaagaagcaactgaggagagacaaagagtagtaaaggaaatacaagtagcagtctcaggtcaaaggaatcaaggaagaatttcttctgatattgcggttactcttccagaatctcatcctgagacctaagtatgccattctcttcgtcaagaaagatcgagcagcatagaagccttgacttcaagcttaggtcttttttttgaaaaagggaactaaggcaacttttaggtgcagggaaagaggttcgctagccttttccctagctttttttgtcaactatctatctttccgaactagattagacggacttacttaaaatgaaaaaagggctaaaaaagaaggacgaagtaatttcgtatataaagatatggctttccgggtttagatcgaaatggaatccccgaaaaccagggctggagtcttagacttcttctgcttcgatagagggactgacagcctaagtggaataagaatcattcggccgattgctctgactcttatccttccttcgctgacagagaagagagcactcccaagccaaggatgagtgccaaagagaagatgggcaagcaatgcccactcccatgctttccgttggtcaacaaccaaccaaagtgctctatacttcttcactactcgtacaggcttgacggagttaagctgtattgagggaatcgttttgtctcaatcaatcaatatgtttccgaaaattccacgtatcttttctttgatgaagagagtctaaattccagtgctacatcctctcaaactcgagtcaatccacgacaactattagcgattttagtcttcaatcgtccgatactcaaggttcttctaatggtattttgaggatcatccaggtcttaacccttccagtgaacgtatagtagagcttcaatgttgtatacgcgaaagattcgaagagttgctgcctaacaacaatgccgaagcccaagcccaagaggctctggtagcggccgaagttttacatggcgaaagcaacgatatcgccgagctggaacacctttgacagatttgaatcttcacggagtactaagtgaagcctttctagaggcgatgcatctagtgaaggagctcaccagcccccaacccacctaccgtccccagcccacttgaacaatttgaaataatcccattgattcctatgaaaataggaaacttatatttctcattcacaaatccatctttgtttatgctactaactctcagtttggtcctacttttggtttattttgttactaaaagggaggaggaaactcagtaccaaatgcttggcaatccttggtagagcttatttatgatttcgtgctgaacccggtaaacgaacaaataggtggtctttccggaaatgttaaacaaaagttttcccctcgcatctcggtcacttttacttttcgttattttgtaatccccagggtatgataccttatagcttcacagttacaagtcattttctcattactttgggtctctcattttcgatttttattggcattactatagtgggatttcaaaaaatgggcttcattttttaagcttcttattacctgcaggagtcccactgccattagcaccctttttagtactccttgagctaatcccttattgttttcgagcattaagctcaggaatacgtttatttgctaatatgatggccggtcatagttcagtaaagattttaagtgggttcgcttggactatgctatgtatgaatgatcttttatatttcataggggatcttggtcctttatttatagttcttgcattaaccggtctggaattaggtgtagctatatcacaagctcatgtttctacgatcttaatctgtatttacttgaatgatgctataaatcttcatcaaagtgcttatttttttataattgaacaaaagcgagtctgaatgggtatacttagtcgtggagcattccgagtatttgctttagggatcgttcctgcgcatctccttactttatagcagttattgctccggttccagaaggtatagctcttggctcagcttttcttagaaattggagactgttccaatttcctactgagataggcaagcggagggagaactagacgtatcttgctaggcaaagacaggttagaatggatagctcgcgggtgggattgacgggatagatcactattgcagaaggaggtagaaccggggaagaattatggctataaaggtcctcgccctcttaggcacatggttctaaagattcaatctcaaagcggtactaaagattaggcagaagcagaactagaactagaattcttcgcccctcccttgtaccaagaagcaagttcagaacataaggataatgggctcgtctattagaagttattagtttacggagctatctcagatatctcgagtaaggagacggggcgggtttgatagttagagttctatttctaggaaggaagagactatcgggaagctcactctcggccgggctcgaagcagaaggtagaacgtaatatctcttgttggttcagctcatcaagctattacaaaagagtccagcggagacaaagaaagaagccattttacggtattttcgcttccagtccgtaattagatcttcaagcttagtccagtccggatccatcctaaaccaaagagcggggctaagcgaggggcatagcgatacagtgttcatactcgagttgctcaaatccagtaggaatatcaggaatagtaggatctagtaggagcttgccttggaatgcagtgagggagcccggagctattgaattctttcataacccaaggagaagaataggactctttaccagtatcataacctctcgatgggaaatggaacttagatcacgatgtgaacctacttatgagtggaatttcgttgacaagcaaattccccggaaaacgaacttttctccaattgagatgctttcttcatttatggattctatgcgagattcggttagtgtgaagtgtgatcctggctcagaaggaagagctatatgcttaacacatagagttcgatgtaggtaaggatgtgctccaaagttttcaattccaccttatcaacctgaaaagagctaatacgggcttagcctgccttttatcttatccttctattctaggcgaggaggtttatttttaaatagtaaatagccccataaaaacaacaaactagtcaaaggacagcctgccttattcttctcccgttcgggacccctattttctcggagatagcctggtctgagctagaacagcagattcgtgagcaagagcgtatttcacagctgattcaacaacagccattttttctggggaactttcatatgagtctgttctttcttttaatccactataaaggttcttaattttctctttaatatgaaggagaattacattcttgaaaggatcaagggctctaccctctcgcataaagtcttacgctcttatcgtcaaccttcgtggcttttgctcctttggtctcgctatttcattcctggttctctctttcaagcttctttccatcctggggatttcttctcattccgtccgttctgctagctggtgtcgccttctctcttacttatctattcccatccatctttacctctcctactccactacttccctccttcaaagcgtgattaatgcgccttaaacctctctcttgaaaagagcattttttagtggagccttagcacgtgaacccataggaacagggcccttcttctttgcaaaaaagcttctgaattatcatcacatcagtaggcgcagaaagcaaatcttggtattgacttattgaaaatctctttgagattgcttagacaaatcttttgtgtgaggccgctgttccccacctttcttaccttgttttttgggcttaaaattctgtgactcataagccctccatatctaaagatagatggctaaagggcgggttccgcagttaactaagaaggcgatcgattggcttggagaggaaacgaaacccggactgaaaacaaaaggataggaatgaattgaataaagaaagaatatatagaaccttgagcattttctcttctcggcaatggttgagagtaaaaaagggtatccgcatagaaggattgctggtataccgggtagatgtttatcttttcgacttcagcgaaaatgtaaaagcacaaatttcgtaaattttctttctgtcgaaagggaagaggacagggtcttacttacttaaaagtaaaaaaaaaaatggaagtttcctgtcttagtttcacttccttgaactggctactaccgcgcaacgtgcccttgcttggtgggtcgttaattaatcagttttaaaagagggatggatttcgaccttgctttgagtcgtcaggctagtaaagcgctacttctaaaacgatcgttaaggtcattcactcgattccctcggtggctctgctaccgatggatcaagatatgctgcctgcctatcatgccaaaggcgctgctggtggatatgccaaagatgtcctggctctgaaccgggtacttgaaatgctaaaggtacttcttatggtcctgcttcaaccacccttccttctctaccttttcttcaaaacttaagctacttagactgatgctggcgatctcgaagggagatatctggacctggagctactcatcttgatctttattatattaggatgcgaggaaagggaaagaaggtgataagcaagaagaggaaagaagaatgttaaagaagtccctataagtacttcacttagcctttctatagtctgtctttcttccctcttccctcaaagcgctctttcatccatgcgcatggttcttactttcatttcccctcctcacgtaggagcgcatcttgttttcaaagatgagttgtagatgagtcggttcgatcaccccacatatcgacggtttttaatgccttatcctaagcccatctagttgatcgagggatagacgagtataaagaagggatggagaatcttttatttgatcttgatttgatgtatatgttacgatgccttcgtattcaggaggattggggtacggcagataagaagagcgacccaaaacggaaagaagagtatgaggggcagcggctcaccgataataagaagaactcacattctcgtcctgacagatgaccaacctgttaaggcatctttctcaatgaccatcctctcccattccagttctttctctttttttagggacaagttcattttcattccctcgatatggccaggtgtgaagcaacttcacgatccaatgaattccctaaaatcggatgacacaaggcgaactagaataggctgatttatccacaagaatgtcataaaggttttctccggtcttcctcaaaagacagctttagagcgcaagtcaaactcatgataggcgagaaatcacgcgcacatggtttagcggtttgctgtgctctgtgatcttattcttctcaagacccgatgcttcatctgcttctttagtttagtaggacttctttcacgctattgcgtgaaacatttgtttggtctcccactgctactgctatctatgctaacttgaaaggtatggctactctcttgtttcctgctgaacctccttcccaatacaggcttcgcagccatccctgcttgcattttttaaaaaagtttggtaggggctgccaagcttgactaatagaatagggtccccttaaaaggagaatgcctgccctgtgccaccttggtagcacaaacaaaggtcctgtgtaccagggatgtacgaatcatagtaataaactttacaaactttattagttgcaaggcgactttgctgtaaagtttattatactcttaaagtatattctaaagtaaaagtcttcttagtattcaaatttttgactatgaatattcctacccttgcagtgctaatatattcattagtctgagtcttagtctactaaaagcataggaaaggaagagtcaactcttatgttgcaaggttccaccccaaccaagtaataagcactaaactgaactctataaggatagacggggtgatttctcactacaaagaaaaaggctgaggatttgaaatagatagaaaggagtccaatctaagcaagcgtagtggaggaaaaaaatcctaaaagtaagcaagtagttgaattagtccctgctagtattggttggtcttactttattatacaaagsthhgdggcaacgcgthtghvgtcadchgcdtdbgvvgtacdvhvcgaaggcccctcgaatcttccttgagttgacgtcactgggacatctaccgcttggatcctgccttgttagtcatccgtagagctaaagggaattttttgaagccattcccattcccacacaccaataccaaccagggtggctgttcagtaagtcctacccctaatagaaaggataaattgcttgcgcgcttcgtcaagtaagagagggatcttaggccgaacagatcaccggctccgaaggcctgcaatcgtgactttagttccggtggttcgctttgctgccggggtgcaacagcctttgtgacacttcgaatggagtggtccgtacgcccctcccctcgccaagcctgaagaaaggagcaacttagatacctctttgttaactagattcctggtttgctaaaagggtccttgggcccaatcaatctctatactcttgatgcaatggactccccaaagccactaaaccgctctcttccacccgatttgaacagaacctcgttctagtgagattttatcccttttaaacggaaactcagttgcctatctgatccttggtctaattgggcctttctctatagctcgaatcgaatagctgggctaccccttcccttggcttggttggttatataagagaatcccaggagaaagcaagttagaccttacttagggcgaaagattttttggatggttcattccagtctgaagtcagtcaagtcatggaattggcagaagttccccttaaccaaccctaagagggaattcttctattcattaagatgaagccattcagtcagctctgaatctgaactcaatgattgcttttcaagaagggcatgaagctttggctcagtacagtagcatttgactttgggaaagagaatcgatagaatcgatcgcttaccttgctttggcatgccagaagcatttcgctgtggttctcattgattgagtcgatcccgagacaaagcaaagggagttccgtgggttcagtttgcttagaggcagaaagcctagaagaggcctagaagtcataaggaataggcaatgtaccggcaactctaaggtttggctttttcttttattgacttttgagtcaatgtcgcatttcgcgtgcttggttagatctcctaacctaatgtaatgaaggagaaggcagaaaaaaagatgcctttatccctagagatgcaggagcttgccttaggacagaaatgatatccgaatggcgtacggagctgcttaccctaagacttcaactccatcttacatcgaagtcagttcggctggatcgagagaatctggataggcatgatcgaaagaggggcaactctgtctccgcctctgctcgtgcactcgttaaagtcatggcctagcctagttggtgaaggagcctacaagtggtaaccgctctgtatccgtcatctctttgaagaagcagttgggctacaagcggcgctttcaaaatcccgtgactctcagtcatctatcttcttttcacctgaaaattttggattggggaagcagagaatcaaaaaaaaaaaaaagtcatgcttactataagaaggaagcgggcggagacccgtgcgtgcagcaggtgtagagtcagtcgaactagtcctgcgaatatgcgaaaatgttctttatgaatggagaccagacacaattgctttagcggggactgaaatcgtgactatgtgttcatgctttcgaaaagaaaacaaccatctacacggggcgctatttgtctacttattgcattagtcacgtctattttgaagtcttatttaactcgttcgatgtgaagcccttccacacctgtatgaagcatctcctctcgggattcaccggacttcgtagcttgaaacaacctgtccttttcctatgctgaggcagcaccaacaaatcaatccatcgaagttcctattgacatacataaaaatatagggatgcccttgatgattcggatcatctcaatcaattgattgggaagagattacttatgagcaaagggaggacgaagtcgcaggagattaggtattatttaaactgtcaaaataagggatatcgttgactggtacaagaatagaattccttgcttacactttctttctactggttggcttaccctgtatttcaagagtaaataccgcagtgaggaatagcggttcctctctttgtttggtctaataaaaagattattcatcaccgcaaccactctcgcttagctaccacttgtctttgcttgcttacttctaaagcaaaccagactgaagacagtagagaaagacttttattacgttatccagaatgcgatgccccaaggcaagaaagtagcaatcggctttcaatcctatgattttactcgaatagctaatatcagagtagcagatatggttttagcggaagctgctttccccggatgcggaattgaaagaaccatgccttttttcttataaaagcctcctcatcaactctctatctttcgaacccacctcaccgagcttaacgccctgtggacttttttacgaaggcctaacttgacaggcccggacggccgattcataagggtctgagccttggtcggctgccctactaggtaaggcaagcgctcaccgatttctttacgtcttttcgatcgtgctttccgtgaattgaaaggggaattaattatccagcagagatggcatccattagcttattgtcggctctcactctggctcatcatccagaggcgggttgagccccttgcacagcttttagcagatgattccaggcaagacaagatcagggtcaatgaagtgtttaaggacaatcaatggcactgggattgtctgcacactcaacctccagactttgtgaagaacatcatctcctctatgcagcttacactcagtccagatgaagatgatttggcaattttgtctccaactgcatcaggtaaattctctcttgcttcagcctggaatatgcttaaacataaaaaagggtgtccttttagattcaaagatatggcataaggatgtgccttttaaaatggcatttcttacctggagagcagtccatgataaactcccaactgatgggagagtgtccaggtttggtcattctctttccctaaatgttattgctgtgttgactctactgtgaactcaagcttagaatctgttgagcatctcttttgctctggtgtttttgctcaactggtttgggaacatcaattgttgaatgctacttcttaattggtggaaccacaaggtccttaatcctgtggcttcatatattactaaggtcatgcctcctttggtttgctgggagctgtggaggtccagatgcagcaataaatatggttctgagaaaccatcactcaatagatccaaggcattgatcacatactccttatctcacctgctgcattctcagtttggcaaggttagagtaggtgagagctgggagagtatctgtcatctgtgtgatgcttcaatgacttagaaatctgtggctttggttaggtggatcaagccaccactgcttttgtcaagcttaatagtgatggtagctgtagagatggtatttgtggaggtggtggtgttgtcagagatagtatgggtgctcttattatggcttactccattcccttgggtgctggaaccagcaactgggcagaagcaaaggccatgcttttggccttaaatggtgcattgaaagaaggtacaggttggtgatagggagactgattccttattgctgtcaagctgcatttcaggagaagtgaagtgatccccacccgggaatcacgaacgggaatctaaatagaaaagaaggccctggcaaagcctctcctaggcacctaagggcggataatagcagcggatatatcgctttctgtttccgctctatctgccaagggaaatcccggtaaagggaaccccgaccccgagaagaccgtactcatgtgcaactaattcaataggaccggttatgaacccaagagaagagcggataggagtactcatactcaaggacaggaagctctcacagcgtgaaggcaaagaataactcctattggaagaagagcgtttacgatcagagctggaagagtgggagggaatgaaatagcaatagccgctacttctgtctgcggctatcttctcctattgattaagcccttcaaaggaatttcttctatttcttctttctaaaggcaaggctaagccatccgcccttcattgctgggtaaaaggggagacggttcccaaggggtggctagttcgagtaagagagacggatacagataaggtcctttttctgagagacccgctcttgacttttatcatacccactagtaagcgcagtggatgctccttcatacagggacagagaggcgagtgatgggcactactcatcataagaaagcagtcatgcagatagaaagagtaaaacaatgactctgactaagtaaagagatgaggtttttttctcatctattttccataccacagctctagacatgcgccccgattcaaactatgtttcaatcataccacccttgtggggtgttcgcaattcacattaaagaccctttccaaaggttgagtaccttggctcgggtaggtggtgctgggttccgtgtccttggcaggctcgaccatcggagatccgttcattacgaacgttttttctcgatgtggaccaagctccgacttccttttagctttggctcggaagaggccggcctttgagcccgtattggaagggatcttggtttcttttagaaaagaaaccccaagagttacgtcttattcccgaggagatgtttgatctcctagtctagggacttcttgtaagggccccttatttatggaatgggtaatgtgttaaaggatagcttaggtactgcagtaggtttggaattagactaccttaatatcagacatcaaagacaacacagaatccaagtccaagacttgagtgataatgctagagaacgtatccttcttggcaaggcaaacaacctttgccaaggttccgaaggaaagatagatctgaactaacacaatcactataatcatccctcttgtatgtatataagttttcgatgaaagaggggattatcctacgataccctaggagcgtgtcagaaagatgggtacgcgaagtgagtaatggtgaaattctccgccacaagccctctgaagcgaggatgcacactgctttaaatagaaagcgcaatgcaacatccccgaacgtcgggccgtcctcattaccgtaagagcaaacaggtaagctccaatacagaactccttagtaagaccgtcagcggctatcaagatcgctttgttaagcagtgaccttaagaaccgagagtcttctaaaactctctgccacaaactaaagaattgaattaccttgcgccggtatcatttcgcttgagccgggaactcctgtttaccttgcgacaggtattccttcttatagataccaccgaaaaagcggaagactaagaagacttttctttgtctcgtccacacccaggaaagaaaagatcagatcagcaacggctttcgagtagaggattttttgcttttaattattccctcggagttgagttagagttagcagatgggatctaattcattagaggaagggatggtgattaactgatagaacctcttctcttctttcaaatcgcatctctcaagtgagaagaaaaggccccacggagcggtgggaaagcaagggcgtagcaggaagaagaagtatgaaagcagcaaatctttcctcctcgggctgggatcacgaacgggaatctaaatagaaaagaaggcccaggtcgagvgttcgctccctctctctcagctaaggaaagagatagagaattcatgtacatcgctatttcctgcggatctatcgtatccttacttctctctgattgtgatttcccttgtgccgtactataccgctaaggaaaacaaacaagaaccaggctaggctactcctcttcccctttctgaatcaacttgtccttgcgcttaccacttcttaaaacttgcgagcgagtgtcgatcgctcctttgcctgggcaagatctgacgactcctgcccaaggcgggttacgaattcagattagctactgccaaagaggccaggaacgagcttccgctttatctaaagaaaaacctcttcctttctctcttcctgatcagcggattcagagtgatcaggtgaagccccttctcgttggatgaccggccctttcttagacttggtgaactcctgtcgcgatgaattaaactccgttccatgccccgctgcttgtcaatcacatcggaaagtcgttgggtcggcggagacctctttcggcaaagaattatatcacaaagaaagccccaactagggactaccacttataggagtcttctttgctagtagaatgcccccacgagaagaaagaatagtgggatgctcacgctctcgttggacgtgacagtcagttacagtgggtaaactaacgaagggaagaattttatttcatcacagaattgaatcgggtctcatcccttcgattcctcgctgcatacttcaatgagaaaggaaaagagctttgttgcgtgcttcttcgggtgtggttgcaagatctcgctttcagttcgaaaatgtgtacgtagcttccttgtacaatagctctctctctgagagagtgatcgggaagcattctctcttcccctccgtatctgaccctgacccacgctctagccctctttcgtcgtccaagtcgcatacctcctaaacagtctatttggttttaaacgcgatctatttaactgattaactgtgaactaggtgggacttgattcttttgctgaaaagagaaggtacgtaggcagctctcctaaaagagtgaagttccgcccgcgtttgaaggctagctcctgcttcggagcttcatccccacatctcacatattggaaaaggcaaacaaaaaggggaactcagtcaatagacaaagaaaaaacggatatgttacacaaaacaatccaatctttgtctttctaaggattgatttttcttgtcgtagttcatattcatattcaagttggaaaaattcttcttttcttcttattgtggaaacggagggaaggcaaaggtccgtagaagctagctctcttatccgcttgcctcttttaatgaagaagggttggtttaattgatagctttggaataggtagtcctatggactgctcttttcttatgccccggagtggcgagaatacgaagctagatcagcaggaatgacagcggtctcttccaaaagtgggtacaggactcggatcccatttccaaggtgaattggaggagaaatggatactggtattatagttgttgaaagacctattaattacatgccaaaagagcaaaagttgaatcatcggcttggccaccttatccttttatacaaagattttccttgttgatataccgtccgatgcgcttggtgtcgactctgatcttccttcacttgacaatggggcgaaggaacgacgtcctgactaaacaaaagtttctttcttcaataatggcttggtcgaaagtcgtaaagaaggcaccggataagcagctaacataaacaactaccgtacagcgcatcccgtgggcggccttcaaaggctatcattcgtaggacgagacgctaacctacgcccgtacattccaacctgcctccttgggacttagctctgaagatgaattcccggttagccgattaccttgcccggttaggagaacagttagaagtaggaaaagatgccgacaccgaacagttaaagaattctccgttgcttcaagactgccagcctattcgctttgagccgaagcagacgctgcccatggagagccttttcctttgtgaacatttgtgtgcgtgcccataagacatgacaaaaaatacaaaaattgggcttctagacgccttacaataaagaagccccggcccctcggtgtcttacacgtcttcttcgatcctgccgaagctgctttctttcttcaggtagtgaagtcactccggtttgtgtatgacttgacgctctaaagtctctatcttgcccctagttacttaatcgtattcgacttctatcgcagatcttttatttcttacgcatttctttccattagctctccaagcttcctatctttccattcctctagctctcatttcgcgcatgcgctttgcgctcttggcttaataacatcaaagaggaatcgaacctcttccagttctgtgagaacaaaaatccatttgatgtgtagagtagagactgttagataatcttctctctcactagaaagtatatgtgtatatatactttaacaaagccgacctggacgtccacgaccctgagtaccatgaggaacagctctaactggctatgtatgctggaggaggtgcggtaaccatagtaccctgctgctgcgtgcctgtctgaccagtaccactatctcgagggcaaaacctcgtaatgtgaccaacctctctgcaagtgtagcaactttgagatgtaccccaacactcgccacgatgagtgcggccacaagtagaacatgaacgtgaccctgtctgagatgatccacctctctatctctgagtctgctgctggccctgctgggctgggggtgcctcggaagtaacctgaagtgctatctgagtaggtctagactgaccacgaccatgcttgcccttgctcccagatggagcaccactctgtcctcctgtagtcttgacctcttgctctccctctcggctatgtcccgcctcttagatgccttgcacctaagggtggtatccaacacgtcggcataagaaccggtccgaacaatcccagcaattgccatacggtaagccctccttttcttgaaaaaaaaaatgaagcttagaactgccagagccaattattgtgctttttaaccctgttttcgtgatactctcacattaaaccctactgttccttaaggtaacggaaagcaaaactgaattcctaaggtggagagcaaaagcaataaagaaaagaagttaaagaacatttcaaatgcgtcgacataaatatgactgattctgtgtcaatacattgtaaattttctcaagttgtactgtgacaaacagctcaatcaatagccgacatgtttatccaaaaaggattctgatgaaaaatgttattacctcattttgatttctggtctactggaaatttagttaatagtagagcttcaaagtggaattgatgtgcacccaattccacggacattgttgatatagtttgctactacttgtgtagcttgttttttagtgccgcttactctactctattgggtaattttagagtgtctttattgatgtttccttgacaggattagaatagattcatactcaacatgacaatgatgaaaatatctttatgaaatttctcgaaatctttgaatgaatcttcattttggacagttcttaggctaccctaacagacgtgtgggaatgaagctactactatcttttttacacgcataaatatacatagtaaaaattcatcgcaattcattcttgaacccgttgtgtttagtctaaatccgccactagaagaatcccaacgtatcagcctctttagtaacttgataataactataaggtattttgtgtatcataaaaacctatacgtagctcaagacgaggggtcatctttggcaactgaatagggtcagggaggtatctccttgattaatagttgaacatgcttgatgaacttagggacatgtatatacaatacctcgaggtacaagcactaaaatggcaattttttgttgtgttgttctatgatagtggtttcatcttctagattaggcactgaaactgatcatttttttattccttcaaatcttttattcaggggcctggatttttggctgtattctgtaatggttttactaccttttttttttcaactcttattcattttttcagatttaacactaacttactgtccacggattcagatattcaatcccacaatgattggaaatttttgctttcagtaccccactcttttgaaaaataggcttctgtgcaaaaaatggggtgtagaatgtggaaccaaatcccactagcaagagcctattccataataaggtttctagaggattttaagtgcttgttaattgctttgcctctgtgggcattggaagagccatattttacctctcattttggaaaatgacagcttcagatattttctcttactccctcttctatcttatcccttatagtcgaaattttcttggggcagtggtacatgcccataagctacagtactaacagcaaaaacaataccaatttatttaagggaagaacaactaaagtatcttgacatggaaaagaaatcactttagaaaccaaacagtcattcaactagatcaaaacctgtaagtagttaaataggagaaatagaacaaatcgcttaacacattactcttgttagtgaatagtgaatctccatcttttttttttgaattcaaacgtttaagtaccttctcctttgctgagctagacctgatttgaataccggttttatggcctcttctcctgggacctgcttcgtcaaattcagcaacgggagcccgagagggttaagcagcgtcaggagcattggaagtttcattcctgaaatgaacaaatcattaatgggcactttgaagcaagttgatcctagaagactaacctcgtagctcacttagatcaatcagttcaagcattgacaaacccgccttccttctgtgttcaggacggagactctttctgcctttgtcgaactgccttgacgccttggcaggctttgacctgctttccttcgcttaccggagagcggattctttattactgacttttcgcggttgatcgcacctcgcacctaaaggagccggtccttgtgaggaggaggactcttctcttgctgtcaaaagtgcttactcatggtctatcgtgcagttgatgatatcattctggactagtttccaggcatacgccaaccatacataccgctttctcgttcaggaatttcttaagattaaggttcgaaaggaccaggcggcgatgaagtatgagtctaaaacactatatgcagagctgccttagctcaatagatcaacgaatcaggagatgacttcttaaacgttcgcgaatggaaaagagttgctttaggcacggaccacaaacccacgaacctaatagttggatccatgaggagacaggagaaagccattcattccggtcattgagcccggattgaggattgattgatctaaaccaaagacttgattatataggagaaaggcgttctcataccctgataccgctttgtggaaacctagaacagaagaaagtctctttaggatggctctgtcctagctagaccgagtcacaactacttattatagaagactcaggcacacttccctatacttctcctaagtgacatcaaaatcctctttcagccgattcgaaagcagtaatagatgagattgaatcagacagaaggttcacccctcaccctgggggattggggagttgagagggatttggacgcggtagtatcctactattcgttggcgctccgtaaggcccaaagtcaacgagatcttctttatccggtgcggggcatgtactatcttctgccttctgctaggggttgaaggtcttctctctcgtttgatgatttgagaagccatcttctctccctcccaatgcttcattctctgctttttgtactcgttcgataacacgaaacgaagaaaactcttagccccaacgaactgattcatgttcttgacaggcttcttgactccactgctacccacccggagtcgactattgatccgtcgcccgagccccttttcctttcgtccttgcctgaggtacgttgttcttatttgtgacacccatatggtttgtgtctgacccagcatagtgcttttctttccattgttcattcttctttgaagccgcaaaatgatagtgaggcagcaaggatccctcagtgtcagcaggccatatctgaggaattgccagtcttgcagaagacgtcgttcattaccatatcagatagagaggggttccaaacctcttcctgacggaaagaccactattgaggtgagggaaattcagactcactcttggtatcgatctgagaatacttttgccccactgtaaaaggttacttttgtagggctctgattgaagttgccacggaaagaaagtagcctttgttccagtgagatgtggggaatctttttctgaattgaaaactacatgaggggatttacatgccaccttcgccagggcgatcagtttcttcacatctagttagtcgactcaggaaggcgttgtatggactaaaacaagcaaactccggctcgaaagcaagggaaggccctattattggggatcttccttgaccgggtggaaaggtctcttttttctatgtgtttcgcccattcgagtgttctttgacgatgacatcataggcaccagaccctcggtccgtctgtgctgcttcgaatgatcgggtttcaacggcttccctagctgtactgatctatctggcagttcactacgcgccgaatgattctttgctatttcctctttctcctccctattatttgattggtgctgcctgaaaagagttccctgtaagagggacagtcataacaagattattatttgcggtttcatcagacgggatcaaagatttcgaaattcgccgatcataggtaagcggttctacaaaggtgaagagaattcctaaaattctcggaggaaattttttgcttagaatggggattctgtagggccttggcggcccgtaaggggttcatccctgtggtataaatatattccactcttttttttttttcttctgggtcggcaacttgaattccgttcctttgaaggaattggtcggcttcctcgctttcgcgagtgtctagctgttctaacttggtgacctctactttcgagagattgttaggctccatggcattcctagactaactatcacttctgatcgggattccaagttcatgagtcactttttgtgcacactttggagaaagcttggaactcgtcttcaatttagctcaacttgtcacccacaaacggatggccaaactgaggttgttaataggattttggggattcttttacggagctttgggggtgaaaatattcggcaatgggacttgcttttagctcaaatagaatttgcttacaatcagtccactagccaaactactggttttagtcctttttaagctgtttatggccaaaatcccgagagtcctctggacttagctccacttccagctactcacaactttagtggagatgcgggtgaagaaaatgaagaagttgcatgagcgagaaaatttctaagcaaaatgagaagtatcaagctcaagctaacaagcatcgcaagttttctgagttcaaagaaggtgatctggtctaggttcatcttcgaaaggagcctttcccgcgaggacaatttgctaagctcaagcctagagctgatggaccattcaaagttctcaaacgcattggtgaaaatgcctacaagattgaactaccagctgagtatgaggtttcagaaactttcaatctttctgatctttctccttattatggtgaagaaagcactaacgactcgggggcgagtcttcttcaacttgacggggagaactagaaataaaggaagttgttttggctgtagtttttccaggttgggtaaatttctttagaaatgtcataaaagagaggggctttctttcttcagcatgtgagggaaatgccccgggtaccgaagttagcggatagagagggcggcgggtgggcacggtagcagatacgtgaaatgagatcttcttggaacaaggtcagaggcgttggacggaccagtttcttcagattccaatgatagatggatggtcaggtcggtaacatatggatggaggacttctacagggtcttctcgtgcgctcgactagaaaggtggttttgtaggcgaacgaaataagtttttggaggcgagcggagtgaggcaatgaaattgtttaggcgaaagaaaggagagaacgagtggagtatactccacgaggtaggtgggcatggaagcacgagaggtgttggtgagtggggaaggtaaggtagtcgacctacgggagtcgcgagcgttagtgagttgacaaactcgccatgcattcattcgtggttggaacttctctctgcagagtagccttgtgcatagaggctcgcgcccttgattgattgattgaccgggcccctaaagctgcacagctatggcctgtaccgctaactctcatgatgcttctttctgggaaaggaagaaaactaaagcaagctacctttactttttgaaagaggaagacataaaacaaagccgcttctcctgattgaatagctcgtcatgcagcaagactaaagaaggctctgaatggccgctaaattaagtcaaagactaagtaagctggtacgtcaggtcttgacctatcattctgttatcgtgctttgacagctataaaatagccctttcttaaagattgtgagagcttccgttttagttgttgattttgaagcattataataagaatcatcctttccacaaatagatcctcaaacatagaatcatgggcagctagcgataggcagggtggtcacgtcaaagtgtgccaatcatggtgatcaaaccctctttttgttagagctcccagccttgctaagctaagaaagatgcccttcatcctcctttcttccctttacccttccctctcgttccttctctctttctcgtctggcttggtctggtggttcgcctagttggaggctttcagctccatgccgtaggtcaggggtcggtgctaattttcctgatctttctgatcttgttgatttttctttcgatagagtgtgaatcatacgccggatctaattagatatatatcataccataatctagagtcttgtggagtagcctccgtgccacatatactgggcgatttagttcgttcgggacacgtgggccaagaagctctaggcaattctcacgatcacggtcgatcatggttcaactccatgtcgtgaaagtgaaagcaatcatttctttcatcaacatcaacgaatcactatctctctttcatcggtagggcgatcagtcttttctttttgtgtctaatcggagtctagtacctctctggcccttatgggcctccacagatgtaaccaaaaaaagaaagtctaaaaagttttttatcctcgttggtctataagcttgtgacttgatccgctagcgcaggttcgattcctgcttgcgagaaacgaaaaatgaaacgatctacagggatttcatgcttctcatccattctttgagtgagtcgggtcatcggtaggcttgcttcaccggtatggctcatcggcttattaatgactaagcggagtcaggagtcgatcgagcctttattagatatgttctatttcattggcagttccgatccgattaagactggaaaatccatcaataagagagagaagctaccagcaagaatcatatcaatgttgggcaaaggaaggtactttggacaagcttatatctccgaattcactgccgattctgatgcccccagtttcctcggccactgggacaaggagatccgatcttcataatcaatgggacgaatgttttgatacctcaaagagcgaacgaattcctgcctttgcaataacagcccatcttgtgccacagaatcggttgtgctctgcctcttcccctctatcagaagattgccttgtgtggaaggttgactctgaacttcagtcaatgggaggtatccccttatctaaggttctttgtatggcactctaaactctctttcttacgcgagacagaaagtctaactaccgaagctctttcaacttgtcctgtctttggataagtattgcgcttaagtcagttaacaagatgagagtcggaaaatggaaataagaactgtaaagtgattcttgaatccttctacttatgtagatggagtccagtacgctactatatagactgaaaattcccaagacaatatcgggagtacccatcttatcagatatttaaatatatcgtcaaactctttcccgctgtacccagccgattctcaaggacaaaaggtatagcattacattttaacagacagatgaaagctaggtctctactccttcttcatgaggaagaaaggccttcttatcatctagatcgacgtaaggtgcgtagcggtctagagtccaactaagacttccatgaaaggtctcattcatgttgattgaggagtttcttactgaccgctaaaccttctctactttagaagatagactggaaagcaagctcagagaatagctaagtggaagtcagagactcccttttttaggaacttagactacctatgtgctggtaaactccacctagactgagattcatcagttcgatcatttagtttgtgtcctaagtcctatatccttcaggaaaggatcaattccttctctaacttctacttggggtcactcctcggaaagattcttcattcgagttagcttctttcgctccttcacccttgactgcattcccggaaatgccattcccatccgctaaacctgctccttctgagaatggttttaccccgctcctcaatcttattcagtttccgatcctgcttcagattctctttcagttgtggaaacaaacccctattcctatcggttgagtagcccaagctccttaagagcgtattgtcccctctcctgtgaaagaaagaggttgatgcacccagctacccgaagtagagctttctttgtcccacctttccttactgactttcctagtttagatagcgtattgagaatcatgtcaaaatacaccaagacctgggcccaggttctctttcttcaagaaagggttgctttaaacaacccggttccaaacacaccaaacaagcaagcgactccccttccttagcgtacccgtccattaaggcattcttccttcttgcgtatgtgttatagctcatagctctaagccccaattccttggctcataactggaaaacataacaacaatgtctcctagctgcaaaagaatggctcccaactgaaaatctctcttgatcactctctaacagaaagccattttccctttcgcaaaaagtaaacttggacttctttcctaagcggagatttggactacatggacctaagcaacccgccgacaggggcagcctttcactgttggaaactttgattttgattggtaggattctgtctaatctttcctaatttagaaattgcactcaatcaacatagtttccactcattccttctcgaccgcctcttttctagtcacttttgatcaaatctttcttgtgattttctattatcttatgagaaatggtttgcttcgtttgagccgtcgtcgcttaatgcatgtaggggggctggggcttttcccccacgaccccttttaaaggagaaccagaagaacaacaatgaactcaaagctaatgaaggagatccgcaacttgaacaaggtacacgggatctttcctacccctttctatttcgacttctttgaaaggtgaaagagtaagaagctagaccgacttgctcttaaattaaaagcagcaagagcaagtaagtaggcttttctccgcaagaacaatcttgactttctttatactttagaatataaggccctttaaacgatcgtaaatggcctgaaatgtaacgacctatgagagaagggtttttagaaaagaaagcgtaccaatccggcaaacaaagcaaaaacaacggctcctacataaatacaatagaattgaaatgctgtcactagaacggaccacacaaataacatctttctagccgcctaaaggaagtattcaaagataagataacgctatgcgcacacaagcaaacttcaggtatgcagttagttctcaagcgattccttcggatcttaggtgcgaccttagggagcttgttttggcagctactctcttatagttatgtgtcctggtttccgagttctagttcaaggcagggcaggacgggactcacgggggttggggggagccttcccccagggaaaacctaataagactcattcgaatacttgagttcaagctcctacttcgaagtaagcctatgggttgtttcgaagcttagcagctaaagcgtacttgcgtgttaaagtgggtacgcggatttaggctactaagtggaaccagaccattcaacttgccatttgcactctcctagggtgcgatcgtaggaagctctattagcgaatgcaattccccgcccgataagactgatcatgccctgctgcttggcttggaatcaaactagcctatcatgccctttcttcattcctatatggacccatattcctatgttcttccaatgtttactgtattactgggattcctatttactgaaccatatcaaagaagctactttctttctggcttttatacccaggtataaagggatagacagtctaagagagtgccaagaaagaacacatacctatcacttttggaaggtttggaaccctcgattcatccgactcaaggagaaaaagagaacaagatgggtttggctcgctgtgcctccctcttgccttaagcgactcctagtgagcttttgaataatttaatagctctgcccttctctcttatacctttatcgcttatttccaccctttgacttttgagccagcgacacctctccacgaatcaagcctataccgtgcaataaagacttttccttatctttcttcttcaaattacgagtagagatttggggagagtggataggacagggtggtggatgacgtaaaggaagggaaggcccatcccgtgctttcgagcgattcttcccgcaaaaggcagatctttttctttccgtcccaaatagaacaatagaatagggacttagatgtgaccaaggtgcttgcaagcttagggttagcaggttgttggctgggagagctggtaaaagaatgaaaccttcaagagaccgtggttaacaagccagctgaggaagaacaatctcccccagcaataccgatcctccctagttcaatcagaatcgagaactgcggagaggttctaaccggcctagcctaaccaaccgctacaagcgggcaggaaatagatgtggtggagactcaagtcaaggcgatggatcactatcactatagatagatgctttccctggactgtgttcaatggcacctgatatgccaacaagggcttactaagagatcttgcatgttttatagggtgcttcttatgtctttccataagcagaagtctgagtagagcagctcttcccctattcttaatcccacttcttatgtctgtcaacaagagcccagcccctggttcaatcgatagataggccgaaaacttctttctggacaaatgaacagacctttccttacttgacttgccaacaaagcggtcaaaccagtaagcaagttcatgcgtcagtaccacgtccaggatcttaggaaaggggaagctcaaatgatatctaatgggatgggcatgctccccactgctctatgatttattatagtcatactcagtttcgtacctggtagctagcctttcgcttcctccttgtactagattttgacttgaattccccctgaaagcgagaacgcactatatgcctttaaaataaaaagaaggctggaaaaaagagagagctcctttcttttctagctttggcgggaggaatgaaaatcctatcctatacgaaggcctatatacaaaaaaagcactttgcctagaatcccaagttgcctcccctctcctctgaggccgatcgcatccacttttggagcccctcgccagtacggcagcagcccagacatagaccgaattaggggcctaaactcttgagtagattgcccatggaaaggagcttactccaagatctgactccccccgtgtaggagttcgggaaggccagaagtaaagaaagagcggtagaagagaataaagtgttgcgcccattcttctttttcatagctggagcaaatggaaggagacgtcgtgcaagccgaagactttgacaggtgtcggtaggcacgcctctgataagggctcgatcctgagaatcaatcccaatcgaatctatggaagggagaccctctatcctcttaatctgtagagtatatatttattttaggataatcagtccactgcggtgcccaagacaaggcaagatgaataggaatgttgaagggacataaggctcagctaaggtaaggaaagaccctgaccatctaggtcaccaagtactcttcttttttagggagttggagacgatcgaagaggcagcaaaataggaactttcgatcagggagagctcaacaaggtcgagaccaagatgatggatattccaaggaagatcgaagaagatgaatgaaggtttatacctacccctaactggcactatgaatccaatcccatctacatagatgttcctagccacgagatgagggggttctctcttactgttaagccgtcttcaactcttctttctttactcctttccgcatcggggctgataattggatagaatctccttaaataaagaaagggggcgtaaaaatagggtttttggctcgcaataaagctagggtcctgatcgagcaactagtagtcctatctatccacctctccagacacaatatcttgagtacctatgatggtgaccacatctgctggcatgtgatgtttggacatagaatcgagtccttgtgaatgggcaaagccaggtgctcttattttacgacggtagggacgattgcttccattactgaccagaaagacaccaaattctcctttaggtgcttcaactgcggtataggtagaaggagctggtacggaaaaaccttctgtataaggttcgaaatggtgaattgaggtagagtagaccgatgatcctgtagtcatttggccggctattgaaagaaaaagcttgcatctgcttcccctattatataaccggtcccatctctctccaaacctaacgtggtagtttcccatcatagggctttctatctatagattaagccattaccaaggagctaattcgttcagaactcagttgactgcttctatagagaaggcggagcgtccttggctcagcattatagcacatagggcttcggcgctactacagcgcttcgctaactcgaagcgcctcgctatgagaatctagcttcgctaacgctcggctaagtcttgaaccttcgcgctgaccgttcgctttctcagtagcaaaagcgcttctctttgccccttaaccttaagtagaaggacaagaaagatattattggttttcttgcccccgcttcctcatctgcgctcatcaagccaactttgctctttgggaggtgaaacagcggttgaagcggacatttcgaaatgacagcatcgaagatagatttctatatatacacggttagggttatctcggactgcgttccggaaaaagcagcctacttgtggggcactgtgtacttacagcctctacgataagcaagtgaatgtggccggtgcgtggcgaacggttcatcaagccatttttcgcctcaactccctaaataggaataggggttgtttacaaaaaggggtaagaatgactgtgatagccctctcgataccttattggagctttgtaactagtggccggtttcccgtcgcgtcagccttttcccagtgcgcggagccccaacgaggaaggtgttagtgctttatcattgggtcaataatgctaatccctctttttgtgctactcctagggcgggaagaagataagaaaacgcgaagcgttctcttgctttcccaacctgttctttctaaagactgccctctctcggctggatcttggtccagcctactacgaggatcccgtatccagcaacccaacctatacaaagggcatcaaagccccttgactaggttggagctataaagcttaccttatttattattattaaaaggggaaagggccttttcagctggtgcgcaggagcgcacttccgttttccctttacgagtagggggtcccgtggttcctatgccgccgcgtttcccggtccttttcttttagtgcttcgacccgaagcgatagcttctagctagttcagtggataagatggctgcgctccagctcactcaagaatgggacggcagtggtccgccggcaagctcgttctgatcttggacgcagtacattggaatcctgaagcaccaccacgaacgctaccgcgcgtccgcctgcggtgcggtaaggcaccaccctcttgtgccagcagccaactccggcgtgtcagcttagttatcctcatcaaaccacttacttgatgtctagcttcccaactggtagacggttccttttcccccaaatcaatgaagaagggagacataagttgattcttccgaagaaccggaagcgaagcgctatgccggggcggggggacggaaaaagaaacggctccgaagaaaaaaattggggttcccaatgcttctccacgctcaacgagatgcgccaacctcgggatgctttactcctaaccccacaaggttccgagacggagcttaacctgagtctcggttaagaacggcgatgatatacgtttcacacggcgcacgattccatggatagtttcattcgagatcgtgatggaggacatagcttacgatcatcggctttgatcatgccactaggcatttgattaagacattgcacaatgatccgaacactttgtcgcatctcttcgatacgaatacagtaacgatcatagcgatctcctctggtacctactggtatgtcaggatccaattggtcatgaacatcgtaaggtgctgcttttcgcaaatcccagcataccccagaacctcttaacattacaccactgaatccccaatcctttgcttgctgtgcagtgacagtaccaatatccactaatcgttgtttccagatacggttgccggttgacatctcttctaattcgtcgatacgagaagcaaattgttgtgtgaatgaatcaatatctatacataagccaagaggcagatcttgtgccactccaccaggtcgtatgaaactggcatgcatcctggctcccgagactctttcatagaattccaacaatttctcccgctcctcaaaagcccacaggaacggagttgatgctcctacatccatagcatgagtagttaaagcaagtgaatgatttgaaattcgagttatttcacggaataacactcgtatatattgagctcgtaatggtacctcgcaattcaaaagtctctctacggctgaagaatgagcgtgttcttgggccatcatagaaacatagatagggtcgacgacggaacgaagaacgaaactttacgacagctttttcgtagacgttcacttgcatcacatacacaagtgctctctgaaccgtgcaataaggtcacccataacacggctctcccacttgagttatcttagccccaggccatgctattcaataatctaggaaaaatggcagcgtaaggtaacaacgagtatggaaagctggtcgcctttggaagccttcgccggtaaccaaagcgtatcgttcccgcaaccactttggtactttgtttctagcttttttaagttatgcaatagaagggggggcttgcgcttgaattgaagtagcgcctttggaatatgagtagggctcctaagtggcgcgttcgtggaggcaaaccgaaggaagagcaaaaggaaggttgggtgcttgtggggcgaggccatccggcctcgaataggagggggcttagctctggagcctccctgcttgcagaaatgaatggatcagaaaggggcttggttctctatttccgggcggggggtgaaggccataagagaagattgccctaccggtaaggaagaggggaaaaaggtgctgtcatctatctcgaccagtttcccgaggcgttggaaatccagaccggctcagagaatcactgtcgctatttagcccttcgttccgccaacaaagaagtcatccttgacgatttcccattccttccccgccgagccgcctctcttcgccattcgatgcttctgccttccctttctataacatacccaggcgccctcctttccaatcactaagaaaaaaaaaataccaataaaagccctatctaagtaaagcttcgtctgttatttttccggccccaggggagtttattcgacccattccccagtctcccgcactgctcaagtaagtgtgcgactccgtatgaggacctccttctcttctgcccactctccgttcacacggttctcaaagcagaggaggaagggtgggcagcaggtaccacgagccctctgtcccacacatctatccagaagcaagtgtagttcaccggttccaccgaatgctcctatctctcggcaaagatcgtgtgagtgtgcagttatgcttcggatgcttcaccatagaatagatcgatccagttcccgttcttttccggtgcactcgctttatatctccgacacacaaggaaggacgcggtgggaaggaagcagccctagcctctgtccggccgatcattccgctggcatctcgcattcacgcccccgtttgactgccgctcggggatgtagttgtagataggttagtcttagtgggtcgttggctccacctgttatctccttctacgacatgctgttgtcgtcgccatattctatatgtcacttagtcatctctgcctcgctgcgggtcagcacctccgaaagaaacggaggacttcattcagtgaccccgcgatcgccctctgaacgatcagaataaggtaaagcttgaagataagttttgtactcaattaatttctcagttcctctagtcgggtgggcgccggccggtttttcgaccagatccccctaaaaaccgtacgtgcgggtctccccgcatgcggctcacgccattcgaggtggcccagcccagcattcattcgcaaatcctgtagtgaaattgagactgctcaacctcggaagctaattcgcgtgtaggcagcgctgtctgtcgtaccgttgactctatctattcatggaattttcttttttttttttcattttcgattttatataggctcgctccctctttttccaagaattcatccacttccctttactccatagggccttctctaatagggaaaagccttccatttccgtcaaatgacccggcctcccctggctcttccaccgtccgggctccctttcttccctatggtatgctcctccggcgcaggcctaccacgcttcgcgcctgcggcgttttcgccagacggtctttgccagtagtgccatcctccccgctggctgtatgggcgggttgtccctcgctgctgcgttcttttaagctatggattaaaggaacaaatgtagttgaatggaacagcaggcgggttacacgttccactgtgccgagatgtgaggtgcaggtggtgatgatcaccccggggtatgcgctagcgcccttgacaggcactccagaacccgccaacgctcgtgaaaacccgggtcggtcggtcctccattcatccgaccggaggtatggataacgaggccaccttcacaaccttctcccttctgtccctatgttggaataaggtaaggcggttcgcttgagttgctcaaccgccccttagcccggtgctcatgacgtgctacggaacctccaccgtgccgggggagggggaccaagcagggcatagctagcggcataggagccgactcggcatcagcggcttcgtgccgcactggagtaatccaatatgtggttccgcacgttccaccacttctccgttcatttccaatactgatcgtgaaacaccatgagcagcaggatgttgaggtccgaaattcgaagtgaaatttttgatttgcctgttcttagtcgtcatgggaaagaaatacagaaataagaaagagattattcccttagagcttgtccaataccaccagtaccagaaatgcatctccttcgcccgcgcgagagacttctatgccagccgggaataacggctctgttatgaaagaaagcggcagacagagtaatttggccggtattccctaatgagtagctttaggagataaaggtcccccttatattctccacccatctgcggagggtttccgtatccgtctccgcggagatctccagatcataagacattatcgccttcgcggcactggactatatttccgtcatttccggaaagtgcacggacagccgccatttccccctttcacaatgttctcgtgaagttgctcacgaatcaaagtgtgaatgtcccttcgaagtctcgcatgctctttttgatcgggagcggggtgggctatttatgtcggtgctggcgcctgcggcagcgcctctggagccgcccccccgttatggagccagcgggttctgaatgacctccctctcacggttaaaaaagtggttaactatctcgaaaaaatccatatcgtccatccgaaaaacgtgtctcaattacagccaactccccctcccctgtctctttacctatcgaaaaaccagccctacttattttgttctacaaatgctaaccaagtgacacactggggccatgggtcatgaaagaggttgacccccatcctccttaactatgtatggctaatgaactcctcgctttagtccgttcttttccttctttgggctcgggtcgatagtcgccgtggtagtaatgccccggagcccagctaccgacctgaggcgccgatcgggaaagtcataaagggacgttaaacgtaattctagaagggccttcccgcaaaaaaaccgagtcttggcagttcaagtgaaagttttttagactagtcccactaagatggcgaggaaactgacttccgagagagctgctttcgcctcggtaattacctaacgagagagagccgatgcaaaagttgtcctttacgcgaggaaacgccagacagactgacctctgctaactacgttttctatagactggaagctagagagatactaaggtatagtgctgctaccagagaaggctctttcatgctaggcgtccagacctactatacccccccggcacatttgctatatctactaacgcttcatcctaaccaactatacctgatagaaagccgttctataaaaattcaagacaagaagaaagcaagaaaaggatagcgatcgctttgggaacgtcacgggggaggaagatagaaaggtaacctatgacaccggggaattaggctttttctcccgcctcagcttcgcggatggaaggagggcgagagcgtagcacgcacgctctatgcttttcgccagctttccctctagtaaaagattagctcgtaccctctctctgtgtctagggattcctggggcatgagttaaggttaagcatatagttgattgctctttctttcgattgagcgtcggtacttttggagtctctctctgtaggcgtgcaaaacaacagagccactgctcttcggggtgatgaggtggacaattccttactccagcttcaaaggagcatctttgcatgaatcaatactaactcctcagtcagctgaccttcgatttcggagattagagcagaagaactccgtaagggcggagaggggtttcgcctcgaatccaaatgatttctcttcttctcttaagatatttctagttaggacttgatcgagggatcaattgactccgaaagataaagtaacaagaccataaccccgtgcccccgccttaaaggatcccaactcatcaccctcatctccaacttattcgtggttttaaggtgcttttgactattctaaaaacttatttggagaccaaggcgaggggtcatcttcggcaaccaaccggggtcatggagccggcctccccgccgtcccccctgcccgcaccctccataacggaagtacgtagaaaccttgatctgtttacttcctcctttaataagatcgggatgaggagtgaccttttactggacctcgaggatcggcttaaacttgaaactgcctcagaagcaaagagacgcaaaataattgaattcatggagatcttggcctttgatgaagatgaactgatatactggcattctcttccaactccgtatcctaactcagggcaaactatctctagatggcaaagtgaaaagtcgaattgatctgcacatccctctattccaatagaaaacgttagccttcatccatgagatcggggtatcactaccagtaggggcccgcttccataatagactttgaaacctcgccttccctttcgatgtccgatcccggataccatgacttgccttcaaacgggcttcaccttcaaaggagagtaatcgatctgcggacagcaaggccaatgaagatcaaattgaccggggtctgagtcgtgtcttgtccttgagtcctctctatgcctctcatgtccttctttccttcgcttgggactcactagcacactccttgctgctttcgtgcttgatggcttctgatgaaccaatgatagagatccttccctaacagctgctgttcaatccgtccctgagagtgagaggagtcgtaggaattcacattgccttttacggcttggaattcctattgtatagaataaatgtattgggcaatgtcttttcttgaattcaaaaattctccgccttttctcagcttgacacctactttagaaccatccttttctaagtacgacaaagcttccttgtaaactaaggctaaggcacgctcgatagcaagaagctagtgacttctttcaggtcattaactagaacttgcacgaggtatcacagtggggtctgtcttctgtccggttcttggggccggtcgagcctctttgaaattacatccctgcctctcgtcttgccccgctcctttggcagttaaagtagctcgcttcaagaagtaagattatatccctaggggtatgttacgagcagaagttctcttgctagtggaagtaagagtagcaaggttaggaccgcatataaatagaatagggggttcgaaagaaatttgattccctagaagttttgtccggttgggaaagccagaactcttgtaaaccagcttgataaagggtagtggtagggacagtctcagtaccactgaaagtgcgatagtgcttcaagcaagggacttgggcaaacaaagtccttactcgtattccaccaacaactcgcgtatcgtatagagctttttcctatcctttccgcatagacttgcttcgcacctgtgtaaaaagccagtttagttttactcaagagtaagaatgataaagcatttcgtaagcttgaatccctataaaaagtccgtcccttaaatttagcctgaaaagaaaaaaagggggctaacctcccctccaaactattctaggccagtcccagtgagtgagtcagtcaatcctgttcaaaaactagcgcccgctctcgctccaatatacgtgtagggggaagcaccaatgaaagtgaacctttattctttcgtttccttttctcttcgaaccgattggaaggaaggcagtagctcctcctacatacgagtagggagatcctgaactaaggtatgattccattttcctttgacgacaaagaaagttatagtagcttattccatttggaaggttttttgtttaagacagcttttcgtgcccttacttttgagtctatcagctgcaacaagggctgcgggaacgagtgctgtgcttgccccgaccgagaccaccattcattaccgtgaaccggccttggccttcacttaaaagtcagatgagtcctctgatgaacttgggtccatactctagtgaaaaaaggaaattaggcttctctttccgcttcttaacttctatcctttttcgtacttagcccttctttggcatccttccctatgaatctctcaatctcgggagttcctgccgattggttagtccctcgcgttttcttctttcctttctttttcactcttgttaggttaggaaggagcaagccttttagactatggaaggcaagccagctgaagaagtcaagcctgcagagcagtcacaaagaagaggttgtattcactggaacaagagtcaccttcatcttctcgggtcaggccactgcccttccatagtgaagactctttccaggcctaacgataagattccctggtagagctccagatattcgaatatagaaatatctttatccggtggggacaaacctataagtagaagatcatggtaataggctataagatagctatataatagactattctaatagttactgactctaataaaagtaattgccgttcaaagggcaagctcaccccagtcactactttcttcccctatccctaaacaaatagtcagaatagtgactagtctcagtcctacttacatccattgctctttcctctccttgcttagggcggcttcgttccccgctagccagttcctgtaagctgaactatatcttagtcatactctaagcccgtggtagttccattccatcccgcctagtgcccagtcatgcattttttgtcttaagctaagcgcttttcattccttctgcaagccatccagttctaaggtcagccctgccctttttgttgggttagagcgagtatgaagtcagggaggaagaagaagagagggaagaaataatatagtaatatttacctttcccagctctcagaaatggagaaggaatcaaaaatctagtcaacccctcaaactccgtaggtaattcgagacaattcaagaagaataagataagctaacacaaagaacttgaacattgacaatagaaagttgaatactaccattctttcgcgttgactcttccgcggagtagcctaaagaatcccctttcgcttattactcctatagagcgagagattcggcaacattcactgagtaaaaacaaacctccactttctttcataagaaaacttcttgtaaactaagattagtcttagattaggtaggaaaggggatcgcatcaccgaccatatctattattagtaggaaggtaagtacaaaaaactagatttctctatttgattgacaatgtaaatctattcggatgatgtgataatttatgtagccgagtcacgaggacttcttcttctactcccttcccggaagatagagggaacttagcctctgacaaagtagtagctgacataggaatagctggcaaaggaagagcttccgctaagattctgacttatttggaaactagatttgctgcccctgcagactcttcttttgaagaatctgattcgctaacattggttgaattttcggcatggcatagaatagaacatgaatgggtcttccttgccaaccttcgcttctagaaggaagtaagtagaagctgaccctccaacatacattgcagggaaggacccctccagtggcatactttatggagaaaggcttccatcagcaggcaggtatttacttttctgataccttcacgtcttgttgtcaaaccataaactattcgtattattcattctctcgcgcttgcacatataattgggctcttaagcaactggaggtctgtaatgcctttttacacggaactcttgaggaggaggtctatatgtctcaacctcctggttttctggataccgctcatccaggatatgtctgccgacttcacaaagctctttatggactgaagcaagctcccagagcttttttcacttgtttcagcactatattgtgctctaaagggattccgtggcagtgcctgtgatacctctttattcattcgtcacacatctggggatagtatctaccttcttttttatgtcgaagatatttttatcacaggtagtgatcaacagggaatacttgctcttctttcgttcttgcatgctcatgaaaatatgaaagacttgggccttctccactactttcttggtatggaagtgtatcggcaggggcgcactcttatccttcgtcagcagaaatatgccctagatctcttgcctcgtgcagacatgcttgattctcgtcctttggccactcctcttactagtggtaccgagcttcccaagttggatgtcacttccctctctgatcccaccaatttcattcttctattgagtcggctaactgtaactataagctacacgcctcgaactcgtataaagattcttcctctagggcctcctttcaccttttgttagcgacccttaaacgggttccagcagtgccagttcaagccttacctttttcgtttagtctgactattttccgaattctatatatgaatgaaagctacgtttcggcaaataggtctatttatataaactatcatcctaaggaagaaactgaaaaacattagtttcacagccgaggtcagagcttcaagtcagtaatgtctctttagcgccccataccctactacaattcttattcaaataatattactacaatgtcgtgccgatgtctcccttacgaaattgaagataagtcttttgattacgggggtgacaaccgaggcttttaagagaagttgccatagaggctataaagagctatctcatatctaataggaataatcaaattgttatgtctactgtgggaaatggggtcccaagaccctctcttcgacgacgtagacaaggggtcccatcatgggcgatctgagaagagagatgcagaagaagatgtcctcctcaacgggtcaagccctcgctcagaactaaaggatccttaacatcggcactcactgcataagctcatagggcaagatgaagatccggaaaaaggttaaacagatcgtcaacttcaccttggcatgcttccatcagcgctgaaaagacagcattgaacgagaagagaactaaggcaaggctggtgatgtgccactgtatggagggctcagagagagtagaagcactttctttcacgctgagtgtgaacttccgatttcaggctgctcttagaccaggaagattgcttatgacatcaatcagctaggtccgtcgtatgtcgaatagtttgtcaatgcatgcttccctttcttatgctaaagttagtctttagaaagttttctgatgagcaaactctttttcttcagatcccttttagtaataaagaaatgtttgaggccttttatctcgtccaaggcctcaaacctgatatctgagaggagatgtctttgggagcagctaaagaaagtgtctaaacgcatccagggaccatggttggtcaccggggacttcaattggtcctttctctctcctctttcaccagtgagtggtgagtttccctttttttttctaggtaggtacctcttggattcggactttgttccaacagctgccatacgtgagatcctgatcgtcttcctcccagtgttgttgcctgctgggggaaggaaggaaagtagggcttccttccaggaccggagaaggtcaaactctgggcgggctgccaggtttcgcctacgcaacggtttcacaagattgaaccttttttgttcaacccaagtgttggagttccagagcacgagggaatggactttcattcccaggaccgcctcgtctatgtattcggcgcctcccccgattgcttgaagataggcgcgcgatacgataaaggcccctgggagaaaccaatgaaaagccagggtagagcctcggagccgacccaagcgaagatcggcactcgattgaggagcagcccgaaaaagggaaagccgtggagacggcagactcgccagtcaggcacagcgtgaggctgactacagtagaccgggaggttacaattcctgtttcaatttccgggagtgaatgtagtaagtgcagacggtggatcaggtgtaaacatcaaccaaaggcgtcttggggatcggcaatagctaaacattgtggccatcacagttcaagctacgtatggctggcgtacaacctacgggctttttagccaaaataaaaagaacaaaaaaggatgcctgctttggtacctttagtccaatcttagacaaagagcaatttggatatgaagcactgctgggtagaccatggctccaaccaggtgattcatgactgggctaataaaaaaagtctcaagcagggaaaggcgggatggaaggcggaaaaggcttggctttgtttcacagaaaaaggactaaggaaatttcctttccctagtgttggagctggctcattcatgctagtcatcttagagctatgagtcagaacaatgttcaccaactcctccatagtaatcttgttcatatatcgaaaaagctttagaatattcgtttttttatattaaagtgttatatctcctccccaaggtagcattgacgagcgggcgatccctgtcttgtttatccagctagcttttttccgtggtactcaaattcgatttgtgagagctctttcggctcggctactctttttttttaaggtaaggtaggacctttaaaccgacaaaagtaataaaaaaaaaaatgcctatctataaagcgctgagttgaagagggaacaagtcccacagagagatgataagtgggagaaagagtgaaattacaatctcttctggaatggaagacctcccatccactgactacaagactgcagcctaacacccaagttagcctgacggtcagctaaatgagtcccttacctcttcacatgatgaatttgaactcaacatatattgagaaatgttttatcaggagaaagcataggcaccaaggttcttgattattaccattcgcccatctaatcattgttaagagaacccctttttgtttgatatgatgacttgaaaagaatcaatagtttggacaaaactatggccatgcaggagagtttctgcttctgcaaaggttgcatctttaatccctagaggagatctgttcaattccacatgacagcaccattgccatctcttatgacccccaccataatccgaattcccagagtagccttccctactccttcaaagttcatcttgatgtgatttgaagaggaaattgccgcaagattgagatagatatgtttgaatttttttttcttttaattaagtaatgcaataaaacctcgtcatgttcatccttactaacatcccatacaaaaaagaaaatcttttatggtctggattttttcaatcaccttaacgcttaacgaaggaggtggacttcaaccaaatcagcccttcttatgaagtggctatggaaatttccaaaagaaaagaaaaagccatggtgctcatatttggctgctaagtgcctctccaatggcaaaaatggattgaccaacccacctcttaaatattctgcatctaaaaaggtattatttttaatagagagactttcaggcagaacttgggctagactttggttgggcaatggtaagctgattcgcttctgggatgatgtttggccgcgccactctcctcagagatgcatgccataatttatatcaaatcacaaggttctcatgacctcaaagtgattgactacattcaatataaaggagaaaaaaggatttatccccctattcaactacccatccaagagcatttggcttcagaatactttcttctttttctttttctatggactgcgtaaatcttctcttccagcccaaaggaggataatctcttttggcagctcaatcctcacggtaataattatgccaattctgcctaaaaatctcttcaggtgatcaagggggctccctttttcagtagatgagattaggatgaaaggtattatctaaacgcttcttttctctggcttgctctttcaaatccaattttggcctgcagtaatgtaatcgggatttcatctcctaaattcttttttctatgaaagcaagaggtggaaagttttgttaaaaattctgccttattccatgagatctagaagcacttctgcaactttctctcttccctagcgctagcgctctttttttttttacttttttcaaagggcaatgaaggccttccttataagttctcgctcgatcgaaaggatataacacatacgaaaccttagcttcgctgactttatgaggtctaaccttcgccacgacattagtggcttagctcttcgcgcttcccgcaggcttttttatagagagagagtaaggggggggggcggtacggaagattggtccgctccgaaaagctgagtttttcggttcgccccccctatgtggtcggccttcttaccagtctgcctcctttctcttgatggaatatatcaatacccgagctccagctttgcttgcgttcttcaccggcgctcgccagatgtatcactcatcccgctcctaaggtaaggagtcttcttgtgtgttataatctttacgggaatgaatcgcatatgttggttgagaattgctcgggaattcattgataatgactttgccaggttctagggaggctactcttcttttttgtcgatcgagccgctttccctcattccactcgtccagccctcttcacgaacttgtacaatcgatgccacaaagatagccaactctattatcaaagaaataaggaaaggggcgacaatttggcaccagatatccggaggtgtggaaagagcagctgtgagaagcggaaaaaccatcaaaaaacgacgattgttcgtggaggtttctacagaaagaccccttggttctggcaaacggatcacaattacaggtacctgggagcataccgatggaatgaacgaaatacgaacagttaacataatatggtcatagatcttaggttgtaacttgatcatgagcgaatttgttgatgttgcacccatgaagtatggaaagtgccaaacattgggaactacccggggaggagttaggaacaggaacaaggagaagcgagaaccacttaaatggaggaatcgattgtatttcgtcctttgttccccatagcaactggggatcaaaaagcaccaaatttgatgacttattaagggaaagacgaagtaagagcatgctattggagacgttgcaacatatgtagggaaggcctccgttgattgtgtacgaacaaaatacgaatccaaaggcagggtaagaaagggtttagctaatggagatattaactcttccgggaaccagtaacgcgtaaaccatgtcaaaccaagaccaatcaatatccgaacggaacggattcgaacttctcctagaatagtttccggtgcgaaatgaaattcataggatatatatgagtaattcaaaggataaatataaatatttgataggattcgattcattttagtaatgaacaaaacaaataggattttttatgtatcacaatttcatcactacatcgaaggctcttttgtaaatatattgataagatagcttggtatccaaactaaaataattatgatccttattgtgtacataagaaattgggtgggtatagggcatataacaaaaaggtttcctcggtcataaaatgaaaaaagaaaaagcagacaggaacagtttgattctttaaacaagcaggttttggcttcttttttagcaccctaattctcttgttggctttgataccatgaaataaaatagagaaaaagaccttcaagagaataaataaataaaaccattttcaagagacaaactccagtgaacccctttcctcccattcattgccctttgaaagaagtaaaaaaaaaaaaaagaatctaacgctctagtcgaattgaagactttcaacgctcatgctatttgaaagagctttcaacatggagtggagactccataacgtacacaaagagtaagcgatctatgaatatcatcccaattcaggtcttgttccgcacttaaatggataactcaaacccttaccttgaccagtttgtagtggaaaacctcaatgacataatcgtttatagtcactcactggaggtttggaaccctgagtacagtgttccgggtgtagcaggaaaagaggctgtacgtgaaacagtactcagacgaaagtgctatttcttggccattggatcagcaagggtgtgattcagatggatcaagagaagaccaggtctgttgtggactgggaagtgccgaagaaggagagagcaggcagcagtggtgaagctggatgctcgaagtcattttagatacggcaagacagctcaggaggagtcgaaagttgccacaacctaggaggggtttctaggaagccaaaaaaggggagcctttttacatacttcttaaagggggagagcgccaggagaatgtcgagacgccatcagtttggagcgcgaggccagcagagcttgctgcagaggagataagaaaaggctcagcagaggggatctggtaactgttatgaatgtggaggagtggggcatttttctcgttactcttccaatgttcagacggacgaatgctgctaggggagtgcagaatagaccagctgaagatggaagagtgaacgttgtcgagcctagagcccgggaagctctaaaggtaagttcaagtcggaaacatagcgggggttctcaagcttaggagaggagactgtttcgctgtcgttagattgtgtggcaacgtgagccaacgtcagcagaaaggaggagaagacggaaggctgtattcaaaatctatgtcggaattggccagtgcaaagataatcattgatgctgggagtttggataagatagcgtccacggagatggtagatcagttggggctgaagcccttttaagtaagggcctcatccagagccctatcgaatcagatcaaaaagggcatgagcggcgggccctatgttgagtaaggggggagaaggtgccccttctgctaagttggagctagggaagttaaagcaggacgtctggtgtgacgtcgtccttatggacgtattacatatcctactcggaagaccttggtaatacgagtagggttctacctgcgtagagagaacaccggtttacttttaaggggaaaggcggttattgccatcagaagactttggttggctaaggagaaagggtgtttgttggcataccatttctggacgtgggaaagagtccatagaatgctatgccttgatagcaacaaagccaactagcagagccgattcggggatcggtgggatgccgtagctttaagagataggggcggaggcaatcagaaaggctttttaggaacgaggccccctccctcctatgttgtaaaagggaagtgcagatctttatctttctgcaacactcttccgacttgatgccgcccctgaatccacaagtaccggcttgattaccctctaagataagaggaggatatagaagcagatttagttgcaggtaggagcgagtctaccctgcaaagcggcttctcgcttatccccattttcaaatgaggagatccgacgtcaagtgcaggaattgctgtcaaaggggcgggagagtctcagtccgtgttcaacgcctgcttgactagctcaaaaggaagcagctggagtgtgtagatgggctttgaataagagttgggtgatttatttccaataatgccaacgatggatgatattatggattaattgcctgtcgggagcgtgttacttttcaaagcttaccttatttagaaaaggggaaagggcttttttttatagagagagagtaaggggggttttctggggctttgaagaagggccacttatattgcaaaactttcagagacgggatggaaagtctttcgtgagaagagatggtaggcttgatacggatacagctgcttatcacccaccttagaatcaagcagttcagttcgactatacccgccttaattccctcattcaggacagatggaagcaggttatggatctgttcaagttggtcgatcaatccctcccttctttcccctgcctccggacaccttagaatagatttgattggaaggagggtgaggaacgaacacagtggcttgactgctgggatcccaatcggcctgcatcagcagaaaatggaactatcgaatcacgggtgactcgctttatcgggatgggaagaattgcttaattggcatttctttccttccctaaatcgatccactagtaggtagcggtagtagagatccattatggtgggatggaccgttctcgaattccggccggcatttctgtcaatcggcggaagactcacgcatactgggagggtacgacttcaagggatggactcgatcgaacggccaaccacttgccatttttgtaggagatgaaatccaaaagaccattattagcgtgtagtagattggcccgagtgcgtaataggccagtcgagaagaaattcaatcaatagattgaacggtagataaaggatcagaggatgagaggggtagatctacccaatatggaccgataacggatggtccccgccaactgcttatctctcttcctcgcattccattcatgacctaacgactatccctgtttcggggagggaatcacttgctggatcgaacccaaggataggtttgatcggccgggtgttgggtcgaatgaacactcaaccgcgtcatcacggcagcgatggatgtccaacctttagatctcttctttctcaataaaggcgggtaaggaaagtccgaaggctaatccggcaactgctggctagaaggcgaaaaccgcttttgccaatcaaagccccaaaactagtaagggcactcgtgccccagcaagccaccccaaccctaccgccaaagcttgactttactaaacaagcgagaaaggctctttctatcttattagtcaagcgctaacgagcaagaaaacggatatgccctaagaagcaagggctttcgtgcagctgctgcgcccttgcttcttgctttagaaagattgctcgttagctaggccgttttcaataaggctcgcgctaggcgctcaccttttttggctgagccgtatcgtatcttgctggtaatggattgattcttgaatcttgcttggtttaggcaggtaagtgttaagaggctctttaaggctttcgttaggtacacataggactttcttgcaatacatagtggttggcttcgaatcacatgaagcccatatagatgtccactcctatttcctctaaagctctccctgtggggaacacaatcagtccatacaaggacctactgagtcatccacccttgcatctatttgatgcatcatcacatggccgtcgtctaactcctcgagaatcatgtcattcgcctgtcacgtgttgccaccagagtcataaatactcgaagtaagctcctggctcgcccctatctctaaaggggcttacgaacgagcggagtgcttacggccgtggtagctgcgagcctcctgggtcttgctctctcgtcttttttcctccgccttcctcttgtaattgaccctttcttttctgctacgcctatccatccgtcagattgacatccagccgggtgagcgatagcggctcctgtttactaatagatctgccgccgctagtataacaaaaaaaagcacataaggatccagaatattcaaatatactgatcactgatcaggatcatataaagcccggtattaccagaaaggatagtcgtgatgtcccttcatggccggcgttttcagtatagagccgaaggcgagggtttccagcaggcccccttctctggctttccctttaagtgacaaggggggtgaggtaaggagtagtataagagtggttcggtcatcgataagcctctccttattcattctatagggcggggctgcggaccaacaatccagcaaaagggctgaaaagctcctttattaaaccttccccttttaataataagaaggtaagcatcaaagcccagaaaacccaacctatacaaagagctcttttcagcccctactcctaacaagtgaaagttgctggcacccaccatatcttgcttcggggccgatctcttgtatcggagcaaagaaattcaatgattttctatattctatttctttctttttttgttgagttttttccaccacaaacagatttgccgcatggattggatagagtcccctgatctcgacattcaagcacgaatcccttgagcgcttcggcggcggatagcagcatgggcaaagcactctgctgcggcgagcagccggttcttattgcattcaccaagatagtcttgctcgctcctgaactctgcggcgagttcagccaccacctccgggtctgagctctgctcgagcgtagtcagccagcttcgtgactttgcttagcttccagccttgcaaagggataacctttcactatctaggcgccctcgaaggaggggtcccacggacttcttccccgaaggtcaagccgtagttcctgtccctgggagaagtggaaggagttaggaggatggagcgccctttgccctaagaaataggcggcttcgccttcaagccgtcaataaaatcgagctaatatgtggtcatgacagtacactgatgcataggtcttctttactttacggccttttgattatgatgcatcatgaacgtgccaatatgtgatcggggtgcgcggtggttagatataggggcggcttcgccggcttggattggaaggaagggcttcgctttccgatcgctttttgaggccgctttggatgagcgtgggcaagttagggattcactatcgctttccgcttggagcggctcacccccttgtcacttaaagggcgaagtcgccgaagcgagtctaaaggccaaagagtcatctttgaaggctactatgcatccttattcatagtagagtgtaaggtaggtttgggtatagcaggacttgaacctgcgaccattaggttaaaagcccaatgctctaccaactgagctatacacccaaaaaaagatgtagtagtaaataaggattggtacggaaaagaggccggccccccttcttctcatcatattaaaggagcgcggctctgtatgaggctcgtactgcagagcaggcggaagaaaacgtaaggtcgcgcgttagcactcctgcaagaaaacggatgcgctaaggcgcaagggctttcgcgcagctgctacgcccttgcttcttgccccttatttcaaactcttgatcgatatgagaaagatgcgctcaagcacccaacctatacaaggggcttgggctcgaaagccggccttactcaacaagcacctttcttagtaaggttgcttctttccactcattgaagattctatctacaaaagaaggtcaacgggggatactcaaattgctctcactgacaccagagaaggtgaggtcgtctttctttccagccgccatacggttcgccttaaagccttaaggagaaggggaggagcagttatctatgtaattacggtctttgttggccgttgttccggtcgagcactctcttttctttgtccaattccgtcttaccaaacaagactgacttcttaccaacccgcgaagggttgtgaggctggaccaggtacgaagaatgaatctatatctgtgcacggaagttgctggccggcggccgctcaactgttcgagcgcaatgcagtggtgttggttccgattcgacaaaggtggaatgcctggtcgaaggtccagtacagtaggtagcaggcgtgttcgttttggctcccgagcgagaacgataaataggcgatgcaccatccttgctgctacgtacgttttccttgacttgacagattcattcaattgaacccacactcaaaggaggaccacaagctcggggctcgacgaaacagaaagtttcagcatgttgaaacctcttggggttagcagtgaaagaaagagcccggcattcatttcttcatgaatattcatagctgagtctactaaaagagggaccagcctcgtcgtggtgattagaggacacctctgatcgttcacctctaatgtgacacgttccctcccagttatatgatcaacgggatcagtcggctagagagcggggctattcttcttccggggagacaaagtcgtcccttctactgaccgaaccctcagttcgggggccttcgtcaacatgttacgaagctccagtcttcggtgggtcaccattacttgacttcgaaaggcgaacatctgggcaagggaaagcgcagtgcgcctggtgcaaatggctttcttttttcatgatataccaatcagaatggagggtcctacctacgtacatgattgatagaatcactacgtagggggggcggtcaacttgatgcgggagaggcatgagtgcagttcgatcttgtggtgtattcgtttgtagtgagtagggcctctttctcgttgatcagtccgcctccgctctattgaaaagtcggaattcctacggcggttttgtcaacgaacgcgtctcgggccggattgactaacctaacccacccttaaggaggcttttccatagttgggtgtccgctttagtgtgatttacgaaggctaggctaggtttggtaatatccaaaacaaatgaaaagagatcggggtcgataggtggcagctggcaaggaacttgatcccccccaaaaaaagggggaagccgcggtcgaactcgaattctggaaataagtcggggcccttttaccaagtctaccagatagaagatgatagagggccaactatcgttgccttgcacaagacggtgccctttcacttcgagttccttccttcgtagtcaaatctgatgatacgctttggcgatgttacctaccaaataaaaggcctgctaggtgatcgaaatcgctcaggtcagtgaggactcactcactcacctactccttatctatttaatactttcttctatctacttaatttaaaaggcgacccgccgcgccgggctataagataagatacagttcttgtactacttgattgactggtaagaaagagcttccgtaagaactggaagactcttgtatgtacggtaaccctctcttccgctactggtggactgttgcacagaaagggcgacagaagcaacctttcttagcgcgcttttcaagcgcttagcttctgctagtggcggggcggcaaggccattaagttcagttggaagcctaagccaagaaggtacgaacgaagtgacgggcccctttagaagatagggggcggctttcttgtggtagtaattgcgaacatctctcctcttctcttagcgtgcacagtttgcttacatgccgccttaggcacatctctctttcttagtttcacgctggactaatgataatgaatgaaagtcagtcttttagtaaacgtatataagcagctgtttagtgtataagcaattctttagtggtcgcaccgaaagtacggtggaggttggttgaagatgatcttacgcggcgttcagaaccagtcttgaagtgaatgaattagaaagaacgaagaagtaaggaaatgagacgactctttcttgaactatatcataaacagatcttcccctccacaccaatcacgagtttttctctattcctctcgtatatcgtcgtaacgcccttaatgctaggttttgaaaaagactttttatgtcattcccatttaggtccgattcggatccctccgttgtttccttttccttccgcaccttttcctcgaaatgagaaagaagatggtacacttgaattgtattatttaagtgcttattgcttgccaaaaatcctacttctacaattggtaggccaccgggttattcaaataagtcgtgttttccgtggctttcccatgttacaacttccgtaccaattcggtcgatccggaatggatcggttaaacattccattagggagcctggtcttgactcttctgtgtggtattcattctcgttcggctcttggaatcacatccagcagtggttggaacagctcgcaaaatccaaccacttcacctacttcattgcccccaaccgtttctcgtacctctattgaaacagaatggtttcatgttctttcatcgattggttattcctctccgttcgtatctctttttccaatttcggtctcgattagttcacaagattgaatggccaattctcctccgaaccctcgattcgattgttttccaagaatgttgagccgggtatgtaagccatgtatctgggaggaacttaataaaaagaagggctttcggttttttgcaccccgttttggtcttgcagctatttttaaaatatacataaaagtctcttttttttattaaaatgattatatatatgtccaatctctagtggtggtggaaccaaccaagatgtatgtcgtccgacccgacctcagactccttcttcccgacctatttgactctctggccgtagttatttaggtggtattccgagatcgaattcctcccaggaacacacgaaacaaagatatgaactgggtaaatagaaatggaaaagagatctttctatttcatccaaattagaagctttttctacatccatatgatctactaaagtagatcggtattgaccatataataaaagcagatcttggtccatggagtcccaagaaggtaagaactccaacctgtccgatgcttcttcggccaaatacgatatacaagtgggacctgcactatgagcaagctgtgcgaaaaaccgcttcttttttccggttccgaaagaacttgggcgaaatagggttctaccgggaaaccatgaatttttgagttttcgccattggttactggttgagccactggaatggaatgagataagaatctctggagatctttcctctccacttactcgtaacaggcttttcttctgtagaagactttttccgaatggcataattgtccgacactacgttcctcgatcttcaaagaaaactgactcctcctactccaccttctcctttaggataggatcctccttggtccttctttcactaatggtctcaccattttctagtagtagttcgcgcgagggactatcctttctatcgcttgcccttgcctttcactctcatttggtctctttcttatagaaaataaagcgaagcaaagcgcatggcaaagaagcagccagctgactgcccccttccactcggcctttcttcgctgtgtgaataaggtcttagtctgtatgggcattctgggcaggtcgcaataagtcgctagtcgaaggtttagaccaatcgcaattcatcaccatcttgcccgcttccaattgatgactggctattatataagtgttgacctaagcccctgcgcaggggctcggctcccgaaccgtacgtgagctgtctcgtacggctcttcctaagaacttgaagccccctctctctaaatagaaaaaaatgaatttacaaaacaaaaaagactttttcaaaaagccttcgccctcctattcaagggggctattagagaagcagcttcgttccttgacttcttttctcagtcaagcttccttgttccttagtgtagtctcggtccatagtttaagactccgttccttatagcctagtctatatccacagctgacgtgactccgtaccgacgcctttccctttgtatagtatacggctaagtgacttcgtaaccttaacgtactttttttcttactgtagcataggccttcgtcgggctttcgtcccttcgcctatagacggcggcttggcttctagcactaaataataggcattaggcattctgagctgaaaggaggcaagcaaatgaagggaggcattacgggccgactacaagaaaagcaaagcttcgtagactcggtcaagtcgcttatagaatgccgacgacgattttccacttaataagtgaaggggagagggaagcgaggcttagcgagctttataaggccgaccactacataagccgctggcggagaaagctcgaagagcttcccttcattcattactaagccaaggtcccaggtctccgagtcagcccgcgctttttcgaagaatcctgcacccatgggcatacggcctggcaggccttccctttccgccggagcttcatgggcgttgccccgttccccaatcagatgtttggatgtgagctatactccgcgaggagccaaacgggcgtatggccttgccttgccatttgacctcttttcccgtgtgactaggaatgctcagtgacaacctctcaattgtcaccgcctggcctctcttgctaccacggtagcacctagtgtggtcagcaccaatcgtgttcgggcaacgaagcttacactcattcacattggttcatcctgctatgccctgggccttttgctcttctaacgtaaaaggtggccggccattcgtcaaggcccaggaatccgctggacatctcagcggcgggatttgatacccgcatccgatcgaagttgcattttagtgctcccctaacataaaggggagctttttcaaagtgggtcgcttcgcgcaagacattgcttaggaccaacgggtcacacgacaggtgcacgatctactttgcacgttccatccttcagcccttcgcctatcggcttggcaggcaagctaccttgatccgtcttcggcttcgattcgttacgctcagaagctccaacaagccctaaagtctcttgccgcctaaaactctgccaagagagcgctgctttacgtttgatcctatgtacccatagaatgctatgcgttctccactttcggatctcgcaaagagataacgtgttttttcctctgactttctctctcattcgcggagcgaagaaagcgggctttgccccagctaccgctatccttgggaaaccaaaagagctaccgaaggaaagggatgcagtctctcccttggcctttggagaggagagggcagagaagaaaacgtccttcgcgcaagtttttttgcttcctgcgtccttactagtaaaaaaggggctcttcgagcaagaaggcattttggtaggaaggccgaccactacataagtcgccatccgtccaggagagaagcaagctacctttctttgatcccccttttcgggcagggaagagaacgaaaatggaccgcagatggtagtcgtggttgattcgaggatcttacgcggcggagcgaactcttctatcgtgttgcattttctctggcggaccccccccccggtccatcgtactggagcgattcgagaagaacgattaggctcatattctatcctttctacaatgcctatagacgaagtgcttcgtttcagatcaattcttcgctgcaatcgcttcgatccaccccctcggtgaaaaaccgtaatacgccctgaggaattcctaccagcagacttccctgtactcaaagtgaattgtctaagtgctctcctttgtctcattgtttatctcgtaatcattcgattccgcccctaaagctagcgcctactcctcctccttctcctcctgaatcctccttggtcctttttacataacactctcggccgcccaagaggactggctatctttctctttatacgcacaatatcttgaaaggcaaagaaaaagatctaccttggcaacgaagacgtcattgactgatatattcattgcatggaatgccacactcaattgtcagcgactggggacccggtcttcattagcaatttatggcatgagctctttcgtttacaagggacacaatttaacatgagtactgctttacactcttttcccgggtggggcttcttatacctaaacgcagcaggccccgcgagtagtcgaacaaatgagaggttgtcgacgaaggggtcaaaggttgcgcttgcgagaatccgaaggttgcgcaagaccccttcaacctcgcccgcgtcttagcttgcttgtactatcgctcgcctgcctgacctgctttctggctagcttctttatggcaagcgctaccgtaacctagctagcgctacatcttgctaacgtcgtctgaattgccttgcaagcgctacatctatatggcaagcgctacccgtcgcttgcactacattgtctgacgataaccttgcctgaccgcttccgctctgactgagctgaccgccgcacctgacttctatatcccattatccatagatctccttccttatcgttgccggtctaagcagaaggttgctaagtcagatgtctggtgaacacattcgtaatgagtatgggtctagtaggtgtactagtaaggaagcgaggtactgagtttagcgtcgacaaggcaagtagtggatctttattctcgaatgatatgggagacagtcaaagcatcagtctcagcatcaacagaagaaaaggactgaccgaccgccgttcaagagagatcccgaaggctcgaactttttgctagctttgaaacatgggccgaaggaaagaggaagaccaaacaaagtcgcggtcaaagcaaagaaaaagatgccaaaaaagattcactttagcttctagctcgcttagtgtaggttgcttgcaagactttcgatagctggctcggccgaacggaatcaccgatctagatagaagggtcgttcactccctattctttgagaggttgcttgcgacggtagcattagctaggcaatcaaggcaggtcgaacagagtcagtcctagggtgaagatcatcggatggaaaaatggattgagctggctaatcacttgatgacccggtggagaatgggaacagagagtcgctcccataaacgaatgaatgggactcctggtcctgatcgaaccagagattccgacaacccggggaatcggcagaaagagatggttcggatactggaatctgcccaaaagtcctgactttttcgaggcagggcttcgacccgtatctggccaactcctcgaactgctgggtgcggcatattcatggactggcaaagcgaactctcaatttgatcaggagagcctagagagctctctatctttccccaaattccgactagcgcggttctttttctcgaccaatttgaattccatttcattttttattttaagttaagtagagtagtaagtagctaggcggatttcagcgcatgctgcattgagaatctccaaagaaattagaagggcctatgagagcgtattattcttcccatttgtgaccgacggttgcttgcaagaggtggcgatcggcagtgttccaaagcgccataacgacgtgcgttagagcgttatgccaaacgatccccagcaccagtagttatggggatcgccttcggcttgctatactctttccctaacgcatgctggttaccataaagacaccgagggatatcgcatgcgctagtttcggggatgttgtttacactactattggtaacaactcaaagtgccggaacgactctagtggtgcaagcgaaggtttcagtcttgtcgagcgaagcaaccactagtcgcccttagtgctccaaaacaccctttcgcttgcgtgagcaacggcccctagcgcccagagcaagcgcctttagtgttcccgaccgcctgcctttcggccttagcgttccaaacaaccagtagtgtgaccgatctgtgttcaaaacaaccgatgacgctagcgacgactcgtggggccccctaacgccgaacaaaaaggactagtgctataacgacgagtggtgtggtcctaacaaccgactacggtaacgacaactcgtagtggtcctaactactagcaacaaccactacggcaagcgccacaacgacgataggtgaggctagaccgtaatataggcttgcgaagcaagcactcgttgtcctttagttgtccgtcactcgtagtctctgcgtcagaggtggttgttcggaagggtttgacaaggcaacagacagccaggcagttactacgcaacacacattggggtggtgcaacaatggaacgactagtagtctacgactagtggtgttacggaacaactacccgacgagtggtaataacgacaactacagtaggtttgacagtagcgttaggacgactggttctcgtagttgtattgccctaaggcaacgactcaaacaacaacgagtgctcccaagacgatgagacgcatgcgctataccgtcgagtattgcttgcgaagcaaccgcaactcgttgtaggtcctctccaaccattacagtcgagtagctttcactccttcgcttgaaatgtgcggttggtttacctaacgcatggcttccccaacgccaatagtcgcatgagttctcctaggccataacccatgcgttgaaagaaagcgcatgatgcgttccggagttgccgtagttccgttaccgccttgtcgtcttgggttgggaaggatacgacaggctcaattcaaggacactcaatttcaagctcaatttcaggctttcgaagctctgacgctttctgtcgcatttgttctctcttttgtttacctttcattttcactttctttaaccgtacttaggtagctcttcgttcggtagaggcgtagagtcctagaacgctatctacttggtcgcgactggctctgctacgctaggttctccctatggcgctacgcatcgttcccttcggtcgagcgaatcccgttgttccggtccgagaatccctatgtctgaggtcgagcagctaggctctcgttggtcgaggttagatcctcgtatgtcgccactctcgtcactgggcgttgtcactgatgtcttgttatctcaggacactctgccaggttgttccttgttgaccggccttgtgattctcgttatagaatgtagtgcccaacagtttaaaggaacgggtgaagtctcgggatccgctctagtcgagttgttagatgtctctctccggagtcgctcctctatctttcgtgaaagcatacgagtcgttatgttaagcatctaatcctagtctttatgttatctgtgttagaggagttagatgtccctcatgttgaacagtctgacatcaagttgttaggaccttagtcgctatgcgaacacttaacacaagactgaaagcgttagtggtttatgaatcagtcatcaaggatcttagccaaacggtgaccggctacgtaagcactttgggcgcaggtttctcgatcggacttgacgaattgtcataaagacatcactctgctatatatataagaaaattggattctaaaaaaagattcaattaattagaagcattcgcagttttcagttcgtttgtcatcatctaaaagaaaagagaaaacgaaagtcattttgaaagacaaaactgctaagctataagtagaagttgttgaagtagaaaatgcttgctgctcgcttagcgcacggatcataggctatctcatcactcactaaggctagcgaaaagtgatcgaataaagcatttgttcgtacagctctcgaacctcacgctctatcacgcacggaaaagaagctgactcaaagaaactagctctcgcttaatccgcatatctggaactccttgatttgaactactccgaatccggcgatgaactcacatttcccccctggggggactcttgcttctgtcttcctctttctggcatctggtggaaatgttatctcgatcgatcagtttcttctactctatgcctactaaaagcttaaccatgccctaccaccaagaacagattctcgccatctatttataggaaaaacttcgcaatatgccagagctatcattacctttagttgattatgtccagactgggaacaagaggcctggtttttttcctgtgtctgattccagagtatcagcaccagttgttcttgtaatagacgagtgtttagatgaacctcatctccagcatctacaaagctccttgcatgcatttgtagattcattacccccaacaacaagactcgggattgtcacgtatggcagcacagtgtcagtttatgatttctcagaagagtctatggcatcagcagatgtatttccaggtaaaaaatcaccaaatttggagtcattgaaggcattgatttatgggaccgggatatacttgtctcctatgcacgcatcacttcctgtcgcacactcaatattctcatcattgaggccatatagactgaatatcccggaagcttctagagaccgttgcctgggtacagcagttgaagttgctttggcaattattcaaggtccatcggcagaaatgtcacagggtgttgttaaaaggcccggtggaaatagcagaattcttgtttgtgctggtggacccaatacttgtggccctggttcggttcctcattctttcactcatccaaactatgcccatatggagaaaactgcattgaagtggatggaaaacctaggtcgtgaggcttttaggaagaagaagactttgatttacatattttgtgcaggcacatgtcctgtaagagtgcctgtcctgcaacctcttgccaaagcctccgggggtgtacttatactccacgatgactttggagaggcttttggtgtgaacttgcagagagcatctgggagggctgcaggttcacatggtttattggaggtccgctgttctgaggatatttttgttagtcaagttataggccctggtgaagaggcacatgtggacagcaatgaaacttttcaaaatgacgagactcttgtcatacaaatgttaagcatcgaagaaacacagagctttgcattatccatggaaaccaagagagacattaagcgcgattttgtgtatttccagtttgcatttcaattttctgatgtctaccaatcggatatcaccagagtcattactgttagattgcctactgtagacagtgtttcatcataccttgagagtgttcaagatgaagtggctgctgttcttatcttattgccaagaggacaggagagccaagaatgccaatgatgcacttgatatgcgagtcacggtcgatgaaagaatcaaagatattgcaagcaaatttggttctcaaatgcccaaatcaaaactctatcggttccctagggagctctcattgttaccagaactcttattccatcttagaagggggccacttttaggaagcattcttggtcatgaagacgagagatctgtgctgcggaacttgtttctgaatgcagcatttgatttgtcccttcgaatggtggcatctcgctgtctgaaaaaaaaaaagttcctattgtaagaacataaaagaagcattccacagtcgtaggttcttctctttctctggcataaacaataaaaagcttcaactaatccgatctttcaaccgcacttcatggcaaagcggtcttctttcaaagaatctccgtccctagtccatacccacgtctggggaacttcttcacttcatgttcacatctttgtctccctctttcaagtgagttcagttagcccttagggtcagaagagagctcatctttacttcctttcctatagaaagctactgattctcttatagccttcgttcattttgtttaagaaggctgcgacatatacagcatctttccttatactttttcttgcctggatgaaaatacaatagatgaatagtcattccctcacaaattctttatttgaatatctttgctttgttcgttctacagatatagattcaacttcctttcttggcaccatccctattctgatggctcagtacaagaccgacggaagagaaggggtgaaaaggctagcgaggcagaattctttttctctttcatagcgccgcacaatggagacattgtagtgctagaccagatttaccagcggacagttgaaaaacgatacgacccaggacctccctccactcgtgggacggggttcttctttctatcaaaataaatcgaattcgaaagcgcaccacccttctttactttacaaccagcctccgacccaaggtgcttttagaaaaggtcagcggggcaatcaaaaaagacttgcttttgacgccccgctgtgccgaccagcagcgggatgctacttacgagctggtcagggacaggttccggtcactctttcgatgccatgccattgtggtggcacgggaaccactgaatgggggctgttttcatctcatcgctggcgtgtggaagactagtgcatccaagcacagcgcagccaagagggtccaagattgcttcgtcgaatgggacggacatcgatcttcgcttctacaaggcctggtcgactctttgtaggagcctttttttatcaaggggtgacctggcttcctttcctttacctttaaacagttagagcctcttctcttatcagtcctttcagtcagttccttttcggttagctacttaggatgaatcacacagaggcgatctctaacataagaatacaatattttcaagagacagaaggcttaagagagatggggaacttctctcctataaatcttctttgcacgagcttctgtaagccccgaaacagactccaattacatgtgttaagcatcgtgccatttcaaaaaaaatcaaataatagagaaaaaacggctagaaagaaggtcaagtgaggaagccataatcttcataagcagacgtgtgagtctagctttcaattagcgaagaaggaaggaggcaaagcaaggctttcttctttctttcagagtgagaaacgaatcgaagcggggaggcttgaaaggtccttcgaggctcgtcaatggcttggcttcaggtcgcgaatggaagcgcggattagcgggtgtccgcttgactcagtcatagtctcgcctggtacgcactcgaagcctatgttcactagaaaaatggaaaaaaaaaaaaagtgtgaagatccgcccatgattcatggaaccattccttcgcgtgccgtagcttaggattcgtgctattgctattgtttaggggcgtcaagaccgggttccgactttttctttttgagaaagaagaggttactggacaagcgaaagagatgccgaaagagcagatgcttttatttgaaacaaaagcattagccgagacatacctcccgctaaagaacactattgacaatggggtccgggaggccctcaaaaaaagcgatagagcaagaaagaaagaaaggatcaaaacatcacgcacgggccgcacgcaaaagaagagagaggatagccagaattgtattgaggccgcagcagcaagaaaacaagaagagcacgtcttcccaaacaaagcagccttcagcaggagctgcactacaatgcctcagctctgggaacaggaaggaactgagcgccccggcgaataaagaaaacctagaacaaaaatggaagcctaagccttcacatccgaaactgaaaaatcatcagttggagaatcgtttttacagggtaggcatggtgaaggcagaatggaaatagaaaacaactaaatgacttagtcttggcttcttcttcctttatggagagaggcccctttagcttcagggggaaattcctatgtctttctttcatcctctctgtctatggcctatgccaattggtcttattcggatgagttgcatttcgttttccttttgttagtttctcagtcagggccaaatccttctccctaaaaattccagattttctttcctcggcgagtgaagtttctgcccttgttgagtgagtaaggcccgatcgagcttatgtgcttgccaggtctttcaccatctgcttttcctcgagaatgtgagactgctcaccctcagtaatcgtattgtccgctcttttcattgattgtacagctttctctaaacaaggaatttctagggagtcctcccagtcggctaaaggcgcaatggcttttggttttgaatccggctaaggttgaatttgcttttgctttagttgttgtcgtagagcgaccttctgttctttcagttgtgtaagccttccacctctctcttagctttgcatcttttccattcggtccaagaactaagagcggtcgaagtcctgtctcagggaatgggcttgaaggctagtggtcatattagtcgtctaaggggaaatgccttttccgggcctatccccattcgcctatcgctttcttgagttgatgtttaacttgcacctaggggattaaatcttccttgaggttttagtgggagttcctttttgatgcccattcgcgagtggctaaagggaaatttgcttgttccgatagttagtctaacccctttcccgcagcattccattcgaagtcgtcgaaaaagtctaagacggagaaagtggtgatgctctttgattgcatccgcttgcttgatctttgatcgtctagctgtcccctaagcccctctctttagcctatgttgtctcagtcttggatagagtccattacctatctttctttgtttgaatgagactatctgatgtcctttcatctcaaactgaatgtaataagagtgaaaaattaggaaatttcgtacgaaaaggaggctatgtagtatggcccctatcccttctttttacgccagttgctctgctccttatccctttggggctagacctcagttcagatcatccttggatgctagcgatcctttcaccgaagaactcttcaaagaggacactggctttctatctttgaagggtttacccacagaccagagggttaaggctctcaccttcttttcaaatcaaagaaagaagagcccttcgattcgggccctttcccacctccttagtatgaatttgatttatcctttttctttgttgcgtacttaacctgaaccctgtctatgagtatagcaatcctttgaatctttcctaatccgctttctctttttcttatgccttgggagcccagtctttaggagaagcagctgctcactcgtgacaatggatgcctgcttatgtcaaactatcctcaatctctttcccctaaagctaggatttttttcttagcttccgctatttcaagagtttgctgagcttcttgtggatcaatgtcactacccttctccgcatcatttactaaaacagtgatctcattattgcctattctagcaaaaccacccatcagagccatcgttaaccattggtcgttaaggcgtattctcaaaatccctatatctacagctgtggcaataggggcgtgacttggtaatatgccaatttgaccactatttgtagataaaatgatttcttccacttctgaatcccaaacaattcgattaggggtcagtacactaagatttaaggtcatttcttcgcattgctctccatttctaagttcatagccttcgcggtagcttcatcgatattacctaccaaataaaaggcctgttcaggaagaccatctaattctccggaaaggatcaattgaaatcctcgaattgtttctgctagaccaacatatttccctggcgaaccggtaaacacttctgctacgaaaaagggttgtgataagaaacgctcaatttttcgcgctcttgctacgactaaacgatcttcttcggataattcgtccaacccaaggatagctataatgtcctgaagttctttgtaacgttgtaaagtttgcttaactctttgggcagtttcgtaatgttcctcaccaacgatccgaggttgcagcatggttgacgttgaatctaaaggatctactgctggataaatacctttggcggccaatcctcttgatagtacggtagtagcatctaaatgtgcaaatgtcgtagcaggagcagggtcggttgataacccacagcggaaggcattctacccaataaggccgatacttcggatcctgcttggacgaaacggaagatattgtcaataaatagaagtacgtcttgttcattaacatctcggaaatattccgccatagttagggcagtcaaaccaactctcatacgagctcccggcggttcattcatctgaccgtaaactagggccactttagattctgcaatattttcttcattaatcaccccagattctttcatttccatgtaaagatcatttccttcccgagtacgttcacccactccgccaaatacggatacacccccgtgagctttagcaatattgttaatcaattccataatgagtactgttttacccactccagctcccccgaatagtccgatttttcctccacgacgataaggggctaaaagatctactactttaattcctgtttcaaaaatcgctaattttgtatccaactgtataaaggcgggcgcagatctatgaataggagacgttgtactagtatctacaggccctaaattatcaacaggctctccgagcacgttaaaaatccgtcccagagtcgctccaccgaccggaacacttatagcagctcctgtgtcaatcacttccattcctctcgttagaccgtctgtagcactcatagctacagccctaactcgattatttcctaataattgctgtacctcacaactcacattaattggttgaccaacactatctcgaccttgaactaccagagcgttataaatattcggcatcttgcccgggggaaaggctacatctagtaccggaccgctsgtaacctcgctcctgactattcatattcacggcttattcataataaaggctgtaacctcctaatcaaggagtggaattctctgctcccctcggaaaaccccattgctttgaccatcctcaatgacctgaggatgcttctagccttcaaagaagagcaattgaccactactactataatggagaaaggacaatctgccttctaacccgaggtccaggtattccggccccagagagagagcgtgccaaagcccgatgaatagacaggggatggacagtcctcccgttcagggaagaggaagggggggaagtccttggcattcctgcctttctgtcaaaaagacaataaacatagaagagaaaaagactggcgtcctcccggaggtctagccggtgaaggccaacttaagtactgacctggcttacttaacttaataggcttgcagaggaaaggcctagcccttggagccgtaccaccaagaagaagatcaggggaatctctaccatcaggcttcgaatctgaggttgaggtctagcctctcttttcagtggaagttgagctcgtcggatctgctgcccgtgacgtgagtgatcgttgaccctgccccttcttattgctatttgtgacatcgagtgcttaagtgagatcagcggtctggcaggtccttggacgctggcccttatagtctagtctactcggacctctactagggctagagctagccggaaaaagaaaagacttagccaaaaagaagtacataataagaaaatgctccacgctctaccttccgtcctccttaaactaggctttcttgcacagtagcctacctttggtctcaggttcgctacttgctagcctagagctgaccctggctgtgatcaagaagtctgcagctaattctagtttcggggtcgccaaagcattgagagatggaaggaatgctctgtctaaccgcaatgcttgtctggcctctccagccaaattgagaaattctgagagaaattcatccttccttctatcttttttttctgaaaggcgggtcttcctagtgggctcgtcgccactaggcagtcatctttgatcctgatcggccgacctttccgatcccgaaacaaagagagttcggctctcttttttcgctcattcagatgaataaattccgtgaagacgacgagagatgccgcctgctctttccgttccttctctttcggagtggagcactcctctttgttctgttcctttctaataaaagcttggtacgtgttctgagcgagccttcacgtgacgtgaacggtacctatgaagtggaatccgtttgtcttggcttccaactcataagggagttgcgttctgagggactcaaaatatccacagctattgtcaagcttgggcatactaaagaatgacccaattgagaccgtggccacaccttgataaaacagtgatgatgtggtcaaccctggatacgtggctcttcgatgggggaaggaccacgctagtcgtctgagtgtgtggtgtgtagtgggtgcgtcttagtgtcttcttactacgaaaaagaaatgagaaaatagatgattctcgttctcgaaactccactctttttctctttcaaaccaggaggattggcatttggccaagatgtgatctatctctttccttggccttctttctatttagatccccgttcgtgatcccagccctggaatcacttcactctttattcaagagaataataaagtaaagaagaggttcaagacagaactgtgagcagggatatttagctatttagccttagagaaaggctgacttgagagccctagtcccttacttttagagaagaaggacaactccgttcgtgattcccgggtggggatcacttcactcctgcgcctgtagagtctttaagcatctttccttgaaaatcgactaagcgggaagcctacttgtgaagtgggctattgcagagtgaaggaaggtgggttccagagaggattgcgcctaccaaagctttgactctgagagtgagagttgttctgtttgagttctgaactagaggagagatttcgattatcttcgattctagggtcttgtgcttacctaagtgttgaagcgtggaagcggaagatcaccctaggtgacttagtttaagagcttcggtatatagaaagcaaaagcatatttttttttagaaatttctttcactttcccccctccaaaagagttctttcttcctccattagcatagttccaaacctctattgcttggatgaagagcttgatgccaaagcaatagtgcaataggagacgatggccagtatgaagagattcaaaaaggatgcttcccgagaaagctttttgctttctttactcaactcgtcgcggcgagctaggagcatctagaatagcataatggctatcttttatttataggcttcaaacaaagagtccaaagattgaaagggcaccaaaggtgaaatagccgggataagggctttggctttctctctaatatgccagatgccggtgaaaggaagggaatgaaagatggcatgaacacaaaaaactgccatttccccctagttggagtcttagcataaaatagaaaaggaatggctgccttaactttactaaaagtaaagttaagaggcagattccggactggagcattaaaaggaagacttgaagccgctttagaataaagaaattttttctatggggaaagcatcgaatcctctcttttcacgaatccgcagcaaaaagacgcagatattttcatgaagaataagctcttagatgtagcattaccggacgtgaatctaaaggttagaactaataatctagctctttgcaataagggcttttttcaggacaaatgccaaacgcaaagaaagcagaagatgcggcttagccagctcgctctagtcccctacaataaggatgagaaaaggccaaggagtgaataggagggaataggggcaatataggggcatcagtcttagctcttactgttcgagaatcaactgtacatgaatgcccatttataggctcttccttaggccatcaaggaggaagcgagggtgggacaagtgaatccgatgtgagggaaggattgcagctagagtcgaaactagggcttatgcaattgaatcagaaaaggctgcacatgtaatataagaatgggaggagacagccaaagctgggattgattgatctattccaaaaccactaggaagggacctattcctaagccattttcagtagacagacagggaaaaggactaaaaagattcttcgcaagatgagagcaagcattagatgaagccgactttgtccatctcgcatatcaacatcctctatcgatagcctaatatagccccacacagagaacgaagatggtcggtaggtccttcctctatttcaagagttctagtacttgcattgcggtccgtccattagttcgatgattcttcttcgcctttaagttaaggctttttcaatcaatctcataggttcctatagctcgtcctataagaaagtgttggattcaaagctggtgttaaagagtacaaattgacttattatactcctgagtaccaaaccaaggatactgatatattggcagcattccgagtaactcctcaacctggagttccacctgaagaagcaggggccgcagtagctgccgaatcttctactggtacatggacaactgtatggaccgatggacttaccagccttgatcgttacaaagggcgatgctaccgcatcgagcgtgttattggagaaaaagatcaatatattgcttatgtagcttaccctttagacctttttgaagaaggttctgttaccaacatgtttacttccattgtaggtaacgtatttgggttcaaagcccttcgcgctctacgtctggaagatctgcgaatccctgttgcttatgttaaaactttccaagggccgcctcatggtatccaagttgaaagagataaattgaacaagtatggtcgtcccctactgggatgtactattaaacctaaattggggttatctgctaaaaactacggtagagctgtttatgaatgtcttcgcggtggacttgattttaccaaagatgatgagaacgtgaactcacaaccatttatgcgttggagagaccgtttcttgttttgtgccgaagcaatttataaatcacaggctgaaacaggtgaaatcaaagggcattacttgaatgctactgcaggtacatgcgaagaaatgatgaaagkaatgttgtgttgtaatggcttgtgctaaaggaactgagagatgccatgccacgatctttagtattcctgctatcccaaagggcgggaaggaagagagcattacgaattgccctatttgagatagtctctataattaccaagacccgtacatactaagatcgttctagcgaagtacgagtttacgaggcaatttccttccgagctcacattcgttctagactctatttagattattatatctcataagagaagaaagatcgtaggaaaggtgaagattcgagaaaacgtccgttcacgtcaggcaatgtttcgtttcgagattggcttcagccttctgcttaacacatgcaagtctactagttgatcgaccgattcccccgagcttaggggtcaattacgggggaatcggaaactattgtatcttttctaaagtggcattctcccttttgaggaccggctttcctattgatttgacttttgcgggattatgaatatatcaatcgactcttgcattcctcccttgctttccaccggccttggcctgaaaatgaagagtcttctctgctgacctatagagaggtaggaaagattttccctacactggcttcctcccctagctactgaggaagagggatctcgaatcaatcaattcctgggttgttgtattaaagaaagcttttagtgcgcgttgcatgctttgtaatagtacgaactcattatgctcgtcaactaggtcaagcaggtgaacccccttacgctgtctgtgactttttttgccttcaaaaaccgatgcttaaaacatagaattctatcttctcagtcgtcgatcgatcattctctgcggccaactaaaaaggatggaaaatataggcaaattctgaaatggaccgagatggcctatacaccaattgactgagaaaggaagattgttgcaagcccttaaaagtactctaaagcaagccttgttccaggcagaggcccacggaacggtaatgaaattccctgcctgcttcacttctttctttattccaaaaaaaggtccaatcagaacttttgctaaagctgtcgatcaggtcggtcaggcaacgataagccaataggcgatcctaagagccagatttctttcttcgagctaaagaaggttcacctaagaaaagacaatgtctgagatttccgtcaattgacttttggttggctaatagctcgtcaatttctagattttccatggtacccgctcattgatggaattgatgcgtggaatgctaaacccaagagagtgataccagcgagtcgggcaagagagctaggaatagttagttagccattcaagtgtgctattcctatggggaaggataactcctttctctgacgagaagaaggtttgctttcgaataaataagccgataggcgaaagaatagcacgagcgctagagcggtagggacggggactaacccaccatctttagattttggcattctttcttgtgacctaacaatttagatagtgtggaagagcaggactatggtcaagtgatccctcgcataagagcgtgttaccagggtcccccagttggagaagaaaaggcttgcattcacccattcgattcgactcgaagcagacagttcaattgaagcgcgaacttcattttcaccgcctaaaggccgaaaaataggactttgttaccggaaaggcgggaacaggcgcctaagaaagagagccatctttgttgacagtagcatatacctcaatctgacctaccagccttcgtatttaaacggatgcgtaaagaaagaaaaaagacagacgacgcttgtagtaagccgaaggagctagcccaaccaaagtctgcctttattcgctaggctcagtctcatatgtaacgatacctggctgacaatccattctctctcatgggatataaagaatatgtgaattagaagcatccgaggcaaaaagaggtcaaatcccctagttgggctttcttcgagcaagctcttagcgacgaagggactcgttttctattaattgttggtgtgatcgtatcagctgtgattgagtatgtcagtgtgaaagaaacccctgcagatctgatcgtatcgggtgctttagtatgagtacgagtaggaactcctgcagttgccgttgctagtgttttcgtaaccggtcttcttcttagagtaagcgctgaaattgaatctactcttggcctatcagctcttgtgcactcattggcagttctcgaagaagcagctcttgaggaagcatccaattcccagtctctatccaatccatgcggcaaatctatttgtggtggaaaaaagtcaacaataaaatataggaacttattctattttgagaataacaataaaaagaattgcttaagtaaggtagtcgtttctttttttcggtataccccgctctgcgagtagagcgaatgaagataaatcttacctaatctcatgaatatccttcactcaatttctcgtctttgtctgcatgtgtcaaaaaacctacttgttccaaccaatctattttttagaaagaatatcgtccgttgtttctccccctgtctcctccttcttgtctttctaactatcatctttctagttcttggcaaaagtgacctctttcacttttacctttcgaaggcattcatagccgcggtaagccgcaccctctcgtctttattaatcaagatgggcttctcgggcgtgctagccttggccgttgcatggtctctgaaattttttttcattgcagactcatgtaacatgatggctccttcgggggcctctggctcaggatcaggggagagcgctggaggaaggggcttcaggtggactgatttatttggaagcagttcccctgctaattccgaagcgagtctggaccaaccggccccggactctcccaaccctggtgaacccgcagcgcctattgctgaggtttatcatccgttacaggaggacgaacagaggcgtcgggagctcagtgatcgtcttgcactgaatacaattaaggagcccttgagcgaagagatttttgaggcaattatagaaactcaattccaaacggaattgaaaattgagaaagctcttcgctcggacatggttcaggagggttccattttagagaagaggcacaaaattagaggggcgctcttctattctaaaggaaggccattatcattggcgacctatttggaccaccttaaccaaatggagaaccaggggacccaccgtagcccgccttataaaaaccttatgaaagccatttttgataagatggaatttgacctggattttaaaggaatcaaaaaaaggagatactggtagagctcatctttgtcagcggcattctccctttactttctaataattagatagattattatggaactttctccccgagctgcggaactaacgagtctattagaaagtcgaattagcaacttttacacgaattttcaagtggatgagatcggtcgagtggtctcagttggagatgggattgcacgtgtttatggattgaacgagattcaagctggggaaatggttgaatttgccagcggtgtgaaaggaatagccttgaatcttgagaatgagaatgtagggattgttgtctttggtagcgatactgctattaaagaaggagatcttgtcaagcgcactggatctattgtggatgttcctgcgggaaaggctatgctagggcgtgtggtcgacggcttgggactacctattgatggaaagggggctctaagcgatcacgagcgaagacgtgtcgaagtgaaagcccctgggattatagaacgtaaatctgtgcacgagcctatgcaaacagggttaaaagcggtagatagcctggttcctataggtcgtggtcaacgagaacttataatcggggaccgacaaactggaaaaacagctattgctatcgataccatattaaaccaaaagcaactgaactcaagggccacctctgagagtgagacattgtattgtgtctatgtagcgattggacagaaacgctcaactgtggcacaattagttcaaattctttcagaagcgaatgctttggaatattctattcttgtagcagccaccgcttcggatcctgctcctctacaatttttggccccatattctgggtgtgccatgggggaatatttccgtgataatggaatgcacgcattaataatctatgatgatcttagtaaacaggcggtagcatatcgacaaatgtcattattgttacgccgaccaccaggtcgtgaggctttcccaggggatgttttctatttacattcccgtctcttagaaagagcggctaaacgatcggaccagacaggcgcaggtagcttgaccgccttacccgtcattgaaacacaagctggagacgtatcggcctatattcccaccaatgtgatccccattactgatggacaaatctgtttggaaacagagctcttttatcgcggaattagacctgctattaacgtcggcttatctgtcagtcgcgtcgggtctgccgctcagttgaaaactatgaaacaagtctgcggtagttcaaaactggaattggcacaatatcgcgaagtggccgcccttgctcaatttggctcagaccttgatgctgcgactcaggcattactcaatagaggtgcaaggctgacagaagtaccgaaacaaccacaatatgcaccactgccaattgaaaaacaaattctagtcatttatgcagctgtcaatggattctgtgatcgaatgccactagacagaatttctcaatatgagagagccattccaaatagtgtcaaaccagaattactacaatcctttttagaaaaaggtggcttaactaacgaaagaaagatggaaccagatacattcttaaaagaaagtgctttagcttttatttaatacaatacaagaaaaagcaaaaatagctaaaaacagcctgcctcctttatcatatatatgagatgggcgggcctttttaagcaaaagatgatccgatccactatcggttgtaatcttcttgacatagaaagtcctttttttccaattgatcgtttatgaaatggaagagtagctcatgttagactgatgtgatgagcgaggcccctagcgatggggggaaaggggagtgggtaagcgggctcctttcacttgactgcttagttaggagtgatctttcccatgctttccgttggtcaacaaccaaccaaagtgctctatacttcttcactactcgtacaggcttgacggggttaagctgtattgagggaatcgttttgtctcaatcaatcaagaatgcctcaactggataaattcacttatttcacacaattcttctggtcatgccttttcctctttactttctattttgcgtgttccatttttaatattcaatataggctttactttctctatgtgatagatcctagatttcagcggatcattttctacttgaaattttttttctttttctttttagtggtgcgcgctggctttctcctttgggaaaacatccatctccttctttttccacgtacctgttttggtattcttccctctgaactaagccttcttcatttctgcttaaaccaaccgcatcaagaccctgagtgggtggaatatgtacatcaagtgctaagaaccacccccaggatgtcggccacatatgaggtcatggtccgaaacgtcctaaacacagagatgtgtttttcgacgcgagaacagatttactctatatacaaacttattttctatggtcgagaggacccttccctctttcttgatcctctcgacctggaaggcatccttcaagtccatctagaaaagatggagtttgatcaagccgctctgaacgaagtattacgaagtctatgtaccgagagggatgattcccccttttatcaagaggtaaagacgactcaagctcattattttcgggactttataaacttaaagaagaaagccgaattggagatgggggaaaagctcaatttgcatagagagtgggaatctctctcgaggaagacagacttcttagagaaggagaactcctctctcagagaaaaacttttgcttctcgagagggggccagtcggaaaaaaagaataataaagtaatataaagcaataaagtagagaaagaaagtcccggtttttttgttgtatagagagaattctccaatttccctttcgttattacttttttttatgtcaaagaccagaagctggaaacatagtttttttcattcttttcttatgaggtcgtgtacaacaaccttaaccgcacaagcctgggctgggcctacctccatccctagaggagccgtatgaggcggaagctccacgtacggttttgaagccgagcctttccagcaatggggcctagggaccgatatgatgattggtttaggtagggcggccggcctactacgggcacctgtagggattagtgtgtgagaccgcgatccacaaactgacgcatgggactcacccctttacttgggaatagagaggggaaacatagcatgtcacaagagcgaggcgaggtttggaaccctactgcgagagggacgcctcgcgagccgggcttttagagatgaggccttttggcgaagccaagtcaatttcgggccaccaaaccctgcaactgatgagaaggccctatggagtaaagggaagcgtgtacgttgtcacactccctgccttccaaaggtgcctagaggacgggccagacgcagcagagcgacgaccggggagcgggttccccactggaagggggacaggagacggccatctcaaggcacatcacgacctacaggcaacaccggcgagacctgggaaggcaacccgattgggtgtcagaggatccatagtacctgcagcctcccggacttcatattcatcatttttgaaagcgaggggaagggatctcttttctgcaacggaaaaaaacggagcagatttgactcggcacaacctaacgatacatccaataccaatgatctgtgcctagaatgcgttgctagatctctgctctagaaagctatacaggcaacaacgaaggcgctttgaccccgggcttccctttcattacttctttcacgacgagagaaccgcgtccgcatcagtcgaagtggtggaaggccccctgagtcaaagggagagcttctgcacttctctccaagagatacgattcggtatctgaataggctgaaggagagtgaagaggcggctactttcccagcccacgggaaagcctcttctttctggtattctttctttggctttggagatcgagagcggggtccggaagagcatgatgtcttcgtctggaacttcctgcccatcaagctcttcggggcgaccgcctatcgatttgaatttgcctcctcagccggaggcggaaccggctccccctgaaccatcctcggaagagtaagaaaggagaaggaaacgggagtttctcgcctccaaagagtataaagaagcggagtgtcaccccaaaaactagacgcacgcatcaaggcgttctgccaacgagcgaaggcgatcgctcaagaaaggggattcagccccggcaaatgcgatgcagtgaaagacgctgcggactatgtggccggtgacgtaaaagatatgccggcagctagccaactccgctttctaacgaggttaaggcatgacctagaaaacggaaacagcgagacctggggtctcatcgaacgagaagttcgaagatggagaccaggttcggcacgaaatcataaaggtttgaggacccgttggtcaaaggaaagggaaggtcctgcttccgggacggagccgtatgacgcgagagtgtcacgtacggttcctttgagaagggtgtgataccaccacctatcaggcccgacgagcggtccacggagctgcatccctactcacctggtctatgcacatcgctctctccaggaggttggccgcctatcctagatcttcccatttccaagaagatcccgggctcgatctggtttagtatcaaggtgattctttttctgttcctatatatatgggtccgtgcagcatttccacgatatcgttatgatcaattaatgggacttggccggaaagtgttcttgcctctatcattagctcgggtagtccccgtttctggtgttttagtcacctttcaatggctcccttaattatgtgcgaggaattgccctattgagtaatgggaagcgggctagtccccgaaaatgccccgcccgtaagttcgtttgtcgttggggaaaaaaaaagatctttttcaataaataagcccctctctgataaggaaagaaacaaaaaacctaatatcatgaatatccttcgccccctatctcctcctgcattgcgccacttcattctttctgtgattcttcttgcaaggcttatcttgtgtacttggctcttctgtcatttgatcggctttgacccctaccttattattgagaaagtcaaaggttcttttttcctccttgggttacgtgcaatttttaggctctttggtttgcggattccttctgtacttcttctttcgatcgtccctttggtactagattgctgcttgcacatgcaggatcccgcaggaggtcaacctgcagcggagcaaccctccaacctgccttcgggcgaatccagcgaagctagcgtgaatcagcagcctgtgattcccgaactgcagcctccccttctcgatgacaacacccgtcgagcggagctcgctagccgattgaggactcatttttggggggtagcttataccaaccgaattttagactcttttgttcatactcaagtgcaaattgaaaaagatctcgaagccgcacttgtggacgacggctattctcgtgattctcttcttgcgaagagagatcagatcaggggattcattttctacccgaatggacaggcgcttagtgaagacacttacgctttgcatctgaagcaaattctcaattcgggtacacgccaaagcattccataccatcggattgaaagagccatcaatgactagaatctccttttagattcgaaattcttcgtttttttctcccaatttcccactctttctgtgaggcaaaacctcaccacactacactacacttcgacacaagagaagaggaccgggcgctttgtatcttcgggataggagttggcggtcttctttaagagaacttcaatctaatactcattatggatcaactcatgtttccactctattttcattacgaagatgtatcacgtcaggatccgttgctcaaaccgaatcacgccaacgttatggaagttcctggatcgtgtaaaataatagtagtaccgaagacagcaccttctatcaaaaatggaaaattggctatggagattccgtgcggtcagaaattaatacagacacaaagggcttcaacaggaaagtcgtttcgatccaatccattcttggggtcaaataaagacaaaaaaggatatgtcagtgacctagcacgacaaagcactctccgagggcatggaatgtctaattttttggtcagaatatccacagtaatgtctctgttagattctccggtcgaaataagggaaaggtcaattcaattctcgatggaaacggaattttgcgaattctcccccgaactggaagatcatttcgagatcttcgaacatattcgagggttcaatgttactattgtaacttcggccaacacacaagatgagactttaccaccgtggagcggctttttgcaaaaagatgagggggaaactcagtaagatgtcggagaagagaagcgaaatataggagatcacaaacgtagattgctcgcggctaaatatgaattgagacgaaagctttataaagccctttgtaaagatcccgatcttcctagtgatatgcgggacaaacatcgttataagttgtccaagttgccaagaaatagttcctttgcacgagtaagaaaccgatgtatttacacgggtcgccctcgttccgtatatgagttctaaaaaatttctcgtatcctttttcgtggattagcatctcgaggtcctttgatgggcataaagaaatcgtcttggtagcaaccaccaaaccaatagaacaaggggtagctccgcagcaggtctacaagcaaggtaagtaggtccattaccagccggctccggaccgaaaagacctaacggactaatcccttatctcggatcgtagatgctaacggggcgggaatcgaagtgggggacccctctaccgcctgtgtctatctcctgtcaagtatgctccccagacatagactacgtacagggtagtactcttggaaagatagaatatcaccgcgtgaacataacattacattaagttacgaatgtaactcccgaaggatcgaccacttttctaaatatagtaaggcggagaactgttgttcagtggagcgccggagtgcggaggttgttcccatcattgaagtcagggtgtgggactgagccttccgaatgagaaagaagaaaagtgcttagtttcgttggaaaaaccaacgcaaatatcatattgactttctctcgccctacttctaaagatagatagaaaaggttggaaagaatgactttctgaaattctctcctttctaaagctgcgcaaggycgtggggccccagaacaaaagcccacccctcttttcccctttaatgaaggaccctcgwrkwctattcatttgtgggtctggatbcgvdgtctbtddttttttttttthbtnnaggtgatttcgaaaatcaaccaacggaaaaatccgtagcccaggtgactcacagcctccctctcgcccaaataaatgaaatgggatgaatcaaatcaataagctttttgattgattcagggcgcagcgaagccaaattcaatcaaggcaagggggcttacttttcctgaggctgattcatcctattcaaatttagctatgctaatggaagaggaaaagttttcagatgagatggacccccaagagatgagcgagaacccccaattgcttaggggtcgcactctgtcccgcttggtggacgaaatcttctctccttttagaattctttctcccacacaccttttttgccctctttcacttcaccgaggaggaaagaataatcttccaagcggacagagacctaaatttccattagattcattcctaagcttgctttgttgcagcaagatgatcagtccgagagtgctggagagaagagaaagcggtaaaaacctctcttattcggtcaccgagaagtcggacgactcttcagtaacccagggtgatccgaccccttcgacgcttttttcgctgtataccccctccatccttcggaggtggaagaaagggtactctaattttaataatagtagggccccagaacgctaaaaggtgggggaacaagagttgtcacgatagaaaagataaaaaaataaatgactataaggaaccaacgactctctcttcttaaacaacctatatcctccacacttaatcagcatttgatagattatccaaccccgagcaatcttagttattggtggggtttcggttcgttagctggtatttgtttagtcattcagatagtgactggcgtttttttagctatgcattacacacctcatgtggatctagctttcaacagcgtagaacacattatgagagatgttgaagggggctggttgctccgttatatgcatgctaatggggcaagtatgtttttcattgtggttcaccttcatatttttcgtggtctatatcatgccagttatagcagtcctagggaatttgttcggtgtctcggagttgtaatcttcctattaatgattgtgacagcttttataggatatgtactaccttggggtcagatgagcttttggggagctacagtaattacaagcttagctagcgccatacctgtagtaggagataccatagtgacttggctttggggtgggttctccgtggacaatgccaccttaaatcgtttttttagtcttcatcatttactcccctttattttagtaggcgccagtcttcttcatctggccgcattgcatcaatatggatccaataatccattgggtgtacattcagagatggataaaatagcttcttacccttatttttatgtaaaggatctagtaggttgggtagcttttgctatctttttttccatttggattttttatgctcctaatgttttggggcatcccgacaattatatacctgctaatccgatgtccaccccgcctcatattgtgccagaatggtatttcctaccgatccatgccattcttcgtagtatacctgacaaagcgggaggtgtagccgcaatagcaccagtttttatatgtctgttggctttacccttttttaaaagtatgtatgtacgtagttcaagttttcgcccgattcaccaaggaatattttggttgcttttggcggattgcttactactaggttggatcggatgtcaacctgtggaggcaccctttgttactattggacaaatttctcctttagttttcttcttgttctttgccataacgcccattctgggacgagttggaagaggaattcctaattcttacacggatgagactgatcacacctgattagtgagaaattctgacaccaatcatttacgagtgagtattacaccaagaatttacaagcggatcgaggaatgaagggagaggaattagaatagaaagaaagagagggatttcgaattagagtaagggcacgctaagacattccttttcgtgctttcgatctgcttactttgaataaagagaaaaaaaagaatagaatagataggcggaaaggctttacacaagaccacagagcgagagagagagccttcgcttacctgcttaaccgtaccctcctatcgtacctatatagcctttccttcagttatatccagtttcagttctgcttccaactaccgatgggagaaggcttggacgtatagcaagattaaataagaggtattgcatacgggaatgataaaaaaaaaggttggaaacagagctggagatgagcgctagccaatggttaagacttcagaaagcaccttagcaattaccagtaatgcccctatcgacctcagtcttgttttttgctagcttgagttcataactttactatttttcattaaacgtagaatatcccgacttcgctagccagaacgaaatggacataggagcgatcgattacgagagctcgaccgatcagaccgggaagaagagaaagaaaggtcaatctccgaaaggccttcgcagagctgagctttaggggggaatactttttgtggtcttgcacatggaaaagtcaagtattctacgcaggcttgatttaccggaatttttgcttcaaagaatgctttcaagctaggaatttaagcacggatagctttatttgacaattagctggaagtcgggtatgccataaactaaggcgctgggtagatcgtagattgccgggtatgaattcgattctaagtcggagaatgcccatgaatagggtcttattacagaatccgcagttttgaaagtagccctagacagatcattgctaagaggagagcagggaatttcttgctaatctggtgctatcatcgtattctaatgattattccgacgtcagagcagacgggactaccaatcccagagtgaattaaccttgtctgcactaccaccttagtttactagaccttggggaattggctagttaccttcactccgcgtggcagcctacctacgttttgtctttttcctacgagaccttagagtttcccagcctttctccgcctacatgccccccgaaatcagattgggttttttcttgaggaaggtccatctgcttttgttttcgaataagactaaggcgtgagcgagggtctctttgtggtggtctttcaccatcttccttttgattggcctatatcttggaataaggtctttagctattcccacagtaccttagtcccgtaccggctgtcggtctatctcatattcgcagaagaaggaacttgcttaatgccatgccggaagtgtaattaagtaggcggctggtcgtagaatagtcttttcagtaagtgctgttgcagttgtagaaccattggccattgattcttcctcgcaaacctttcatccccgctgtctagctctctcgtagtccaaagcgaattcaatcgtatccgcctttgaggaaaagaccgaatcagtctttgagccatcctaataaatcctcgtaggtaatgctcttggtctgccttcaatcagtttatcagcctaaggcttcgctctattacctgtgttgtaagctttccagtctttgaagtaaggttcaatgctaggaaaaatgcttttgcttcgcgggtctatcgccccaataggttttgttaggaaattttttatatgagtatgcccctatcccgtaagccttccatcgttgcaagccccttccattcggcccaagctttctttcgattacgtctgcttccgattctgttattccgttagcctgagttagtcgtttagtcaaagccgtacgtatgcccctttcgaatcgttctatcattcgaagtaggagctggggttgcgggcagagaactattggtatagcgagttcatgtgcttgcagttgggttactaccatccccctaaccattagtatcacactctgtgaagtgtctctctggtattgggataacttcaagccccttagctcgcttgtatcggggggagcttacttcacttgttttcttttagtcacttgccaggagggaaagcagcagataaagagcaccatcaccttacttaacaaagggcttatgcgaaagagagcaccgcttccccgataagataatccgctttcctaaaatccctactttattgctctagctcttgactcatatggcactgaaattggataggttcacgcttaggcctggttatggaaactctttaagcataggaaatttttccttttccataagaaactccaacttaaacaggaactggcctggaactatatgtaagggcactctcatccactggctgcaaggaaacaactggattggcctttctaactctctttaaaagagactgctttcaaattcacttgccctagaacctgctttttattgagattgatctagaatccgctattcctagtttttttattattcctagccagagaaataaaacaaatctcgagatccagaaacctatctatacgcctagccttaagcaaaagaaatctccttagccctaccatagaaactattacctcgacttggattgaaaggaagaacttaggactttgggacttcccctaggactccaacccctagcattccaattgaaactcaaggagatggaactaaacaggcttaggcccttttcctctttcaaggagactagagggaatgcaactactgagacagcaactcaaacaaaatcccgagagaaaataaaagattagtgaggtaaggtctatagactgtaaggcagaaggcttgaaaggaagagcactcctacttacttttcttttgggagaaatcctagacaccttagacaccggatcctcggtaggactcttatttgataggcattaggggatttgaggttttggggtttcacttgcagacccagccctgctgcttccataagtctcctatcctaagtttctttctctgcatgaatcaagttcttcgacaggaccatcccgaccgagggctaatcatagatctactatggtcttttttttttttttattcttttatcttatttccggttaaaagccttttctggaagcattatgttgagtcactccaagagtagaatcagcagctcacctcacgttttaggaaccaaatgaggaatcacacgtagacggacctgagcattctcctgctctacggagccctctggagctagagttggggctgcttgacgctcttctcctttcgagtgaattgaattacttcggctcggatgcctttgatcaaatggaaggatggatgcctgcctttagcgacttcgttcggtcattccttctttacttgttcgctatggcttgagagttaatcgcacgagagagtaagtaagagattgaaaggaggatcattggacctcgctctcgggcccagaggcagagcaaagaaagccttagatctttgcttgtttcgtggtatggaccaaagcaaaggttctgctgctatcgacacctacccaattaaccaaaagtataatcgatcgagaccgaagcttatgcaattgtggaattccgttcaaatagaaagctttttggccagttcaaggtcagtcgtgagctgtaggaaaagatagtagcgaaccagaagaaattcccgtagttgcataagggggacgttgaaaacattccagcagatagtatgtaatactcttctcaaaacgagcactatactctttcttagtttagggcagaaacatactcaaggaatgcaaagctaaccctaaaaatggaatattacctcagctcaaaggttgtttactcagatatttcttatcaaagcgagggattcgtttcaggcgaaatcaaatcagaagctatttccgctctaccattaattgttgctatttccgcacccctgtccggtggtttgagaaagaaagtcgagacattcagaaagagagttatggcatttctaggattctaatatggtcctattgattcaatctttatgcttggcccggaactcttgtttcgagtgaaagggagagcagtggcccgcaccgcattcaccggtaaatttccctctacggggcggggtgtggaaagcactataagttagttgacttctcgaccaaaggtagtctagctcaacctccaagtaggaatagattctatgagtcgtgatccagttaagatagggggcatttctagcattgaaaatccctattcttattgaatagttcaaataactagttgaacatacctattcttttcaagaatagcctccccttatcgaaaagaagggtccgaagaagacagaactggccatccttctcatccccctaaggaagtagagcgcggtgaaagaattccgtcgttcagtcgaaggggacaggttagcagcttcaggataacccgagcagtgaaagagaagtagggttcagkytgwtagatttttatttattatttatcgtgaatgggggaatcattacacatagtatatcaaaccggcgtatttttttgttttacgccccgtaactcttcctcagccaggcttgggcagaatagcagagcaagtattagtagcataacaaaaaggccttcctcatcaaagatgcagtgctagtacatctgagacttcttaattggctagttgtaaatagccccagggctatggaacaaaggattatctcggacctagaccgaggcattgatggtgattttctaatctcgcagaacagaatgtgatacgatgagatagaatgcaatagaaacaaagactgggaacgggttacctactcttaacgggcaaagcgagcccctttattttattctgaattctttaattcagaatcaatcaaatctccccaagtaggattcgaacctacgaccaatcggttaacagccgaccgctctaccactgagctactgaggaacaacaggagattcgatctcatagagttcaattcccgttcccaacccatgaccaatatgagctcgaagcttccttcgtaactcccggaacttcttcgtagtggctcccttacatgcctcatttcagagcatcymggacaasgaggcggcgatsaaccatccrctctcgagattcatattgatcaatagatctccgcgtcctgccagttcgctaagtagactcactctaccgaggggcaacaaaggctggaactcttcctgccaaaaacaagggacctacttctcatcctaggagttagcaggtatgaaagagtcccctctctgtctgtctctccgagtttctactactaagtagcacttctgctattcaatcatagaatcgattccgatcaagctgaaaaaagtaagccctatatatgttattagtaaagcgctaacgccctatctatagtaaggggccctttcttgctcgttagcgctcttttttgattgcagctagggcgccccttttctttctcaaagtcaactttctcgcttgttagtcaagctttgaagtccctactttatttagatttatgggatatttgaagaagggcaggtttggaaccctatacctatacaaggggctggtctcgatctcgcttggtggtacccctctcgatgattgttgactcaacattgatttcgtgcttgagttggagggctctccctccatccatccatcgagtcaagtaattcgctatcggaaattgatccgccgcctatctcatgccatgcttcttctttctccgaatcggtttctagtgtcagtcaatcaagattcgccatcaagagagggaagagccttgactttaggttaggccggtctcatcattcacgcaattcccccgtccatcgattgatcacgcgagtacgcatccagtcagcgcatagcgaatgaaaaaagcgttcatcctggattctcttcctcaagaaaaatggctatcaattgatccctattcattcggtcaaagtctccacttttcacgcccctctactaagagatgcaccatgttgataggaatcggcaaagaccttcttgtacacgtcctcgagggcagcattcatggcaatcatcactactttctcccgagggcatggtatggctttgttcttggtcttgtttaatagatgtcgagtgccgcttttccccgtccgagaatctccatctgctctaagtgggcgcgagctagaatccttatgtcagcttggttgttcaaaagactgtctctttaccccttccatcttcatcttttctaaagcccagaccattcttctggatctgcattagtcctatttcaggtgcaaagcctcttcaataaagacctcttttttttctttctcccccatttctcattttgttgattgaaagagaataagcgctatccattgagtaaagagagggtttgctacagtgattcgggcggttggtggccccttcgagagttgcgggtccttgccgctgcatgagtgttagctcacgctcaaaactcctccgacacgagtcctagtcgttgcgctgcggtccgtttcccggcttcgcttgcgcgatttgcacttctgattggttccagccatccccaaccttaatgaatggactatgaaggggttagtcaagcggttcgggttttcggtcggttcccgttcgccttccccccccctcatagtccattagtgggtagggtggtcaacttagagggcgcccgcctcctcttcagacgtgtcctcgacaacctggcggttcttcggtctccgcttttgggggcgggagtgcttggtcgctggggtttccttttccccaaccaattcggttgtgtcagccctgagattggtctaacattttgttatgagctggctggacaaagatggattgaaggtcagatagatttgagttcaagtggcacagcaccttcgatcgaccatagggcctattctacccttaccgaattcattctattgaagcgtaaggtaaaaagctccttctcatcttgcatttctttggtttggaagttccagaatgttgtctgtggatttctataacaaaggaaagcctcctaccctaatactatgccatttgattgattaaagttccgtgctgctcaccactcctcgaggccaaggacggggtcgaaccgtcattccaggatttgcagtccgatacatttccattatgttacctagccaaacccgccacctcatgtgccaaagtcaaagggttgttcttccttctccgctccttctttttctacatatgcggcggcgggttaccagagaagaggggacaacttctttctcctttgccttgctcaatcttccttttctgattgaaagttgcaagccactcgactattggtacagaggccagatagaaggttgctcatccagcccagcggatccattgtttatgcggcagtgcaatgcagctgaaaaagggaagcccctttttattagtaaggtataggttggttggggaaaactccaaaactagggttccaaattaccttatattatagaaaagtttgagaaaggggcacccctactatacccctaaactacaagctagcgcgcaagggctgaaaagccgttgttgcttgctgcttgcaggctcgaaaatctctctttctcctccctgtctcaattctgattgattagcttcttccttcgcgcaagctacggtctaacgacccccttgttgtgttgcattttgtgatcttccgcttcagtctgcgtttttcggatagccgggacccgatgttgatttccgatttaaatgtcagctccaggtttggggcggcccatctgattagttcagctatcactgctggaaaccccagcggttgttcggctgcgtactccccgtctgcctatctcacactcccaaagcaaatttggatttcttctttcattttcctttcctgcatctttcttttttttaagtcattgatctcatatctataagcaggggggtctgcgttcactattaagcctacgcccgtccattcctttcaagcttgatccttcccttagactcgttaccttgttcgactgaactcgttggttccgcgctctattcggtcgtaacccggttcgagaaccttctctcatagattccctttaccaagtcatcgccagcaatcagctcttatcccttggtgtcaaagggcgagttcctttcttgtcttgcccaaaaactttctttattctcattggagaaagactctcccgcggcaaggttttacacatagggccagctgctttctttatctcgcttgcccttagtccgtctagcgcctttcggttggggtccgccctgggggttaggttagaccgcttgggtttttttctagtatcgaaggcagtcaacgtgtcagccattcttcccccattagacttgtcaatcctttgctctttttccttttctcttccagttctccccctctactttatttgacaggggcggagaataccactctatcaataacaagaaaaaagtagcaattccctttcaaatggtttgagcttggaagcaacctgctatctatcgataggcgagaacagactgctattgactgcttcgcctatctattctattatggccggcttggagacatcagaggaagaccatcatctctatccgggtacgatcatagcttcattcattcgttgaaccttggggatcaccattagcattgaggtcaatcaccacactacctctatcatacatacgacattacacgaagcgagagtgcatggtcaacacacacctaaagcgcctacgttccgcttgcagccaatacaaccacaacctaacttgcacgagattcaacaaccgaagctactggtagtcccgagggggcggcatcctcctataatagttagcagtactgaacaagcgagtcatcggtccgaggaaagaaaaggaccgcctttgaaaaaaaaaaggaactcgctaggccttcagaacaaaggcgattctgttcatgcttcagacgatctggctaattctatatacaactatctaattttcttcaattatatagaaaggcgtaaaggcgaaggcctatttagcgcctttccaaaggtaaccggttaggttgactttggaaaggctactaaggaccgggtgaagaatgaaaaacgtccgctaaagcccacgggataaggtttgcagatgcgatcatgaatcgaaccagatcgaaacattcagctgtcgacggacaaagccggaacgtcgaccgcaaacgaaggatggccaggccccggttcccagggttagggtattccctattatgagcctactcagatcagaactaaactagttgattctctttggccggccggctttaagcaaccttcgcatttcctgctgagatcccaagtctccaagtgggccctcttggccacccacgaccttggctttttagagaatcccgctcctgtgtcgtaggacttgtagctcggcagtccaccgggtgggtttgtttatccttccagtttcgagtgtcttcttggatagttatagcggcccataggcgcgagatgtaccttgtgggggggggcggcggtcccctggacatagtcctttcaggcagtggccgtttagtccatggtccattggatggtcggtgcaaggccagaaattggaacacattgattccgctcgttcccgtccttcgcttcagggcctgtccctcggtgtggtcagtactccatactgtcgggcagcgaagcttacacttgttcactaattatgacggttcaccagggcctctttcctcctcccttttctgctcactcgtaggggtcgggacccccacaaagggggagggagtcgactgaacatctcagccattggcgggaatttcgcccgcatccgatccccaattcttgttcaccccggatgatcgtgtcgggtgaattgtgacctcgtacgatcgtgtcgggtgagcaacagccgcttcgtcacagtacttacttatgggctaacaggtcacactttggccaagtatcctacaaagagactcccgagagccagaagtattaaaggaatggccataggaatgggcgcatcatgacatcgtaagatgtctcgcccgaatgaattagttggtactagaaatgttagaaaaagtgaacgaaaggagtaataagaagtgaaaaggacagagacacttcccaaccagaaagcaaagttcccactgatggtatacttagtgtaagcgagctctaagatcacatctttggaataaaatccagttagaaaaggaaatccaattagagataagctgcccatgagcatcatggcataggtaaaagggaacgaggaggcaagcccccccatcttccgcatatcttgctcatccgacatggcatgaatcaccgaacctgcactcaggaatagtaatgctttgaaaaaggcgtgattcattaagtgaaagacgctaaccgaatagttagagatgccgcaagcaaagatcatatagcctaattgactgcaagttgaataagctatgaccctctttagatcattctgtaatattccagtggttgccgcaaggaatgacgtcatagctcctgcaaaagtaataacaatcaaagccgtaggtgggtattcaaataaaggggagcaccttgctatcatgaaaacgccagctgttaccatagtagctgcatgaatcaaagcggatactggagtgggaccctccatagcatcaggtgaccaagtatgcgatcctatctgtgcagatttcccaacagcaccaataaaaagtaaaatacaaataagagttatggcattcaatctcatattgcaagaaatccaagaatttctgggggcactagcacgagcaaaaatggttgaaaagtctactgtttgaaatagagtaaaacaacccaaaatcccaggagctaatccaaaatcacctactcgattgacaagcatagcttttatagctgctttatctgcctgaagtcgtgtaaaccagaaatgaattaacaaatatgaagcaagacctactccctcccatcccaggaataattgaagagagttatctccagtcaccaacattggcataaaaaaagtaggaatggataaataacacataaatcgagggctatgcggatcctcagacatatatgaaatggaataaagatggaccaagctacttatgaatgtaaccacaattaacatcactacggtcgggctatcgaacacggggtcagaagtgaattacgagtcggaccaatctgcgaatcgagcgagctccccttgcatgcaatgatgtggtggtaaacctctcattctaattcagtgctctccgaaccgtgcgggaaggtttcccatcacacggctcaccaacttgatcttccgcgggaaccgtatgtccgaacaggcctggaaaaaaaggtaaggtctcgctttcctttgccactcaagtgtacggcatctgccgtgcttaggccccttcttcccttacctaatgaaagagtccaccgcctgccttagtagtctcaaataaggcgtgcaggcctgcccctttagtaggtgattcactaccgaagcgaagaaaaggctggatcaatcaaagggggtactacgagccctctgccccacgcatctaaccagctcgcgtggttcaccggttccaccgactagaccaaaagagtgattcagtcgatacagaggtgcgcttgaagtggggggtgtgctgtccctattgggctgggcccttccccataaggccccaccgtcggggcataagcgccctcttgctacccatatgcgaggcgccgtcttagccttccctgaccaggatcgctcccacacctgtagcgttcgtgatcggcctcctcaactgtgtatcgatcgaaaggcagggcggcacagcccccaaccaagggagtggttacgtccagtatgtccccccttattcccgacatgctatggtaccccggagtgggtaggagcgggtcgagtccgtatcgccgcggagcaacagccgcgtccggatctgatctattgactcggcaattcatccggtgacttcacggtcgccaaagaagccccaagaagcatcaaacatttccgatgagatccatggagcaattcttagatagcaagcactagctcccggtgcgacttcataaaaagcaatcaaagagaagatcgaagagaatgaaacgcacgtagtggttattatagcggttccttcttttcctagaaaacgtccgaaacaacctgctacaaaactaccgagcaggggtaaaaatacgataagtagatacataatttcgagtgtgatcagacaaccaaaaatcagacaatgacagagcggcctttatacaagctgtatattggtttggtatattatcctatggctcgctagcttgacggtcataaaatgcgagtcttcttcagagggggaaaaggcaagtcaaggtcatattgggaccgtgcttttagaatgcacgcatataatttgctacggtgggccccacagttctctatttgattcaggtggttcaagtacgtacccaatgtaagaggttttccttgaggatagaagaggatacctctaatctggtgccttttcgcgacaagttgatcgtcggacaccaagtcagaacgaagtgctctttctatatgaagttctgctttcgcttgggcctcaattatttgatcaaaaatactatcgggcaagggacgccctatagtatttatgctcagacgatctgtcagctccagacgcctctccccttcttcctgtaatgggtggtaaacctcagcctcgggcaaaataggcgccgcgggttcgctaggtgtttcgccggtttcagtggaactgctaccgaataaatcgctccaccttaattcacctgagccagaggaagccatcatgttacacatgttacaatccccaatgaagaatttttgggacaatgtaatggccaaggctagtccgcctgagaagcccatcttgatcaataaagacgagatggtgcgccttcccacggctatgaaccctttccaaaagaaaaagtgaaaaacttcaccttccataaagattagagctataattagcacaatggctattattagcacaatacggtaaaaaaaaaccgcttttaaacctgtttgcatcggctcgtgcacagatttacgttctataatcccaggggctttcacttcgacacgtcttcgctcgtaatcgcttagagcccctcttccatcaataggtactcccaacgcgtcgaccacacgtcctagcatagcctttcccgcaggaacatccacaatagatccagtgcgcttgacaagatctccttccttaatagcagtatcactaccaaagacaacaatccctacattctcattctcaagattcaaggctattcctttcacaccgctggcaaattcaaccatttccccaacttgaatctcgttcaatccataaacacgtgcaatcccatctccaactgagaccactcgaccgatctcatccacttgaaaattcgtgtaaaagttgctaattcgactttctaatagactcgttagttccgcagctcggggagaaagttccataataatctatctaattattagaaagtaaagggagaatgccgctgacgaaaagatttctcttagagagtaggtactgtctatgccattggtaagtagatctaaatagatcttttgtagtccgagaaatttttcttgccaagactcgtctccattttgcttcaaatccggagtttcgtttcactggttgtgttaaaataatctttcaatcctattagtaaactattagcgtaccaaagctcaagcgagcggccacttcttcctctattcgatttttcttcttcccaggcccgggtagctttggctcttgttgaagcattgccggaagcttcactctgtgtaaagtaaggacttagcttttacggggaaatccccgaatggggaccttaggagctttgttcagcactgaccttttctagaccgatccctgcgtagaagtgaagtttcaaagcgctaataatcccatcttttcacgaataaactgattctctgcttgcttttggggaagcccctgcttggccctttactggcagtcctttgtaatgcccgaacccgggctactaccgattctaaattctacgggtaacccttcccatgactacttcttgtcgtaagacagttcgcttacccgattggctggggcttagacaagacttaaaaacaatcactaaaggcctggtgaagctccaccttttccatccgctgtctctcttctcgctaccatgttgaaaaagaaaattcgtatttgagagaatcgtaaacagaggatttcggtggcaccatctatccatgaggaaaacctttaacagtagactagttccatagtatggtcagtcactcatgaattccttctcgaatcactactggaatatagcaacaaagcttgaagcaagtggaaatgcgtcaagggcatttctttctcactggaagcctacttgagtagtgcgttggatctacacttggacagcttcatcgagacttcacatacgtagcatacgtagattgccatgtttatatccgaacgaaaacaccttactgatgtttttgtttccagacttaaatctttaactataagaagggaatcgattcaagccagattacttgaccggtcttaagcttaagctaactaagtatatgtatgtgaggacggccatccggttagctgcctctgctgttcttccagtccttctatttacttttttgccttttataatctatatcgtatatcggccttataaacttctaaagcggtaaagatctaaaaagatataaatagaacctcgtttggagagtaattgcttgttaatgcagtaagcagttcgttcgactcgctcaaagattcgtctcactaataaggaatagtcacttcgtacctcttcgaggaacgaagtcccgcgaccaaatgagttgaactatgttcaacgaattcccgtagggagagggaatgtggtaccgaacggttattgtgtgtcaccaagtacttccacttgtcactgagtaaggtaaagccacgagggtaggtgggaatctttcctcaaggcgcaaccaacccagtaagaagcagctccggggaacctctagctagttatgaaactacgtttcataattacaatgaatcaacaccaacccagaatgtggacaacgtcttttccgaccggagaatacgttattaggtaactagagtcaagtgaggaatgagaggtactcgctcttatccaaagacgatctagctgcttatccgggccttcaagcaagttcaaaaactctcactatgtgaaatcaacgaatcgttacactctagccacttcgtacctagtcgctagagattcctctcccgttggtcgagagacttcgtacctctcccgttggtcgaattcgttgttcgttgaactatgtgaaacgaacttcgtacgttggtcgtacctctttcgatagatagtcagagttcttatttctttgacctttgacacttgctggattccttctggttgtcacatcttgtcaccctgtctgctttggctatctgttcgtaatgcttccttcttttcttcgatccttcttaacttgaatcatgaattggattcgaaccaatatctctccaggatctcggcatccctcccacctttcggcgagatatttgccgtgagcaatgcgacattcccaagacctaacgagagatctctctctccctctctttttgggcagagattactgcttttagtttccattgccctaagcctgtcgctcggcccgggcgcccatgaggtgtggttcgggttcctcctcaggcgaacatgaaaaaaaaaaaggggtttagtcaagggccaaaatttggttttatgccatgttgtctttacacagctctgaaataccccccacctaatatatatataatatatatatatagaaacaaccaaccaaagagtaccagacagataacgtcttgcaaatgcaagtagcatgtaaaacaatcaaagataagatcgaagagaatgaaacgcacgtagtggtcattatgaatgaatctcccagaaaacgattgactatatatactggtgataggaaacaagtcaaattcatgacgaaggctatcatatagagtcgaacaaatttggggcaaagccacatcggggctatgggagtcgaacccaattcaattcttccgcgaccctttctcttttctacgaaaatttctgtttcgctgcttttctaaactagacagagtgcggtaaaatcaatctcgactgttcactacgtacgatatttcttgaaattttgcatgaagatgtgatcaaagctacatgttccgcttttcctcaatgaaattacagagagagtggaattggaatttagcactgtgcggagctctcgctccttctttgcttttctgatctcattctggacatatagaggagataggaaccttaccttatctatgaaattatgaaataatgatctcacactcttcaagacagattcgtgaaaggtatatctacgccatggaagtttcatggctgaatgatttgtctgctaccaactccttcctctatgtctatgctatgggcaggatctctctctctacatgtgaaatcttgtataataatttctcacataccagattcccgaggaagaaagcaagcaagcctataaagatacgaggtttcaccagattacaggtatggatccggtatgaaatagatccctccttttttttatcccttaggagctaactaagagggcaggcggacacttctcttcgttagacaaggaaatgctttcaaaataaaagcattatgtgattggttgtccttcttcacttcaattcttcaagaaggacctcgccaacttatgttgttcacccacccccttcggataggcgcttccgttcttttttcatatccgcgagaatgggaggtaagtaagaagtaaggtggagacttacatatattatattatgcaacttatgcaactcagtgacctatcctgttcttgggatgaggcttgacttctcagatgctgcttctcctttcttgtcttgtggcaggggaaagacggaaaaaaaccttcttcgcgaacctctcttcgatgccgtcttctttgcgcccctctcccgttggtcgaatgagtttcactatgtgaaacgttggtcgagtgacttcgtacctcctattagggacatctttgtgaatttaactcacgagatggcctcatttatgtttcatttaaacaaaaccctgatccctctattctatgggccgagtggatcatatatccattcgatcccaggaatacggctatagctaattggtgccttgattggtttgagcgacggaaacctatcaaggtatcccattagttacaggtaggttagcgcagacactctcaggggctgggaactttgctatatgtaactatatcaagcaaagacttcttgctcccgtcaatgaatgtattatctacaatagagatggatagtacgtatgaccaagagcggcccattcttaggttagctcgtaagggttaaagggttataataatacttattgttatgttgttatgacctgaaaagtgcgaccgacagatggttatctatcattttgattcgggacaacatatggtcaactatccgttgactaagaagattcatgagatttcattcttggcaggtcaacctttaggttacctcggctcctggtcatttctcaccactttgtcatgtgattggcagcacaaatgacgtatccagaacggtcaaggactatgccatattaggtgatgatgttcttatcactgatgatggggaattataggatgagcttggtgtgtctatctctgataggaaatctattattatatcaaatggcgtacggagctgcttaccctctttggatcgacagcgggggggaaactggctctggctttgttgtaatgagcattttttctacaattgcctctacggatacaactttcgccatctagggtgggctgcttcgcctagcagcacgttttcacggttttcgctcgccgctactattttcctctagatcttcctgcccatggattcagcagttgccctattcgggaatctccggatctatgcttcagatacccgttttggtctcctttggaggtctgacgacttggtcgcgttgaagggtatagatttcaaagtgctttctcgatgtgaatcatagctagaaattacattatttctcattcactcggactcttagatcaaacggaacgattcgttgaacatagttcaactcatttcgtaccttctttttttctgattttttagcaaaaacctgttgataaacggttgataaacggttgataaacgaccggtcgactcacggagttggcactccaggagatcgaggagtcccctttgactgattcgtgattccgtacaacgggacggcgggtccaactgaccatcttctccactacaggaatatcatggatcagaagactatctgatgtgccgtgtctcccagccagcctacgcgggatcccagcgaaatcttcctagctgtaaccggaggatcttgactacctcttcaacctgaagaagaggattccactaagcgattctgagcttcagcccttcgggttgacaactgcaacgagcagccagcagtggtagcctacaagaaagggctacccgtagagtccaagctctaccagtctctggtcgattcttgaccagagaccctttaaggccctccccaacagctgtcccttcttaagcaatgaatatgcatctttgactaaacggttaatagaaatattcttaatgaacctttagtgggatggggcaaagccctgggataaccctatccatgagctgcaagatcaattgtccagtacgggttactccagccggttattcatattattcatactagtaatggaactctagtgccctatatactttgacacatacatctctgtctgaacgagcaatttcgatgcttcttctggcccaacctttaggtttaggtacgaagtcactaatatagtaatatagctagtatagctagctatattaggaagagatcccattcgtaggaatctccactccattcaccgaagcagaagcgcctgatcccacaggatctggggtaatttgtcagcttgcctttacatggaaaaaccccattccttagctgagagtgatgcagctggcgcagaagacgtcgttcattaccttatcagatagagctgacggaaagaccactttggtatcgattctgagaagacgccccactggccagttgccacggaaaactacatgaggttcgccgagggcgagaggaggcaaatcactgagatttccgagacaaagtcttcttcggatgatttcactgtcttctcgaattgtatttgctgttggctcttgcctattatatcagtcatgccattctggtcttcctttcctgcctttagttctctatcgaaatcacaagcagaggggaactcggactatgacactttgtttggaccggggaattgcaccgacaagtcacctgctctgcttagttttcataatatctggaagtaggaaagacattcccttgtcgtttactgcgcgaactcatacgcatactttgatgctaactcgaatgatggatgtctcgggataattcctttttcaaggacctcctgcaggactggatcctcattctggacaaaaagcaatctcaaaataggaaatctactcttagagtaactaggatctcgccttgaccactaactagacttgcctattcttcgctaaccacctactgtctagtgtacgcttagttaacgaataaatccttttgcaataacagggaatagcaatctaaatattgcctccccctttaacatctttcaattcccgactccatcagtattcactggaatgcggctatgaagtgtgacctgacgggcgaacatgatctttacaatctttacataaccaagagtttggtcggttctccgatccaccttgaatgagctaaacaaagactgggaacgggttacctactcttaacgggcaaagcgagcccctttattttattctgaattctttaattcagaatcaatcaaatctccccaagtaggattcgaacctacgaccaatcggttaacagccgaccgctctaccactgagctactgaggaacaacaggagattcgatctcatagagttcaattcccgttcccaacccatgaccaatatgagctcgaagcttccttcgtaactcccggaacttcttcgtagtggctcccttacatgcctcatttcagagggaacctcaaagtggctctatttcattatattccatccatatcccaattccattcatttaatatccctttggtgtcattgacataacagatgtcgtttctagtctatctctttctatttcgtttctatatatggaaagttcaaaaatcatcatataataatccagaaattgcaatagaaaagaaataagggaggtttgtgatgatttttcaatcttttctactaggtaatctagtatccttatgcatgaagataatcaattcggtcgttgtggtcggactctattatggatttctgaccacattctccatagggccctcttatctcttccttctccgagctctggttatggaagaaggaaccgagaagaaggtatcagcaacaactggttttattacgggacagctcatgatgttcatatcgatctattatgcgcctctgcatctagcattgggtagacctcatacaataactgtcctagctctaccatatcttttgtttcatttcttctggaacaatcacaaacacttttttgattatggatctactaccagaaattcaatgcgtaatctcagcattcaatgtgtattcctgaataatctcatttttcaattattcaaccatttcattttaccaagttcaatgttagccagattagtcaacatttatctctttcgatgcaacaacaagatcttatttgtaacaagtggttttgttggttggttaattggtcacattttattcatgaaatggcttggattggtattagtctggatacggcaaaatcattctattagatcgaataagtacattcgatctaataagtaccttgtgttagaattgagaaattctatggctcggatctttagtattctcttatttattacctgtgtctactatttaggcagaataccctcacccattcttactaagaaactgaaagaagcctcaaaaacagaagaaagggtggaaagtgaggaagaaagagatsacggtctggggctggagttctaaggttgaattctgggcatgtggataatccgaatcttaaacaactgacctggaaggctttactaccactggggaactaatccctgaaaagagctcttgcgaactctgacttagaaagcattgtactactcagctgttagagtccattagagtgtttgaaatccctgaatccttactctgtacagagcagtaggcttgagttagaagtccgtatcccgttggagtgtggagtcttttaccaggccgttttctagcctttacagctggtgtaagagtagtggcattctcaccagcctgaatagcaagatttcctccagtagagggctatagataagattataaggtagggttatacggtagaatcattaaaatgtgaattccttgtgaggatctaaggtagtaatagaatatcatagcgctagagctgggtcaagagtaaggggcaagtgcctatagaaagccaatttcttttattagaaccctgggaaaattcatattttgcatttctacttcctccatcagacaagggagctgatgggttttaaatcagagcagaagtacctctttcagccagttttcttacaccccggccagcctttttttcatctctctcttttgtaagacgccctgcctgaaaataataccttatcctggcctgttggagtggtagttcacagttttccaagcgcatctagctccattctttcttgttggaaggctacctcgggatatggcaatgaagcctatctgtggctatagtttcctgagtgaggggattggagagtacgacatatcctttgaggcagcttattttcagatatttaatttcctaaaagataagcctatctagttgaagtgtaagtccccccctttttttccagttggagtttctttccccggtataactatgaccggctataaagcagttgattagggcagaggttttctagtaggcgctatctggctgaaattctaagtcaaaagagatcctggtgtgcagtccatcatctttgttagagggctcccagcggatttgttagctgctacaaatagggaagaaatcacgaaatggaataggatcgagagttttcgttctctttagccacagtcttagtcttagacttttgagttcttctcctcgcgatccagtgccgttgcagcaaatgataaacccagtgaaagaaagtttgccattcctgcgcgtgtaattccttcttcctactaggattttcagtcctaagctaagcacatgcagtctaagtttcggaggaatctacttgaagtgcttccccatcttgcttgactcaagtttgaactttcttactttacttatggataaaatagaatctatcttaccctacttcatatgaatagaggagagggatgaagatgaagacgagatttcttttacgatatgtctctgggttgccctacatagagggattctaatgggatttctaaagcgagaaacctatccaattgctgcagtttcttattctgtagttgcctgccgctgtataacgagttgtttccgatgggtaagccgtggaaagaagactctggctaaggcatttgactactccttccgaacagctatagaacagcttattcaatagcagcagattcgagagaatttcctattatggaaaggtagtcttcagactcccagatattggaatgccctaggattggattcatatggaagtcaagctcgacaacaagaagagaaagtcactgaacacaaactatctttctcatgtcttgcaatagacgattcaaaatgaaacaaacgatagaacacttatataccgaactttccatcaacttcttatttcttcaactactatattacatactatactatatgtatatatgtttgagatttgctccgagatgatagattgtatgaaaacaaaagagaaagggcatcaccccagctccggttccggcaacgctaggcgattcatctctctcaattcctgaaccaaagctaattcaactaccttccccctcctgtttagacatctagcagccagaaaatttgataactaagaaataagggatccttttgcaaaaatagcaattggattgagatggatggttgtgctttcagtcttttccatgccgaatagacaactgcctcttatgagtgattgctctacagccaaggcagactgaggaatcccctaaaaagagatctccatagtaaatagaatcgtacatccaagaagcaagactgacagagcgagctgtaaatgccataccattgattcttgcttttttacttattagcattaagtggactaagggcaccaatcaatttgaacccaacgctcgggaatccattcttctatagcagcttgccggaatgccttcaagcctttgaaactacccgggaatttaaaaaccttccttccttcaagtcttctatgagggatcgatcttgggtaaatacactaggggatggtcccataccaaagagaacctcgagcggacggcttttccgcagtcaaatgacttattgcttgacagcttcaacaatagattgccttttcttttttctttagtgactcagtccctccgcagccccttacttagtctaattttttgatagaatcgtggtaatggctgaagatcgagttcacgcttttgggcttgtgtaaggatttccctatcagttagccggagaaggtaatcaaggagttccgtcttctacgatgtatgctctttaactggttcatactggaagaatggatggcgcaggagtctctcttctgagacttggactgatgaactctgtaacctatattctccaaccttcctcgataccctagaggtcgactcttgccacaaggaatgtcatcgcttttcggctgttctacgatattccttggaggatgaaacttttctgttgacctaactttccagtgagcggacctactcgaaggaaggaaaaaaaagggggttgggggtgcttctatataatctctaatccgagtcttacccctatatatgtggaaattctgctacaaatggattggatgcacggaactcacctaaaaaccccaacctgcgtgcagtcgaactgctttattcaacttggcaaagacaaagcatgacctctggaaccaaatcgttcttgtctctggattgcctcaactcgaagcatgaggcctggacccatcggtggataagatcacctcttcatgacaaaaggtgtacacgttaggcctcactcaaggtaatgggccaaacctaacgagtccaaacaaattggatctttttgtatgacaaaaccacagattgggcttaattcaaagcccacaaccaatggaagagcctacaacttgaccatgcacttacacataccaacactaggttctattcgaaggtctcgaccaccgatgggtcttgttctaagcccaatcctctcgtcttaggataggatatccataaaccgggaacttctcctttttagttgacaacctatgttgggctgactaagcccactatcctaatagggtcccagggttaaggctccacctcatcttgggttaagggcttagttgaacccaatttcttcttttcctatgattgttccgtgatgggttttctccttctaggattagctttctatccccgtgttgtgctaagctcatttctcttattaggtatgaccttttgtactctgtggatgttcagattgcataccttgcaagtcattcattatccacacatgtcatacatctttcatataggatgattttagaaagcacctaagtgttggacatttgtcacccctacactcagctgaggccacaggtctagtcgacgtggccattcatattctacagtaaactactagtcacaccaccatctttctttcagctctctctcttctgtcatgtgcttaaagaatttaaagtcaaaaagacgtgatcaactttctcgatctggttcagactcatcactctaactaatgtctcgtccaggtcggggggtgaattgggccctctgaatgaatggtgaaccagtcctacgagtgggtggatccgccgcaattattgttatatatatatataagtcctgacccggaaaggtaccgccaccttgttcaggctttccaaagaaagcccatcaagtgaatgaagtctaattcccattccgggccggcccaggcctgctcgctatccgagtgtagtcagcaaaagctagtttagaactaccatccggccttaaaaaaaaaccactcgacatgtgctcttattcttctgtcaaaagtagggaacagcaagtgtctgatcagatcaatcaagcgataggggcagagactttacttcgctaggacggagctgctgtcgattgaggattggccgaggggccctttttcttttctaagggaatagattgtagctgggtacaaataggccgggacgagtaggcagggtacgacgaagcccgcggggtgacacatggttgtactggtcagctttgggctggagattgacgattgactgagcgtgctttggcagctcgtggtggagtactctctgacggattcgctctattattgcctcctattcttgagggagtgatcgggattaagccgcgtggcgaaaaagcactattcgctctttggggtgggcctttcgtactcaaatccgtacggggaaaggacaattattcagcgcactaaaatctagtgaatggggttccatattcatgaaaagccaggtttgaaatgatccatgttacggaaccaagacaacctatcttactaataataagaaagggttaagggcctccaacgcctataaatagaagcttctttcagtctctatttggcaaagggagacggagaggaacttagaagtcggcaaaaaaaagctttgagtgtagccatggattcttttataagacttcaagaaatttcgcaagaaatctctcaagtggaagaggagaagctccaatcggagcaaaccctggctgccttttgggagcacctgcctcccatcgatcctgcacttgtggctgcagccatgcagcggatccgggaccgcattagcgtcctggaagacaggaaacgggccctcctccaaaaacaggaagacctaattgtgggtgctgtcacccgtggtcgccagggagactagaatagaagagtccgtcgactctttttagttttagaaggtttaaataagtgtctgtagacgcaaagtagtgtgtttcttctttttctttgtttggtggagatctactcctatcctaagtagattgctttttttgggtgtgtttgcatgtatcactagtagtcttcaatgcttccgttgttaactttgtaatgttgtctttagttgtgtggctggtctatgtgtgtgtaagcttcctatttgatgtattcccatgtaacggctattaatgaataaaaagtgctggtctgctttgttaaatattccttatgtatacgtaattaataatcccagagggaatccggatcttgagtgaacctcaaagccatgccagcctggagttaattctttctatggacagccttttttttaagacctaatctaggcattagccatttaaaaagatggatttaggtttcggaggtagatcgaaaacctcagcgaaggtcaccgaacacgaacaagatacgaaagatgttagacagcggaccacttaaactacttagttagagattctttgctattgcttatgcctcagcagagaagtaaagttctgctctcctctctttctcttgcgtatctagttctatagcttaaccctgacttttacgatgtaagggcggaacgtaatagtaataaaggaaaagcaaggtgtggcggtaagtcaaaactttttggtctccatgttccggtcccggaagaagcttatttttatcgctataaggcataagtagtgaaagaagtagacctataaagagaaaaggaagcgctatccctcctacttatgattcaacatttagctcgatctattctagatgtcttttttacatcaatggcatcagctggagcttgcaccgaattgcttacccgcggaactcatttaacccgaccctgcataagtaccaatgccccttcccctttcacctctaggaaaaacttctgggatgagcccttctactcgtcatttttatattagagggaaaattctcgatcccagaccaggctccgatcaaggcttataaaagcatcaacctcatcctaaaaggactcctttagctttggggttgatttacgtggctcaagactttgagtcaagaggtcaggtgttcagaaaggtggtgatgcggcattggcattttcagcaaattcatcagatagcttgccttcttttcgtttacgtggctacatacttgtagcgatcaaagggcatatttattcttttttattatttatataaggaaaaggtaattgtatgggcctttgcttcgagaacaatcgtattagcgccttcgcagcctgcctttccattcttcgagtgcagttccttcttgagccttttctttttgactcctaccgaagcaagcctctcaagtgctgacctttcttcccacccggaaatcgtagtaagccgggagaaagacattcatatattccccaggcacgggataaagagagagccgagagccgggaacgcaacaaaaagaatttccctctccctgtaggtcgagcctccttttcagtcgccctctcacgggaatcttcttctttataatacgtacgagactaccaaagaaaatgaaacttctttccccggagcagcaactgaaagagaaaataccgctttcttcatctgcaccggaaaagagctaagcccggaagtcacggagctctcttctctttcaatggcagcagctagtttaagttcaatgtcagccggatttctaagcactagtctttccttctcacctgctaactcatagaaagaaatagagtcaacccatgcgcctttcgcggggtgagcaaaaagcctttccctggatcctggtatgaactcaaaaaaagcatttacccgtcgcctgcttcatctgcagagcttcctcttgttcacagcaaagagagcggattcgttcaagcaagctaatcacattaccctttctagggtaggggtaggctacgatgtcattactctcgctccctcactccttaaagggatcaaacgactttgagctttggcattaagtacgcgtgggaaggaattccattcaactagttcaatgaccctagagggaatgaacgcattaagcttgaaagcattaaatttagttgctagctggactgactgtcttctctctctttcggtttctagtctttgcttcagaaagtcatttagaaagacccgcttttaacagagaggatttccttacattacatacgatatttgagtggggattcactaagcgtaagttcttaacccggtatgatgcgacgatgacttcttgctttgtttccgtctctcctgcctttgttagtctttaatcgtctctaaagcgagtgaagtcacctgagggttagaatccgatgtgatcttagagctattgaccctacccaactaactctctctaagtaagagctcgccctgacttattagtcttatcgaagtcgatagggaaaagagaaaaggtcagtgcttctcctgtgagcgactccgaagtgggctcctttcacttgactatttctcttttttaggagggagagactgaatccacctaaaagctaagggaagcccggaagtattcgaaggctgataaaaagagacgtgtactacgagaccaccaagactgataggcattccgaccaaaaggggcaagtttcttataggatccaccctcccaacaaaaaaagaattccttgctgtggaaaagctgttcaagttgaaaagcataaaggttgaaggaaatgcaccttctccgattagaagggtacgggactccttttcctacgcaatttcctacgatagggtagggatgaattgaatgagagactacgaaagtgaggcaaacccacataaggaaagaaatcaatctaatcactccatttcaagccttagagaatccgactaaaaagcctaaattagcgaattcacctccctctgagtccgattagaaaaacagggatgaaaggcctagttttcggtgagctagtgggattcaagtatgaatttgaattttcctcgatccggacttattaccgtgatcaattcactaccagtgcccatgtggccgaggttgtcccgaagcggatcaccccgatgcctgtaatgaaaggacagactttcatcagctgcaaactggaagcggtttttcgttagtgcgttaaggttgcaagaacctactcctaactaaacaaagactcatccgaggagccaccatcggtactagtccaggaggtcaatactagcgagagtcccacagctacgctagttatttaggtataacgtgtttcggtcagctttaaaggccaaactaacccagtcgcttttttgcagccctgtggagtcaaggcgaatcgaatggtcaggaaggaagcaagcaattcggacagaattaagagggcttgaaagaataagatacgtagagcgtgaaccaaggttcataggcggatcaaagtcgaaaggcaaagctgttggttagacgtagacgaagccaaagtatagttagacgaagccgtaggaactcttgcaacgcaatcccagctacaggaagctaactccctaagacgaatgagtcactttctgatccttactccccgaaggaactcttagcctcatagctacatgagctacattaggttccgtagggttagcaatacaagaatctcgattggaaaatacctgaggtaggattactcaacgatccttgttaccttaactcccttctcccgggatgaagccttagaaggaaaagtataggggaccccaaaaactctttagctttagatgttatatgaacccctaacaaggaaccgtaggcatagagctatcgggtcataactcttctcactctggccttagggttcttctttcaacaatctaaaatcctttcttcatttgcaaacacttatgtgataatattcctaacaaagattccgtttgacttgaccgtaggacatcgcgttcctcaatgcaatggaaaactaggagcgcggaagcgatgaaagcatgcccactttcgccggctaacacaatggatcaatacaggggaaactggccgagaagcctaagctagctatcagctgccctagcgaacgaagtctagtcttcttatcgagatgagcatgagtggtcaagccctgcaatgagatcatgcgccctaacctaagcctgggctactgttgtgtgttccgatccttctagtgagagcttgtgaccatcgcagtgaccgcagtatgcttaatcgactgtctctctaccttcttgatcgttgcatcacaagttcgcacgacaagccgcattgtgcactcaagatgatgaatgcctttgaaagatagaggatttgaacctgtaatgtgtacctaagggctagatacacagatgccttcctatcttccttctttactggaccaatcgaagactgaaaagacaaagagatttcgcttagccaatgcttactgatagactagatggagagcctggtgcaaggtgggaagactgagtgagaactagccctttgaggagctctctaagctgtctaactctctattaccataggcagagggaaaccaggttcaatagccggatagagtaagaaaacaagaaatttgacgatcaactatgtaaaccccccgaagggggaaggtaagcccgccgctgatcccgctttaccttcgcctaccgtgaaaagagagtcccctatcacgataggccctcccagctcccgaacgtgtctttctatcaatcgagagaggtacataaaagaagagcaactaaactgtgaaactaaaagcatgggaaaaagaaagcggtgaaaagcatacatctactaaggaccctcatactagaagacatagtttatactatcgagaaaattacagagatcttctacaagccaactcgaacccccccttaaaagaacatcgtaatagatatcttggaggtgtcctggaatttgaaaagcctcgtctcccataacagcctgaacaagatctgctatgttccactccggaggtaattccctacctctgagtcgaagcaactccgcgctattttggcagattctatcaaatacctgttctaactcaggtggagcgctttgcgcgtccgacctagttgaggaaagagtggaagtgctactagcagaagggaacgaagaagtggaactttgcaaaaagtgaagatcactaggggtaggatctccatagagtattacagcattatttcgaagaatcatttggtttggttcattctttcactgctctgctcccccaaaaaaagaagagagactgaatttcttccaccttccctgtacgagtagtgaagaagtatagagcactttagttggttgttgaccaacggaaagcatgggagaaaaaaagatgcacaaaggaaaaggagtctcattaacagctgaatgtgccaaactagtagcccgaaatagagatctgatttaaaggaccaggtacagcgagttcgatccattaggttctttttttttttcagaaaagaaacgagagacaagaaaacatctttgattacgattaaaaggaacaatctcaaatagaccaagatccaatttcgggtcatttcttggtgaacatgatctgccataatctcttcgatcccttcatttatgtgccagaatagagagagatttggtaggaaagtggaagagacctttttgtatatgataatcaaagggagtgggaaagctgcagtaattctttggaaaagcccggttctctttgtcttcgaactttcattcctcaatccactgattccttccttcatatacctccccaccaatagatagagacaaatgggaataaccgaaccacgtctacaaaatgccagtaccatgcagctgcttcaaagccaacgtgatgctccttggtcagatgaccaagatattggcgaatgccacatatgatcaagaaaatagtacctataatcacatgaaaaccatgaaagccagttgctaagaaaaaggtagaaccataaatactatccgaaatagtgaagggtgcttgataatattccattccttgaaagcctgtgaatactagagccagtgaaacggtagctactaaagcgtaaactgctcgtttttccttccccgcgagtatagcatgatgagcccaagttacggcagctccggatgaaaggggaataagggtattaagaaaagggatttcccaaggatctaaaactgcaatccctttcgggggccaaatacctccgatctctaccgtaggcgccaaggaagaatgagaagaagcccgaaaaagagcaaaaaagaacataacctccgatacgataaacagaataaaaccatatcgaggtcctaattgtacgactttggtatgatgtccttcgaacgtggattcacgtagaacatcgcgccaccatacgaacatggtatataggataaatatgaggcccaaactgagaagtgttgcacccccttgaaatgagtgcatgtacatcacacctcctacggttgttgccaaagctccgagtgaacccgaaataggccatggacttggatctaccaaatgataagaatgcctctgagattcaatcataaaccactttgcctcggttctatgtaaacccccccttcacccccaccccctaaagtagtaaagtaaagaagggctctttggggtcttattttctttctatctgacaggacaaacaaagaaataggaagggagggttctttcattccattgatagaagtctaactagaaaaagactctctctattactttgagaagagaatcgttggtttgaccgacgaactacgtgggaaaatagaccttctttctttgatttgaagcaagatttttggcaagtaacaattccattcagttcgctttcggaaaacttgctggtcgcggattagttcgttctgcgccgccagcggcctcaactcaaaggcgcaggttgaactctctggttgaggctgcattcatttattcatattcaacttgacacgtgggaagggcttactctactagtggctcggcttggtctcgctcccttcccgcactattcctccccactaaaaagagcgattgagaatctcgagaacctttccgaacgtctgtcttcgcggggcgattggaaaagaaaggagtcttcaattcttttactgccttccattccactattttgatcgaattaattgctcttccgaacgaccaagtcataatgagattaaaaaccgatgcttccttggccgtgtggaacatggattagcattatgtcattcctacaagtgatgacccacccaggattgctatgtacggacttagagatcaaatataatatgtttctttccattcctcgtgagccacttatttctccgaaacaagagattaaagtcatcttcctcctttttcccaagaagtcgacggccttacaccattgggatacttcgaataaacttgagtacatataggaaacaccggtgctaaaaccttttctcaagatatcttccaaactgttggggtcgttgctccggatcttgttctcccggtgtgaaaccagttggttccgtagttttagaattctgctgatcccaagtactccatctccatcattgcatataggaatatagaaagtaaagaggaaaaggcatgaccagaagaattgtgtgaaataagtgaatttatccagttgaggcattcttgattgattgagacaaaacgattccctcaatacagcttaaccccgtcaagcctgtacgagtagtgaagaagtatagagcactttggttggttgttgaccaacggaaagcatgggaaagatcactcctaactaagcagtcaagtgaaaggagcccgcttacccactcccctttccccccatcgctaggggcctcgctcatcacatcagtctaacatgagctactcttccatttcataaacgatcaattggaaaaaaaggactttccttttcctttctggtggaaaaacgaaagaaaaggtgttcccccttattgtaatgctccagttgaagtgcttccactcttgaaagcagagctttagaaaagccaactgtcgcattattcaagtgaaggggttcaatataggtcgaaaacatttcatcggacagcgttttttttcgacctatattgaataggtatcgcaattgttcgttaatatgtcttaacagacagtccggcgctagttgattctcgggaagagaaagcgccgtttcccattccggcttggcttggaaaaggaggtagaggcttccgagcttgatgggcaggaagttccagacgaagacatcatgctcttccggaccccgctctcgatctccaaagccaaagaaagaataccaagaagaatgagacttgcgcccccctcccatccaaaagccctactacaaaataaggcgagggatcgcctccccacagagaacccaaccctttcaagtagggcctgaaagaaatcaattgaagccattttcaaacaaagaagataaaataagaaaactatagtggctaggaacagtaacggaatacggcgttttttcataatcgaaccgagatgcatcatattaggtaagatgtatcttcattcgctctgcgagcagagcggtataccgaaaaaaagaaaagccttatggccactaccttacttaagcaattctgcttattcttattctatcttagaataagaataagttccccctctccggatcccgataagaatggaagatggtgcaagatcgaatcctgttaccttacttcgaatggaatcttagcccgcctcacttgctttctttactgcataaataagggcataagcgaagtcaagggatttccgtctaactagtgtctgagagtaagcaagctaccttcattcaacagatttgtggttgagtcaataacatgctctgctctgggtcgggaatctttgctcttctcttttgcatttccgctgcctgcctaaaggcttattgctagctcttaggttctctgtcagtagagtgattgccaaaacctaggtatgttttcggagaataataagaagagacggttgtagcttttagagactatcctctgcagctgtagctacgtggaagccagctgcttaaagacaagccccctaaccattctgctattcctgccctaaagcaagggaatccgctctgacccaccaccctggtaggaattgccagatttacagtttatgaatccttgtaatacaagttctttcctctaacgatggctacgaactacgcgaactgaactgtcaaggctttcaaaccaagactgagaaagctcaatcaaaaaagagtattttagtggaatggcttaacgaagttactccccatacgagaccggaaaggaagctagcgaacctagggtcaacaccaaggtaggggcgaaagggaaaagaacgatgtttgatgtgaacggaagcaagcatttcgctaagaaagcaaaacaggaagcggcgatagcaaacattaccctgactcagaacaatatgctcttgggagacatgaagcacaatcaacctctctaccttaagacttctaacatggtcgattctagatagagcacggtaacccacaaccccctactctacaaaacaaagagtggaaaatctcttcatagggtactgtagctgtacagccatagtaccatagggatggtgagagttcataagagcccgaatttagataggtgaaagatccttactcaaattacgaaccctgaacctctttgcgaattcacagctgaaccttgatgggaaatcatagatttctgataggaaagaaaaagcccaattacccacaattttttcatatacacgagcgtcctcctacattgtcccctagtacagcatacttaataaagcggtttccagggtcaacctgtttaactgcatgccagaccactaagtgatgagaccatgcaaacaaaggcaacgaggagcgctagccggaactggacaatgggtgggtgtccaacaaacattccttagctaagaaggattcattcaccgcagcttctcttactagcagatgaaactagcaacatcacatcatatagaataccgattgacaggcattccagtctatcttatagtttatgttgatgatctcattgtttccgcgagcgcatccttcatttccaagctttatttctatcgtaatttttccatgcctattcattcttttttggggtgtataatataaagccacggagcgattcaggcatctatcttattgtattgacgcaattggaagatcaggatttctccctaccgctcaagcgggatcagatcgggctttagcgagaacagctgtaattgaatcgggaacggaaagacttcacttcaactcaataaatgacgtctacttcgtaagtgctaaggcaaaatatatcaccgaaaggaaaggtgataggggagcctagccatttcactctacctgagtaataaagtggaaacccccctcacgatcgattaaaaggaaagtcgcccagagatatttgttcaaatccaattcgtgaagacagagtaaattcaacaaatctaagaaagcaagtcctaggcctcactatctatcaatcaagaaggtaaaggagagaaggtttgattgaaagtagtacgtctgcagggatctgtcgttaacgatttgaccgggacacatccaattgaaagtctaatcccaacctctttggaaggagctccaaaaaagacttgacttcagagcggggaatcttcctacaagtgagcaccaagtcaaatgtatgaaaaaagggctatacctctgcctagacaaagaggactttaagacagcctcgtaggagacattggatgtaaccagccttcaaaggcggaggagtcaaaagcgactttcgattcaaattagagaaatgctgagctttatccgcttcaattcattaaggtattattttttccttctaaatagtcagagtgggaactcaaaagcaagaactcttaaccatcattccttaactctaaagggcgtgaatgtgtggatcaaggaagaagggtgggatagcgcccgattgattgagcgtcttacagcccgtcatgcaagctagcaaagccagcgcagaagcagccctttccatcgtctttcgctgaccctggttctatcaaaccagcttcttcaatcctggtgtgaacttcttcctgccttcttacccaagagctctgattccgcttaaataaaagcagcccttcttccttactctttcgagtaagcattttgaaacttccttaaacatctgcttcaaagagctaagccccggtctcactgaactgggtcaaagaactaccttcctggagctacctccttacttagatcgttcgttccccaattcaaactcggatcagttggcaagtggattccatgcctgggtacgaaactcgaaattcgatcttgaaagagtgaaatctagccttttgtctttatcctttataggtctgggctaattcttgaaagcagcaactcctacacctaccgaaactttaacagaacaactacggattctcaccctcgagtcaggagctcgctttcaatctctaagagccgattcgatggcatctttttttatgatctttctagttagcacgtagtgggaatagtccctcatcgacacgggaagagagcttcaagcaaaaagggcttgtgcaagcaagtgacactttacttcaagcgaatagtgctgcctcactttctttagctaggctgagaagccgattcccgacatagactatttccttctcatcgaaagatgcctaagaccttttcaccaaaacaaaacctctaccccctactctagtcagctttctatctctttctccaaccttcgatgatcctcctgcaggcaaatcatcgaagtcaagaagaagtgatgggcctgatcttccgatatcgatatctgatccctaagctgagctccaaagtctagatttcttcctaaagctaaagtaagggcaaggccccggtcggttctccctttctttctttcctggttctctgttctctagtcgtataatcataccattctgccatactattttcagaattcattccacgtggaaaatcgtctagctagggaactcttcatcagacgatttctcatatgattattttcgtgaattcgacgtagaagaagttcgccttgcctccctttattaagtactgggctaagggcggacccccccttctatctgggtcctagtctcgtcccttgttagtgcaataaagagaagtgtattaaattccaattcttttccgcccttcctaaccttgctcgatccaatagcccgatcctagcccactcacctttctccaagattgaagttagaactaggagtcctaaaatcttaatgaaaaggagcttggcatccatgtgttcgagaggtagaaaacgacccctgtggcggggtttaccaggtaggtataattcaatgggaccctatcccgtcctgtggtcctgaacaaaggttccatcctaaaaagaaaagagagccttcacggaaaaactgttggaacgagatctctcatacaaaaagacctgaactaactactcgctcaatgcgcattgaaattctaatgaatgcccttatttagcatctttgagttgagcttagccctcttcctatcctaaatccctagaatcataaggaacgattgatggttgatctggcaattctttttagtaattagttagtctatcaagcagaaaactatgactgaggaagtctcagggagggcacccccttttaaggtaattatatgccatttgtggccccccacgttagaactctctttaaccggaatctttatggctaaacctttttttttaaccgatttaatcgtaagttgcatcctcaacttctggacgggttcgagagtttggttcgactgagactgatgtctcatcgggttcagaaggggatgggaatgcagattttgatgcctcgtatcgtatgacaaagaagagagtttttacaaagccctagagctagagcttgttgagaaagtagctttgaagatgggcttcctatgggaaatagggaagtttaaagcgataacaaaggccttagggaataggatctctttctgcgtctactgatgcttttgaaaaaagcctttggtttggcttgtttaattgattcgtacgtaatccgagagcttcatacgtgggatttttttggcaaaggaaagtcaagagaaaaggtggtagctattctagcaagtcttctgtggaggagtagcactaggctagtaacttattacactagtctcgattcctcaaggttgtacgagctgtaatagtagttgaaaaacctcccgtcccgagttggcttaagccatgcctttactaaagaattctcgccatctctgataaaatctggtgtggagcccaggctagccaacaatgagaaatgccttcctcttttttgttgatttaggtgacgtagtcttatccgatgaatggcagtgagaaggcggaaaaggtcgtaaagggctaagctaagggaggttggcattccgaagtcaagtgggcttttctcacaccgcatggggtggtttcctacgcatatgcaacaagctcttatttggatctccctaatctagagggttctcacgccaaggttcctttgtttcgggcaagtccaattacaaacaaaagagaaggtcggtcccgtcccacgggttaggtgcttagctgaaggtggaagtccaaagcttaataaggtggaaggcgaagccgaggcaagagcaagggttgaaagacaagagagaagaattcaatctcccctatttgttccattctcaatggttggccaggatgctttggtttatcggatcgatcgcagtggtcaagtgcgctggacgacacggcattctcgtttaaatagtaccatcgactggagaccggattgctaccagagagaggaatgactataggcacggaacttacttttgaccctttctttgccccttggttcgctagctgacttgccagcgcttggattctcgaactctaagagcggatttcaggaatttgttcacatccgattcgatggcatctgtctgctttccaccctttgcaagcgtgctactgactcgatggacaaactcaaggaactgctttgcctctaggttgacttggatcacatcatcctgaacttttgatcgtatgtcgtccagctttgttggtgctgtgggtgtcagtcttctaatgtcagctctctggtaggccaatcgatctctgcttgattggccgtaactgcatgatcgatctgacgaagattcccatgtagatctatgaaactacagccgaaccaaatgggaatcctaggtataggcaaaggtgggagggatgagagagcaagctggcgtgggggcaagggcaataacatccgagcaaggcaagccctagaaatcggcagggtatgatgaaaagctctcaccaggattgtgtttccagatcgattgatcaacatttccctctttgtgatagctgagaagcgttctaaatacttttcgacaaggagagagttccaacaaagacgcgatcttctgcaacggaagctaacgtggatgttccaccggcaccggggttcgaaggtcacgatcatcggagcaatcaacggagtgtttccttcagtcagtaaggggagaaatcccttattctaaggaaatgtttttggtaagaaagcctgtcctagaaggaagcctgcccgcaagaactctggttaagtgccctccaccgcaaccgacataacataaagaaagaaggaaccggtccccatggtcgccttcgttcgtaaggtaaaaacgaatagacattcttgtcttggcccaggtgacgcacatgaccggtcaagaaagttcttatttttggatttcgctttcgctacggctacagtcaagtggctccccctttacaagactccctcccaccagaagaaagattgatcgctttcggtaacccagggctccattgcgtgtgctcgaggtagaagttttttttttttttagatgtgaatgggaaaaaattctgaccaccggtagcgaatgcttttgaaaagatttgaaggtagaaggctgtttcagtctagctccggaagcattgtctgaagtaataagaagaaggaagtgaccactctgaagttctttttctttgattccaatgaccgatatcgtacaagacggaagtcatgagcgatagcgaagataggtataggtcttagattagagtgccagtgcccctcgggaaaaaggaaacctagctattctttttgttcttaagaaaggttgcggtaagggtgggcgtcaatcggccattcctccatcataacctttggaactctacgcccgcgcttggttctcatgcactaggtgcacccgagtcgactatagcactaaccaacttgccattgattacaacatcgacctttgaatcgtatcatccatggtgagtggtatcatatataagtataagagcaacctttaggaaggatctttctctctaactagaaattttagaagaaagcgtagaaaatcaaggttttgattcaacaacggataaccccgaaaggcaaaaaaactcgaactgaatcaaagtacaaggctgacgtacttatataagtgatgaatatgtagttaatcagatatttccatttggagactgattcatgtattctatctttatctaccgctacgccctggaaaagcagtgaaacttctaaagcttattagcacagaaaaaaggatttgaataccctagtttataagggaatcaccaatccctctatataagctatcgttcgaaactacattcatcagttgtccaaggaggcaaacatggaatggagatagaaagattcagtcggtctatccctgtggatcggtatatgcacctatagttgagttgagttggttgattcaatccacaacaccgccaaccagaggggaatcaaactcgcttagcaaagtgcaaaaagaaaaggaatcgaaagtatgaatatcataaagcagcagctgctcccctagccttctaaagagctagtcccgaagtagcaacagagctcttcttccctattagtctatgaactatggatgctactaactagcaatgtatataggtaagctactaaccttatggatgatatctactctttgctgtataagtctttctcattcctcttctcttaataagcctagcagctttcttttcttcactgggaaatatccataggaataagaatctctatatatcaaagatcttaaaatccctctacaacgggaaagcgacggaaaagccgtttcaccaccgaagcgaactaccttaggccaatgggaaatgccagagtagagcgcaaaagaaagggattttcaatccacttcaggtgggactaagaaaagaaaatctgaacctgggaagcagatttacaggttgtacttttcccgttagtccataaggatcggacacccatattccaggaccatacaagcctgttacatgaaatgcaccaaaaccaaagcaagccaagtagccttccattaatagcctctctttcaggctcttctgtgggaatactttcaatcgttggcattcccctaggcggagacagttttcgcaatagctagattctcaagctctgattcacttgcacccttcttcttgaaatggcattagctgctctttctattccatcaaagatccaagcaggagattctgtaagaaaaagatcgcttaggccgacataacatatgtcacttccacttcctttaggagatgtttttcagggaccaaagagaaggcgatttggtcaaattgatcctttttcatttccatgccatgacatgagacagatctctcgcaactagttcctttgctgatgaaatgccttagtcagtagcctgccttacgactgaaaatggttcacgttcacagccctatagcgctagtcttgctaaaggaatggtgaagaaaatccccctatagctagtgagcatctttacttttagtaggtaaagagcctcaatgaaaggggaattgccgccctcaagggagaactaagatagtggttgattgtctacggtctcgttacaggatgaagctacagatagaacagatagagtagaagagtcggtggggcttacctttcttgttgaactagagtagagggtgagcagagaaatcccttgaagaaagagcttattccacctcctggatcggtaagggcttcggttccatcaattcgatgttgctcgataagcaggattacgattctagtttagttcatcagatctacgctctcaggcacacccaccaacgtaagacaggatcaaagtccaatagaatagctcgggcatgaataaagataggaatcgacgagaccttttcctacttaaaacaattcgaaatctcgaacccctggtatttcattgaggagacaagacaaatagggacctaaaaacgccctgagtgggacgcccccttcgggctgagatgctttccggacatgctattctttttatataagacttcgctacacggcttagccgacctttccgagagaacttcaagacatactttgagtattctataaatatcctaagtcgagttataggccaaatgccctaccagatcagtctcgaagaaatagcaaaaggatggctacgggatcccactctacctttccaggatgaacttcccttcctgcttctgtagcactggaagtgacccgtgtttggatctaggattcaattcatccagctttcatttaaagtaaactctttaagataaggctttttccctcgcctaagttatgaatctattgcaattgaaaactccctcgcgactgatttgccatttggatcgatttgagatatagagagttgtgtctttctaacgctaacgatgctaagcttaagctctttcctttagcttaaacaggaatagctcttccagcttgttcgttgcactcaccctcaccctgaccttctcccagaaacaaaggaaaaaacctaacattcgctccttcacccgcgagggattctcttcatcgctactaactagaaaaagttcctgggctaagaagagctccgttaaaggatatctatagctgcggagagggaagcgcttagaagctatgctcttcttcagctttctaagcttctactttcgtgagctcttattgctcttttagtcgagaatgctaccattcatccctaaaagaggaagatagtgaatcagtgcttactttagaggaagagtagtttagctagacagattatatagagaaagggaaggggcttgcttactcggaagagaaaggactgaaggtgaatgtattcatggatatgattcgattctctgatcggagaatgtaaggtatgaactcctaagaggaggagagggaagatctacatttttaaaagaaagatgtatatcagacattatgctgtgcttactaaggtctttagtctttactttagatagaggttcatctgtcctttctttcctctagcaaagcctacttcctgattaaggatttgaagcttcatggccttcttttcttcctcagaaacacagaaagaaagatttaaaaaagcaacaaaatctgtatttaacacaaaacggaaactaaggagagagctggtcttactgttagacacagtaaacataggagacaccttatacacgttaggaatttaggaagagtagtaccgatagccttagtatgagttgaacctttcttattcttagtcctcttatacaagctagctctcttatccgcttgcctcttttaatgaagaagggttggtttaattgatagctttggaataggtagtcctatggactgctcttttcttatgccccggagtggcgagaatacgaagctagatcagcaggaatgacagcggtctcttccaaaagtgggtacaggactcggatcccatttccaaggtgaattggaggagaaatggatactggtattatagttgttgaaagacctattaattacatgccaaaagagcaaaagttgaatcatcggcttggccaccttatccttttatacaaaaattttcyttgatgatataccgyycraggsgawttstcwcgacntcctctgcyagamaaagaaaahagaaacccvscagbtsccwcctcwsatcamwgaaraaaccaaawcacyacamwavachaaccgcaaaahgctcccactcbtstdtgtyctmgratsctgcttgtattcaancttatrtttnygkaancctctnchdctyswtmwac